European Patent Application EP 4 741 425 A1, published May 13, 2026. Title: 降低肿瘤内中性粒细胞水平的抗肿瘤细菌. Applicant: 深圳先进技术研究院. The sequence listing filed with the application follows.

SEQUENCE LISTING (123 sequences)

SEQ ID NO: 1 - DNA, 3977 bp, synthetic construct
  source 1..3977: mol_type = other DNA
ttcacagaaaagtgttgcccccttccatggcggaagggggacaaaggtgaatttgtcctactcaggagagcgttcaccgacaaacaacagataaaacgaaaggcccagtctttcgactgagcctttcgttttatttgatgcactagtgccgatcatattcaataacccttaatataacttcgtataatgtatgctatacgaagttattaggtctgaagaggagtttacgtcccatatggagtcccgctcagaagaactcgtcaagaaggcgatagaaggcgatgcgctgcgaatcgggagcggcgataccgtaaagcacgaggaagcggtcagcccattcgccgccaagctcttcagcaatatcacgggtagccaacgctatgtcctgatagcggtccgccacacccagccggccacagtcgatgaatccagaaaagcggccattttccaccatgatattcggcaagcaggcatcgccatgggtcacgacgagatcctcgccgtcgggcatgcgcgccttgagcctggcgaacagttcggccggcgcgagcccctgatgctcttcgtccagatcatcctgatcgacaagaccggcttccatccgagtacgtgctcgctcgatgcgatgtttcgcttggtggtcgaatgggcaggtagccggatcaagcgtatgcagccgccgcattgcatcagccatgatggatactttctcggcaggagcaaggtgagatgacaggagatcctgccccggcacttcgcccaatagcagccagtcccttcccgcttcagtgacaacgtcgagcacagctgcgcaaggaacgcccgtcgtggccagccacgatagccgcgctgcctcgtcctgcagttcattcagggcaccggacaggtcggtcttgacaaaaagaaccgggcgcccctgcgctgacagccggaacacggcggcatcagagcagccgattgtctgttgtgcccagtcatagccgaatagcctctccacccaagcggccggagaacctgcgtgcaatccatcttgttcaatcatgcgaaacgatcctcatcctgtctcttgatcagatcctgatcccctgcgccatcagatccttggcggcaagaaagccatccagtttactttgcagggcttcccaaccttaccagagggcgccccagctggcaattccgacgtcattgcgttgctagccaagcttaggatccggaacccttaatataacttcgtataatgtatgctatacgaagttattaggtccctcgaagaggttcactagctatctagagcttggactcctgttgatagatccagtaatgacctcagaactccatctggatttgttcagaacgctcggttgccgccgggcgttttttattggtgagaatccaagcccgggaaacgggatcctgatcttgatcaggctgtgggtcaggccactcttggcatcgacaccaatgtgggccttcatgccaaagtgccactgattgcctttcttggtctgatgcatctccggatcgcgttgctgctctttgttcttggtcgagctgggtgcctcaatgatggtggcatcgaccaaggtgccttgagtcatcatgacgcctgcttcggccagccagcgattgatggtcttgaacaattggcgggccagttgatgctgctccagcaggtggcggaaattcatgatggtggtgcggtccggcaaggcgctatccagggataaccgggcaaacagacgcatggaggcgatttcgtacagagcatcttccatcgcgccatcgctcaggttgtaccaatgctgcatgcagtgaatgcgtagcatggtttccagcggataaggtcgccggccattaccagccttggggtaaaacggctcgatgacttccaccatgttttgccatggcagaatctgctccatgcgggacaagaaaatctcttttctggtctgacggcgcttactgctgaattcactgtcggcgaaggtaagttgatgactcatgatgaaccctgttctatggctccagatgacaaacatgatctcatatcagggacttgttcgcaccttccttagcacgttaattatctatcgtgtatatggaggggatctagaatgaaaaaaataatgctagtttttattacacttatattagttagtctaccaattgcgcaacaaactgaagcaaaggatgcatctgcattcaataaagaaaattcaatttcatccatggcaccaccagcatctccgcctgcaagtcctaagacgccaatcgaaaagaaacacgcggatgaaatcgataagtatatacaaggattggactacaataaaaacaatgtattagtataccacggagatgcagtgacaaatgtgccgccaagaaaaggttacaaagatggaaatgaatatattgttgtggagaaaaagaagaaatccatcaatcaaaataatgcagacattcaagttgtgaatgcaatttcgagcctaacctatccaggtgctctcgtaaaagcgaattcggaattagtagaaaatcaaccagatgttctccctgtaaaacgtgattcattaacactcagcattgatttgccaggtatgactaatcaagacaataaaatcgttgtaaaaaatgccactaaatcaaacgttaacaacgcagtaaatacattagtggaaagatggaatgaaaaatatgctcaagcttatccaaatgtaagtgcaaaaattgattatgatgacgaaatggcttacagtgaatcacaattaattgcgaaatttggtacagcatttaaagctgtaaataatagcttgaatgtaaacttcggcgcaatcagtgaagggaaaatgcaagaagaagtcattagttttaaacaaatttactataacgtgaatgttaatgaacctacaagaccttccagatttttcggcaaagctgttactaaagagcagttgcaagcgcttggagtgaatgcagaaaatcctcctgcatatatctcaagtgtggcgtatggccgtcaagtttatttgaaattatcaactaattcccatagtactaaagtaaaagctgcttttgatgctgccgtaagcggaaaatctgtctcaggtgatgtagaactaacaaatatcatcaaaaattcttccttcaaagccgtaatttacggaggttccgcaaaagatgaagttcaaatcatcgacggcaacctcggagacttacgagatattttgaaaaaaggcgctacttttaatcgagaaacaccaggagttcccattgcttatacaacaaacttcctaaaagacaatgaattagctgttattaaaaacaactcagaatatattgaaacaacttcaaaagcttatacagatggaaaaattaacatcgatcactctggaggatacgttgctcaattcaacatttcttgggatgaagtaaattatgatcctgaaggtaacgaaattgttcaacataaaaactggagcgaaaacaataaaagtaagctagctcatttcacatcgtccatctatttgccaggtaacgcgagaaatattaatgtttacgctaaagaatgcactggtttagcttgggaatggtggagaacggtaattgatgaccggaacttaccacttgtgaaaaatagaaatatctccatctggggcaccacgctttatccgaaatatagtaataaagtagataatccaatcgaataagtcgacctcgaggactagtgaacctcttcgagggacctaataacttcgtatagcatacattatacgaagttatattaagggttattgaatatgatcggctcgagattacttcgcattgcaatcagctacggactcaagcttacgtcaggtcatacgatgaaggcgataagtcgcgtaagttgctagcccacgcggctcaccttcacgggtgggcctttcttcggtgtttcaatctcgattaacaggtaacgcaaaattgctgtgtacgtcaga

SEQ ID NO: 2 - DNA, 2716 bp, synthetic construct
  source 1..2716: mol_type = other DNA
ttggtttcagtgaatcccgttatcagcagttttttgatgaggtgtagtctatttgtcctactcaggagagcgttcaccgacaaacaacagataaaacgaaaggcccagtctttcgactgagcctttcgttttatttgatgcactagtgccgatcatattcaataacccttaatataacttcgtataatgtatgctatacgaagttattaggtctgaagaggagtttacgtcccatatggagtcccgcttacgccccgccctgccactcatcgcagtactgttgtaattcattaagcattctgccgacatggaagccatcacagacggcatgatgaacctgaatcgccagcggcatcagcaccttgtcgccttgcgtataatatttgcccatggtgaaaacgggggcgaagaagttgtccatattggccacgtttaaatcaaaactggtgaaactcacccagggattggctgagacgaaaaacatattctcaataaaccctttagggaaataggccaggttttcaccgtaacacgccacatcttgcgaatatatgtgtagaaactgccggaaatcgtcgtggtattcactccagagcgatgaaaacgtttcagtttgctcatggaaaacggtgtaacaagggtgaacactatcccatatcaccagctcaccgtctttcattgccatacgaaattccggatgagcattcatcaggcgggcaagaatgtgaataaaggccggataaaacttgtgcttatttttctttacggtctttaaaaaggccgtaatatccagctgaacggtctggttataggtacattgagcaactgactgaaatgcctcaaaatgttctttacgatgccattgggatatatcaacggtggtatatccagtgatttttttctccatgcgaaacgatcctcatcctgtctcttgatcagatcctgatcccctgcgccatcagatccttggcggcaagaaagccatccagtttactttgcagggcttcccaaccttaccagagggcgccccagctggcaattccgacgtcattgcgttgctagccaagcttaggatccggaacccttaatataacttcgtataatgtatgctatacgaagttattaggtccctcgaagaggttcactagctatctagagcttggactcctgttgatagatccagtaatgacctcagaactccatctggatttgttcagaacgctcggttgccgccgggcgttttttattggtgagaatccaagcccgggaaacgggatcctgatcttgatcaaccgaggtcacaacatagtaaaagcgctattggtaatggtacaatcgcgcgtttacacttattcagaacgatttttttcaggagggcctacttgtcacacaggacggtaatgtcgtgcccggttattgagctgacacagcaacttattcgtcgcccctccctgagtccggatgacgcaggctgtcaggcattaatgattgaacgcctgcgtaaaatcggttttaccattgagcatatggattttggcgacacgcaaaatttttgggcatggcgtgggcgtggcgaaacgctggcgttcgccgggcatactgacgtcgtaccggctggcgatgtcgatcgctggatcaatccgccgtttgagcctacgattcgcgacggaatgttgttcggtcgcggcgcggcggatatgaaaggttcactggcggccatggtggtggctgctgaacgttttgttgcgcagcatcctcatcaccggggccgcctcgcatttttgattacctctgatgaggaagccagcgcaaaaaatggcaccgtaaaggtggttgaagcgctgatggcccgtaacgagcggctggattactgtctggtcggcgaaccttccagtactgaaattgtgggcgatgtcgtcaaaaacgggcgtcgcggttctctcacctgtaacctcactatccatggcgttcaggggcacgtcgcctatccgcatctggcggataaccctgttcatcgcgccgcgccttttcttaatgaactggtcgctatcgagtgggatcggggcaatgactttttcccggccaccagtatgcaggtagccaatatccaggcaggcaccggcagcaataatgtcattcccggcgaactgttcgtgcagtttaacttccgtttcagcacggaactgaccgatgagatgatcaaagagcgggtacatgcgctgcttgaaaagcatcagctacgctataccgtagactggtggctttccgggcagccgttcctgaccgcacgcggcaagctggtggacgcggtggtaaacgccattgagcactataatgaaattaaaccgcaattactgacgacgggcggtacgtccgacggacgttttatcgcccgtatgggagcgcaggtggtagaactggggccggtgaacgccaccattcataaaattaatgaatgtgtgaatgccgccgatctccagctactggcccgtatgtatcaacgcattatggaacagctcgtcgcccatcaccatcaccatcactaagattacttcgcattgcaatcagctacggactcaagcttacgtcaggtcatacgatgaaggcgataagtcgcgtaagttgctagcccacgcggctcaccttcacgggtgggcctttcttcgtgagcgttccggtaagaggaaataagcatggactggctggcaaaatattg

SEQ ID NO: 3 - DNA, 6750 bp, synthetic construct
  source 1..6750: mol_type = other DNA
catggtcatagctgtttcctttaatgcccatggcgtttaccaatgcttaatcagtgaggcacctatctcagcgatctgtctatttcgttcatccatagttgcctgactccccgtcgtgtagataactacgatacgggagggcttaccatctggccccagtgctgcaatgataccgcgacttccacgctcaccggctccagatttatcagcaataaaccagccagccggaagggccgagcgcagaagtggtcctgcaactttatccgcctccatccagtctattaattgttgccgggaagctagagtaagtagttcgccagttaatagtttgcgcaacgttgttgccattgctacaggcatcgtggtgtcacgctcgtcgtttggtatggcttcattcagctccggttcccaacgatcaaggcgagttacatgatcccccatgttgtgcaaaaaagcggttagctccttcggtcctccgatcgttgtcagaagtaagttggccgcagtgttatcactcatggttatggcagcactgcataattctcttactgtcatgccatccgtaagatgcttttctgtgactggtgagtactcaaccaagtcattctgagaatagtgtatgcggcgaccgagttgctcttgcccggcgtcaatacgggataataccgcgccacatagcagaactttaaaagtgctcatcattggaaaacgttcttcggggcgaaaactctcaaggatcttaccgctgttgagatccagttcgatgtaacccactcgtgcacccaactgatcttcagcatcttttactttcaccagcgtttctgggtgagcaaaaacaggaaggcaaaatgccgcaaaaaagggaataagggcgacacggaaatgttgaatactcatactcttcctttttcaatattattgaagcatttatcagggttattgtctcatgagcggatacatatttgaatgtatttagaaaaataaacaaataggggttccgcgcacatttccccgaaaagtgccacctgacgtctaagaaaccattattatcatgacattaacctataaaaataggcgtatcacgaggcccttaggccaaataggccgttcagatccttccgtatttagccagtatgttctctagtgtggttcgttgtttttgcgtgagccatgagaacgaaccattgagatcatgcttactttgcatgtcactcaaaaattttgcctcaaaactggtgagctgaatttttgcagttaaagcatcgtgtagtgtttttcttagtccgttacgtaggtaggaatctgatgtaatggttgttggtattttgtcaccattcatttttatctggttgttctcaagttcggttacgagatccatttgtctatctagttcaacttggaaaatcaacgtatcagtcgggcggcctcgcttatcaaccaccaatttcatattgctgtaagtgtttaaatctttacttattggtttcaaaacccattggttaagccttttaaactcatggtagttattttcaagcattaacatgaacttaaattcatcaaggctaatctctatatttgccttgtgagttttcttttgtgttagttcttttaataaccactcataaatcctcatagagtatttgttttcaaaagacttaacatgttccagattatattttatgaatttttttaactggaaaagataaggcaatatctcttcactaaaaactaattctaatttttcgcttgagaacttggcatagtttgtccactggaaaatctcaaagcctttaaccaaaggattcctgatttccacagttctcgtcatcagctctctggttgctttagctaatacaccataagcattttccctactgatgttcatcatctgagcgtattggttataagtgaacgataccgtccgttctttccttgtagggttttcaatcgtggggttgagtagtgccacacagcataaaattagcttggtttcatgctccgttaagtcatagcgactaatcgctagttcatttgctttgaaaacaactaattcagacatacatctcaattggtctaggtgattttaatcactataccaattgagatgggctagtcaatgataattactagtccttttcctttgagttgtgggtatctgtaaattctgctagacctttgctggaaaacttgtaaattctgctagaccctctgtaaattccgctagacctttgtgtgttttttttgtttatattcaagtggttataatttatagaataaagaaagaataaaaaaagataaaaagaatagatcccagccctgtgtataactcactactttagtcagttccgcagtattacaaaaggatgtcgcaaacgctgtttgctcctctacaaaacagaccttaaaaccctaaaggcttaagtagcaccctcgcaagctcgggcaaatcgctgaatattccttttgtctccgaccatcaggcacctgagtcgctgtctttttcgtgacattcagttcgctgcgctcacggctctggcagtgaatgggggtaaatggcactacaggcgccttttatggattcatgcaaggaaactacccataatacaagaaaagcccgtcacgggcttctcagggcgttttatggcgggtctgctatgtggtgctatctgactttttgctgttcagcagttcctgccctctgattttccagtctgaccacttcggattatcccgtgacaggtcattcagactggctaatgcacccagtaaggcagcggtatcatcaacaggcttacccgtcttactgtcaagaggacatccggtcagataaccgtcatcttcggctactgtctagggcggcggatttgtcctactcaggagagcgttcaccgacaaacaacagataaaacgaaaggcccagtctttcgactgagcctttcgttttatttgatgcactagtgccgatcatattcaataacccttaatataacttcgtataatgtatgctatacgaagttattaggtctgaagaggagtttacgtcccatatggagtcccgctcagaagaactcgtcaagaaggcgatagaaggcgatgcgctgcgaatcgggagcggcgataccgtaaagcacgaggaagcggtcagcccattcgccgccaagctcttcagcaatatcacgggtagccaacgctatgtcctgatagcggtccgccacacccagccggccacagtcgatgaatccagaaaagcggccattttccaccatgatattcggcaagcaggcatcgccatgggtcacgacgagatcctcgccgtcgggcatgcgcgccttgagcctggcgaacagttcggccggcgcgagcccctgatgctcttcgtccagatcatcctgatcgacaagaccggcttccatccgagtacgtgctcgctcgatgcgatgtttcgcttggtggtcgaatgggcaggtagccggatcaagcgtatgcagccgccgcattgcatcagccatgatggatactttctcggcaggagcaaggtgagatgacaggagatcctgccccggcacttcgcccaatagcagccagtcccttcccgcttcagtgacaacgtcgagcacagctgcgcaaggaacgcccgtcgtggccagccacgatagccgcgctgcctcgtcctgcagttcattcagggcaccggacaggtcggtcttgacaaaaagaaccgggcgcccctgcgctgacagccggaacacggcggcatcagagcagccgattgtctgttgtgcccagtcatagccgaatagcctctccacccaagcggccggagaacctgcgtgcaatccatcttgttcaatcatgcgaaacgatcctcatcctgtctcttgatcagatcctgatcccctgcgccatcagatccttggcggcaagaaagccatccagtttactttgcagggcttcccaaccttaccagagggcgccccagctggcaattccgacgtcattgcgttgctagccaagcttaggatccggaacccttaatataacttcgtataatgtatgctatacgaagttattaggtccctcgaagaggttcactagctatctagagcttggactcctgttgatagatccagtaatgacctcagaactccatctggatttgttcagaacgctcggttgccgccgggcgttttttattggtgagaatccaagcccgggaaacgggatcctgatcttgatcaggctgtgggtcaggccactcttggcatcgacaccaatgtgggccttcatgccaaagtgccactgattgcctttcttggtctgatgcatctccggatcgcgttgctgctctttgttcttggtcgagctgggtgcctcaatgatggtggcatcgaccaaggtgccttgagtcatcatgacgcctgcttcggccagccagcgattgatggtcttgaacaattggcgggccagttgatgctgctccagcaggtggcggaaattcatgatggtggtgcggtccggcaaggcgctatccagggataaccgggcaaacagacgcatggaggcgatttcgtacagagcatcttccatcgcgccatcgctcaggttgtaccaatgctgcatgcagtgaatgcgtagcatggtttccagcggataaggtcgccggccattaccagccttggggtaaaacggctcgatgacttccaccatgttttgccatggcagaatctgctccatgcgggacaagaaaatctcttttctggtctgacggcgcttactgctgaattcactgtcggcgaaggtaagttgatgactcatgatgaaccctgttctatggctccagatgacaaacatgatctcatatcagggacttgttcgcaccttccttagcacgttaattatctatcgtgtatatggaggggatctagaatgaaaaaaataatgctagtttttattacacttatattagttagtctaccaattgcgcaacaaactgaagcaaaggatgcatctgcattcaataaagaaaattcaatttcatccatggcaccaccagcatctccgcctgcaagtcctaagacgccaatcgaaaagaaacacgcggatgaaatcgataagtatatacaaggattggactacaataaaaacaatgtattagtataccacggagatgcagtgacaaatgtgccgccaagaaaaggttacaaagatggaaatgaatatattgttgtggagaaaaagaagaaatccatcaatcaaaataatgcagacattcaagttgtgaatgcaatttcgagcctaacctatccaggtgctctcgtaaaagcgaattcggaattagtagaaaatcaaccagatgttctccctgtaaaacgtgattcattaacactcagcattgatttgccaggtatgactaatcaagacaataaaatcgttgtaaaaaatgccactaaatcaaacgttaacaacgcagtaaatacattagtggaaagatggaatgaaaaatatgctcaagcttatccaaatgtaagtgcaaaaattgattatgatgacgaaatggcttacagtgaatcacaattaattgcgaaatttggtacagcatttaaagctgtaaataatagcttgaatgtaaacttcggcgcaatcagtgaagggaaaatgcaagaagaagtcattagttttaaacaaatttactataacgtgaatgttaatgaacctacaagaccttccagatttttcggcaaagctgttactaaagagcagttgcaagcgcttggagtgaatgcagaaaatcctcctgcatatatctcaagtgtggcgtatggccgtcaagtttatttgaaattatcaactaattcccatagtactaaagtaaaagctgcttttgatgctgccgtaagcggaaaatctgtctcaggtgatgtagaactaacaaatatcatcaaaaattcttccttcaaagccgtaatttacggaggttccgcaaaagatgaagttcaaatcatcgacggcaacctcggagacttacgagatattttgaaaaaaggcgctacttttaatcgagaaacaccaggagttcccattgcttatacaacaaacttcctaaaagacaatgaattagctgttattaaaaacaactcagaatatattgaaacaacttcaaaagcttatacagatggaaaaattaacatcgatcactctggaggatacgttgctcaattcaacatttcttgggatgaagtaaattatgatcctgaaggtaacgaaattgttcaacataaaaactggagcgaaaacaataaaagtaagctagctcatttcacatcgtccatctatttgccaggtaacgcgagaaatattaatgtttacgctaaagaatgcactggtttagcttgggaatggtggagaacggtaattgatgaccggaacttaccacttgtgaaaaatagaaatatctccatctggggcaccacgctttatccgaaatatagtaataaagtagataatccaatcgaataagtcgacctcgaggactagtgaacctcttcgagggacctaataacttcgtatagcatacattatacgaagttatattaagggttattgaatatgatcggctcgagattacttcgcattgcaatcagctacggactcaagcttacgtcaggtcatacgatgaaggcgataagtcgcgtaagttgctagcccacgcggctcaccttcacgggtgggcctttcttcgcgatccacatg

SEQ ID NO: 4 - DNA, 5456 bp, synthetic construct
  source 1..5456: mol_type = other DNA
catggtcatagctgtttcctttaatgcccatggcgtttaccaatgcttaatcagtgaggcacctatctcagcgatctgtctatttcgttcatccatagttgcctgactccccgtcgtgtagataactacgatacgggagggcttaccatctggccccagtgctgcaatgataccgcgacttccacgctcaccggctccagatttatcagcaataaaccagccagccggaagggccgagcgcagaagtggtcctgcaactttatccgcctccatccagtctattaattgttgccgggaagctagagtaagtagttcgccagttaatagtttgcgcaacgttgttgccattgctacaggcatcgtggtgtcacgctcgtcgtttggtatggcttcattcagctccggttcccaacgatcaaggcgagttacatgatcccccatgttgtgcaaaaaagcggttagctccttcggtcctccgatcgttgtcagaagtaagttggccgcagtgttatcactcatggttatggcagcactgcataattctcttactgtcatgccatccgtaagatgcttttctgtgactggtgagtactcaaccaagtcattctgagaatagtgtatgcggcgaccgagttgctcttgcccggcgtcaatacgggataataccgcgccacatagcagaactttaaaagtgctcatcattggaaaacgttcttcggggcgaaaactctcaaggatcttaccgctgttgagatccagttcgatgtaacccactcgtgcacccaactgatcttcagcatcttttactttcaccagcgtttctgggtgagcaaaaacaggaaggcaaaatgccgcaaaaaagggaataagggcgacacggaaatgttgaatactcatactcttcctttttcaatattattgaagcatttatcagggttattgtctcatgagcggatacatatttgaatgtatttagaaaaataaacaaataggggttccgcgcacatttccccgaaaagtgccacctgacgtctaagaaaccattattatcatgacattaacctataaaaataggcgtatcacgaggcccttaggccaaataggccgttcagatccttccgtatttagccagtatgttctctagtgtggttcgttgtttttgcgtgagccatgagaacgaaccattgagatcatgcttactttgcatgtcactcaaaaattttgcctcaaaactggtgagctgaatttttgcagttaaagcatcgtgtagtgtttttcttagtccgttacgtaggtaggaatctgatgtaatggttgttggtattttgtcaccattcatttttatctggttgttctcaagttcggttacgagatccatttgtctatctagttcaacttggaaaatcaacgtatcagtcgggcggcctcgcttatcaaccaccaatttcatattgctgtaagtgtttaaatctttacttattggtttcaaaacccattggttaagccttttaaactcatggtagttattttcaagcattaacatgaacttaaattcatcaaggctaatctctatatttgccttgtgagttttcttttgtgttagttcttttaataaccactcataaatcctcatagagtatttgttttcaaaagacttaacatgttccagattatattttatgaatttttttaactggaaaagataaggcaatatctcttcactaaaaactaattctaatttttcgcttgagaacttggcatagtttgtccactggaaaatctcaaagcctttaaccaaaggattcctgatttccacagttctcgtcatcagctctctggttgctttagctaatacaccataagcattttccctactgatgttcatcatctgagcgtattggttataagtgaacgataccgtccgttctttccttgtagggttttcaatcgtggggttgagtagtgccacacagcataaaattagcttggtttcatgctccgttaagtcatagcgactaatcgctagttcatttgctttgaaaacaactaattcagacatacatctcaattggtctaggtgattttaatcactataccaattgagatgggctagtcaatgataattactagtccttttcctttgagttgtgggtatctgtaaattctgctagacctttgctggaaaacttgtaaattctgctagaccctctgtaaattccgctagacctttgtgtgttttttttgtttatattcaagtggttataatttatagaataaagaaagaataaaaaaagataaaaagaatagatcccagccctgtgtataactcactactttagtcagttccgcagtattacaaaaggatgtcgcaaacgctgtttgctcctctacaaaacagaccttaaaaccctaaaggcttaagtagcaccctcgcaagctcgggcaaatcgctgaatattccttttgtctccgaccatcaggcacctgagtcgctgtctttttcgtgacattcagttcgctgcgctcacggctctggcagtgaatgggggtaaatggcactacaggcgccttttatggattcatgcaaggaaactacccataatacaagaaaagcccgtcacgggcttctcagggcgttttatggcgggtctgctatgtggtgctatctgactttttgctgttcagcagttcctgccctctgattttccagtctgaccacttcggattatcccgtgacaggtcattcagactggctaatgcacccagtaaggcagcggtatcatcaacaggcttacccgtcttactgtcaagaggacatccggtcagataaccgtcatcttcggctactgtctagggcggcggatttgtcctactcaggagagcgttcaccgacaaacaacagataaaacgaaaggcccagtctttcgactgagcctttcgttttatttgatgcactagtgccgatcatattcaataacccttaatataacttcgtataatgtatgctatacgaagttattaggtctgaagaggagtttacgtcccatatggagtcccgcttacgccccgccctgccactcatcgcagtactgttgtaattcattaagcattctgccgacatggaagccatcacagacggcatgatgaacctgaatcgccagcggcatcagcaccttgtcgccttgcgtataatatttgcccatggtgaaaacgggggcgaagaagttgtccatattggccacgtttaaatcaaaactggtgaaactcacccagggattggctgagacgaaaaacatattctcaataaaccctttagggaaataggccaggttttcaccgtaacacgccacatcttgcgaatatatgtgtagaaactgccggaaatcgtcgtggtattcactccagagcgatgaaaacgtttcagtttgctcatggaaaacggtgtaacaagggtgaacactatcccatatcaccagctcaccgtctttcattgccatacgaaattccggatgagcattcatcaggcgggcaagaatgtgaataaaggccggataaaacttgtgcttatttttctttacggtctttaaaaaggccgtaatatccagctgaacggtctggttataggtacattgagcaactgactgaaatgcctcaaaatgttctttacgatgccattgggatatatcaacggtggtatatccagtgatttttttctccattttagcttccttagctcctgaaaatctcgataactcaaaaaatacgcccggtagtgatcttatttcattatggtgaaagttggaacctcttacgtgccgatcagacgtcattgcgttgctagccaagcttaggatccggaacccttaatataacttcgtataatgtatgctatacgaagttattaggtccctcgaagaggttcactagctatctagagcttggactcctgttgatagatccagtaatgacctcagaactccatctggatttgttcagaacgctcggttgccgccgggcgttttttattggtgagaatccaagcccgggaaacgggatcctgatcttgatcaaccgaggtcacaacatagtaaaagcgctattggtaatggtacaatcgcgcgtttacacttattcagaacgatttttttcaggagggcctacttgtcacacaggacggtaatgtcgtgcccggttattgagctgacacagcaacttattcgtcgcccctccctgagtccggatgacgcaggctgtcaggcattaatgattgaacgcctgcgtaaaatcggttttaccattgagcatatggattttggcgacacgcaaaatttttgggcatggcgtgggcgtggcgaaacgctggcgttcgccgggcatactgacgtcgtaccggctggcgatgtcgatcgctggatcaatccgccgtttgagcctacgattcgcgacggaatgttgttcggtcgcggcgcggcggatatgaaaggttcactggcggccatggtggtggctgctgaacgttttgttgcgcagcatcctcatcaccggggccgcctcgcatttttgattacctctgatgaggaagccagcgcaaaaaatggcaccgtaaaggtggttgaagcgctgatggcccgtaacgagcggctggattactgtctggtcggcgaaccttccagtactgaaattgtgggcgatgtcgtcaaaaacgggcgtcgcggttctctcacctgtaacctcactatccatggcgttcaggggcacgtcgcctatccgcatctggcggataaccctgttcatcgcgccgcgccttttcttaatgaactggtcgctatcgagtgggatcggggcaatgactttttcccggccaccagtatgcaggtagccaatatccaggcaggcaccggcagcaataatgtcattcccggcgaactgttcgtgcagtttaacttccgtttcagcacggaactgaccgatgagatgatcaaagagcgggtacatgcgctgcttgaaaagcatcagctacgctataccgtagactggtggctttccgggcagccgttcctgaccgcacgcggcaagctggtggacgcggtggtaaacgccattgagcactataatgaaattaaaccgcaattactgacgacgggcggtacgtccgacggacgttttatcgcccgtatgggagcgcaggtggtagaactggggccggtgaacgccaccattcataaaattaatgaatgtgtgaatgccgccgatctccagctactggcccgtatgtatcaacgcattatggaacagctcgtcgcccatcaccatcaccatcactaagattacttcgcattgcaatcagctacggactcaagcttacgtcaggtcatacgatgaaggcgataagtcgcgtaagttgctagcccacgcggctcaccttcacgggtgggcctttcttcgcgatccacatg

SEQ ID NO: 5 - DNA, 76 bp, synthetic construct
  source 1..76: mol_type = other DNA
ttcacagaaaagtgttgcccccttccatggcggaagggggacaaaggtgaatttgtcctactcaggagagcgttca

SEQ ID NO: 6 - DNA, 68 bp, synthetic construct
  source 1..68: mol_type = other DNA
tctgacgtacacagcaattttgcgttacctgttaatcgagattgaaacaccgaagaaaggcccacccg

SEQ ID NO: 7 - DNA, 72 bp, synthetic construct
  source 1..72: mol_type = other DNA
ttggtttcagtgaatcccgttatcagcagttttttgatgaggtgtagtctatttgtcctactcaggagagcg

SEQ ID NO: 8 - DNA, 68 bp, synthetic construct
  source 1..68: mol_type = other DNA
caatattttgccagccagtccatgcttatttcctcttaccggaacgctcacgaagaaaggcccacccg

SEQ ID NO: 9 - DNA, 85 bp, synthetic construct
  source 1..85: mol_type = other DNA
gcaggggtaaaagtgacctgacgcaatatttgtcttttcttgcttcttaataatgttgtcacaaaaagtgagggtgactacatgg

SEQ ID NO: 10 - DNA, 85 bp, synthetic construct
  source 1..85: mol_type = other DNA
cgccgcaaagtttgagcgaagtcaataaactctctacccattcagggcaatatctctcttgcaggtgaatgcaacgtcaagcgat

SEQ ID NO: 11 - DNA, 85 bp, synthetic construct
  source 1..85: mol_type = other DNA
tcagaagaagcaaaaagacactttaccgaagggtttaacattttttcgtgatactcatcaccatgacgcaaatgcgttgcataaa

SEQ ID NO: 12 - DNA, 85 bp, synthetic construct
  source 1..85: mol_type = other DNA
aaccgaggtcacaacatagtaaaagcgctattggtaatggtacaatcgcgcgtttacacttattcagaacgatttttttcaggag

SEQ ID NO: 13 - DNA, 54 bp, synthetic construct
  source 1..54: mol_type = other DNA
ggataaaagtgacctgacgcaatatttgtcttttcttgcttaataatgttgtca

SEQ ID NO: 14 - DNA, 35 bp, synthetic construct
  source 1..35: mol_type = other DNA
tgtaagtttatacataggcgagtactctgttatgg

SEQ ID NO: 15 - DNA, 74 bp, synthetic construct
  source 1..74: mol_type = other DNA
ttaaatttcctctcgtcaggccggaataactccctataatgcgccaccacactgatagtgctagtgtagatcac

SEQ ID NO: 16 - DNA, 58 bp, synthetic construct
  source 1..58: mol_type = other DNA
aaaattgatctgaatcaatattttgacaaaaattgatctgaatcaatatttactgagc

SEQ ID NO: 17 - DNA, 44 bp, synthetic construct
  source 1..44: mol_type = other DNA
gttaataaaatgttattgacagttaataaaatgttatactgagc

SEQ ID NO: 18 - DNA, 30 bp, synthetic construct
  source 1..30: mol_type = other DNA
ttagcacgttaattatctatcgtgtatatg

SEQ ID NO: 19 - protein, 118 aa, synthetic construct
EVQLVESGGGLVQAGESLRLSCAASGSTFDFKVMGWYRQPPGKQREGVAAIRLSGNMHYAESVKGRFAISKANAKNTVYLQMNSLRPEDTAVYYCKVNIRGQDYWGQGTQVTVSSGSG

SEQ ID NO: 20 - protein, 122 aa, synthetic construct
EVQLVESGGGLVQPGGSVRLSCVASGRIFSSNAMGWFRQAPGKEREFVAAITWRSGGSAYYADSAKGRFTISRDNAKNTVYLQMNSLKPEDTAVYYCAAGGSSWLSFPPDYWGQGTQVTVSS

SEQ ID NO: 21 - protein, 126 aa, synthetic construct
EVQLVESGGGLVQPGGSLRLSCVASGSIVRINTMGWYRQTPGKQRELVADITSGGNINYIDAVKGRFTISRDNTKKRVYLQMNSLKPEDTAVYYCNAEIVVLVGVWTQRARTGNYWGQGTQVTVSS

SEQ ID NO: 22 - DNA, 354 bp, synthetic construct
  source 1..354: mol_type = other DNA
gaggttcaattagtggaatctggcgggggattggttcaagccggtgagtccttgcgtttgagctgcgccgcatctgggagcacatttgatttcaaagtgatgggctggtatcgtcagccgcccggaaaacagcgcgagggtgtagcagccatccgcttgagcggaaatatgcactacgccgagtctgtaaaagggcgctttgctatttccaaagcgaacgctaagaacacagtgtatcttcagatgaactccttgcgtcccgaagacactgccgtttattattgcaaagtaaacatccgtgggcaagactactggggtcaaggaacgcaggtcacagtctcttctggctctggc

SEQ ID NO: 23 - DNA, 366 bp, synthetic construct
  source 1..366: mol_type = other DNA
gaggtgcagctggtggagtctgggggaggattggtgcagcctgggggctctgtgagactctcctgtgtagcctctggacgcatcttcagtagcaatgccatgggctggttccgccaggctccagggaaggagcgtgagtttgtagcggccattacctggaggagtggcggtagcgcgtactatgcagactccgcgaagggccgattcaccatctccagagacaacgccaagaacacggtgtatttgcaaatgaacagcctgaaacctgaggacacggccgtttattattgtgcagctggtggtagttcctggttaagttttccgccggactactggggccaggggacccaggtcaccgtctcctca

SEQ ID NO: 24 - DNA, 378 bp, synthetic construct
  source 1..378: mol_type = other DNA
gaggtgcagctggtggagtctgggggaggcttggtgcagcctggggggtctctgagactctcctgtgtagcctctggaagcatcgtcagaattaataccatgggctggtaccgccagactccagggaagcagcgcgagttggtcgcagatattaccagtggtggtaacataaactatatagacgccgtgaagggccgattcaccatctccagagacaacaccaagaagagggtgtatctgcaaatgaacagcctgaaacctgaggacacggccgtctattactgtaatgcagagatcgttgttctggtgggagtttggacccagcgtgcgcggaccggcaactactggggccaggggacccaggtcaccgtctcctca

SEQ ID NO: 25 - protein, 613 aa, synthetic construct
AEEAFDLWNECAKACVLDLKDGVRSSRMSVDPAIADTNGQGVLHYSMVLEGGNDALKLAIDNALSITSDGLTIRLEGGVEPNKPVRYSYTRQARGSWSLNWLVPIGHEKPSNIKVFIHELNAGNQLSHMSPIYTIEMGDELLAKLARDATFFVRAHESNEMQPTLAISHAGVSVVMAQTQPRREKRWSEWASGKVLCLLDPLDGVYNYLAQQRCNLDDTWEGKIYRVLAGNPAKHDLDIKPTVISHRLHFPEGGSLAALTAHQACHLPLETFTRHRQPRGWEQLEQCGYPVQRLVALYLAARLSWNQVDQVIRNALASPGSGGDLGEAIREQPEQARLALTLAAAESERFVRQGTGNDEAGAANADVVSLTCPVAAGECAGPADSGDALLERNYPTGAEFLGDGGDVSFSTRGTQNWTVERLLQAHRQLEERGYVFVGYHGTFLEAAQSIVFGGVRARSQDLDAIWRGFYIAGDPALAYGYAQDQEPDARGRIRNGALLRVYVPRSSLPGFYRTSLTLAAPEAAGEVERLIGHPLPLRLDAITGPEEEGGRLETILGWPLAERTVVIPSAIPTDPRNVGGDLDPSSIPDKEQAISALPDYASQPGKPPREDLK

SEQ ID NO: 26 - protein, 346 aa, synthetic construct
PEGGSLAALTAHQACHLPLETFTRHRQPRGWEQLEQCGYPVQRLVALYLAARLSWNQVDQVIRNALASPGSGGDLGEAIREQPEQARLALTLAAAESERFVRQGTGNDEAGAANGPADSGDALLERNYPTGAEFLGDGGDVSFSTRGTQNWTVERLLQAHRQLEERGYVFVGYHGTFLEAAQSIVFGGVRARSQDLDAIWRGFYIAGDPALAYGYAQDQEPDARGRIRNGALLRVYVPRSSLPGFYRTSLTLAAPEAAGEVERLIGHPLPLRLDAITGPEEEGGRLETILGWPLAERTVVIPSAIPTDPRNVGGDLDPSSIPDKEQAISALPDYASQPGKPPREDL

SEQ ID NO: 27 - protein, 230 aa, synthetic construct
RHRQPRGWEQLPTGAEFLGDGGDVSFSTRGTQNWTVERLLQAHRQLEERGYVFVGYHGTFLEAAQSIVFGGVRARSQDLDAIWRGFYIAGDPALAYGYAQDQEPDARGRIRNGALLRVYVPRSSLPGFYRTSLTLAAPEAAGEVERLIGHPLPLRLDAITGPEEEGGRLETILGWPLAERTVVIPSAIPTDPRNVGGDLDPSSIPDKEQAISALPDYASQPGKPPREDLK

SEQ ID NO: 28 - protein, 22 aa, synthetic construct
MKYLLPTAAAGLLLLAAQPAMA

SEQ ID NO: 29 - protein, 32 aa, synthetic construct
MGLKMKKRSGKKAWMLLVMSLLIAAVPITASA

SEQ ID NO: 30 - DNA, 5512 bp, synthetic construct
  source 1..5512: mol_type = other DNA
tggcgaatgggacgcgccctgtagcggcgcattaagcgcggcgggtgtggtggttacgcgcagcgtgaccgctacacttgccagcgccctagcgcccgctcctttcgctttcttcccttcctttctcgccacgttcgccggctttccccgtcaagctctaaatcgggggctccctttagggttccgatttagtgctttacggcacctcgaccccaaaaaacttgattagggtgatggttcacgtagtgggccatcgccctgatagacggtttttcgccctttgacgttggagtccacgttctttaatagtggactcttgttccaaactggaacaacactcaaccctatctcggtctattcttttgatttataagggattttgccgatttcggcctattggttaaaaaatgagctgatttaacaaaaatttaacgcgaattttaacaaaatattaacgcttacaatttaggtggcacttttcggggaaatgtgcgcggaacccctatttgtttatttttctaaatacattcaaatatgtatccgctcatgaattaattcttagaaaaactcatcgagcatcaaatgaaactgcaatttattcatatcaggattatcaataccatatttttgaaaaagccgtttctgtaatgaaggagaaaactcaccgaggcagttccataggatggcaagatcctggtatcggtctgcgattccgactcgtccaacatcaatacaacctattaatttcccctcgtcaaaaataaggttatcaagtgagaaatcaccatgagtgacgactgaatccggtgagaatggcaaaagtttatgcatttctttccagacttgttcaacaggccagccattacgctcgtcatcaaaatcactcgcatcaaccaaaccgttattcattcgtgattgcgcctgagcgagacgaaatacgcgatcgctgttaaaaggacaattacaaacaggaatcgaatgcaaccggcgcaggaacactgccagcgcatcaacaatattttcacctgaatcaggatattcttctaatacctggaatgctgttttcccggggatcgcagtggtgagtaaccatgcatcatcaggagtacggataaaatgcttgatggtcggaagaggcataaattccgtcagccagtttagtctgaccatctcatctgtaacatcattggcaacgctacctttgccatgtttcagaaacaactctggcgcatcgggcttcccatacaatcgatagattgtcgcacctgattgcccgacattatcgcgagcccatttatacccatataaatcagcatccatgttggaatttaatcgcggcctagagcaagacgtttcccgttgaatatggctcataacaccccttgtattactgtttatgtaagcagacagttttattgttcatgaccaaaatcccttaacgtgagttttcgttccactgagcgtcagaccccgtagaaaagatcaaaggatcttcttgagatcctttttttctgcgcgtaatctgctgcttgcaaacaaaaaaaccaccgctaccagcggtggtttgtttgccggatcaagagctaccaactctttttccgaaggtaactggcttcagcagagcgcagataccaaatactgtccttctagtgtagccgtagttaggccaccacttcaagaactctgtagcaccgcctacatacctcgctctgctaatcctgttaccagtggctgctgccagtggcgataagtcgtgtcttaccgggttggactcaagacgatagttaccggataaggcgcagcggtcgggctgaacggggggttcgtgcacacagcccagcttggagcgaacgacctacaccgaactgagatacctacagcgtgagctatgagaaagcgccacgcttcccgaagggagaaaggcggacaggtatccggtaagcggcagggtcggaacaggagagcgcacgagggagcttccagggggaaacgcctggtatctttatagtcctgtcgggtttcgccacctctgacttgagcgtcgatttttgtgatgctcgtcaggggggcggagcctatggaaaaacgccagcaacgcggcctttttacggttcctggccttttgctggccttttgctcacatgttctttcctgcgttatcccctgattctgtggataaccgtattaccgcctttgagtgagctgataccgctcgccgcagccgaacgaccgagcgcagcgagtcagtgagcgaggaagcggaagagcgcctgatgcggtattttctccttacgcatctgtgcggtatttcacaccgcaatggtgcactctcagtacaatctgctctgatgccgcatagttaagccagtatacactccgctatcgctacgtgactgggtcatggctgcgccccgacacccgccaacacccgctgacgcgccctgacgggcttgtctgctcccggcatccgcttacagacaagctgtgaccgtctccgggagctgcatgtgtgatgcctccgtgtaagggggatttctgttcatgggggtaatgataccgatgaaacgagagaggatgctcacgatacgggttactgatgatgaacatgcccggttactggaacgttgtgagggtaaacaactggcggtatggatgcggcgggaccagagaaaaatcactcagggtcaatgccagcgcttcgttaatacagatgtaggtgttccacagggtagccagcagcatcctgcgatgcagatccggaacataatggtgcagggcgctgacttccgcgtttccagactttacgaaacacggaaaccgaagaccattcatgttgttgctcaggtcgcagacgttttgcagcagcagtcgcttcacgttcgctcgcgtatcggtgattcattctgctaaccagtaaggcaaccccgccagcctagccgggtcctcaacgacaggagcacgatcatgcgcacccgtggggccgccatgccggcgataatggcctgcttctcgccgaaacgtttggtggcgggaccagtgacgaaggcttgagcgagggcgtgcaagattccgaataccgcaagcgacaggccgatcatcgtcgcgctccagcgaaagcggtcctcgccgaaaatgacccagagcgctgccggcacctgtcctacgagttgcatgataaagaagacagtcataagtgcggcgacgatagtcatgccccgcgcccaccggaaggagctgactgggttgaaggctctcaagggcatcggtcgagatcccggtgcctaatgagtgagctaacttacattaattgcgttgcgctcactgcccgctttccagtcgggaaacctgtcgtgccagctgcattaatgaatcggccaacgcgcggggagaggcggtttgcgtattgggcgccagggtggtttttcttttcaccagtgagacgggcaacagctgattgcccttcaccgcctggccctgagagagttgcagcaagcggtccacgctggtttgccccagcaggcgaaaatcctgtttgatggtggttaacggcgggatataacatgagctgtcttcggtatcgtcgtatcccactaccgagatatccgcaccaacgcgcagcccggactcggtaatggcgcgcattgcgcccagcgccatctgatcgttggcaaccagcatcgcagtgggaacgatgccctcattcagcatttgcatggtttgttgaaaaccggacatggcactccagtcgccttcccgttccgctatcggctgaatttgattgcgagtgagatatttatgccagccagccagacgcagacgcgccgagacagaacttaatgggcccgctaacagcgcgatttgctggtgacccaatgcgaccagatgctccacgcccagtcgcgtaccgtcttcatgggagaaaataatactgttgatgggtgtctggtcagagacatcaagaaataacgccggaacattagtgcaggcagcttccacagcaatggcatcctggtcatccagcggatagttaatgatcagcccactgacgcgttgcgcgagaagattgtgcaccgccgctttacaggcttcgacgccgcttcgttctaccatcgacaccaccacgctggcacccagttgatcggcgcgagatttaatcgccgcgacaatttgcgacggcgcgtgcagggccagactggaggtggcaacgccaatcagcaacgactgtttgcccgccagttgttgtgccacgcggttgggaatgtaattcagctccgccatcgccgcttccactttttcccgcgttttcgcagaaacgtggctggcctggttcaccacgcgggaaacggtctgataagagacaccggcatactctgcgacatcgtataacgttactggtttcacattcaccaccctgaattgactctcttccgggcgctatcatgccataccgcgaaaggttttgcgccattcgatggtgtccgggatctcgacgctctcccttatgcgactcctgcattaggaagcagcccagtagtaggttgaggccgttgagcaccgccgccgcaaggaatggtgcatgcaaggagatggcgcccaacagtcccccggccacggggcctgccaccatacccacgccgaaacaagcgctcatgagcccgaagtggcgagcccgatcttccccatcggtgatgtcggcgatataggcgccagcaaccgcacctgtggcgccggtgatgccggccacgatgcgtccggcgtagaggatcgagatctcgatcccgcgaaattaatacgactcactataggggaattgtgagcggataacaattcccctctagaaataattttgtttaactttaagaaggagatatacatatgaaatacctgctgccgaccgctgctgctggtctgctgctcctcgctgcccagccggcgatggccgaggtgcagctggtggagtctgggggaggcttggtgcagcctggggggtctctgagactctcctgtgtagcctctggaagcatcgtcagaattaataccatgggctggtaccgccagactccagggaagcagcgcgagttggtcgcagatattaccagtggtggtaacataaactatatagacgccgtgaagggccgattcaccatctccagagacaacaccaagaagagggtgtatctgcaaatgaacagcctgaaacctgaggacacggccgtctattactgtaatgcagagatcgttgttctggtgggagtttggacccagcgtgcgcggaccggcaactactggggccaggggacccaggtcaccgtctcctcatacccctatgacgtgcctgattacgccggctctggccaccaccaccaccaccactgagatccggctgctaacaaagcccgaaaggaagctgagttggctgctgccaccgctgagcaataactagcataaccccttggggcctctaaacgggtcttgaggggttttttgctgaaaggaggaactatatccggat

SEQ ID NO: 31 - DNA, 5500 bp, synthetic construct
  source 1..5500: mol_type = other DNA
tggcgaatgggacgcgccctgtagcggcgcattaagcgcggcgggtgtggtggttacgcgcagcgtgaccgctacacttgccagcgccctagcgcccgctcctttcgctttcttcccttcctttctcgccacgttcgccggctttccccgtcaagctctaaatcgggggctccctttagggttccgatttagtgctttacggcacctcgaccccaaaaaacttgattagggtgatggttcacgtagtgggccatcgccctgatagacggtttttcgccctttgacgttggagtccacgttctttaatagtggactcttgttccaaactggaacaacactcaaccctatctcggtctattcttttgatttataagggattttgccgatttcggcctattggttaaaaaatgagctgatttaacaaaaatttaacgcgaattttaacaaaatattaacgcttacaatttaggtggcacttttcggggaaatgtgcgcggaacccctatttgtttatttttctaaatacattcaaatatgtatccgctcatgaattaattcttagaaaaactcatcgagcatcaaatgaaactgcaatttattcatatcaggattatcaataccatatttttgaaaaagccgtttctgtaatgaaggagaaaactcaccgaggcagttccataggatggcaagatcctggtatcggtctgcgattccgactcgtccaacatcaatacaacctattaatttcccctcgtcaaaaataaggttatcaagtgagaaatcaccatgagtgacgactgaatccggtgagaatggcaaaagtttatgcatttctttccagacttgttcaacaggccagccattacgctcgtcatcaaaatcactcgcatcaaccaaaccgttattcattcgtgattgcgcctgagcgagacgaaatacgcgatcgctgttaaaaggacaattacaaacaggaatcgaatgcaaccggcgcaggaacactgccagcgcatcaacaatattttcacctgaatcaggatattcttctaatacctggaatgctgttttcccggggatcgcagtggtgagtaaccatgcatcatcaggagtacggataaaatgcttgatggtcggaagaggcataaattccgtcagccagtttagtctgaccatctcatctgtaacatcattggcaacgctacctttgccatgtttcagaaacaactctggcgcatcgggcttcccatacaatcgatagattgtcgcacctgattgcccgacattatcgcgagcccatttatacccatataaatcagcatccatgttggaatttaatcgcggcctagagcaagacgtttcccgttgaatatggctcataacaccccttgtattactgtttatgtaagcagacagttttattgttcatgaccaaaatcccttaacgtgagttttcgttccactgagcgtcagaccccgtagaaaagatcaaaggatcttcttgagatcctttttttctgcgcgtaatctgctgcttgcaaacaaaaaaaccaccgctaccagcggtggtttgtttgccggatcaagagctaccaactctttttccgaaggtaactggcttcagcagagcgcagataccaaatactgtccttctagtgtagccgtagttaggccaccacttcaagaactctgtagcaccgcctacatacctcgctctgctaatcctgttaccagtggctgctgccagtggcgataagtcgtgtcttaccgggttggactcaagacgatagttaccggataaggcgcagcggtcgggctgaacggggggttcgtgcacacagcccagcttggagcgaacgacctacaccgaactgagatacctacagcgtgagctatgagaaagcgccacgcttcccgaagggagaaaggcggacaggtatccggtaagcggcagggtcggaacaggagagcgcacgagggagcttccagggggaaacgcctggtatctttatagtcctgtcgggtttcgccacctctgacttgagcgtcgatttttgtgatgctcgtcaggggggcggagcctatggaaaaacgccagcaacgcggcctttttacggttcctggccttttgctggccttttgctcacatgttctttcctgcgttatcccctgattctgtggataaccgtattaccgcctttgagtgagctgataccgctcgccgcagccgaacgaccgagcgcagcgagtcagtgagcgaggaagcggaagagcgcctgatgcggtattttctccttacgcatctgtgcggtatttcacaccgcaatggtgcactctcagtacaatctgctctgatgccgcatagttaagccagtatacactccgctatcgctacgtgactgggtcatggctgcgccccgacacccgccaacacccgctgacgcgccctgacgggcttgtctgctcccggcatccgcttacagacaagctgtgaccgtctccgggagctgcatgtgtgatgcctccgtgtaagggggatttctgttcatgggggtaatgataccgatgaaacgagagaggatgctcacgatacgggttactgatgatgaacatgcccggttactggaacgttgtgagggtaaacaactggcggtatggatgcggcgggaccagagaaaaatcactcagggtcaatgccagcgcttcgttaatacagatgtaggtgttccacagggtagccagcagcatcctgcgatgcagatccggaacataatggtgcagggcgctgacttccgcgtttccagactttacgaaacacggaaaccgaagaccattcatgttgttgctcaggtcgcagacgttttgcagcagcagtcgcttcacgttcgctcgcgtatcggtgattcattctgctaaccagtaaggcaaccccgccagcctagccgggtcctcaacgacaggagcacgatcatgcgcacccgtggggccgccatgccggcgataatggcctgcttctcgccgaaacgtttggtggcgggaccagtgacgaaggcttgagcgagggcgtgcaagattccgaataccgcaagcgacaggccgatcatcgtcgcgctccagcgaaagcggtcctcgccgaaaatgacccagagcgctgccggcacctgtcctacgagttgcatgataaagaagacagtcataagtgcggcgacgatagtcatgccccgcgcccaccggaaggagctgactgggttgaaggctctcaagggcatcggtcgagatcccggtgcctaatgagtgagctaacttacattaattgcgttgcgctcactgcccgctttccagtcgggaaacctgtcgtgccagctgcattaatgaatcggccaacgcgcggggagaggcggtttgcgtattgggcgccagggtggtttttcttttcaccagtgagacgggcaacagctgattgcccttcaccgcctggccctgagagagttgcagcaagcggtccacgctggtttgccccagcaggcgaaaatcctgtttgatggtggttaacggcgggatataacatgagctgtcttcggtatcgtcgtatcccactaccgagatatccgcaccaacgcgcagcccggactcggtaatggcgcgcattgcgcccagcgccatctgatcgttggcaaccagcatcgcagtgggaacgatgccctcattcagcatttgcatggtttgttgaaaaccggacatggcactccagtcgccttcccgttccgctatcggctgaatttgattgcgagtgagatatttatgccagccagccagacgcagacgcgccgagacagaacttaatgggcccgctaacagcgcgatttgctggtgacccaatgcgaccagatgctccacgcccagtcgcgtaccgtcttcatgggagaaaataatactgttgatgggtgtctggtcagagacatcaagaaataacgccggaacattagtgcaggcagcttccacagcaatggcatcctggtcatccagcggatagttaatgatcagcccactgacgcgttgcgcgagaagattgtgcaccgccgctttacaggcttcgacgccgcttcgttctaccatcgacaccaccacgctggcacccagttgatcggcgcgagatttaatcgccgcgacaatttgcgacggcgcgtgcagggccagactggaggtggcaacgccaatcagcaacgactgtttgcccgccagttgttgtgccacgcggttgggaatgtaattcagctccgccatcgccgcttccactttttcccgcgttttcgcagaaacgtggctggcctggttcaccacgcgggaaacggtctgataagagacaccggcatactctgcgacatcgtataacgttactggtttcacattcaccaccctgaattgactctcttccgggcgctatcatgccataccgcgaaaggttttgcgccattcgatggtgtccgggatctcgacgctctcccttatgcgactcctgcattaggaagcagcccagtagtaggttgaggccgttgagcaccgccgccgcaaggaatggtgcatgcaaggagatggcgcccaacagtcccccggccacggggcctgccaccatacccacgccgaaacaagcgctcatgagcccgaagtggcgagcccgatcttccccatcggtgatgtcggcgatataggcgccagcaaccgcacctgtggcgccggtgatgccggccacgatgcgtccggcgtagaggatcgagatctcgatcccgcgaaattaatacgactcactataggggaattgtgagcggataacaattcccctctagaaataattttgtttaactttaagaaggagatatacatatgaaatacctgctgccgaccgctgctgctggtctgctgctcctcgctgcccagccggcgatggccgaggtgcagctggtggagtctgggggaggattggtgcagcctgggggctctgtgagactctcctgtgtagcctctggacgcatcttcagtagcaatgccatgggctggttccgccaggctccagggaaggagcgtgagtttgtagcggccattacctggaggagtggcggtagcgcgtactatgcagactccgcgaagggccgattcaccatctccagagacaacgccaagaacacggtgtatttgcaaatgaacagcctgaaacctgaggacacggccgtttattattgtgcagctggtggtagttcctggttaagttttccgccggactactggggccaggggacccaggtcaccgtctcctcatacccctatgacgtgcctgattacgccggctctggccaccaccaccaccaccactgagatccggctgctaacaaagcccgaaaggaagctgagttggctgctgccaccgctgagcaataactagcataaccccttggggcctctaaacgggtcttgaggggttttttgctgaaaggaggaactatatccggat

SEQ ID NO: 32 - DNA, 5512 bp, synthetic construct; identical to SEQ ID NO: 30
  source 1..5512: mol_type = other DNA

SEQ ID NO: 33 - DNA, 4493 bp, synthetic construct
  source 1..4493: mol_type = other DNA
ctggaagatccgcgcgtaccgagttctaattcactggccgtcgttttacaacatacgatgaaggcgataagtcgcgtaagttgctagcccacgcggctcaccttcacgggtgggcctttcttcgcgatccacatgcatggtcatagctgtttcctttaatgcccatggcgtttaccaatgcttaatcagtgaggcacctatctcagcgatctgtctatttcgttcatccatagttgcctgactccccgtcgtgtagataactacgatacgggagggcttaccatctggccccagtgctgcaatgataccgcgacttccacgctcaccggctccagatttatcagcaataaaccagccagccggaagggccgagcgcagaagtggtcctgcaactttatccgcctccatccagtctattaattgttgccgggaagctagagtaagtagttcgccagttaatagtttgcgcaacgttgttgccattgctacaggcatcgtggtgtcacgctcgtcgtttggtatggcttcattcagctccggttcccaacgatcaaggcgagttacatgatcccccatgttgtgcaaaaaagcggttagctccttcggtcctccgatcgttgtcagaagtaagttggccgcagtgttatcactcatggttatggcagcactgcataattctcttactgtcatgccatccgtaagatgcttttctgtgactggtgagtactcaaccaagtcattctgagaatagtgtatgcggcgaccgagttgctcttgcccggcgtcaatacgggataataccgcgccacatagcagaactttaaaagtgctcatcattggaaaacgttcttcggggcgaaaactctcaaggatcttaccgctgttgagatccagttcgatgtaacccactcgtgcacccaactgatcttcagcatcttttactttcaccagcgtttctgggtgagcaaaaacaggaaggcaaaatgccgcaaaaaagggaataagggcgacacggaaatgttgaatactcatactcttcctttttcaatattattgaagcatttatcagggttattgtctcatgagcggatacatatttgaatgtatttagaaaaataaacaaataggggttccgcgcacatttccccgaaaagtgccacctgacgtctaagaaaccattattatcatgacattaacctataaaaataggcgtatcacgaggcccttaggccaaataggccgttcagatccttccgtatttagccagtatgttctctagtgtggttcgttgtttttgcgtgagccatgagaacgaaccattgagatcatgcttactttgcatgtcactcaaaaattttgcctcaaaactggtgagctgaatttttgcagttaaagcatcgtgtagtgtttttcttagtccgttacgtaggtaggaatctgatgtaatggttgttggtattttgtcaccattcatttttatctggttgttctcaagttcggttacgagatccatttgtctatctagttcaacttggaaaatcaacgtatcagtcgggcggcctcgcttatcaaccaccaatttcatattgctgtaagtgtttaaatctttacttattggtttcaaaacccattggttaagccttttaaactcatggtagttattttcaagcattaacatgaacttaaattcatcaaggctaatctctatatttgccttgtgagttttcttttgtgttagttcttttaataaccactcataaatcctcatagagtatttgttttcaaaagacttaacatgttccagattatattttatgaatttttttaactggaaaagataaggcaatatctcttcactaaaaactaattctaatttttcgcttgagaacttggcatagtttgtccactggaaaatctcaaagcctttaaccaaaggattcctgatttccacagttctcgtcatcagctctctggttgctttagctaatacaccataagcattttccctactgatgttcatcatctgagcgtattggttataagtgaacgataccgtccgttctttccttgtagggttttcaatcgtggggttgagtagtgccacacagcataaaattagcttggtttcatgctccgttaagtcatagcgactaatcgctagttcatttgctttgaaaacaactaattcagacatacatctcaattggtctaggtgattttaatcactataccaattgagatgggctagtcaatgataattactagtccttttcctttgagttgtgggtatctgtaaattctgctagacctttgctggaaaacttgtaaattctgctagaccctctgtaaattccgctagacctttgtgtgttttttttgtttatattcaagtggttataatttatagaataaagaaagaataaaaaaagataaaaagaatagatcccagccctgtgtataactcactactttagtcagttccgcagtattacaaaaggatgtcgcaaacgctgtttgctcctctacaaaacagaccttaaaaccctaaaggcttaagtagcaccctcgcaagctcgggcaaatcgctgaatattccttttgtctccgaccatcaggcacctgagtcgctgtctttttcgtgacattcagttcgctgcgctcacggctctggcagtgaatgggggtaaatggcactacaggcgccttttatggattcatgcaaggaaactacccataatacaagaaaagcccgtcacgggcttctcagggcgttttatggcgggtctgctatgtggtgctatctgactttttgctgttcagcagttcctgccctctgattttccagtctgaccacttcggattatcccgtgacaggtcattcagactggctaatgcacccagtaaggcagcggtatcatcaacaggcttacccgtcttactgtcaagaggacatccggtcagataaccgtcatcttcggctactgtctagggcggcggatttgtcctactcaggagagcgttcaccgacaaacaacagataaaacgaaaggcccagtctttcgactgagcctttcgttttatttgatgcactagtgccgatcatattcaataacccttaatataacttcgtataatgtatgctatacgaagttattaggtctgaagaggagtttacgtcccatatggagtcccgctcagaagaactcgtcaagaaggcgatagaaggcgatgcgctgcgaatcgggagcggcgataccgtaaagcacgaggaagcggtcagcccattcgccgccaagctcttcagcaatatcacgggtagccaacgctatgtcctgatagcggtccgccacacccagccggccacagtcgatgaatccagaaaagcggccattttccaccatgatattcggcaagcaggcatcgccatgggtcacgacgagatcctcgccgtcgggcatgcgcgccttgagcctggcgaacagttcggccggcgcgagcccctgatgctcttcgtccagatcatcctgatcgacaagaccggcttccatccgagtacgtgctcgctcgatgcgatgtttcgcttggtggtcgaatgggcaggtagccggatcaagcgtatgcagccgccgcattgcatcagccatgatggatactttctcggcaggagcaaggtgagatgacaggagatcctgccccggcacttcgcccaatagcagccagtcccttcccgcttcagtgacaacgtcgagcacagctgcgcaaggaacgcccgtcgtggccagccacgatagccgcgctgcctcgtcctgcagttcattcagggcaccggacaggtcggtcttgacaaaaagaaccgggcgcccctgcgctgacagccggaacacggcggcatcagagcagccgattgtctgttgtgcccagtcatagccgaatagcctctccacccaagcggccggagaacctgcgtgcaatccatcttgttcaatcatgcgaaacgatcctcatcctgtctcttgatcagatcctgatcccctgcgccatcagatccttggcggcaagaaagccatccagtttactttgcagggcttcccaaccttaccagagggcgccccagctggcaattccgacgtcattgcgttgctagccaagcttaggatccggaacccttaatataacttcgtataatgtatgctatacgaagttattaggtccctcgaagaggttcactagctatctagagcttggactcctgttgatagatccagtaatgacctcagaactccatctggatttgttcagaacgctcggttgccgccgggcgttttttattggtgagaatccaagcccgggaaacgggatcctgatcttgatccgccgcaaagtttgagcgaagtcaataaactctctacccattcagggcaatatctctcttgcaggtgaatgcaacgtcaagcgatggcctacttgcggccgcaagattaaagaggagaagg

SEQ ID NO: 34 - DNA, 5518 bp, synthetic construct
  source 1..5518: mol_type = other DNA
tggcgaatgggacgcgccctgtagcggcgcattaagcgcggcgggtgtggtggttacgcgcagcgtgaccgctacacttgccagcgccctagcgcccgctcctttcgctttcttcccttcctttctcgccacgttcgccggctttccccgtcaagctctaaatcgggggctccctttagggttccgatttagtgctttacggcacctcgaccccaaaaaacttgattagggtgatggttcacgtagtgggccatcgccctgatagacggtttttcgccctttgacgttggagtccacgttctttaatagtggactcttgttccaaactggaacaacactcaaccctatctcggtctattcttttgatttataagggattttgccgatttcggcctattggttaaaaaatgagctgatttaacaaaaatttaacgcgaattttaacaaaatattaacgcttacaatttaggtggcacttttcggggaaatgtgcgcggaacccctatttgtttatttttctaaatacattcaaatatgtatccgctcatgaattaattcttagaaaaactcatcgagcatcaaatgaaactgcaatttattcatatcaggattatcaataccatatttttgaaaaagccgtttctgtaatgaaggagaaaactcaccgaggcagttccataggatggcaagatcctggtatcggtctgcgattccgactcgtccaacatcaatacaacctattaatttcccctcgtcaaaaataaggttatcaagtgagaaatcaccatgagtgacgactgaatccggtgagaatggcaaaagtttatgcatttctttccagacttgttcaacaggccagccattacgctcgtcatcaaaatcactcgcatcaaccaaaccgttattcattcgtgattgcgcctgagcgagacgaaatacgcgatcgctgttaaaaggacaattacaaacaggaatcgaatgcaaccggcgcaggaacactgccagcgcatcaacaatattttcacctgaatcaggatattcttctaatacctggaatgctgttttcccggggatcgcagtggtgagtaaccatgcatcatcaggagtacggataaaatgcttgatggtcggaagaggcataaattccgtcagccagtttagtctgaccatctcatctgtaacatcattggcaacgctacctttgccatgtttcagaaacaactctggcgcatcgggcttcccatacaatcgatagattgtcgcacctgattgcccgacattatcgcgagcccatttatacccatataaatcagcatccatgttggaatttaatcgcggcctagagcaagacgtttcccgttgaatatggctcataacaccccttgtattactgtttatgtaagcagacagttttattgttcatgaccaaaatcccttaacgtgagttttcgttccactgagcgtcagaccccgtagaaaagatcaaaggatcttcttgagatcctttttttctgcgcgtaatctgctgcttgcaaacaaaaaaaccaccgctaccagcggtggtttgtttgccggatcaagagctaccaactctttttccgaaggtaactggcttcagcagagcgcagataccaaatactgtccttctagtgtagccgtagttaggccaccacttcaagaactctgtagcaccgcctacatacctcgctctgctaatcctgttaccagtggctgctgccagtggcgataagtcgtgtcttaccgggttggactcaagacgatagttaccggataaggcgcagcggtcgggctgaacggggggttcgtgcacacagcccagcttggagcgaacgacctacaccgaactgagatacctacagcgtgagctatgagaaagcgccacgcttcccgaagggagaaaggcggacaggtatccggtaagcggcagggtcggaacaggagagcgcacgagggagcttccagggggaaacgcctggtatctttatagtcctgtcgggtttcgccacctctgacttgagcgtcgatttttgtgatgctcgtcaggggggcggagcctatggaaaaacgccagcaacgcggcctttttacggttcctggccttttgctggccttttgctcacatgttctttcctgcgttatcccctgattctgtggataaccgtattaccgcctttgagtgagctgataccgctcgccgcagccgaacgaccgagcgcagcgagtcagtgagcgaggaagcggaagagcgcctgatgcggtattttctccttacgcatctgtgcggtatttcacaccgcaatggtgcactctcagtacaatctgctctgatgccgcatagttaagccagtatacactccgctatcgctacgtgactgggtcatggctgcgccccgacacccgccaacacccgctgacgcgccctgacgggcttgtctgctcccggcatccgcttacagacaagctgtgaccgtctccgggagctgcatgtgtgatgcctccgtgtaagggggatttctgttcatgggggtaatgataccgatgaaacgagagaggatgctcacgatacgggttactgatgatgaacatgcccggttactggaacgttgtgagggtaaacaactggcggtatggatgcggcgggaccagagaaaaatcactcagggtcaatgccagcgcttcgttaatacagatgtaggtgttccacagggtagccagcagcatcctgcgatgcagatccggaacataatggtgcagggcgctgacttccgcgtttccagactttacgaaacacggaaaccgaagaccattcatgttgttgctcaggtcgcagacgttttgcagcagcagtcgcttcacgttcgctcgcgtatcggtgattcattctgctaaccagtaaggcaaccccgccagcctagccgggtcctcaacgacaggagcacgatcatgcgcacccgtggggccgccatgccggcgataatggcctgcttctcgccgaaacgtttggtggcgggaccagtgacgaaggcttgagcgagggcgtgcaagattccgaataccgcaagcgacaggccgatcatcgtcgcgctccagcgaaagcggtcctcgccgaaaatgacccagagcgctgccggcacctgtcctacgagttgcatgataaagaagacagtcataagtgcggcgacgatagtcatgccccgcgcccaccggaaggagctgactgggttgaaggctctcaagggcatcggtcgagatcccggtgcctaatgagtgagctaacttacattaattgcgttgcgctcactgcccgctttccagtcgggaaacctgtcgtgccagctgcattaatgaatcggccaacgcgcggggagaggcggtttgcgtattgggcgccagggtggtttttcttttcaccagtgagacgggcaacagctgattgcccttcaccgcctggccctgagagagttgcagcaagcggtccacgctggtttgccccagcaggcgaaaatcctgtttgatggtggttaacggcgggatataacatgagctgtcttcggtatcgtcgtatcccactaccgagatatccgcaccaacgcgcagcccggactcggtaatggcgcgcattgcgcccagcgccatctgatcgttggcaaccagcatcgcagtgggaacgatgccctcattcagcatttgcatggtttgttgaaaaccggacatggcactccagtcgccttcccgttccgctatcggctgaatttgattgcgagtgagatatttatgccagccagccagacgcagacgcgccgagacagaacttaatgggcccgctaacagcgcgatttgctggtgacccaatgcgaccagatgctccacgcccagtcgcgtaccgtcttcatgggagaaaataatactgttgatgggtgtctggtcagagacatcaagaaataacgccggaacattagtgcaggcagcttccacagcaatggcatcctggtcatccagcggatagttaatgatcagcccactgacgcgttgcgcgagaagattgtgcaccgccgctttacaggcttcgacgccgcttcgttctaccatcgacaccaccacgctggcacccagttgatcggcgcgagatttaatcgccgcgacaatttgcgacggcgcgtgcagggccagactggaggtggcaacgccaatcagcaacgactgtttgcccgccagttgttgtgccacgcggttgggaatgtaattcagctccgccatcgccgcttccactttttcccgcgttttcgcagaaacgtggctggcctggttcaccacgcgggaaacggtctgataagagacaccggcatactctgcgacatcgtataacgttactggtttcacattcaccaccctgaattgactctcttccgggcgctatcatgccataccgcgaaaggttttgcgccattcgatggtgtccgggatctcgacgctctcccttatgcgactcctgcattaggaagcagcccagtagtaggttgaggccgttgagcaccgccgccgcaaggaatggtgcatgcaaggagatggcgcccaacagtcccccggccacggggcctgccaccatacccacgccgaaacaagcgctcatgagcccgaagtggcgagcccgatcttccccatcggtgatgtcggcgatataggcgccagcaaccgcacctgtggcgccggtgatgccggccacgatgcgtccggcgtagaggatcgagatctcgatcccgcgaaattaatacgactcactataggggaattgtgagcggataacaattcccctctagaaataattttgtttaactttaagaaggagatatacatatgggcctgaaaatgaaaaaacgtagcgggaaaaaagcgtggatgctgctggttatgtcgctgctgattgcggcggttccgattacggcgagcgccgaggttcaattagtggaatctggcgggggattggttcaagccggtgagtccttgcgtttgagctgcgccgcatctgggagcacatttgatttcaaagtgatgggctggtatcgtcagccgcccggaaaacagcgcgagggtgtagcagccatccgcttgagcggaaatatgcactacgccgagtctgtaaaagggcgctttgctatttccaaagcgaacgctaagaacacagtgtatcttcagatgaactccttgcgtcccgaagacactgccgtttattattgcaaagtaaacatccgtgggcaagactactggggtcaaggaacgcaggtcacagtctcttctggctctggctacccctatgacgtgcctgattacgccggctctggccaccaccaccaccaccactgagatccggctgctaacaaagcccgaaaggaagctgagttggctgctgccaccgctgagcaataactagcataaccccttggggcctctaaacgggtcttgaggggttttttgctgaaaggaggaactatatccggat

SEQ ID NO: 35 - DNA, 5530 bp, synthetic construct
  source 1..5530: mol_type = other DNA
tggcgaatgggacgcgccctgtagcggcgcattaagcgcggcgggtgtggtggttacgcgcagcgtgaccgctacacttgccagcgccctagcgcccgctcctttcgctttcttcccttcctttctcgccacgttcgccggctttccccgtcaagctctaaatcgggggctccctttagggttccgatttagtgctttacggcacctcgaccccaaaaaacttgattagggtgatggttcacgtagtgggccatcgccctgatagacggtttttcgccctttgacgttggagtccacgttctttaatagtggactcttgttccaaactggaacaacactcaaccctatctcggtctattcttttgatttataagggattttgccgatttcggcctattggttaaaaaatgagctgatttaacaaaaatttaacgcgaattttaacaaaatattaacgcttacaatttaggtggcacttttcggggaaatgtgcgcggaacccctatttgtttatttttctaaatacattcaaatatgtatccgctcatgaattaattcttagaaaaactcatcgagcatcaaatgaaactgcaatttattcatatcaggattatcaataccatatttttgaaaaagccgtttctgtaatgaaggagaaaactcaccgaggcagttccataggatggcaagatcctggtatcggtctgcgattccgactcgtccaacatcaatacaacctattaatttcccctcgtcaaaaataaggttatcaagtgagaaatcaccatgagtgacgactgaatccggtgagaatggcaaaagtttatgcatttctttccagacttgttcaacaggccagccattacgctcgtcatcaaaatcactcgcatcaaccaaaccgttattcattcgtgattgcgcctgagcgagacgaaatacgcgatcgctgttaaaaggacaattacaaacaggaatcgaatgcaaccggcgcaggaacactgccagcgcatcaacaatattttcacctgaatcaggatattcttctaatacctggaatgctgttttcccggggatcgcagtggtgagtaaccatgcatcatcaggagtacggataaaatgcttgatggtcggaagaggcataaattccgtcagccagtttagtctgaccatctcatctgtaacatcattggcaacgctacctttgccatgtttcagaaacaactctggcgcatcgggcttcccatacaatcgatagattgtcgcacctgattgcccgacattatcgcgagcccatttatacccatataaatcagcatccatgttggaatttaatcgcggcctagagcaagacgtttcccgttgaatatggctcataacaccccttgtattactgtttatgtaagcagacagttttattgttcatgaccaaaatcccttaacgtgagttttcgttccactgagcgtcagaccccgtagaaaagatcaaaggatcttcttgagatcctttttttctgcgcgtaatctgctgcttgcaaacaaaaaaaccaccgctaccagcggtggtttgtttgccggatcaagagctaccaactctttttccgaaggtaactggcttcagcagagcgcagataccaaatactgtccttctagtgtagccgtagttaggccaccacttcaagaactctgtagcaccgcctacatacctcgctctgctaatcctgttaccagtggctgctgccagtggcgataagtcgtgtcttaccgggttggactcaagacgatagttaccggataaggcgcagcggtcgggctgaacggggggttcgtgcacacagcccagcttggagcgaacgacctacaccgaactgagatacctacagcgtgagctatgagaaagcgccacgcttcccgaagggagaaaggcggacaggtatccggtaagcggcagggtcggaacaggagagcgcacgagggagcttccagggggaaacgcctggtatctttatagtcctgtcgggtttcgccacctctgacttgagcgtcgatttttgtgatgctcgtcaggggggcggagcctatggaaaaacgccagcaacgcggcctttttacggttcctggccttttgctggccttttgctcacatgttctttcctgcgttatcccctgattctgtggataaccgtattaccgcctttgagtgagctgataccgctcgccgcagccgaacgaccgagcgcagcgagtcagtgagcgaggaagcggaagagcgcctgatgcggtattttctccttacgcatctgtgcggtatttcacaccgcaatggtgcactctcagtacaatctgctctgatgccgcatagttaagccagtatacactccgctatcgctacgtgactgggtcatggctgcgccccgacacccgccaacacccgctgacgcgccctgacgggcttgtctgctcccggcatccgcttacagacaagctgtgaccgtctccgggagctgcatgtgtgatgcctccgtgtaagggggatttctgttcatgggggtaatgataccgatgaaacgagagaggatgctcacgatacgggttactgatgatgaacatgcccggttactggaacgttgtgagggtaaacaactggcggtatggatgcggcgggaccagagaaaaatcactcagggtcaatgccagcgcttcgttaatacagatgtaggtgttccacagggtagccagcagcatcctgcgatgcagatccggaacataatggtgcagggcgctgacttccgcgtttccagactttacgaaacacggaaaccgaagaccattcatgttgttgctcaggtcgcagacgttttgcagcagcagtcgcttcacgttcgctcgcgtatcggtgattcattctgctaaccagtaaggcaaccccgccagcctagccgggtcctcaacgacaggagcacgatcatgcgcacccgtggggccgccatgccggcgataatggcctgcttctcgccgaaacgtttggtggcgggaccagtgacgaaggcttgagcgagggcgtgcaagattccgaataccgcaagcgacaggccgatcatcgtcgcgctccagcgaaagcggtcctcgccgaaaatgacccagagcgctgccggcacctgtcctacgagttgcatgataaagaagacagtcataagtgcggcgacgatagtcatgccccgcgcccaccggaaggagctgactgggttgaaggctctcaagggcatcggtcgagatcccggtgcctaatgagtgagctaacttacattaattgcgttgcgctcactgcccgctttccagtcgggaaacctgtcgtgccagctgcattaatgaatcggccaacgcgcggggagaggcggtttgcgtattgggcgccagggtggtttttcttttcaccagtgagacgggcaacagctgattgcccttcaccgcctggccctgagagagttgcagcaagcggtccacgctggtttgccccagcaggcgaaaatcctgtttgatggtggttaacggcgggatataacatgagctgtcttcggtatcgtcgtatcccactaccgagatatccgcaccaacgcgcagcccggactcggtaatggcgcgcattgcgcccagcgccatctgatcgttggcaaccagcatcgcagtgggaacgatgccctcattcagcatttgcatggtttgttgaaaaccggacatggcactccagtcgccttcccgttccgctatcggctgaatttgattgcgagtgagatatttatgccagccagccagacgcagacgcgccgagacagaacttaatgggcccgctaacagcgcgatttgctggtgacccaatgcgaccagatgctccacgcccagtcgcgtaccgtcttcatgggagaaaataatactgttgatgggtgtctggtcagagacatcaagaaataacgccggaacattagtgcaggcagcttccacagcaatggcatcctggtcatccagcggatagttaatgatcagcccactgacgcgttgcgcgagaagattgtgcaccgccgctttacaggcttcgacgccgcttcgttctaccatcgacaccaccacgctggcacccagttgatcggcgcgagatttaatcgccgcgacaatttgcgacggcgcgtgcagggccagactggaggtggcaacgccaatcagcaacgactgtttgcccgccagttgttgtgccacgcggttgggaatgtaattcagctccgccatcgccgcttccactttttcccgcgttttcgcagaaacgtggctggcctggttcaccacgcgggaaacggtctgataagagacaccggcatactctgcgacatcgtataacgttactggtttcacattcaccaccctgaattgactctcttccgggcgctatcatgccataccgcgaaaggttttgcgccattcgatggtgtccgggatctcgacgctctcccttatgcgactcctgcattaggaagcagcccagtagtaggttgaggccgttgagcaccgccgccgcaaggaatggtgcatgcaaggagatggcgcccaacagtcccccggccacggggcctgccaccatacccacgccgaaacaagcgctcatgagcccgaagtggcgagcccgatcttccccatcggtgatgtcggcgatataggcgccagcaaccgcacctgtggcgccggtgatgccggccacgatgcgtccggcgtagaggatcgagatctcgatcccgcgaaattaatacgactcactataggggaattgtgagcggataacaattcccctctagaaataattttgtttaactttaagaaggagatatacatatgggcctgaaaatgaaaaaacgtagcgggaaaaaagcgtggatgctgctggttatgtcgctgctgattgcggcggttccgattacggcgagcgccgaggtgcagctggtggagtctgggggaggattggtgcagcctgggggctctgtgagactctcctgtgtagcctctggacgcatcttcagtagcaatgccatgggctggttccgccaggctccagggaaggagcgtgagtttgtagcggccattacctggaggagtggcggtagcgcgtactatgcagactccgcgaagggccgattcaccatctccagagacaacgccaagaacacggtgtatttgcaaatgaacagcctgaaacctgaggacacggccgtttattattgtgcagctggtggtagttcctggttaagttttccgccggactactggggccaggggacccaggtcaccgtctcctcatacccctatgacgtgcctgattacgccggctctggccaccaccaccaccaccactgagatccggctgctaacaaagcccgaaaggaagctgagttggctgctgccaccgctgagcaataactagcataaccccttggggcctctaaacgggtcttgaggggttttttgctgaaaggaggaactatatccggat

SEQ ID NO: 36 - DNA, 5542 bp, synthetic construct
  source 1..5542: mol_type = other DNA
tggcgaatgggacgcgccctgtagcggcgcattaagcgcggcgggtgtggtggttacgcgcagcgtgaccgctacacttgccagcgccctagcgcccgctcctttcgctttcttcccttcctttctcgccacgttcgccggctttccccgtcaagctctaaatcgggggctccctttagggttccgatttagtgctttacggcacctcgaccccaaaaaacttgattagggtgatggttcacgtagtgggccatcgccctgatagacggtttttcgccctttgacgttggagtccacgttctttaatagtggactcttgttccaaactggaacaacactcaaccctatctcggtctattcttttgatttataagggattttgccgatttcggcctattggttaaaaaatgagctgatttaacaaaaatttaacgcgaattttaacaaaatattaacgcttacaatttaggtggcacttttcggggaaatgtgcgcggaacccctatttgtttatttttctaaatacattcaaatatgtatccgctcatgaattaattcttagaaaaactcatcgagcatcaaatgaaactgcaatttattcatatcaggattatcaataccatatttttgaaaaagccgtttctgtaatgaaggagaaaactcaccgaggcagttccataggatggcaagatcctggtatcggtctgcgattccgactcgtccaacatcaatacaacctattaatttcccctcgtcaaaaataaggttatcaagtgagaaatcaccatgagtgacgactgaatccggtgagaatggcaaaagtttatgcatttctttccagacttgttcaacaggccagccattacgctcgtcatcaaaatcactcgcatcaaccaaaccgttattcattcgtgattgcgcctgagcgagacgaaatacgcgatcgctgttaaaaggacaattacaaacaggaatcgaatgcaaccggcgcaggaacactgccagcgcatcaacaatattttcacctgaatcaggatattcttctaatacctggaatgctgttttcccggggatcgcagtggtgagtaaccatgcatcatcaggagtacggataaaatgcttgatggtcggaagaggcataaattccgtcagccagtttagtctgaccatctcatctgtaacatcattggcaacgctacctttgccatgtttcagaaacaactctggcgcatcgggcttcccatacaatcgatagattgtcgcacctgattgcccgacattatcgcgagcccatttatacccatataaatcagcatccatgttggaatttaatcgcggcctagagcaagacgtttcccgttgaatatggctcataacaccccttgtattactgtttatgtaagcagacagttttattgttcatgaccaaaatcccttaacgtgagttttcgttccactgagcgtcagaccccgtagaaaagatcaaaggatcttcttgagatcctttttttctgcgcgtaatctgctgcttgcaaacaaaaaaaccaccgctaccagcggtggtttgtttgccggatcaagagctaccaactctttttccgaaggtaactggcttcagcagagcgcagataccaaatactgtccttctagtgtagccgtagttaggccaccacttcaagaactctgtagcaccgcctacatacctcgctctgctaatcctgttaccagtggctgctgccagtggcgataagtcgtgtcttaccgggttggactcaagacgatagttaccggataaggcgcagcggtcgggctgaacggggggttcgtgcacacagcccagcttggagcgaacgacctacaccgaactgagatacctacagcgtgagctatgagaaagcgccacgcttcccgaagggagaaaggcggacaggtatccggtaagcggcagggtcggaacaggagagcgcacgagggagcttccagggggaaacgcctggtatctttatagtcctgtcgggtttcgccacctctgacttgagcgtcgatttttgtgatgctcgtcaggggggcggagcctatggaaaaacgccagcaacgcggcctttttacggttcctggccttttgctggccttttgctcacatgttctttcctgcgttatcccctgattctgtggataaccgtattaccgcctttgagtgagctgataccgctcgccgcagccgaacgaccgagcgcagcgagtcagtgagcgaggaagcggaagagcgcctgatgcggtattttctccttacgcatctgtgcggtatttcacaccgcaatggtgcactctcagtacaatctgctctgatgccgcatagttaagccagtatacactccgctatcgctacgtgactgggtcatggctgcgccccgacacccgccaacacccgctgacgcgccctgacgggcttgtctgctcccggcatccgcttacagacaagctgtgaccgtctccgggagctgcatgtgtgatgcctccgtgtaagggggatttctgttcatgggggtaatgataccgatgaaacgagagaggatgctcacgatacgggttactgatgatgaacatgcccggttactggaacgttgtgagggtaaacaactggcggtatggatgcggcgggaccagagaaaaatcactcagggtcaatgccagcgcttcgttaatacagatgtaggtgttccacagggtagccagcagcatcctgcgatgcagatccggaacataatggtgcagggcgctgacttccgcgtttccagactttacgaaacacggaaaccgaagaccattcatgttgttgctcaggtcgcagacgttttgcagcagcagtcgcttcacgttcgctcgcgtatcggtgattcattctgctaaccagtaaggcaaccccgccagcctagccgggtcctcaacgacaggagcacgatcatgcgcacccgtggggccgccatgccggcgataatggcctgcttctcgccgaaacgtttggtggcgggaccagtgacgaaggcttgagcgagggcgtgcaagattccgaataccgcaagcgacaggccgatcatcgtcgcgctccagcgaaagcggtcctcgccgaaaatgacccagagcgctgccggcacctgtcctacgagttgcatgataaagaagacagtcataagtgcggcgacgatagtcatgccccgcgcccaccggaaggagctgactgggttgaaggctctcaagggcatcggtcgagatcccggtgcctaatgagtgagctaacttacattaattgcgttgcgctcactgcccgctttccagtcgggaaacctgtcgtgccagctgcattaatgaatcggccaacgcgcggggagaggcggtttgcgtattgggcgccagggtggtttttcttttcaccagtgagacgggcaacagctgattgcccttcaccgcctggccctgagagagttgcagcaagcggtccacgctggtttgccccagcaggcgaaaatcctgtttgatggtggttaacggcgggatataacatgagctgtcttcggtatcgtcgtatcccactaccgagatatccgcaccaacgcgcagcccggactcggtaatggcgcgcattgcgcccagcgccatctgatcgttggcaaccagcatcgcagtgggaacgatgccctcattcagcatttgcatggtttgttgaaaaccggacatggcactccagtcgccttcccgttccgctatcggctgaatttgattgcgagtgagatatttatgccagccagccagacgcagacgcgccgagacagaacttaatgggcccgctaacagcgcgatttgctggtgacccaatgcgaccagatgctccacgcccagtcgcgtaccgtcttcatgggagaaaataatactgttgatgggtgtctggtcagagacatcaagaaataacgccggaacattagtgcaggcagcttccacagcaatggcatcctggtcatccagcggatagttaatgatcagcccactgacgcgttgcgcgagaagattgtgcaccgccgctttacaggcttcgacgccgcttcgttctaccatcgacaccaccacgctggcacccagttgatcggcgcgagatttaatcgccgcgacaatttgcgacggcgcgtgcagggccagactggaggtggcaacgccaatcagcaacgactgtttgcccgccagttgttgtgccacgcggttgggaatgtaattcagctccgccatcgccgcttccactttttcccgcgttttcgcagaaacgtggctggcctggttcaccacgcgggaaacggtctgataagagacaccggcatactctgcgacatcgtataacgttactggtttcacattcaccaccctgaattgactctcttccgggcgctatcatgccataccgcgaaaggttttgcgccattcgatggtgtccgggatctcgacgctctcccttatgcgactcctgcattaggaagcagcccagtagtaggttgaggccgttgagcaccgccgccgcaaggaatggtgcatgcaaggagatggcgcccaacagtcccccggccacggggcctgccaccatacccacgccgaaacaagcgctcatgagcccgaagtggcgagcccgatcttccccatcggtgatgtcggcgatataggcgccagcaaccgcacctgtggcgccggtgatgccggccacgatgcgtccggcgtagaggatcgagatctcgatcccgcgaaattaatacgactcactataggggaattgtgagcggataacaattcccctctagaaataattttgtttaactttaagaaggagatatacatatgggcctgaaaatgaaaaaacgtagcgggaaaaaagcgtggatgctgctggttatgtcgctgctgattgcggcggttccgattacggcgagcgccgaggtgcagctggtggagtctgggggaggcttggtgcagcctggggggtctctgagactctcctgtgtagcctctggaagcatcgtcagaattaataccatgggctggtaccgccagactccagggaagcagcgcgagttggtcgcagatattaccagtggtggtaacataaactatatagacgccgtgaagggccgattcaccatctccagagacaacaccaagaagagggtgtatctgcaaatgaacagcctgaaacctgaggacacggccgtctattactgtaatgcagagatcgttgttctggtgggagtttggacccagcgtgcgcggaccggcaactactggggccaggggacccaggtcaccgtctcctcatacccctatgacgtgcctgattacgccggctctggccaccaccaccaccaccactgagatccggctgctaacaaagcccgaaaggaagctgagttggctgctgccaccgctgagcaataactagcataaccccttggggcctctaaacgggtcttgaggggttttttgctgaaaggaggaactatatccggat

SEQ ID NO: 37 - DNA, 22 bp, synthetic construct
  source 1..22: mol_type = other DNA
ccttctcctctttaatcttgcg

SEQ ID NO: 38 - DNA, 20 bp, synthetic construct
  source 1..20: mol_type = other DNA
ctggaagatccgcgcgtacc

SEQ ID NO: 39 - DNA, 42 bp, synthetic construct
  source 1..42: mol_type = other DNA
cgcaagattaaagaggagaaggatgaaatacctgctgccgac

SEQ ID NO: 40 - DNA, 40 bp, synthetic construct
  source 1..40: mol_type = other DNA
ggtacgcgcggatcttccagagccggatctcagtggtggt

SEQ ID NO: 41 - DNA, 39 bp, synthetic construct
  source 1..39: mol_type = other DNA
cctgccgttcgacgatatgggcctgaaaatgaaaaaacg

SEQ ID NO: 42 - DNA, 18 bp, synthetic construct
  source 1..18: mol_type = other DNA
tgaggagacggtgacctg

SEQ ID NO: 43 - DNA, 6523 bp, synthetic construct
  source 1..6523: mol_type = other DNA
tggcgaatgggacgcgccctgtagcggcgcattaagcgcggcgggtgtggtggttacgcgcagcgtgaccgctacacttgccagcgccctagcgcccgctcctttcgctttcttcccttcctttctcgccacgttcgccggctttccccgtcaagctctaaatcgggggctccctttagggttccgatttagtgctttacggcacctcgaccccaaaaaacttgattagggtgatggttcacgtagtgggccatcgccctgatagacggtttttcgccctttgacgttggagtccacgttctttaatagtggactcttgttccaaactggaacaacactcaaccctatctcggtctattcttttgatttataagggattttgccgatttcggcctattggttaaaaaatgagctgatttaacaaaaatttaacgcgaattttaacaaaatattaacgcttacaatttaggtggcacttttcggggaaatgtgcgcggaacccctatttgtttatttttctaaatacattcaaatatgtatccgctcatgaattaattcttagaaaaactcatcgagcatcaaatgaaactgcaatttattcatatcaggattatcaataccatatttttgaaaaagccgtttctgtaatgaaggagaaaactcaccgaggcagttccataggatggcaagatcctggtatcggtctgcgattccgactcgtccaacatcaatacaacctattaatttcccctcgtcaaaaataaggttatcaagtgagaaatcaccatgagtgacgactgaatccggtgagaatggcaaaagtttatgcatttctttccagacttgttcaacaggccagccattacgctcgtcatcaaaatcactcgcatcaaccaaaccgttattcattcgtgattgcgcctgagcgagacgaaatacgcgatcgctgttaaaaggacaattacaaacaggaatcgaatgcaaccggcgcaggaacactgccagcgcatcaacaatattttcacctgaatcaggatattcttctaatacctggaatgctgttttcccggggatcgcagtggtgagtaaccatgcatcatcaggagtacggataaaatgcttgatggtcggaagaggcataaattccgtcagccagtttagtctgaccatctcatctgtaacatcattggcaacgctacctttgccatgtttcagaaacaactctggcgcatcgggcttcccatacaatcgatagattgtcgcacctgattgcccgacattatcgcgagcccatttatacccatataaatcagcatccatgttggaatttaatcgcggcctagagcaagacgtttcccgttgaatatggctcataacaccccttgtattactgtttatgtaagcagacagttttattgttcatgaccaaaatcccttaacgtgagttttcgttccactgagcgtcagaccccgtagaaaagatcaaaggatcttcttgagatcctttttttctgcgcgtaatctgctgcttgcaaacaaaaaaaccaccgctaccagcggtggtttgtttgccggatcaagagctaccaactctttttccgaaggtaactggcttcagcagagcgcagataccaaatactgtccttctagtgtagccgtagttaggccaccacttcaagaactctgtagcaccgcctacatacctcgctctgctaatcctgttaccagtggctgctgccagtggcgataagtcgtgtcttaccgggttggactcaagacgatagttaccggataaggcgcagcggtcgggctgaacggggggttcgtgcacacagcccagcttggagcgaacgacctacaccgaactgagatacctacagcgtgagctatgagaaagcgccacgcttcccgaagggagaaaggcggacaggtatccggtaagcggcagggtcggaacaggagagcgcacgagggagcttccagggggaaacgcctggtatctttatagtcctgtcgggtttcgccacctctgacttgagcgtcgatttttgtgatgctcgtcaggggggcggagcctatggaaaaacgccagcaacgcggcctttttacggttcctggccttttgctggccttttgctcacatgttctttcctgcgttatcccctgattctgtggataaccgtattaccgcctttgagtgagctgataccgctcgccgcagccgaacgaccgagcgcagcgagtcagtgagcgaggaagcggaagagcgcctgatgcggtattttctccttacgcatctgtgcggtatttcacaccgcaatggtgcactctcagtacaatctgctctgatgccgcatagttaagccagtatacactccgctatcgctacgtgactgggtcatggctgcgccccgacacccgccaacacccgctgacgcgccctgacgggcttgtctgctcccggcatccgcttacagacaagctgtgaccgtctccgggagctgcatgtgtgatgcctccgtgtaagggggatttctgttcatgggggtaatgataccgatgaaacgagagaggatgctcacgatacgggttactgatgatgaacatgcccggttactggaacgttgtgagggtaaacaactggcggtatggatgcggcgggaccagagaaaaatcactcagggtcaatgccagcgcttcgttaatacagatgtaggtgttccacagggtagccagcagcatcctgcgatgcagatccggaacataatggtgcagggcgctgacttccgcgtttccagactttacgaaacacggaaaccgaagaccattcatgttgttgctcaggtcgcagacgttttgcagcagcagtcgcttcacgttcgctcgcgtatcggtgattcattctgctaaccagtaaggcaaccccgccagcctagccgggtcctcaacgacaggagcacgatcatgcgcacccgtggggccgccatgccggcgataatggcctgcttctcgccgaaacgtttggtggcgggaccagtgacgaaggcttgagcgagggcgtgcaagattccgaataccgcaagcgacaggccgatcatcgtcgcgctccagcgaaagcggtcctcgccgaaaatgacccagagcgctgccggcacctgtcctacgagttgcatgataaagaagacagtcataagtgcggcgacgatagtcatgccccgcgcccaccggaaggagctgactgggttgaaggctctcaagggcatcggtcgagatcccggtgcctaatgagtgagctaacttacattaattgcgttgcgctcactgcccgctttccagtcgggaaacctgtcgtgccagctgcattaatgaatcggccaacgcgcggggagaggcggtttgcgtattgggcgccagggtggtttttcttttcaccagtgagacgggcaacagctgattgcccttcaccgcctggccctgagagagttgcagcaagcggtccacgctggtttgccccagcaggcgaaaatcctgtttgatggtggttaacggcgggatataacatgagctgtcttcggtatcgtcgtatcccactaccgagatatccgcaccaacgcgcagcccggactcggtaatggcgcgcattgcgcccagcgccatctgatcgttggcaaccagcatcgcagtgggaacgatgccctcattcagcatttgcatggtttgttgaaaaccggacatggcactccagtcgccttcccgttccgctatcggctgaatttgattgcgagtgagatatttatgccagccagccagacgcagacgcgccgagacagaacttaatgggcccgctaacagcgcgatttgctggtgacccaatgcgaccagatgctccacgcccagtcgcgtaccgtcttcatgggagaaaataatactgttgatgggtgtctggtcagagacatcaagaaataacgccggaacattagtgcaggcagcttccacagcaatggcatcctggtcatccagcggatagttaatgatcagcccactgacgcgttgcgcgagaagattgtgcaccgccgctttacaggcttcgacgccgcttcgttctaccatcgacaccaccacgctggcacccagttgatcggcgcgagatttaatcgccgcgacaatttgcgacggcgcgtgcagggccagactggaggtggcaacgccaatcagcaacgactgtttgcccgccagttgttgtgccacgcggttgggaatgtaattcagctccgccatcgccgcttccactttttcccgcgttttcgcagaaacgtggctggcctggttcaccacgcgggaaacggtctgataagagacaccggcatactctgcgacatcgtataacgttactggtttcacattcaccaccctgaattgactctcttccgggcgctatcatgccataccgcgaaaggttttgcgccattcgatggtgtccgggatctcgacgctctcccttatgcgactcctgcattaggaagcagcccagtagtaggttgaggccgttgagcaccgccgccgcaaggaatggtgcatgcaaggagatggcgcccaacagtcccccggccacggggcctgccaccatacccacgccgaaacaagcgctcatgagcccgaagtggcgagcccgatcttccccatcggtgatgtcggcgatataggcgccagcaaccgcacctgtggcgccggtgatgccggccacgatgcgtccggcgtagaggatcgagatctcgatcccgcgaaattaatacgactcactataggggaattgtgagcggataacaattcccctctagaaataattttgtttaactttaagaaggagatatacatatgggcctgaaaatgaaaaaacgtagcgggaaaaaagcgtggatgctgctggttatgtcgctgctgattgcggcggttccgattacggcgagcgccgaggttcaattagtggaatctggcgggggattggttcaagccggtgagtccttgcgtttgagctgcgccgcatctgggagcacatttgatttcaaagtgatgggctggtatcgtcagccgcccggaaaacagcgcgagggtgtagcagccatccgcttgagcggaaatatgcactacgccgagtctgtaaaagggcgctttgctatttccaaagcgaacgctaagaacacagtgtatcttcagatgaactccttgcgtcccgaagacactgccgtttattattgcaaagtaaacatccgtgggcaagactactggggtcaaggaacgcaggtcacagtctcttctggctctggccctgaaggtggtagcctggcggcactgaccgcacaccaagcatgtcatctgccactggaaacctttacccgtcatcgtcagccgcgtggctgggaacaactggaacaatgtggatatccggtgcagagactggtcgcattatatctggcagcacgtctgagttggaatcaggttgatcaagttattcgtaacgcacttgcctcaccgggtagcggtggtgatttaggtgaggcaattcgtgaacaacctgaacaggcacgcttagcattaacccttgcagccgcagaaagtgaaagatttgtgcgtcagggtactggtaatgatgaggccggtgcagcaaatgggccggcagacagcggagatgcattattagagagaaattatcctaccggcgcagaatttctgggtgatgggggtgatgttagtttttcaacacgcgggacacagaattggaccgtggaacgtttactgcaggcacatcgtcagctggaagaacgcggttatgtttttgttggttatcatgggacgtttctggaggcagcacagagcattgtctttggcggtgtgcgggcgcgtagccaggatcttgatgcaatttggcgtggtttttatattgcgggtgatcctgcgctggcgtatggatatgcgcaggatcaggagccggatgcgcgtggtcgtattcgtaatggtgccctgctgcgggtttatgttccgcgtagctcactgccggggttttatagaacaagcttaacactggctgcgccggaagcagcaggtgaagttgaacgtctgattggccatccgctgccgttacgtttagatgcaattactggtccggaagaagaaggtggtcgcctggaaaccattctgggttggccgctggcagaaagaaccgtggttataccttccgcaataccgaccgatcctcggaatgtggggggtgatttagatcctagcagcattcctgataaagaacaggcaatttctgctctgcctgattatgcatcacagccgggtaaaccgccgcgtgaagatttaaagcatcatcaccatcatcattaagatccggctgctaacaaagcccgaaaggaagctgagttggctgctgccaccgctgagcaataactagcataaccccttggggcctctaaacgggtcttgaggggttttttgctgaaaggaggaactatatccggat

SEQ ID NO: 44 - DNA, 6535 bp, synthetic construct
  source 1..6535: mol_type = other DNA
tggcgaatgggacgcgccctgtagcggcgcattaagcgcggcgggtgtggtggttacgcgcagcgtgaccgctacacttgccagcgccctagcgcccgctcctttcgctttcttcccttcctttctcgccacgttcgccggctttccccgtcaagctctaaatcgggggctccctttagggttccgatttagtgctttacggcacctcgaccccaaaaaacttgattagggtgatggttcacgtagtgggccatcgccctgatagacggtttttcgccctttgacgttggagtccacgttctttaatagtggactcttgttccaaactggaacaacactcaaccctatctcggtctattcttttgatttataagggattttgccgatttcggcctattggttaaaaaatgagctgatttaacaaaaatttaacgcgaattttaacaaaatattaacgcttacaatttaggtggcacttttcggggaaatgtgcgcggaacccctatttgtttatttttctaaatacattcaaatatgtatccgctcatgaattaattcttagaaaaactcatcgagcatcaaatgaaactgcaatttattcatatcaggattatcaataccatatttttgaaaaagccgtttctgtaatgaaggagaaaactcaccgaggcagttccataggatggcaagatcctggtatcggtctgcgattccgactcgtccaacatcaatacaacctattaatttcccctcgtcaaaaataaggttatcaagtgagaaatcaccatgagtgacgactgaatccggtgagaatggcaaaagtttatgcatttctttccagacttgttcaacaggccagccattacgctcgtcatcaaaatcactcgcatcaaccaaaccgttattcattcgtgattgcgcctgagcgagacgaaatacgcgatcgctgttaaaaggacaattacaaacaggaatcgaatgcaaccggcgcaggaacactgccagcgcatcaacaatattttcacctgaatcaggatattcttctaatacctggaatgctgttttcccggggatcgcagtggtgagtaaccatgcatcatcaggagtacggataaaatgcttgatggtcggaagaggcataaattccgtcagccagtttagtctgaccatctcatctgtaacatcattggcaacgctacctttgccatgtttcagaaacaactctggcgcatcgggcttcccatacaatcgatagattgtcgcacctgattgcccgacattatcgcgagcccatttatacccatataaatcagcatccatgttggaatttaatcgcggcctagagcaagacgtttcccgttgaatatggctcataacaccccttgtattactgtttatgtaagcagacagttttattgttcatgaccaaaatcccttaacgtgagttttcgttccactgagcgtcagaccccgtagaaaagatcaaaggatcttcttgagatcctttttttctgcgcgtaatctgctgcttgcaaacaaaaaaaccaccgctaccagcggtggtttgtttgccggatcaagagctaccaactctttttccgaaggtaactggcttcagcagagcgcagataccaaatactgtccttctagtgtagccgtagttaggccaccacttcaagaactctgtagcaccgcctacatacctcgctctgctaatcctgttaccagtggctgctgccagtggcgataagtcgtgtcttaccgggttggactcaagacgatagttaccggataaggcgcagcggtcgggctgaacggggggttcgtgcacacagcccagcttggagcgaacgacctacaccgaactgagatacctacagcgtgagctatgagaaagcgccacgcttcccgaagggagaaaggcggacaggtatccggtaagcggcagggtcggaacaggagagcgcacgagggagcttccagggggaaacgcctggtatctttatagtcctgtcgggtttcgccacctctgacttgagcgtcgatttttgtgatgctcgtcaggggggcggagcctatggaaaaacgccagcaacgcggcctttttacggttcctggccttttgctggccttttgctcacatgttctttcctgcgttatcccctgattctgtggataaccgtattaccgcctttgagtgagctgataccgctcgccgcagccgaacgaccgagcgcagcgagtcagtgagcgaggaagcggaagagcgcctgatgcggtattttctccttacgcatctgtgcggtatttcacaccgcaatggtgcactctcagtacaatctgctctgatgccgcatagttaagccagtatacactccgctatcgctacgtgactgggtcatggctgcgccccgacacccgccaacacccgctgacgcgccctgacgggcttgtctgctcccggcatccgcttacagacaagctgtgaccgtctccgggagctgcatgtgtgatgcctccgtgtaagggggatttctgttcatgggggtaatgataccgatgaaacgagagaggatgctcacgatacgggttactgatgatgaacatgcccggttactggaacgttgtgagggtaaacaactggcggtatggatgcggcgggaccagagaaaaatcactcagggtcaatgccagcgcttcgttaatacagatgtaggtgttccacagggtagccagcagcatcctgcgatgcagatccggaacataatggtgcagggcgctgacttccgcgtttccagactttacgaaacacggaaaccgaagaccattcatgttgttgctcaggtcgcagacgttttgcagcagcagtcgcttcacgttcgctcgcgtatcggtgattcattctgctaaccagtaaggcaaccccgccagcctagccgggtcctcaacgacaggagcacgatcatgcgcacccgtggggccgccatgccggcgataatggcctgcttctcgccgaaacgtttggtggcgggaccagtgacgaaggcttgagcgagggcgtgcaagattccgaataccgcaagcgacaggccgatcatcgtcgcgctccagcgaaagcggtcctcgccgaaaatgacccagagcgctgccggcacctgtcctacgagttgcatgataaagaagacagtcataagtgcggcgacgatagtcatgccccgcgcccaccggaaggagctgactgggttgaaggctctcaagggcatcggtcgagatcccggtgcctaatgagtgagctaacttacattaattgcgttgcgctcactgcccgctttccagtcgggaaacctgtcgtgccagctgcattaatgaatcggccaacgcgcggggagaggcggtttgcgtattgggcgccagggtggtttttcttttcaccagtgagacgggcaacagctgattgcccttcaccgcctggccctgagagagttgcagcaagcggtccacgctggtttgccccagcaggcgaaaatcctgtttgatggtggttaacggcgggatataacatgagctgtcttcggtatcgtcgtatcccactaccgagatatccgcaccaacgcgcagcccggactcggtaatggcgcgcattgcgcccagcgccatctgatcgttggcaaccagcatcgcagtgggaacgatgccctcattcagcatttgcatggtttgttgaaaaccggacatggcactccagtcgccttcccgttccgctatcggctgaatttgattgcgagtgagatatttatgccagccagccagacgcagacgcgccgagacagaacttaatgggcccgctaacagcgcgatttgctggtgacccaatgcgaccagatgctccacgcccagtcgcgtaccgtcttcatgggagaaaataatactgttgatgggtgtctggtcagagacatcaagaaataacgccggaacattagtgcaggcagcttccacagcaatggcatcctggtcatccagcggatagttaatgatcagcccactgacgcgttgcgcgagaagattgtgcaccgccgctttacaggcttcgacgccgcttcgttctaccatcgacaccaccacgctggcacccagttgatcggcgcgagatttaatcgccgcgacaatttgcgacggcgcgtgcagggccagactggaggtggcaacgccaatcagcaacgactgtttgcccgccagttgttgtgccacgcggttgggaatgtaattcagctccgccatcgccgcttccactttttcccgcgttttcgcagaaacgtggctggcctggttcaccacgcgggaaacggtctgataagagacaccggcatactctgcgacatcgtataacgttactggtttcacattcaccaccctgaattgactctcttccgggcgctatcatgccataccgcgaaaggttttgcgccattcgatggtgtccgggatctcgacgctctcccttatgcgactcctgcattaggaagcagcccagtagtaggttgaggccgttgagcaccgccgccgcaaggaatggtgcatgcaaggagatggcgcccaacagtcccccggccacggggcctgccaccatacccacgccgaaacaagcgctcatgagcccgaagtggcgagcccgatcttccccatcggtgatgtcggcgatataggcgccagcaaccgcacctgtggcgccggtgatgccggccacgatgcgtccggcgtagaggatcgagatctcgatcccgcgaaattaatacgactcactataggggaattgtgagcggataacaattcccctctagaaataattttgtttaactttaagaaggagatatacatatgggcctgaaaatgaaaaaacgtagcgggaaaaaagcgtggatgctgctggttatgtcgctgctgattgcggcggttccgattacggcgagcgccgaggtgcagctggtggagtctgggggaggattggtgcagcctgggggctctgtgagactctcctgtgtagcctctggacgcatcttcagtagcaatgccatgggctggttccgccaggctccagggaaggagcgtgagtttgtagcggccattacctggaggagtggcggtagcgcgtactatgcagactccgcgaagggccgattcaccatctccagagacaacgccaagaacacggtgtatttgcaaatgaacagcctgaaacctgaggacacggccgtttattattgtgcagctggtggtagttcctggttaagttttccgccggactactggggccaggggacccaggtcaccgtctcctcacctgaaggtggtagcctggcggcactgaccgcacaccaagcatgtcatctgccactggaaacctttacccgtcatcgtcagccgcgtggctgggaacaactggaacaatgtggatatccggtgcagagactggtcgcattatatctggcagcacgtctgagttggaatcaggttgatcaagttattcgtaacgcacttgcctcaccgggtagcggtggtgatttaggtgaggcaattcgtgaacaacctgaacaggcacgcttagcattaacccttgcagccgcagaaagtgaaagatttgtgcgtcagggtactggtaatgatgaggccggtgcagcaaatgggccggcagacagcggagatgcattattagagagaaattatcctaccggcgcagaatttctgggtgatgggggtgatgttagtttttcaacacgcgggacacagaattggaccgtggaacgtttactgcaggcacatcgtcagctggaagaacgcggttatgtttttgttggttatcatgggacgtttctggaggcagcacagagcattgtctttggcggtgtgcgggcgcgtagccaggatcttgatgcaatttggcgtggtttttatattgcgggtgatcctgcgctggcgtatggatatgcgcaggatcaggagccggatgcgcgtggtcgtattcgtaatggtgccctgctgcgggtttatgttccgcgtagctcactgccggggttttatagaacaagcttaacactggctgcgccggaagcagcaggtgaagttgaacgtctgattggccatccgctgccgttacgtttagatgcaattactggtccggaagaagaaggtggtcgcctggaaaccattctgggttggccgctggcagaaagaaccgtggttataccttccgcaataccgaccgatcctcggaatgtggggggtgatttagatcctagcagcattcctgataaagaacaggcaatttctgctctgcctgattatgcatcacagccgggtaaaccgccgcgtgaagatttaaagcatcatcaccatcatcattaagatccggctgctaacaaagcccgaaaggaagctgagttggctgctgccaccgctgagcaataactagcataaccccttggggcctctaaacgggtcttgaggggttttttgctgaaaggaggaactatatccggat

SEQ ID NO: 45 - DNA, 6547 bp, synthetic construct
  source 1..6547: mol_type = other DNA
tggcgaatgggacgcgccctgtagcggcgcattaagcgcggcgggtgtggtggttacgcgcagcgtgaccgctacacttgccagcgccctagcgcccgctcctttcgctttcttcccttcctttctcgccacgttcgccggctttccccgtcaagctctaaatcgggggctccctttagggttccgatttagtgctttacggcacctcgaccccaaaaaacttgattagggtgatggttcacgtagtgggccatcgccctgatagacggtttttcgccctttgacgttggagtccacgttctttaatagtggactcttgttccaaactggaacaacactcaaccctatctcggtctattcttttgatttataagggattttgccgatttcggcctattggttaaaaaatgagctgatttaacaaaaatttaacgcgaattttaacaaaatattaacgcttacaatttaggtggcacttttcggggaaatgtgcgcggaacccctatttgtttatttttctaaatacattcaaatatgtatccgctcatgaattaattcttagaaaaactcatcgagcatcaaatgaaactgcaatttattcatatcaggattatcaataccatatttttgaaaaagccgtttctgtaatgaaggagaaaactcaccgaggcagttccataggatggcaagatcctggtatcggtctgcgattccgactcgtccaacatcaatacaacctattaatttcccctcgtcaaaaataaggttatcaagtgagaaatcaccatgagtgacgactgaatccggtgagaatggcaaaagtttatgcatttctttccagacttgttcaacaggccagccattacgctcgtcatcaaaatcactcgcatcaaccaaaccgttattcattcgtgattgcgcctgagcgagacgaaatacgcgatcgctgttaaaaggacaattacaaacaggaatcgaatgcaaccggcgcaggaacactgccagcgcatcaacaatattttcacctgaatcaggatattcttctaatacctggaatgctgttttcccggggatcgcagtggtgagtaaccatgcatcatcaggagtacggataaaatgcttgatggtcggaagaggcataaattccgtcagccagtttagtctgaccatctcatctgtaacatcattggcaacgctacctttgccatgtttcagaaacaactctggcgcatcgggcttcccatacaatcgatagattgtcgcacctgattgcccgacattatcgcgagcccatttatacccatataaatcagcatccatgttggaatttaatcgcggcctagagcaagacgtttcccgttgaatatggctcataacaccccttgtattactgtttatgtaagcagacagttttattgttcatgaccaaaatcccttaacgtgagttttcgttccactgagcgtcagaccccgtagaaaagatcaaaggatcttcttgagatcctttttttctgcgcgtaatctgctgcttgcaaacaaaaaaaccaccgctaccagcggtggtttgtttgccggatcaagagctaccaactctttttccgaaggtaactggcttcagcagagcgcagataccaaatactgtccttctagtgtagccgtagttaggccaccacttcaagaactctgtagcaccgcctacatacctcgctctgctaatcctgttaccagtggctgctgccagtggcgataagtcgtgtcttaccgggttggactcaagacgatagttaccggataaggcgcagcggtcgggctgaacggggggttcgtgcacacagcccagcttggagcgaacgacctacaccgaactgagatacctacagcgtgagctatgagaaagcgccacgcttcccgaagggagaaaggcggacaggtatccggtaagcggcagggtcggaacaggagagcgcacgagggagcttccagggggaaacgcctggtatctttatagtcctgtcgggtttcgccacctctgacttgagcgtcgatttttgtgatgctcgtcaggggggcggagcctatggaaaaacgccagcaacgcggcctttttacggttcctggccttttgctggccttttgctcacatgttctttcctgcgttatcccctgattctgtggataaccgtattaccgcctttgagtgagctgataccgctcgccgcagccgaacgaccgagcgcagcgagtcagtgagcgaggaagcggaagagcgcctgatgcggtattttctccttacgcatctgtgcggtatttcacaccgcaatggtgcactctcagtacaatctgctctgatgccgcatagttaagccagtatacactccgctatcgctacgtgactgggtcatggctgcgccccgacacccgccaacacccgctgacgcgccctgacgggcttgtctgctcccggcatccgcttacagacaagctgtgaccgtctccgggagctgcatgtgtgatgcctccgtgtaagggggatttctgttcatgggggtaatgataccgatgaaacgagagaggatgctcacgatacgggttactgatgatgaacatgcccggttactggaacgttgtgagggtaaacaactggcggtatggatgcggcgggaccagagaaaaatcactcagggtcaatgccagcgcttcgttaatacagatgtaggtgttccacagggtagccagcagcatcctgcgatgcagatccggaacataatggtgcagggcgctgacttccgcgtttccagactttacgaaacacggaaaccgaagaccattcatgttgttgctcaggtcgcagacgttttgcagcagcagtcgcttcacgttcgctcgcgtatcggtgattcattctgctaaccagtaaggcaaccccgccagcctagccgggtcctcaacgacaggagcacgatcatgcgcacccgtggggccgccatgccggcgataatggcctgcttctcgccgaaacgtttggtggcgggaccagtgacgaaggcttgagcgagggcgtgcaagattccgaataccgcaagcgacaggccgatcatcgtcgcgctccagcgaaagcggtcctcgccgaaaatgacccagagcgctgccggcacctgtcctacgagttgcatgataaagaagacagtcataagtgcggcgacgatagtcatgccccgcgcccaccggaaggagctgactgggttgaaggctctcaagggcatcggtcgagatcccggtgcctaatgagtgagctaacttacattaattgcgttgcgctcactgcccgctttccagtcgggaaacctgtcgtgccagctgcattaatgaatcggccaacgcgcggggagaggcggtttgcgtattgggcgccagggtggtttttcttttcaccagtgagacgggcaacagctgattgcccttcaccgcctggccctgagagagttgcagcaagcggtccacgctggtttgccccagcaggcgaaaatcctgtttgatggtggttaacggcgggatataacatgagctgtcttcggtatcgtcgtatcccactaccgagatatccgcaccaacgcgcagcccggactcggtaatggcgcgcattgcgcccagcgccatctgatcgttggcaaccagcatcgcagtgggaacgatgccctcattcagcatttgcatggtttgttgaaaaccggacatggcactccagtcgccttcccgttccgctatcggctgaatttgattgcgagtgagatatttatgccagccagccagacgcagacgcgccgagacagaacttaatgggcccgctaacagcgcgatttgctggtgacccaatgcgaccagatgctccacgcccagtcgcgtaccgtcttcatgggagaaaataatactgttgatgggtgtctggtcagagacatcaagaaataacgccggaacattagtgcaggcagcttccacagcaatggcatcctggtcatccagcggatagttaatgatcagcccactgacgcgttgcgcgagaagattgtgcaccgccgctttacaggcttcgacgccgcttcgttctaccatcgacaccaccacgctggcacccagttgatcggcgcgagatttaatcgccgcgacaatttgcgacggcgcgtgcagggccagactggaggtggcaacgccaatcagcaacgactgtttgcccgccagttgttgtgccacgcggttgggaatgtaattcagctccgccatcgccgcttccactttttcccgcgttttcgcagaaacgtggctggcctggttcaccacgcgggaaacggtctgataagagacaccggcatactctgcgacatcgtataacgttactggtttcacattcaccaccctgaattgactctcttccgggcgctatcatgccataccgcgaaaggttttgcgccattcgatggtgtccgggatctcgacgctctcccttatgcgactcctgcattaggaagcagcccagtagtaggttgaggccgttgagcaccgccgccgcaaggaatggtgcatgcaaggagatggcgcccaacagtcccccggccacggggcctgccaccatacccacgccgaaacaagcgctcatgagcccgaagtggcgagcccgatcttccccatcggtgatgtcggcgatataggcgccagcaaccgcacctgtggcgccggtgatgccggccacgatgcgtccggcgtagaggatcgagatctcgatcccgcgaaattaatacgactcactataggggaattgtgagcggataacaattcccctctagaaataattttgtttaactttaagaaggagatatacatatgggcctgaaaatgaaaaaacgtagcgggaaaaaagcgtggatgctgctggttatgtcgctgctgattgcggcggttccgattacggcgagcgccgaggtgcagctggtggagtctgggggaggcttggtgcagcctggggggtctctgagactctcctgtgtagcctctggaagcatcgtcagaattaataccatgggctggtaccgccagactccagggaagcagcgcgagttggtcgcagatattaccagtggtggtaacataaactatatagacgccgtgaagggccgattcaccatctccagagacaacaccaagaagagggtgtatctgcaaatgaacagcctgaaacctgaggacacggccgtctattactgtaatgcagagatcgttgttctggtgggagtttggacccagcgtgcgcggaccggcaactactggggccaggggacccaggtcaccgtctcctcacctgaaggtggtagcctggcggcactgaccgcacaccaagcatgtcatctgccactggaaacctttacccgtcatcgtcagccgcgtggctgggaacaactggaacaatgtggatatccggtgcagagactggtcgcattatatctggcagcacgtctgagttggaatcaggttgatcaagttattcgtaacgcacttgcctcaccgggtagcggtggtgatttaggtgaggcaattcgtgaacaacctgaacaggcacgcttagcattaacccttgcagccgcagaaagtgaaagatttgtgcgtcagggtactggtaatgatgaggccggtgcagcaaatgggccggcagacagcggagatgcattattagagagaaattatcctaccggcgcagaatttctgggtgatgggggtgatgttagtttttcaacacgcgggacacagaattggaccgtggaacgtttactgcaggcacatcgtcagctggaagaacgcggttatgtttttgttggttatcatgggacgtttctggaggcagcacagagcattgtctttggcggtgtgcgggcgcgtagccaggatcttgatgcaatttggcgtggtttttatattgcgggtgatcctgcgctggcgtatggatatgcgcaggatcaggagccggatgcgcgtggtcgtattcgtaatggtgccctgctgcgggtttatgttccgcgtagctcactgccggggttttatagaacaagcttaacactggctgcgccggaagcagcaggtgaagttgaacgtctgattggccatccgctgccgttacgtttagatgcaattactggtccggaagaagaaggtggtcgcctggaaaccattctgggttggccgctggcagaaagaaccgtggttataccttccgcaataccgaccgatcctcggaatgtggggggtgatttagatcctagcagcattcctgataaagaacaggcaatttctgctctgcctgattatgcatcacagccgggtaaaccgccgcgtgaagatttaaagcatcatcaccatcatcattaagatccggctgctaacaaagcccgaaaggaagctgagttggctgctgccaccgctgagcaataactagcataaccccttggggcctctaaacgggtcttgaggggttttttgctgaaaggaggaactatatccggat

SEQ ID NO: 46 - DNA, 6172 bp, synthetic construct
  source 1..6172: mol_type = other DNA
tggcgaatgggacgcgccctgtagcggcgcattaagcgcggcgggtgtggtggttacgcgcagcgtgaccgctacacttgccagcgccctagcgcccgctcctttcgctttcttcccttcctttctcgccacgttcgccggctttccccgtcaagctctaaatcgggggctccctttagggttccgatttagtgctttacggcacctcgaccccaaaaaacttgattagggtgatggttcacgtagtgggccatcgccctgatagacggtttttcgccctttgacgttggagtccacgttctttaatagtggactcttgttccaaactggaacaacactcaaccctatctcggtctattcttttgatttataagggattttgccgatttcggcctattggttaaaaaatgagctgatttaacaaaaatttaacgcgaattttaacaaaatattaacgcttacaatttaggtggcacttttcggggaaatgtgcgcggaacccctatttgtttatttttctaaatacattcaaatatgtatccgctcatgaattaattcttagaaaaactcatcgagcatcaaatgaaactgcaatttattcatatcaggattatcaataccatatttttgaaaaagccgtttctgtaatgaaggagaaaactcaccgaggcagttccataggatggcaagatcctggtatcggtctgcgattccgactcgtccaacatcaatacaacctattaatttcccctcgtcaaaaataaggttatcaagtgagaaatcaccatgagtgacgactgaatccggtgagaatggcaaaagtttatgcatttctttccagacttgttcaacaggccagccattacgctcgtcatcaaaatcactcgcatcaaccaaaccgttattcattcgtgattgcgcctgagcgagacgaaatacgcgatcgctgttaaaaggacaattacaaacaggaatcgaatgcaaccggcgcaggaacactgccagcgcatcaacaatattttcacctgaatcaggatattcttctaatacctggaatgctgttttcccggggatcgcagtggtgagtaaccatgcatcatcaggagtacggataaaatgcttgatggtcggaagaggcataaattccgtcagccagtttagtctgaccatctcatctgtaacatcattggcaacgctacctttgccatgtttcagaaacaactctggcgcatcgggcttcccatacaatcgatagattgtcgcacctgattgcccgacattatcgcgagcccatttatacccatataaatcagcatccatgttggaatttaatcgcggcctagagcaagacgtttcccgttgaatatggctcataacaccccttgtattactgtttatgtaagcagacagttttattgttcatgaccaaaatcccttaacgtgagttttcgttccactgagcgtcagaccccgtagaaaagatcaaaggatcttcttgagatcctttttttctgcgcgtaatctgctgcttgcaaacaaaaaaaccaccgctaccagcggtggtttgtttgccggatcaagagctaccaactctttttccgaaggtaactggcttcagcagagcgcagataccaaatactgtccttctagtgtagccgtagttaggccaccacttcaagaactctgtagcaccgcctacatacctcgctctgctaatcctgttaccagtggctgctgccagtggcgataagtcgtgtcttaccgggttggactcaagacgatagttaccggataaggcgcagcggtcgggctgaacggggggttcgtgcacacagcccagcttggagcgaacgacctacaccgaactgagatacctacagcgtgagctatgagaaagcgccacgcttcccgaagggagaaaggcggacaggtatccggtaagcggcagggtcggaacaggagagcgcacgagggagcttccagggggaaacgcctggtatctttatagtcctgtcgggtttcgccacctctgacttgagcgtcgatttttgtgatgctcgtcaggggggcggagcctatggaaaaacgccagcaacgcggcctttttacggttcctggccttttgctggccttttgctcacatgttctttcctgcgttatcccctgattctgtggataaccgtattaccgcctttgagtgagctgataccgctcgccgcagccgaacgaccgagcgcagcgagtcagtgagcgaggaagcggaagagcgcctgatgcggtattttctccttacgcatctgtgcggtatttcacaccgcaatggtgcactctcagtacaatctgctctgatgccgcatagttaagccagtatacactccgctatcgctacgtgactgggtcatggctgcgccccgacacccgccaacacccgctgacgcgccctgacgggcttgtctgctcccggcatccgcttacagacaagctgtgaccgtctccgggagctgcatgtgtgatgcctccgtgtaagggggatttctgttcatgggggtaatgataccgatgaaacgagagaggatgctcacgatacgggttactgatgatgaacatgcccggttactggaacgttgtgagggtaaacaactggcggtatggatgcggcgggaccagagaaaaatcactcagggtcaatgccagcgcttcgttaatacagatgtaggtgttccacagggtagccagcagcatcctgcgatgcagatccggaacataatggtgcagggcgctgacttccgcgtttccagactttacgaaacacggaaaccgaagaccattcatgttgttgctcaggtcgcagacgttttgcagcagcagtcgcttcacgttcgctcgcgtatcggtgattcattctgctaaccagtaaggcaaccccgccagcctagccgggtcctcaacgacaggagcacgatcatgcgcacccgtggggccgccatgccggcgataatggcctgcttctcgccgaaacgtttggtggcgggaccagtgacgaaggcttgagcgagggcgtgcaagattccgaataccgcaagcgacaggccgatcatcgtcgcgctccagcgaaagcggtcctcgccgaaaatgacccagagcgctgccggcacctgtcctacgagttgcatgataaagaagacagtcataagtgcggcgacgatagtcatgccccgcgcccaccggaaggagctgactgggttgaaggctctcaagggcatcggtcgagatcccggtgcctaatgagtgagctaacttacattaattgcgttgcgctcactgcccgctttccagtcgggaaacctgtcgtgccagctgcattaatgaatcggccaacgcgcggggagaggcggtttgcgtattgggcgccagggtggtttttcttttcaccagtgagacgggcaacagctgattgcccttcaccgcctggccctgagagagttgcagcaagcggtccacgctggtttgccccagcaggcgaaaatcctgtttgatggtggttaacggcgggatataacatgagctgtcttcggtatcgtcgtatcccactaccgagatatccgcaccaacgcgcagcccggactcggtaatggcgcgcattgcgcccagcgccatctgatcgttggcaaccagcatcgcagtgggaacgatgccctcattcagcatttgcatggtttgttgaaaaccggacatggcactccagtcgccttcccgttccgctatcggctgaatttgattgcgagtgagatatttatgccagccagccagacgcagacgcgccgagacagaacttaatgggcccgctaacagcgcgatttgctggtgacccaatgcgaccagatgctccacgcccagtcgcgtaccgtcttcatgggagaaaataatactgttgatgggtgtctggtcagagacatcaagaaataacgccggaacattagtgcaggcagcttccacagcaatggcatcctggtcatccagcggatagttaatgatcagcccactgacgcgttgcgcgagaagattgtgcaccgccgctttacaggcttcgacgccgcttcgttctaccatcgacaccaccacgctggcacccagttgatcggcgcgagatttaatcgccgcgacaatttgcgacggcgcgtgcagggccagactggaggtggcaacgccaatcagcaacgactgtttgcccgccagttgttgtgccacgcggttgggaatgtaattcagctccgccatcgccgcttccactttttcccgcgttttcgcagaaacgtggctggcctggttcaccacgcgggaaacggtctgataagagacaccggcatactctgcgacatcgtataacgttactggtttcacattcaccaccctgaattgactctcttccgggcgctatcatgccataccgcgaaaggttttgcgccattcgatggtgtccgggatctcgacgctctcccttatgcgactcctgcattaggaagcagcccagtagtaggttgaggccgttgagcaccgccgccgcaaggaatggtgcatgcaaggagatggcgcccaacagtcccccggccacggggcctgccaccatacccacgccgaaacaagcgctcatgagcccgaagtggcgagcccgatcttccccatcggtgatgtcggcgatataggcgccagcaaccgcacctgtggcgccggtgatgccggccacgatgcgtccggcgtagaggatcgagatctcgatcccgcgaaattaatacgactcactataggggaattgtgagcggataacaattcccctctagaaataattttgtttaactttaagaaggagatatacatatgggcctgaaaatgaaaaaacgtagcgggaaaaaagcgtggatgctgctggttatgtcgctgctgattgcggcggttccgattacggcgagcgccgaggttcaattagtggaatctggcgggggattggttcaagccggtgagtccttgcgtttgagctgcgccgcatctgggagcacatttgatttcaaagtgatgggctggtatcgtcagccgcccggaaaacagcgcgagggtgtagcagccatccgcttgagcggaaatatgcactacgccgagtctgtaaaagggcgctttgctatttccaaagcgaacgctaagaacacagtgtatcttcagatgaactccttgcgtcccgaagacactgccgtttattattgcaaagtaaacatccgtgggcaagactactggggtcaaggaacgcaggtcacagtctcttctggctctggcagacaccgccagccgagaggttgggaacagctgccgaccggagctgaatttctgggcgatggtggggatgttagtttttctacccgtggcacacagaattggaccgttgaacggttattacaagcacatcgtcagctggaagaaagaggttatgtgtttgttgggtatcatggtacatttttagaagcagcccagtctattgtttttggcggtgttcgtgcccgtagccaggatctggatgcaatttggagaggtttttatattgcgggtgatccggcgctggcatatggttacgcacaggatcaggaaccagatgcacgtggtcgtattcgtaatggtgccctgttacgggtgtatgttccccgttccagcctgccgggtttttatcgtacctctttaacactggcagccccggaagcagcaggtgaagtggaacgtctgattggccatccgctgccgctgcgcttagatgcaattaccggtccggaagaagaaggtgggcggttagaaaccattctgggttggccgctggcagaaagaacagtggttataccgagcgcgattcctaccgatcctcgtaatgtggggggtgatttagatccgagcagcattccggataaagagcaggcgattagcgcgctgccggattatgcaagccaaccggggaaaccgccgcgtgaagacttaaaacatcatcaccatcatcattaagatccggctgctaacaaagcccgaaaggaagctgagttggctgctgccaccgctgagcaataactagcataaccccttggggcctctaaacgggtcttgaggggttttttgctgaaaggaggaactatatccggat

SEQ ID NO: 47 - DNA, 6184 bp, synthetic construct
  source 1..6184: mol_type = other DNA
tggcgaatgggacgcgccctgtagcggcgcattaagcgcggcgggtgtggtggttacgcgcagcgtgaccgctacacttgccagcgccctagcgcccgctcctttcgctttcttcccttcctttctcgccacgttcgccggctttccccgtcaagctctaaatcgggggctccctttagggttccgatttagtgctttacggcacctcgaccccaaaaaacttgattagggtgatggttcacgtagtgggccatcgccctgatagacggtttttcgccctttgacgttggagtccacgttctttaatagtggactcttgttccaaactggaacaacactcaaccctatctcggtctattcttttgatttataagggattttgccgatttcggcctattggttaaaaaatgagctgatttaacaaaaatttaacgcgaattttaacaaaatattaacgcttacaatttaggtggcacttttcggggaaatgtgcgcggaacccctatttgtttatttttctaaatacattcaaatatgtatccgctcatgaattaattcttagaaaaactcatcgagcatcaaatgaaactgcaatttattcatatcaggattatcaataccatatttttgaaaaagccgtttctgtaatgaaggagaaaactcaccgaggcagttccataggatggcaagatcctggtatcggtctgcgattccgactcgtccaacatcaatacaacctattaatttcccctcgtcaaaaataaggttatcaagtgagaaatcaccatgagtgacgactgaatccggtgagaatggcaaaagtttatgcatttctttccagacttgttcaacaggccagccattacgctcgtcatcaaaatcactcgcatcaaccaaaccgttattcattcgtgattgcgcctgagcgagacgaaatacgcgatcgctgttaaaaggacaattacaaacaggaatcgaatgcaaccggcgcaggaacactgccagcgcatcaacaatattttcacctgaatcaggatattcttctaatacctggaatgctgttttcccggggatcgcagtggtgagtaaccatgcatcatcaggagtacggataaaatgcttgatggtcggaagaggcataaattccgtcagccagtttagtctgaccatctcatctgtaacatcattggcaacgctacctttgccatgtttcagaaacaactctggcgcatcgggcttcccatacaatcgatagattgtcgcacctgattgcccgacattatcgcgagcccatttatacccatataaatcagcatccatgttggaatttaatcgcggcctagagcaagacgtttcccgttgaatatggctcataacaccccttgtattactgtttatgtaagcagacagttttattgttcatgaccaaaatcccttaacgtgagttttcgttccactgagcgtcagaccccgtagaaaagatcaaaggatcttcttgagatcctttttttctgcgcgtaatctgctgcttgcaaacaaaaaaaccaccgctaccagcggtggtttgtttgccggatcaagagctaccaactctttttccgaaggtaactggcttcagcagagcgcagataccaaatactgtccttctagtgtagccgtagttaggccaccacttcaagaactctgtagcaccgcctacatacctcgctctgctaatcctgttaccagtggctgctgccagtggcgataagtcgtgtcttaccgggttggactcaagacgatagttaccggataaggcgcagcggtcgggctgaacggggggttcgtgcacacagcccagcttggagcgaacgacctacaccgaactgagatacctacagcgtgagctatgagaaagcgccacgcttcccgaagggagaaaggcggacaggtatccggtaagcggcagggtcggaacaggagagcgcacgagggagcttccagggggaaacgcctggtatctttatagtcctgtcgggtttcgccacctctgacttgagcgtcgatttttgtgatgctcgtcaggggggcggagcctatggaaaaacgccagcaacgcggcctttttacggttcctggccttttgctggccttttgctcacatgttctttcctgcgttatcccctgattctgtggataaccgtattaccgcctttgagtgagctgataccgctcgccgcagccgaacgaccgagcgcagcgagtcagtgagcgaggaagcggaagagcgcctgatgcggtattttctccttacgcatctgtgcggtatttcacaccgcaatggtgcactctcagtacaatctgctctgatgccgcatagttaagccagtatacactccgctatcgctacgtgactgggtcatggctgcgccccgacacccgccaacacccgctgacgcgccctgacgggcttgtctgctcccggcatccgcttacagacaagctgtgaccgtctccgggagctgcatgtgtgatgcctccgtgtaagggggatttctgttcatgggggtaatgataccgatgaaacgagagaggatgctcacgatacgggttactgatgatgaacatgcccggttactggaacgttgtgagggtaaacaactggcggtatggatgcggcgggaccagagaaaaatcactcagggtcaatgccagcgcttcgttaatacagatgtaggtgttccacagggtagccagcagcatcctgcgatgcagatccggaacataatggtgcagggcgctgacttccgcgtttccagactttacgaaacacggaaaccgaagaccattcatgttgttgctcaggtcgcagacgttttgcagcagcagtcgcttcacgttcgctcgcgtatcggtgattcattctgctaaccagtaaggcaaccccgccagcctagccgggtcctcaacgacaggagcacgatcatgcgcacccgtggggccgccatgccggcgataatggcctgcttctcgccgaaacgtttggtggcgggaccagtgacgaaggcttgagcgagggcgtgcaagattccgaataccgcaagcgacaggccgatcatcgtcgcgctccagcgaaagcggtcctcgccgaaaatgacccagagcgctgccggcacctgtcctacgagttgcatgataaagaagacagtcataagtgcggcgacgatagtcatgccccgcgcccaccggaaggagctgactgggttgaaggctctcaagggcatcggtcgagatcccggtgcctaatgagtgagctaacttacattaattgcgttgcgctcactgcccgctttccagtcgggaaacctgtcgtgccagctgcattaatgaatcggccaacgcgcggggagaggcggtttgcgtattgggcgccagggtggtttttcttttcaccagtgagacgggcaacagctgattgcccttcaccgcctggccctgagagagttgcagcaagcggtccacgctggtttgccccagcaggcgaaaatcctgtttgatggtggttaacggcgggatataacatgagctgtcttcggtatcgtcgtatcccactaccgagatatccgcaccaacgcgcagcccggactcggtaatggcgcgcattgcgcccagcgccatctgatcgttggcaaccagcatcgcagtgggaacgatgccctcattcagcatttgcatggtttgttgaaaaccggacatggcactccagtcgccttcccgttccgctatcggctgaatttgattgcgagtgagatatttatgccagccagccagacgcagacgcgccgagacagaacttaatgggcccgctaacagcgcgatttgctggtgacccaatgcgaccagatgctccacgcccagtcgcgtaccgtcttcatgggagaaaataatactgttgatgggtgtctggtcagagacatcaagaaataacgccggaacattagtgcaggcagcttccacagcaatggcatcctggtcatccagcggatagttaatgatcagcccactgacgcgttgcgcgagaagattgtgcaccgccgctttacaggcttcgacgccgcttcgttctaccatcgacaccaccacgctggcacccagttgatcggcgcgagatttaatcgccgcgacaatttgcgacggcgcgtgcagggccagactggaggtggcaacgccaatcagcaacgactgtttgcccgccagttgttgtgccacgcggttgggaatgtaattcagctccgccatcgccgcttccactttttcccgcgttttcgcagaaacgtggctggcctggttcaccacgcgggaaacggtctgataagagacaccggcatactctgcgacatcgtataacgttactggtttcacattcaccaccctgaattgactctcttccgggcgctatcatgccataccgcgaaaggttttgcgccattcgatggtgtccgggatctcgacgctctcccttatgcgactcctgcattaggaagcagcccagtagtaggttgaggccgttgagcaccgccgccgcaaggaatggtgcatgcaaggagatggcgcccaacagtcccccggccacggggcctgccaccatacccacgccgaaacaagcgctcatgagcccgaagtggcgagcccgatcttccccatcggtgatgtcggcgatataggcgccagcaaccgcacctgtggcgccggtgatgccggccacgatgcgtccggcgtagaggatcgagatctcgatcccgcgaaattaatacgactcactataggggaattgtgagcggataacaattcccctctagaaataattttgtttaactttaagaaggagatatacatatgggcctgaaaatgaaaaaacgtagcgggaaaaaagcgtggatgctgctggttatgtcgctgctgattgcggcggttccgattacggcgagcgccgaggtgcagctggtggagtctgggggaggattggtgcagcctgggggctctgtgagactctcctgtgtagcctctggacgcatcttcagtagcaatgccatgggctggttccgccaggctccagggaaggagcgtgagtttgtagcggccattacctggaggagtggcggtagcgcgtactatgcagactccgcgaagggccgattcaccatctccagagacaacgccaagaacacggtgtatttgcaaatgaacagcctgaaacctgaggacacggccgtttattattgtgcagctggtggtagttcctggttaagttttccgccggactactggggccaggggacccaggtcaccgtctcctcaagacaccgccagccgagaggttgggaacagctgccgaccggagctgaatttctgggcgatggtggggatgttagtttttctacccgtggcacacagaattggaccgttgaacggttattacaagcacatcgtcagctggaagaaagaggttatgtgtttgttgggtatcatggtacatttttagaagcagcccagtctattgtttttggcggtgttcgtgcccgtagccaggatctggatgcaatttggagaggtttttatattgcgggtgatccggcgctggcatatggttacgcacaggatcaggaaccagatgcacgtggtcgtattcgtaatggtgccctgttacgggtgtatgttccccgttccagcctgccgggtttttatcgtacctctttaacactggcagccccggaagcagcaggtgaagtggaacgtctgattggccatccgctgccgctgcgcttagatgcaattaccggtccggaagaagaaggtgggcggttagaaaccattctgggttggccgctggcagaaagaacagtggttataccgagcgcgattcctaccgatcctcgtaatgtggggggtgatttagatccgagcagcattccggataaagagcaggcgattagcgcgctgccggattatgcaagccaaccggggaaaccgccgcgtgaagacttaaaacatcatcaccatcatcattaagatccggctgctaacaaagcccgaaaggaagctgagttggctgctgccaccgctgagcaataactagcataaccccttggggcctctaaacgggtcttgaggggttttttgctgaaaggaggaactatatccggat

SEQ ID NO: 48 - DNA, 6196 bp, synthetic construct
  source 1..6196: mol_type = other DNA
tggcgaatgggacgcgccctgtagcggcgcattaagcgcggcgggtgtggtggttacgcgcagcgtgaccgctacacttgccagcgccctagcgcccgctcctttcgctttcttcccttcctttctcgccacgttcgccggctttccccgtcaagctctaaatcgggggctccctttagggttccgatttagtgctttacggcacctcgaccccaaaaaacttgattagggtgatggttcacgtagtgggccatcgccctgatagacggtttttcgccctttgacgttggagtccacgttctttaatagtggactcttgttccaaactggaacaacactcaaccctatctcggtctattcttttgatttataagggattttgccgatttcggcctattggttaaaaaatgagctgatttaacaaaaatttaacgcgaattttaacaaaatattaacgcttacaatttaggtggcacttttcggggaaatgtgcgcggaacccctatttgtttatttttctaaatacattcaaatatgtatccgctcatgaattaattcttagaaaaactcatcgagcatcaaatgaaactgcaatttattcatatcaggattatcaataccatatttttgaaaaagccgtttctgtaatgaaggagaaaactcaccgaggcagttccataggatggcaagatcctggtatcggtctgcgattccgactcgtccaacatcaatacaacctattaatttcccctcgtcaaaaataaggttatcaagtgagaaatcaccatgagtgacgactgaatccggtgagaatggcaaaagtttatgcatttctttccagacttgttcaacaggccagccattacgctcgtcatcaaaatcactcgcatcaaccaaaccgttattcattcgtgattgcgcctgagcgagacgaaatacgcgatcgctgttaaaaggacaattacaaacaggaatcgaatgcaaccggcgcaggaacactgccagcgcatcaacaatattttcacctgaatcaggatattcttctaatacctggaatgctgttttcccggggatcgcagtggtgagtaaccatgcatcatcaggagtacggataaaatgcttgatggtcggaagaggcataaattccgtcagccagtttagtctgaccatctcatctgtaacatcattggcaacgctacctttgccatgtttcagaaacaactctggcgcatcgggcttcccatacaatcgatagattgtcgcacctgattgcccgacattatcgcgagcccatttatacccatataaatcagcatccatgttggaatttaatcgcggcctagagcaagacgtttcccgttgaatatggctcataacaccccttgtattactgtttatgtaagcagacagttttattgttcatgaccaaaatcccttaacgtgagttttcgttccactgagcgtcagaccccgtagaaaagatcaaaggatcttcttgagatcctttttttctgcgcgtaatctgctgcttgcaaacaaaaaaaccaccgctaccagcggtggtttgtttgccggatcaagagctaccaactctttttccgaaggtaactggcttcagcagagcgcagataccaaatactgtccttctagtgtagccgtagttaggccaccacttcaagaactctgtagcaccgcctacatacctcgctctgctaatcctgttaccagtggctgctgccagtggcgataagtcgtgtcttaccgggttggactcaagacgatagttaccggataaggcgcagcggtcgggctgaacggggggttcgtgcacacagcccagcttggagcgaacgacctacaccgaactgagatacctacagcgtgagctatgagaaagcgccacgcttcccgaagggagaaaggcggacaggtatccggtaagcggcagggtcggaacaggagagcgcacgagggagcttccagggggaaacgcctggtatctttatagtcctgtcgggtttcgccacctctgacttgagcgtcgatttttgtgatgctcgtcaggggggcggagcctatggaaaaacgccagcaacgcggcctttttacggttcctggccttttgctggccttttgctcacatgttctttcctgcgttatcccctgattctgtggataaccgtattaccgcctttgagtgagctgataccgctcgccgcagccgaacgaccgagcgcagcgagtcagtgagcgaggaagcggaagagcgcctgatgcggtattttctccttacgcatctgtgcggtatttcacaccgcaatggtgcactctcagtacaatctgctctgatgccgcatagttaagccagtatacactccgctatcgctacgtgactgggtcatggctgcgccccgacacccgccaacacccgctgacgcgccctgacgggcttgtctgctcccggcatccgcttacagacaagctgtgaccgtctccgggagctgcatgtgtgatgcctccgtgtaagggggatttctgttcatgggggtaatgataccgatgaaacgagagaggatgctcacgatacgggttactgatgatgaacatgcccggttactggaacgttgtgagggtaaacaactggcggtatggatgcggcgggaccagagaaaaatcactcagggtcaatgccagcgcttcgttaatacagatgtaggtgttccacagggtagccagcagcatcctgcgatgcagatccggaacataatggtgcagggcgctgacttccgcgtttccagactttacgaaacacggaaaccgaagaccattcatgttgttgctcaggtcgcagacgttttgcagcagcagtcgcttcacgttcgctcgcgtatcggtgattcattctgctaaccagtaaggcaaccccgccagcctagccgggtcctcaacgacaggagcacgatcatgcgcacccgtggggccgccatgccggcgataatggcctgcttctcgccgaaacgtttggtggcgggaccagtgacgaaggcttgagcgagggcgtgcaagattccgaataccgcaagcgacaggccgatcatcgtcgcgctccagcgaaagcggtcctcgccgaaaatgacccagagcgctgccggcacctgtcctacgagttgcatgataaagaagacagtcataagtgcggcgacgatagtcatgccccgcgcccaccggaaggagctgactgggttgaaggctctcaagggcatcggtcgagatcccggtgcctaatgagtgagctaacttacattaattgcgttgcgctcactgcccgctttccagtcgggaaacctgtcgtgccagctgcattaatgaatcggccaacgcgcggggagaggcggtttgcgtattgggcgccagggtggtttttcttttcaccagtgagacgggcaacagctgattgcccttcaccgcctggccctgagagagttgcagcaagcggtccacgctggtttgccccagcaggcgaaaatcctgtttgatggtggttaacggcgggatataacatgagctgtcttcggtatcgtcgtatcccactaccgagatatccgcaccaacgcgcagcccggactcggtaatggcgcgcattgcgcccagcgccatctgatcgttggcaaccagcatcgcagtgggaacgatgccctcattcagcatttgcatggtttgttgaaaaccggacatggcactccagtcgccttcccgttccgctatcggctgaatttgattgcgagtgagatatttatgccagccagccagacgcagacgcgccgagacagaacttaatgggcccgctaacagcgcgatttgctggtgacccaatgcgaccagatgctccacgcccagtcgcgtaccgtcttcatgggagaaaataatactgttgatgggtgtctggtcagagacatcaagaaataacgccggaacattagtgcaggcagcttccacagcaatggcatcctggtcatccagcggatagttaatgatcagcccactgacgcgttgcgcgagaagattgtgcaccgccgctttacaggcttcgacgccgcttcgttctaccatcgacaccaccacgctggcacccagttgatcggcgcgagatttaatcgccgcgacaatttgcgacggcgcgtgcagggccagactggaggtggcaacgccaatcagcaacgactgtttgcccgccagttgttgtgccacgcggttgggaatgtaattcagctccgccatcgccgcttccactttttcccgcgttttcgcagaaacgtggctggcctggttcaccacgcgggaaacggtctgataagagacaccggcatactctgcgacatcgtataacgttactggtttcacattcaccaccctgaattgactctcttccgggcgctatcatgccataccgcgaaaggttttgcgccattcgatggtgtccgggatctcgacgctctcccttatgcgactcctgcattaggaagcagcccagtagtaggttgaggccgttgagcaccgccgccgcaaggaatggtgcatgcaaggagatggcgcccaacagtcccccggccacggggcctgccaccatacccacgccgaaacaagcgctcatgagcccgaagtggcgagcccgatcttccccatcggtgatgtcggcgatataggcgccagcaaccgcacctgtggcgccggtgatgccggccacgatgcgtccggcgtagaggatcgagatctcgatcccgcgaaattaatacgactcactataggggaattgtgagcggataacaattcccctctagaaataattttgtttaactttaagaaggagatatacatatgggcctgaaaatgaaaaaacgtagcgggaaaaaagcgtggatgctgctggttatgtcgctgctgattgcggcggttccgattacggcgagcgccgaggtgcagctggtggagtctgggggaggcttggtgcagcctggggggtctctgagactctcctgtgtagcctctggaagcatcgtcagaattaataccatgggctggtaccgccagactccagggaagcagcgcgagttggtcgcagatattaccagtggtggtaacataaactatatagacgccgtgaagggccgattcaccatctccagagacaacaccaagaagagggtgtatctgcaaatgaacagcctgaaacctgaggacacggccgtctattactgtaatgcagagatcgttgttctggtgggagtttggacccagcgtgcgcggaccggcaactactggggccaggggacccaggtcaccgtctcctcaagacaccgccagccgagaggttgggaacagctgccgaccggagctgaatttctgggcgatggtggggatgttagtttttctacccgtggcacacagaattggaccgttgaacggttattacaagcacatcgtcagctggaagaaagaggttatgtgtttgttgggtatcatggtacatttttagaagcagcccagtctattgtttttggcggtgttcgtgcccgtagccaggatctggatgcaatttggagaggtttttatattgcgggtgatccggcgctggcatatggttacgcacaggatcaggaaccagatgcacgtggtcgtattcgtaatggtgccctgttacgggtgtatgttccccgttccagcctgccgggtttttatcgtacctctttaacactggcagccccggaagcagcaggtgaagtggaacgtctgattggccatccgctgccgctgcgcttagatgcaattaccggtccggaagaagaaggtgggcggttagaaaccattctgggttggccgctggcagaaagaacagtggttataccgagcgcgattcctaccgatcctcgtaatgtggggggtgatttagatccgagcagcattccggataaagagcaggcgattagcgcgctgccggattatgcaagccaaccggggaaaccgccgcgtgaagacttaaaacatcatcaccatcatcattaagatccggctgctaacaaagcccgaaaggaagctgagttggctgctgccaccgctgagcaataactagcataaccccttggggcctctaaacgggtcttgaggggttttttgctgaaaggaggaactatatccggat

SEQ ID NO: 49 - DNA, 5860 bp, synthetic construct
  source 1..5860: mol_type = other DNA
catggtcatagctgtttcctttaatgcccatggcgtttaccaatgcttaatcagtgaggcacctatctcagcgatctgtctatttcgttcatccatagttgcctgactccccgtcgtgtagataactacgatacgggagggcttaccatctggccccagtgctgcaatgataccgcgacttccacgctcaccggctccagatttatcagcaataaaccagccagccggaagggccgagcgcagaagtggtcctgcaactttatccgcctccatccagtctattaattgttgccgggaagctagagtaagtagttcgccagttaatagtttgcgcaacgttgttgccattgctacaggcatcgtggtgtcacgctcgtcgtttggtatggcttcattcagctccggttcccaacgatcaaggcgagttacatgatcccccatgttgtgcaaaaaagcggttagctccttcggtcctccgatcgttgtcagaagtaagttggccgcagtgttatcactcatggttatggcagcactgcataattctcttactgtcatgccatccgtaagatgcttttctgtgactggtgagtactcaaccaagtcattctgagaatagtgtatgcggcgaccgagttgctcttgcccggcgtcaatacgggataataccgcgccacatagcagaactttaaaagtgctcatcattggaaaacgttcttcggggcgaaaactctcaaggatcttaccgctgttgagatccagttcgatgtaacccactcgtgcacccaactgatcttcagcatcttttactttcaccagcgtttctgggtgagcaaaaacaggaaggcaaaatgccgcaaaaaagggaataagggcgacacggaaatgttgaatactcatactcttcctttttcaatattattgaagcatttatcagggttattgtctcatgagcggatacatatttgaatgtatttagaaaaataaacaaataggggttccgcgcacatttccccgaaaagtgccacctgacgtctaagaaaccattattatcatgacattaacctataaaaataggcgtatcacgaggcccttaggccaaataggccgttcagatccttccgtatttagccagtatgttctctagtgtggttcgttgtttttgcgtgagccatgagaacgaaccattgagatcatgcttactttgcatgtcactcaaaaattttgcctcaaaactggtgagctgaatttttgcagttaaagcatcgtgtagtgtttttcttagtccgttacgtaggtaggaatctgatgtaatggttgttggtattttgtcaccattcatttttatctggttgttctcaagttcggttacgagatccatttgtctatctagttcaacttggaaaatcaacgtatcagtcgggcggcctcgcttatcaaccaccaatttcatattgctgtaagtgtttaaatctttacttattggtttcaaaacccattggttaagccttttaaactcatggtagttattttcaagcattaacatgaacttaaattcatcaaggctaatctctatatttgccttgtgagttttcttttgtgttagttcttttaataaccactcataaatcctcatagagtatttgttttcaaaagacttaacatgttccagattatattttatgaatttttttaactggaaaagataaggcaatatctcttcactaaaaactaattctaatttttcgcttgagaacttggcatagtttgtccactggaaaatctcaaagcctttaaccaaaggattcctgatttccacagttctcgtcatcagctctctggttgctttagctaatacaccataagcattttccctactgatgttcatcatctgagcgtattggttataagtgaacgataccgtccgttctttccttgtagggttttcaatcgtggggttgagtagtgccacacagcataaaattagcttggtttcatgctccgttaagtcatagcgactaatcgctagttcatttgctttgaaaacaactaattcagacatacatctcaattggtctaggtgattttaatcactataccaattgagatgggctagtcaatgataattactagtccttttcctttgagttgtgggtatctgtaaattctgctagacctttgctggaaaacttgtaaattctgctagaccctctgtaaattccgctagacctttgtgtgttttttttgtttatattcaagtggttataatttatagaataaagaaagaataaaaaaagataaaaagaatagatcccagccctgtgtataactcactactttagtcagttccgcagtattacaaaaggatgtcgcaaacgctgtttgctcctctacaaaacagaccttaaaaccctaaaggcttaagtagcaccctcgcaagctcgggcaaatcgctgaatattccttttgtctccgaccatcaggcacctgagtcgctgtctttttcgtgacattcagttcgctgcgctcacggctctggcagtgaatgggggtaaatggcactacaggcgccttttatggattcatgcaaggaaactacccataatacaagaaaagcccgtcacgggcttctcagggcgttttatggcgggtctgctatgtggtgctatctgactttttgctgttcagcagttcctgccctctgattttccagtctgaccacttcggattatcccgtgacaggtcattcagactggctaatgcacccagtaaggcagcggtatcatcaacaggcttacccgtcttactgtcaagaggacatccggtcagataaccgtcatcttcggctactgtctagggcggcggatttgtcctactcaggagagcgttcaccgacaaacaacagataaaacgaaaggcccagtctttcgactgagcctttcgttttatttgatgcactagtgccgatcatattcaataacccttaatataacttcgtataatgtatgctatacgaagttattaggtctgaagaggagtttacgtcccatatgggcgagctcgatatcaaattacgccccgccctgccactcatcgcagtactgttgtaattcattaagcattctgccgacatggaagccatcacagacggcatgatgaacctgaatcgccagcggcatcagcaccttgtcgccttgcgtataatatttgcccatggtgaaaacgggggcgaagaagttgtccatattggccacgtttaaatcaaaactggtgaaactcacccagggattggctgagacgaaaaacatattctcaataaaccctttagggaaataggccaggttttcaccgtaacacgccacatcttgcgaatatatgtgtagaaactgccggaaatcgtcgtggtattcactccagagcgatgaaaacgtttcagtttgctcatggaaaacggtgtaacaagggtgaacactatcccatatcaccagctcaccgtctttcattgccatacgaaattccggatgagcattcatcaggcgggcaagaatgtgaataaaggccggataaaacttgtgcttatttttctttacggtctttaaaaaggccgtaatatccagctgaacggtctggttataggtacattgagcaactgactgaaatgcctcaaaatgttctttacgatgccattgggatatatcaacggtggtatatccagtgatttttttctccattttagcttccttagctcctgaaaatctcgataactcaaaaaatacgcccggtagtgatcttatttcattatggtgaaagttggaacctcttacgtgccgatcaacgtctcattttcgccagatatcgccaagcttaggatccggaacccttaatataacttcgtataatgtatgctatacgaagttattaggtccctcgaagaggttcactagctatctagagcttggactcctgttgatagatccagtaatgacctcagaactccatctggatttgttcagaacgctcggttgccgccgggcgttttttattggtgagaatccaagcccgggaaacgggatcctgatcttgatccgccgcaaagtttgagcgaagtcaataaactctctacccattcagggcaatatctctcttgcaggtgaatgcaacgtcaagcgatggcctacttgcggccgcaagattaaagaggagaaggatgggcctgaaaatgaaaaaacgtagcgggaaaaaagcgtggatgctgctggttatgtcgctgctgattgcggcggttccgattacggcgagcgccgaggttcaattagtggaatctggcgggggattggttcaagccggtgagtccttgcgtttgagctgcgccgcatctgggagcacatttgatttcaaagtgatgggctggtatcgtcagccgcccggaaaacagcgcgagggtgtagcagccatccgcttgagcggaaatatgcactacgccgagtctgtaaaagggcgctttgctatttccaaagcgaacgctaagaacacagtgtatcttcagatgaactccttgcgtcccgaagacactgccgtttattattgcaaagtaaacatccgtgggcaagactactggggtcaaggaacgcaggtcacagtctcttctggctctggccctgaaggtggtagcctggcggcactgaccgcacaccaagcatgtcatctgccactggaaacctttacccgtcatcgtcagccgcgtggctgggaacaactggaacaatgtggatatccggtgcagagactggtcgcattatatctggcagcacgtctgagttggaatcaggttgatcaagttattcgtaacgcacttgcctcaccgggtagcggtggtgatttaggtgaggcaattcgtgaacaacctgaacaggcacgcttagcattaacccttgcagccgcagaaagtgaaagatttgtgcgtcagggtactggtaatgatgaggccggtgcagcaaatgggccggcagacagcggagatgcattattagagagaaattatcctaccggcgcagaatttctgggtgatgggggtgatgttagtttttcaacacgcgggacacagaattggaccgtggaacgtttactgcaggcacatcgtcagctggaagaacgcggttatgtttttgttggttatcatgggacgtttctggaggcagcacagagcattgtctttggcggtgtgcgggcgcgtagccaggatcttgatgcaatttggcgtggtttttatattgcgggtgatcctgcgctggcgtatggatatgcgcaggatcaggagccggatgcgcgtggtcgtattcgtaatggtgccctgctgcgggtttatgttccgcgtagctcactgccggggttttatagaacaagcttaacactggctgcgccggaagcagcaggtgaagttgaacgtctgattggccatccgctgccgttacgtttagatgcaattactggtccggaagaagaaggtggtcgcctggaaaccattctgggttggccgctggcagaaagaaccgtggttataccttccgcaataccgaccgatcctcggaatgtggggggtgatttagatcctagcagcattcctgataaagaacaggcaatttctgctctgcctgattatgcatcacagccgggtaaaccgccgcgtgaagatttaaagcatcatcaccatcatcattaagatccggctctggaagatccgcgcgtaccgagttctaattcactggccgtcgttttacaacatacgatgaaggcgataagtcgcgtaagttgctagcccacgcggctcaccttcacgggtgggcctttcttcgcgatccacatg

SEQ ID NO: 50 - DNA, 5872 bp, synthetic construct
  source 1..5872: mol_type = other DNA
catggtcatagctgtttcctttaatgcccatggcgtttaccaatgcttaatcagtgaggcacctatctcagcgatctgtctatttcgttcatccatagttgcctgactccccgtcgtgtagataactacgatacgggagggcttaccatctggccccagtgctgcaatgataccgcgacttccacgctcaccggctccagatttatcagcaataaaccagccagccggaagggccgagcgcagaagtggtcctgcaactttatccgcctccatccagtctattaattgttgccgggaagctagagtaagtagttcgccagttaatagtttgcgcaacgttgttgccattgctacaggcatcgtggtgtcacgctcgtcgtttggtatggcttcattcagctccggttcccaacgatcaaggcgagttacatgatcccccatgttgtgcaaaaaagcggttagctccttcggtcctccgatcgttgtcagaagtaagttggccgcagtgttatcactcatggttatggcagcactgcataattctcttactgtcatgccatccgtaagatgcttttctgtgactggtgagtactcaaccaagtcattctgagaatagtgtatgcggcgaccgagttgctcttgcccggcgtcaatacgggataataccgcgccacatagcagaactttaaaagtgctcatcattggaaaacgttcttcggggcgaaaactctcaaggatcttaccgctgttgagatccagttcgatgtaacccactcgtgcacccaactgatcttcagcatcttttactttcaccagcgtttctgggtgagcaaaaacaggaaggcaaaatgccgcaaaaaagggaataagggcgacacggaaatgttgaatactcatactcttcctttttcaatattattgaagcatttatcagggttattgtctcatgagcggatacatatttgaatgtatttagaaaaataaacaaataggggttccgcgcacatttccccgaaaagtgccacctgacgtctaagaaaccattattatcatgacattaacctataaaaataggcgtatcacgaggcccttaggccaaataggccgttcagatccttccgtatttagccagtatgttctctagtgtggttcgttgtttttgcgtgagccatgagaacgaaccattgagatcatgcttactttgcatgtcactcaaaaattttgcctcaaaactggtgagctgaatttttgcagttaaagcatcgtgtagtgtttttcttagtccgttacgtaggtaggaatctgatgtaatggttgttggtattttgtcaccattcatttttatctggttgttctcaagttcggttacgagatccatttgtctatctagttcaacttggaaaatcaacgtatcagtcgggcggcctcgcttatcaaccaccaatttcatattgctgtaagtgtttaaatctttacttattggtttcaaaacccattggttaagccttttaaactcatggtagttattttcaagcattaacatgaacttaaattcatcaaggctaatctctatatttgccttgtgagttttcttttgtgttagttcttttaataaccactcataaatcctcatagagtatttgttttcaaaagacttaacatgttccagattatattttatgaatttttttaactggaaaagataaggcaatatctcttcactaaaaactaattctaatttttcgcttgagaacttggcatagtttgtccactggaaaatctcaaagcctttaaccaaaggattcctgatttccacagttctcgtcatcagctctctggttgctttagctaatacaccataagcattttccctactgatgttcatcatctgagcgtattggttataagtgaacgataccgtccgttctttccttgtagggttttcaatcgtggggttgagtagtgccacacagcataaaattagcttggtttcatgctccgttaagtcatagcgactaatcgctagttcatttgctttgaaaacaactaattcagacatacatctcaattggtctaggtgattttaatcactataccaattgagatgggctagtcaatgataattactagtccttttcctttgagttgtgggtatctgtaaattctgctagacctttgctggaaaacttgtaaattctgctagaccctctgtaaattccgctagacctttgtgtgttttttttgtttatattcaagtggttataatttatagaataaagaaagaataaaaaaagataaaaagaatagatcccagccctgtgtataactcactactttagtcagttccgcagtattacaaaaggatgtcgcaaacgctgtttgctcctctacaaaacagaccttaaaaccctaaaggcttaagtagcaccctcgcaagctcgggcaaatcgctgaatattccttttgtctccgaccatcaggcacctgagtcgctgtctttttcgtgacattcagttcgctgcgctcacggctctggcagtgaatgggggtaaatggcactacaggcgccttttatggattcatgcaaggaaactacccataatacaagaaaagcccgtcacgggcttctcagggcgttttatggcgggtctgctatgtggtgctatctgactttttgctgttcagcagttcctgccctctgattttccagtctgaccacttcggattatcccgtgacaggtcattcagactggctaatgcacccagtaaggcagcggtatcatcaacaggcttacccgtcttactgtcaagaggacatccggtcagataaccgtcatcttcggctactgtctagggcggcggatttgtcctactcaggagagcgttcaccgacaaacaacagataaaacgaaaggcccagtctttcgactgagcctttcgttttatttgatgcactagtgccgatcatattcaataacccttaatataacttcgtataatgtatgctatacgaagttattaggtctgaagaggagtttacgtcccatatgggcgagctcgatatcaaattacgccccgccctgccactcatcgcagtactgttgtaattcattaagcattctgccgacatggaagccatcacagacggcatgatgaacctgaatcgccagcggcatcagcaccttgtcgccttgcgtataatatttgcccatggtgaaaacgggggcgaagaagttgtccatattggccacgtttaaatcaaaactggtgaaactcacccagggattggctgagacgaaaaacatattctcaataaaccctttagggaaataggccaggttttcaccgtaacacgccacatcttgcgaatatatgtgtagaaactgccggaaatcgtcgtggtattcactccagagcgatgaaaacgtttcagtttgctcatggaaaacggtgtaacaagggtgaacactatcccatatcaccagctcaccgtctttcattgccatacgaaattccggatgagcattcatcaggcgggcaagaatgtgaataaaggccggataaaacttgtgcttatttttctttacggtctttaaaaaggccgtaatatccagctgaacggtctggttataggtacattgagcaactgactgaaatgcctcaaaatgttctttacgatgccattgggatatatcaacggtggtatatccagtgatttttttctccattttagcttccttagctcctgaaaatctcgataactcaaaaaatacgcccggtagtgatcttatttcattatggtgaaagttggaacctcttacgtgccgatcaacgtctcattttcgccagatatcgccaagcttaggatccggaacccttaatataacttcgtataatgtatgctatacgaagttattaggtccctcgaagaggttcactagctatctagagcttggactcctgttgatagatccagtaatgacctcagaactccatctggatttgttcagaacgctcggttgccgccgggcgttttttattggtgagaatccaagcccgggaaacgggatcctgatcttgatccgccgcaaagtttgagcgaagtcaataaactctctacccattcagggcaatatctctcttgcaggtgaatgcaacgtcaagcgatggcctacttgcggccgcaagattaaagaggagaaggatgggcctgaaaatgaaaaaacgtagcgggaaaaaagcgtggatgctgctggttatgtcgctgctgattgcggcggttccgattacggcgagcgccgaggtgcagctggtggagtctgggggaggattggtgcagcctgggggctctgtgagactctcctgtgtagcctctggacgcatcttcagtagcaatgccatgggctggttccgccaggctccagggaaggagcgtgagtttgtagcggccattacctggaggagtggcggtagcgcgtactatgcagactccgcgaagggccgattcaccatctccagagacaacgccaagaacacggtgtatttgcaaatgaacagcctgaaacctgaggacacggccgtttattattgtgcagctggtggtagttcctggttaagttttccgccggactactggggccaggggacccaggtcaccgtctcctcacctgaaggtggtagcctggcggcactgaccgcacaccaagcatgtcatctgccactggaaacctttacccgtcatcgtcagccgcgtggctgggaacaactggaacaatgtggatatccggtgcagagactggtcgcattatatctggcagcacgtctgagttggaatcaggttgatcaagttattcgtaacgcacttgcctcaccgggtagcggtggtgatttaggtgaggcaattcgtgaacaacctgaacaggcacgcttagcattaacccttgcagccgcagaaagtgaaagatttgtgcgtcagggtactggtaatgatgaggccggtgcagcaaatgggccggcagacagcggagatgcattattagagagaaattatcctaccggcgcagaatttctgggtgatgggggtgatgttagtttttcaacacgcgggacacagaattggaccgtggaacgtttactgcaggcacatcgtcagctggaagaacgcggttatgtttttgttggttatcatgggacgtttctggaggcagcacagagcattgtctttggcggtgtgcgggcgcgtagccaggatcttgatgcaatttggcgtggtttttatattgcgggtgatcctgcgctggcgtatggatatgcgcaggatcaggagccggatgcgcgtggtcgtattcgtaatggtgccctgctgcgggtttatgttccgcgtagctcactgccggggttttatagaacaagcttaacactggctgcgccggaagcagcaggtgaagttgaacgtctgattggccatccgctgccgttacgtttagatgcaattactggtccggaagaagaaggtggtcgcctggaaaccattctgggttggccgctggcagaaagaaccgtggttataccttccgcaataccgaccgatcctcggaatgtggggggtgatttagatcctagcagcattcctgataaagaacaggcaatttctgctctgcctgattatgcatcacagccgggtaaaccgccgcgtgaagatttaaagcatcatcaccatcatcattaagatccggctctggaagatccgcgcgtaccgagttctaattcactggccgtcgttttacaacatacgatgaaggcgataagtcgcgtaagttgctagcccacgcggctcaccttcacgggtgggcctttcttcgcgatccacatg

SEQ ID NO: 51 - DNA, 5883 bp, synthetic construct
  source 1..5883: mol_type = other DNA
catggtcatagctgtttcctttaatgcccatggcgtttaccaatgcttaatcagtgaggcacctatctcagcgatctgtctatttcgttcatccatagttgcctgactccccgtcgtgtagataactacgatacgggagggcttaccatctggccccagtgctgcaatgataccgcgacttccacgctcaccggctccagatttatcagcaataaaccagccagccggaagggccgagcgcagaagtggtcctgcaactttatccgcctccatccagtctattaattgttgccgggaagctagagtaagtagttcgccagttaatagtttgcgcaacgttgttgccattgctacaggcatcgtggtgtcacgctcgtcgtttggtatggcttcattcagctccggttcccaacgatcaaggcgagttacatgatcccccatgttgtgcaaaaaagcggttagctccttcggtcctccgatcgttgtcagaagtaagttggccgcagtgttatcactcatggttatggcagcactgcataattctcttactgtcatgccatccgtaagatgcttttctgtgactggtgagtactcaaccaagtcattctgagaatagtgtatgcggcgaccgagttgctcttgcccggcgtcaatacgggataataccgcgccacatagcagaactttaaaagtgctcatcattggaaaacgttcttcggggcgaaaactctcaaggatcttaccgctgttgagatccagttcgatgtaacccactcgtgcacccaactgatcttcagcatcttttactttcaccagcgtttctgggtgagcaaaaacaggaaggcaaaatgccgcaaaaaagggaataagggcgacacggaaatgttgaatactcatactcttcctttttcaatattattgaagcatttatcagggttattgtctcatgagcggatacatatttgaatgtatttagaaaaataaacaaataggggttccgcgcacatttccccgaaaagtgccacctgacgtctaagaaaccattattatcatgacattaacctataaaaataggcgtatcacgaggcccttaggccaaataggccgttcagatccttccgtatttagccagtatgttctctagtgtggttcgttgtttttgcgtgagccatgagaacgaaccattgagatcatgcttactttgcatgtcactcaaaaattttgcctcaaaactggtgagctgaatttttgcagttaaagcatcgtgtagtgtttttcttagtccgttacgtaggtaggaatctgatgtaatggttgttggtattttgtcaccattcatttttatctggttgttctcaagttcggttacgagatccatttgtctatctagttcaacttggaaaatcaacgtatcagtcgggcggcctcgcttatcaaccaccaatttcatattgctgtaagtgtttaaatctttacttattggtttcaaaacccattggttaagccttttaaactcatggtagttattttcaagcattaacatgaacttaaattcatcaaggctaatctctatatttgccttgtgagttttcttttgtgttagttcttttaataaccactcataaatcctcatagagtatttgttttcaaaagacttaacatgttccagattatattttatgaatttttttaactggaaaagataaggcaatatctcttcactaaaaactaattctaatttttcgcttgagaacttggcatagtttgtccactggaaaatctcaaagcctttaaccaaaggattcctgatttccacagttctcgtcatcagctctctggttgctttagctaatacaccataagcattttccctactgatgttcatcatctgagcgtattggttataagtgaacgataccgtccgttctttccttgtagggttttcaatcgtggggttgagtagtgccacacagcataaaattagcttggtttcatgctccgttaagtcatagcgactaatcgctagttcatttgctttgaaaacaactaattcagacatacatctcaattggtctaggtgattttaatcactataccaattgagatgggctagtcaatgataattactagtccttttcctttgagttgtgggtatctgtaaattctgctagacctttgctggaaaacttgtaaattctgctagaccctctgtaaattccgctagacctttgtgtgttttttttgtttatattcaagtggttataatttatagaataaagaaagaataaaaaaagataaaaagaatagatcccagccctgtgtataactcactactttagtcagttccgcagtattacaaaaggatgtcgcaaacgctgtttgctcctctacaaaacagaccttaaaaccctaaaggcttaagtagcaccctcgcaagctcgggcaaatcgctgaatattccttttgtctccgaccatcaggcacctgagtcgctgtctttttcgtgacattcagttcgctgcgctcacggctctggcagtgaatgggggtaaatggcactacaggcgccttttatggattcatgcaaggaaactacccataatacaagaaaagcccgtcacgggcttctcagggcgttttatggcgggtctgctatgtggtgctatctgactttttgctgttcagcagttcctgccctctgattttccagtctgaccacttcggattatcccgtgacaggtcattcagactggctaatgcacccagtaaggcagcggtatcatcaacaggcttacccgtcttactgtcaagaggacatccggtcagataaccgtcatcttcggctactgtctagggcggcggatttgtcctactcaggagagcgttcaccgacaaacaacagataaaacgaaaggcccagtctttcgactgagcctttcgttttatttgatgcactagtgccgatcatattcaataacccttaatataacttcgtataatgtatgctatacgaagttattaggtctgaagaggagtttacgtcccatatgggcgagctcgatatcaaattacgccccgccctgccactcatcgcagtactgttgtaattcattaagcattctgccgacatggaagccatcacagacggcatgatgaacctgaatcgccagcggcatcagcaccttgtcgccttgcgtataatatttgcccatggtgaaaacgggggcgaagaagttgtccatattggccacgtttaaatcaaaactggtgaaactcacccagggattggctgagacgaaaaacatattctcaataaaccctttagggaaataggccaggttttcaccgtaacacgccacatcttgcgaatatatgtgtagaaactgccggaaatcgtcgtggtattcactccagagcgatgaaaacgtttcagtttgctcatggaaaacggtgtaacaagggtgaacactatcccatatcaccagctcaccgtctttcattgccatacgaaattccggatgagcattcatcaggcgggcaagaatgtgaataaaggccggataaaacttgtgcttatttttctttacggtctttaaaaaggccgtaatatccagctgaacggtctggttataggtacattgagcaactgactgaaatgcctcaaaatgttctttacgatgccattgggatatatcaacggtggtatatccagtgatttttttctccattttagcttccttagctcctgaaaatctcgataactcaaaaaatacgcccggtagtgatcttatttcattatggtgaaagttggaacctcttacgtgccgatcaacgtctcattttcgccagatatcgccaagcttaggatccggaacccttaatataacttcgtataatgtatgctatacgaagttattaggtccctcgaagaggttcactagctatctagagcttggactcctgttgatagatccagtaatgacctcagaactccatctggatttgttcagaacgctcggttgccgccgggcgttttttattggtgagaatccaagcccgggaaacgggatcctgatcttgatccgccgcaaagtttgagcgaagtcaataaactctctacccattcagggcaatatctctcttgcaggtgaatgcaacgtcaagcgatggcctacttgcggccgcaagattaaagaggagaaggatgggcctgaaaatgaaaaaacgtagcgggaaaaaagcgtggatgctgctggttatgtcgctgctgattgcggcggttccgattacggcgagcgccgaggtgcagctggtggagtctgggggaggcttggtgcagcctggggggtctctgagactctcctgtgtagcctctggaagcatcgtcagaattaataccatgggctggtaccgccagactccagggaagcagcgcgagttggtcgcagatattaccagtggtggtaacataaactatatagacgccgtgaagggccgattcaccatctccagagacaacaccaagaagagggtgtatctgcaaatgaacagcctgaaacctgaggacacggccgtctattactgtaatgcagagatcgttgttctggtgggagtttggacccagcgtgcgcggaccggcaactactggggccaggggacccaggtcaccgtctcctccctgaaggtggtagcctggcggcactgaccgcacaccaagcatgtcatctgccactggaaacctttacccgtcatcgtcagccgcgtggctgggaacaactggaacaatgtggatatccggtgcagagactggtcgcattatatctggcagcacgtctgagttggaatcaggttgatcaagttattcgtaacgcacttgcctcaccgggtagcggtggtgatttaggtgaggcaattcgtgaacaacctgaacaggcacgcttagcattaacccttgcagccgcagaaagtgaaagatttgtgcgtcagggtactggtaatgatgaggccggtgcagcaaatgggccggcagacagcggagatgcattattagagagaaattatcctaccggcgcagaatttctgggtgatgggggtgatgttagtttttcaacacgcgggacacagaattggaccgtggaacgtttactgcaggcacatcgtcagctggaagaacgcggttatgtttttgttggttatcatgggacgtttctggaggcagcacagagcattgtctttggcggtgtgcgggcgcgtagccaggatcttgatgcaatttggcgtggtttttatattgcgggtgatcctgcgctggcgtatggatatgcgcaggatcaggagccggatgcgcgtggtcgtattcgtaatggtgccctgctgcgggtttatgttccgcgtagctcactgccggggttttatagaacaagcttaacactggctgcgccggaagcagcaggtgaagttgaacgtctgattggccatccgctgccgttacgtttagatgcaattactggtccggaagaagaaggtggtcgcctggaaaccattctgggttggccgctggcagaaagaaccgtggttataccttccgcaataccgaccgatcctcggaatgtggggggtgatttagatcctagcagcattcctgataaagaacaggcaatttctgctctgcctgattatgcatcacagccgggtaaaccgccgcgtgaagatttaaagcatcatcaccatcatcattaagatccggctctggaagatccgcgcgtaccgagttctaattcactggccgtcgttttacaacatacgatgaaggcgataagtcgcgtaagttgctagcccacgcggctcaccttcacgggtgggcctttcttcgcgatccacatg

SEQ ID NO: 52 - DNA, 6142 bp, synthetic construct
  source 1..6142: mol_type = other DNA
tggcgaatgggacgcgccctgtagcggcgcattaagcgcggcgggtgtggtggttacgcgcagcgtgaccgctacacttgccagcgccctagcgcccgctcctttcgctttcttcccttcctttctcgccacgttcgccggctttccccgtcaagctctaaatcgggggctccctttagggttccgatttagtgctttacggcacctcgaccccaaaaaacttgattagggtgatggttcacgtagtgggccatcgccctgatagacggtttttcgccctttgacgttggagtccacgttctttaatagtggactcttgttccaaactggaacaacactcaaccctatctcggtctattcttttgatttataagggattttgccgatttcggcctattggttaaaaaatgagctgatttaacaaaaatttaacgcgaattttaacaaaatattaacgcttacaatttaggtggcacttttcggggaaatgtgcgcggaacccctatttgtttatttttctaaatacattcaaatatgtatccgctcatgaattaattcttagaaaaactcatcgagcatcaaatgaaactgcaatttattcatatcaggattatcaataccatatttttgaaaaagccgtttctgtaatgaaggagaaaactcaccgaggcagttccataggatggcaagatcctggtatcggtctgcgattccgactcgtccaacatcaatacaacctattaatttcccctcgtcaaaaataaggttatcaagtgagaaatcaccatgagtgacgactgaatccggtgagaatggcaaaagtttatgcatttctttccagacttgttcaacaggccagccattacgctcgtcatcaaaatcactcgcatcaaccaaaccgttattcattcgtgattgcgcctgagcgagacgaaatacgcgatcgctgttaaaaggacaattacaaacaggaatcgaatgcaaccggcgcaggaacactgccagcgcatcaacaatattttcacctgaatcaggatattcttctaatacctggaatgctgttttcccggggatcgcagtggtgagtaaccatgcatcatcaggagtacggataaaatgcttgatggtcggaagaggcataaattccgtcagccagtttagtctgaccatctcatctgtaacatcattggcaacgctacctttgccatgtttcagaaacaactctggcgcatcgggcttcccatacaatcgatagattgtcgcacctgattgcccgacattatcgcgagcccatttatacccatataaatcagcatccatgttggaatttaatcgcggcctagagcaagacgtttcccgttgaatatggctcataacaccccttgtattactgtttatgtaagcagacagttttattgttcatgaccaaaatcccttaacgtgagttttcgttccactgagcgtcagaccccgtagaaaagatcaaaggatcttcttgagatcctttttttctgcgcgtaatctgctgcttgcaaacaaaaaaaccaccgctaccagcggtggtttgtttgccggatcaagagctaccaactctttttccgaaggtaactggcttcagcagagcgcagataccaaatactgtccttctagtgtagccgtagttaggccaccacttcaagaactctgtagcaccgcctacatacctcgctctgctaatcctgttaccagtggctgctgccagtggcgataagtcgtgtcttaccgggttggactcaagacgatagttaccggataaggcgcagcggtcgggctgaacggggggttcgtgcacacagcccagcttggagcgaacgacctacaccgaactgagatacctacagcgtgagctatgagaaagcgccacgcttcccgaagggagaaaggcggacaggtatccggtaagcggcagggtcggaacaggagagcgcacgagggagcttccagggggaaacgcctggtatctttatagtcctgtcgggtttcgccacctctgacttgagcgtcgatttttgtgatgctcgtcaggggggcggagcctatggaaaaacgccagcaacgcggcctttttacggttcctggccttttgctggccttttgctcacatgttctttcctgcgttatcccctgattctgtggataaccgtattaccgcctttgagtgagctgataccgctcgccgcagccgaacgaccgagcgcagcgagtcagtgagcgaggaagcggaagagcgcctgatgcggtattttctccttacgcatctgtgcggtatttcacaccgcaatggtgcactctcagtacaatctgctctgatgccgcatagttaagccagtatacactccgctatcgctacgtgactgggtcatggctgcgccccgacacccgccaacacccgctgacgcgccctgacgggcttgtctgctcccggcatccgcttacagacaagctgtgaccgtctccgggagctgcatgtgtgatgcctccgtgtaagggggatttctgttcatgggggtaatgataccgatgaaacgagagaggatgctcacgatacgggttactgatgatgaacatgcccggttactggaacgttgtgagggtaaacaactggcggtatggatgcggcgggaccagagaaaaatcactcagggtcaatgccagcgcttcgttaatacagatgtaggtgttccacagggtagccagcagcatcctgcgatgcagatccggaacataatggtgcagggcgctgacttccgcgtttccagactttacgaaacacggaaaccgaagaccattcatgttgttgctcaggtcgcagacgttttgcagcagcagtcgcttcacgttcgctcgcgtatcggtgattcattctgctaaccagtaaggcaaccccgccagcctagccgggtcctcaacgacaggagcacgatcatgcgcacccgtggggccgccatgccggcgataatggcctgcttctcgccgaaacgtttggtggcgggaccagtgacgaaggcttgagcgagggcgtgcaagattccgaataccgcaagcgacaggccgatcatcgtcgcgctccagcgaaagcggtcctcgccgaaaatgacccagagcgctgccggcacctgtcctacgagttgcatgataaagaagacagtcataagtgcggcgacgatagtcatgccccgcgcccaccggaaggagctgactgggttgaaggctctcaagggcatcggtcgagatcccggtgcctaatgagtgagctaacttacattaattgcgttgcgctcactgcccgctttccagtcgggaaacctgtcgtgccagctgcattaatgaatcggccaacgcgcggggagaggcggtttgcgtattgggcgccagggtggtttttcttttcaccagtgagacgggcaacagctgattgcccttcaccgcctggccctgagagagttgcagcaagcggtccacgctggtttgccccagcaggcgaaaatcctgtttgatggtggttaacggcgggatataacatgagctgtcttcggtatcgtcgtatcccactaccgagatatccgcaccaacgcgcagcccggactcggtaatggcgcgcattgcgcccagcgccatctgatcgttggcaaccagcatcgcagtgggaacgatgccctcattcagcatttgcatggtttgttgaaaaccggacatggcactccagtcgccttcccgttccgctatcggctgaatttgattgcgagtgagatatttatgccagccagccagacgcagacgcgccgagacagaacttaatgggcccgctaacagcgcgatttgctggtgacccaatgcgaccagatgctccacgcccagtcgcgtaccgtcttcatgggagaaaataatactgttgatgggtgtctggtcagagacatcaagaaataacgccggaacattagtgcaggcagcttccacagcaatggcatcctggtcatccagcggatagttaatgatcagcccactgacgcgttgcgcgagaagattgtgcaccgccgctttacaggcttcgacgccgcttcgttctaccatcgacaccaccacgctggcacccagttgatcggcgcgagatttaatcgccgcgacaatttgcgacggcgcgtgcagggccagactggaggtggcaacgccaatcagcaacgactgtttgcccgccagttgttgtgccacgcggttgggaatgtaattcagctccgccatcgccgcttccactttttcccgcgttttcgcagaaacgtggctggcctggttcaccacgcgggaaacggtctgataagagacaccggcatactctgcgacatcgtataacgttactggtttcacattcaccaccctgaattgactctcttccgggcgctatcatgccataccgcgaaaggttttgcgccattcgatggtgtccgggatctcgacgctctcccttatgcgactcctgcattaggaagcagcccagtagtaggttgaggccgttgagcaccgccgccgcaaggaatggtgcatgcaaggagatggcgcccaacagtcccccggccacggggcctgccaccatacccacgccgaaacaagcgctcatgagcccgaagtggcgagcccgatcttccccatcggtgatgtcggcgatataggcgccagcaaccgcacctgtggcgccggtgatgccggccacgatgcgtccggcgtagaggatcgagatctcgatcccgcgaaattaatacgactcactataggggaattgtgagcggataacaattcccctctagaaataattttgtttaactttaagaaggagatatacatatgaaatacctgctgccgaccgctgctgctggtctgctgctcctcgctgcccagccggcgatggccgaggttcaattagtggaatctggcgggggattggttcaagccggtgagtccttgcgtttgagctgcgccgcatctgggagcacatttgatttcaaagtgatgggctggtatcgtcagccgcccggaaaacagcgcgagggtgtagcagccatccgcttgagcggaaatatgcactacgccgagtctgtaaaagggcgctttgctatttccaaagcgaacgctaagaacacagtgtatcttcagatgaactccttgcgtcccgaagacactgccgtttattattgcaaagtaaacatccgtgggcaagactactggggtcaaggaacgcaggtcacagtctcttctggctctggcagacaccgccagccgagaggttgggaacagctgccgaccggagctgaatttctgggcgatggtggggatgttagtttttctacccgtggcacacagaattggaccgttgaacggttattacaagcacatcgtcagctggaagaaagaggttatgtgtttgttgggtatcatggtacatttttagaagcagcccagtctattgtttttggcggtgttcgtgcccgtagccaggatctggatgcaatttggagaggtttttatattgcgggtgatccggcgctggcatatggttacgcacaggatcaggaaccagatgcacgtggtcgtattcgtaatggtgccctgttacgggtgtatgttccccgttccagcctgccgggtttttatcgtacctctttaacactggcagccccggaagcagcaggtgaagtggaacgtctgattggccatccgctgccgctgcgcttagatgcaattaccggtccggaagaagaaggtgggcggttagaaaccattctgggttggccgctggcagaaagaacagtggttataccgagcgcgattcctaccgatcctcgtaatgtggggggtgatttagatccgagcagcattccggataaagagcaggcgattagcgcgctgccggattatgcaagccaaccggggaaaccgccgcgtgaagacttaaaacatcatcaccatcatcattaagatccggctgctaacaaagcccgaaaggaagctgagttggctgctgccaccgctgagcaataactagcataaccccttggggcctctaaacgggtcttgaggggttttttgctgaaaggaggaactatatccggat

SEQ ID NO: 53 - DNA, 5521 bp, synthetic construct
  source 1..5521: mol_type = other DNA
catggtcatagctgtttcctttaatgcccatggcgtttaccaatgcttaatcagtgaggcacctatctcagcgatctgtctatttcgttcatccatagttgcctgactccccgtcgtgtagataactacgatacgggagggcttaccatctggccccagtgctgcaatgataccgcgacttccacgctcaccggctccagatttatcagcaataaaccagccagccggaagggccgagcgcagaagtggtcctgcaactttatccgcctccatccagtctattaattgttgccgggaagctagagtaagtagttcgccagttaatagtttgcgcaacgttgttgccattgctacaggcatcgtggtgtcacgctcgtcgtttggtatggcttcattcagctccggttcccaacgatcaaggcgagttacatgatcccccatgttgtgcaaaaaagcggttagctccttcggtcctccgatcgttgtcagaagtaagttggccgcagtgttatcactcatggttatggcagcactgcataattctcttactgtcatgccatccgtaagatgcttttctgtgactggtgagtactcaaccaagtcattctgagaatagtgtatgcggcgaccgagttgctcttgcccggcgtcaatacgggataataccgcgccacatagcagaactttaaaagtgctcatcattggaaaacgttcttcggggcgaaaactctcaaggatcttaccgctgttgagatccagttcgatgtaacccactcgtgcacccaactgatcttcagcatcttttactttcaccagcgtttctgggtgagcaaaaacaggaaggcaaaatgccgcaaaaaagggaataagggcgacacggaaatgttgaatactcatactcttcctttttcaatattattgaagcatttatcagggttattgtctcatgagcggatacatatttgaatgtatttagaaaaataaacaaataggggttccgcgcacatttccccgaaaagtgccacctgacgtctaagaaaccattattatcatgacattaacctataaaaataggcgtatcacgaggcccttaggccaaataggccgttcagatccttccgtatttagccagtatgttctctagtgtggttcgttgtttttgcgtgagccatgagaacgaaccattgagatcatgcttactttgcatgtcactcaaaaattttgcctcaaaactggtgagctgaatttttgcagttaaagcatcgtgtagtgtttttcttagtccgttacgtaggtaggaatctgatgtaatggttgttggtattttgtcaccattcatttttatctggttgttctcaagttcggttacgagatccatttgtctatctagttcaacttggaaaatcaacgtatcagtcgggcggcctcgcttatcaaccaccaatttcatattgctgtaagtgtttaaatctttacttattggtttcaaaacccattggttaagccttttaaactcatggtagttattttcaagcattaacatgaacttaaattcatcaaggctaatctctatatttgccttgtgagttttcttttgtgttagttcttttaataaccactcataaatcctcatagagtatttgttttcaaaagacttaacatgttccagattatattttatgaatttttttaactggaaaagataaggcaatatctcttcactaaaaactaattctaatttttcgcttgagaacttggcatagtttgtccactggaaaatctcaaagcctttaaccaaaggattcctgatttccacagttctcgtcatcagctctctggttgctttagctaatacaccataagcattttccctactgatgttcatcatctgagcgtattggttataagtgaacgataccgtccgttctttccttgtagggttttcaatcgtggggttgagtagtgccacacagcataaaattagcttggtttcatgctccgttaagtcatagcgactaatcgctagttcatttgctttgaaaacaactaattcagacatacatctcaattggtctaggtgattttaatcactataccaattgagatgggctagtcaatgataattactagtccttttcctttgagttgtgggtatctgtaaattctgctagacctttgctggaaaacttgtaaattctgctagaccctctgtaaattccgctagacctttgtgtgttttttttgtttatattcaagtggttataatttatagaataaagaaagaataaaaaaagataaaaagaatagatcccagccctgtgtataactcactactttagtcagttccgcagtattacaaaaggatgtcgcaaacgctgtttgctcctctacaaaacagaccttaaaaccctaaaggcttaagtagcaccctcgcaagctcgggcaaatcgctgaatattccttttgtctccgaccatcaggcacctgagtcgctgtctttttcgtgacattcagttcgctgcgctcacggctctggcagtgaatgggggtaaatggcactacaggcgccttttatggattcatgcaaggaaactacccataatacaagaaaagcccgtcacgggcttctcagggcgttttatggcgggtctgctatgtggtgctatctgactttttgctgttcagcagttcctgccctctgattttccagtctgaccacttcggattatcccgtgacaggtcattcagactggctaatgcacccagtaaggcagcggtatcatcaacaggcttacccgtcttactgtcaagaggacatccggtcagataaccgtcatcttcggctactgtctagggcggcggatttgtcctactcaggagagcgttcaccgacaaacaacagataaaacgaaaggcccagtctttcgactgagcctttcgttttatttgatgcactagtgccgatcatattcaataacccttaatataacttcgtataatgtatgctatacgaagttattaggtctgaagaggagtttacgtcccatatgggcgagctcgatatcaaattacgccccgccctgccactcatcgcagtactgttgtaattcattaagcattctgccgacatggaagccatcacagacggcatgatgaacctgaatcgccagcggcatcagcaccttgtcgccttgcgtataatatttgcccatggtgaaaacgggggcgaagaagttgtccatattggccacgtttaaatcaaaactggtgaaactcacccagggattggctgagacgaaaaacatattctcaataaaccctttagggaaataggccaggttttcaccgtaacacgccacatcttgcgaatatatgtgtagaaactgccggaaatcgtcgtggtattcactccagagcgatgaaaacgtttcagtttgctcatggaaaacggtgtaacaagggtgaacactatcccatatcaccagctcaccgtctttcattgccatacgaaattccggatgagcattcatcaggcgggcaagaatgtgaataaaggccggataaaacttgtgcttatttttctttacggtctttaaaaaggccgtaatatccagctgaacggtctggttataggtacattgagcaactgactgaaatgcctcaaaatgttctttacgatgccattgggatatatcaacggtggtatatccagtgatttttttctccattttagcttccttagctcctgaaaatctcgataactcaaaaaatacgcccggtagtgatcttatttcattatggtgaaagttggaacctcttacgtgccgatcaacgtctcattttcgccagatatcgccaagcttaggatccggaacccttaatataacttcgtataatgtatgctatacgaagttattaggtccctcgaagaggttcactagctatctagagcttggactcctgttgatagatccagtaatgacctcagaactccatctggatttgttcagaacgctcggttgccgccgggcgttttttattggtgagaatccaagcccgggaaacgggatcctgatcttgatccgccgcaaagtttgagcgaagtcaataaactctctacccattcagggcaatatctctcttgcaggtgaatgcaacgtcaagcgatggcctacttgcggccgcaagattaaagaggagaaggatgggcctgaaaatgaaaaaacgtagcgggaaaaaagcgtggatgctgctggttatgtcgctgctgattgcggcggttccgattacggcgagcgccgaggtgcagctggtggagtctgggggaggattggtgcagcctgggggctctgtgagactctcctgtgtagcctctggacgcatcttcagtagcaatgccatgggctggttccgccaggctccagggaaggagcgtgagtttgtagcggccattacctggaggagtggcggtagcgcgtactatgcagactccgcgaagggccgattcaccatctccagagacaacgccaagaacacggtgtatttgcaaatgaacagcctgaaacctgaggacacggccgtttattattgtgcagctggtggtagttcctggttaagttttccgccggactactggggccaggggacccaggtcaccgtctcctcaagacaccgccagccgagaggttgggaacagctgccgaccggagctgaatttctgggcgatggtggggatgttagtttttctacccgtggcacacagaattggaccgttgaacggttattacaagcacatcgtcagctggaagaaagaggttatgtgtttgttgggtatcatggtacatttttagaagcagcccagtctattgtttttggcggtgttcgtgcccgtagccaggatctggatgcaatttggagaggtttttatattgcgggtgatccggcgctggcatatggttacgcacaggatcaggaaccagatgcacgtggtcgtattcgtaatggtgccctgttacgggtgtatgttccccgttccagcctgccgggtttttatcgtacctctttaacactggcagccccggaagcagcaggtgaagtggaacgtctgattggccatccgctgccgctgcgcttagatgcaattaccggtccggaagaagaaggtgggcggttagaaaccattctgggttggccgctggcagaaagaacagtggttataccgagcgcgattcctaccgatcctcgtaatgtggggggtgatttagatccgagcagcattccggataaagagcaggcgattagcgcgctgccggattatgcaagccaaccggggaaaccgccgcgtgaagacttaaaacatcatcaccatcatcattaagatccggctctggaagatccgcgcgtaccgagttctaattcactggccgtcgttttacaacatacgatgaaggcgataagtcgcgtaagttgctagcccacgcggctcaccttcacgggtgggcctttcttcgcgatccacatg

SEQ ID NO: 54 - skipped

SEQ ID NO: 55 - DNA, 34 bp, synthetic construct
  source 1..34: mol_type = other DNA
gattacggcgagcgccgaggtgcagctggtggag

SEQ ID NO: 56 - DNA, 39 bp, synthetic construct
  source 1..39: mol_type = other DNA
gccaggctaccaccttcaggtgaggagacggtgacctgg

SEQ ID NO: 57 - DNA, 1128 bp, synthetic construct
  source 1..1128: mol_type = other DNA
atgtcgtgcccggttattgagctgacacagcaacttattcgtcgcccctccctgagtccggatgacgcaggctgtcaggcattaatgattgaacgcctgcgtaaaatcggttttaccattgagcatatggattttggcgacacgcaaaatttttgggcatggcgtgggcgtggcgaaacgctggcgttcgccgggcatactgacgtcgtaccggctggcgatgtcgatcgctggatcaatccgccgtttgagcctacgattcgcgacggaatgttgttcggtcgcggcgcggcggatatgaaaggttcactggcggccatggtggtggctgctgaacgttttgttgcgcagcatcctcatcaccggggccgcctcgcatttttgattacctctgatgaggaagccagcgcaaaaaatggcaccgtaaaggtggttgaagcgctgatggcccgtaacgagcggctggattactgtctggtcggcgaaccttccagtactgaaattgtgggcgatgtcgtcaaaaacgggcgtcgcggttctctcacctgtaacctcactatccatggcgttcaggggcacgtcgcctatccgcatctggcggataaccctgttcatcgcgccgcgccttttcttaatgaactggtcgctatcgagtgggatcggggcaatgactttttcccggccaccagtatgcaggtagccaatatccaggcaggcaccggcagcaataatgtcattcccggcgaactgttcgtgcagtttaacttccgtttcagcacggaactgaccgatgagatgatcaaagagcgggtacatgcgctgcttgaaaagcatcagctacgctataccgtagactggtggctttccgggcagccgttcctgaccgcacgcggcaagctggtggacgcggtggtaaacgccattgagcactataatgaaattaaaccgcaattactgacgacgggcggtacgtccgacggacgttttatcgcccgtatgggagcgcaggtggtagaactggggccggtgaacgccaccattcataaaattaatgaatgtgtgaatgccgccgatctccagctactggcccgtatgtatcaacgcattatggaacagctcgtcgcctga

SEQ ID NO: 58 - DNA, 1428 bp, synthetic construct
  source 1..1428: mol_type = other DNA
atgaaaaaaaccacattagcaatgagtgcactggctctgagtttaggtttggcattgtcgcctctgtctgccacggcggctgaaacgtcctcttcagcaatgactgcccagcagatgccaagcctggcaccgatgctcgaaaaagtgatgccatcggtggtcagtattaatgttgaaggtagcaccacggtgaatacgccgcgtatgccgcgtaatttccagcagttctttggcgatgactccccgttctgccaggacggttctccgttccagaattctccgttctgccagggcggcggtaacggcggcaacggcggtcaacaacagaaattcatggcgctgggctccggcgtaattattgacgccgcgaagggctacgtcgtcaccaacaaccacgtggttgataacgccagcgtgattaaagtacagcttagcgatgggcgtaaattcgatgctaaagtggtgggcaaagatccgcgttctgatatcgcgctgattcaaattcagaatccgaagaacctgacggcgattaagctggcggactccgacgcgctgcgcgtgggggattataccgtcgctattggtaacccgtttggtctgggcgaaacggtgacgtcaggtatcgtttcggcgctggggcgtagcggcctgaacgtagaaaattacgagaactttattcagaccgacgccgcgattaaccgtggtaactccggcggcgcgctggtgaacctgaacggtgagctgatcggtattaacaccgcgattctggcgccggacggcggcaacatcggtatcggcttcgctatccccagtaacatggtgaaaaacctgacgtcgcagatggtggaatacggccaggtgaaacgcggcgaactggggatcatggggactgagctgaattccgaattggcgaaagcgatgaaagtcgacgcccagcgaggcgcgttcgtcagccaggtgatgccgaattcgtccgcggcgaaagcgggtatcaaagccggggatgtcattacctcgctgaacggtaaaccgatcagcagctttgcggcgctgcgcgctcaggtcggcactatgccggtcggcagcaaaatcagcctcggtctgctgcgtgaaggtaaagcgattacggtgaatctggaactgcagcagagcagccagagtcaggttgattccagcaccatcttcagcgggattgaaggcgctgaaatgagcaataaaggccaggataaaggcgttgtggtgagcagcgtgaaagcgaactcacccgccgcgcaaattggcctcaaaaaaggcgatgtgattatcggcgctaaccagcagccggtgaaaaatatcgccgagctgcgtaagattctcgacagcaagccgtcggttctggcgctgaatattcagcgtggtgatagttctatttatttgctgatgcagtaa

SEQ ID NO: 59 - DNA, 1590 bp, synthetic construct
  source 1..1590: mol_type = other DNA
atgaaaaaaataatgctagtttttattacacttatattagttagtctaccaattgcgcaacaaactgaagcaaaggatgcatctgcattcaataaagaaaattcaatttcatccatggcaccaccagcatctccgcctgcaagtcctaagacgccaatcgaaaagaaacacgcggatgaaatcgataagtatatacaaggattggactacaataaaaacaatgtattagtataccacggagatgcagtgacaaatgtgccgccaagaaaaggttacaaagatggaaatgaatatattgttgtggagaaaaagaagaaatccatcaatcaaaataatgcagacattcaagttgtgaatgcaatttcgagcctaacctatccaggtgctctcgtaaaagcgaattcggaattagtagaaaatcaaccagatgttctccctgtaaaacgtgattcattaacactcagcattgatttgccaggtatgactaatcaagacaataaaatcgttgtaaaaaatgccactaaatcaaacgttaacaacgcagtaaatacattagtggaaagatggaatgaaaaatatgctcaagcttatccaaatgtaagtgcaaaaattgattatgatgacgaaatggcttacagtgaatcacaattaattgcgaaatttggtacagcatttaaagctgtaaataatagcttgaatgtaaacttcggcgcaatcagtgaagggaaaatgcaagaagaagtcattagttttaaacaaatttactataacgtgaatgttaatgaacctacaagaccttccagatttttcggcaaagctgttactaaagagcagttgcaagcgcttggagtgaatgcagaaaatcctcctgcatatatctcaagtgtggcgtatggccgtcaagtttatttgaaattatcaactaattcccatagtactaaagtaaaagctgcttttgatgctgccgtaagcggaaaatctgtctcaggtgatgtagaactaacaaatatcatcaaaaattcttccttcaaagccgtaatttacggaggttccgcaaaagatgaagttcaaatcatcgacggcaacctcggagacttacgagatattttgaaaaaaggcgctacttttaatcgagaaacaccaggagttcccattgcttatacaacaaacttcctaaaagacaatgaattagctgttattaaaaacaactcagaatatattgaaacaacttcaaaagcttatacagatggaaaaattaacatcgatcactctggaggatacgttgctcaattcaacatttcttgggatgaagtaaattatgatcctgaaggtaacgaaattgttcaacataaaaactggagcgaaaacaataaaagtaagctagctcatttcacatcgtccatctatttgccaggtaacgcgagaaatattaatgtttacgctaaagaatgcactggtttagcttgggaatggtggagaacggtaattgatgaccggaacttaccacttgtgaaaaatagaaatatctccatctggggcaccacgctttatccgaaatatagtaataaagtagataatccaatcgaataa

SEQ ID NO: 60 - DNA, 54 bp, synthetic construct
  source 1..54: mol_type = other DNA
tacccctatgacgtgcctgattacgccggctctggccaccaccaccaccaccac

SEQ ID NO: 61 - protein, 121 aa, synthetic construct
GGGSVQAGGSLKLSCEASLPSTTTPYSMAWFRQAPGREREAVATISARGGTKLYSDSVRERFTISRDNRKNTVYLKMDHLNTDDTAIYYCAATGSILFNSRPFAESTYPFWGQGTLVTVSS

SEQ ID NO: 62 - protein, 118 aa, synthetic construct
GGGTVQAGGSLKLSCAARGWRFSGYCVAWFRQAPGKEREAVAIIPGAGVMYTDDSVKGRFTYSRDNVKNTVSLQMNSLEPEDTATYYCAVDWAYSHSCPKNTEDYRYWGQGTQVTVSS

SEQ ID NO: 63 - protein, 169 aa, synthetic construct
MKYLLPTAAAGLLLLAAQPAMAQVQLQESGGGLVQPGGSLRLSCAASGRTFSSYAMGWFRQAPGKEREFVAAIRWSGGYTYYTDSVKGRFTISRDNAKTTVYLQMNSLKPEDTAVYYCAATYLSSDYSRYALPQRPLDYDYWGQGTQVTVSSAAAEQKLISEEDLNGLE

SEQ ID NO: 64 - protein, 122 aa, synthetic construct
EVQLVESGGGLVQTGGSLRLSCAASGFTFSSYAMSWVRQAPGKGLEWVSGIKSSGDSTRYAGSVKGRFTISRDNAKNMLYLQMYSLKPEDTAVYYCAKSRVSRTGLYTYDNRGQGTQVTVSS

SEQ ID NO: 65 - protein, 127 aa, synthetic construct
EVQLMESGGGLVQAGGSLRLSCAASGRTFNNYAMGWFRRAPGKEREFVAAITRSGVRSGVSAIYGDSVKDRFTISRDNAKNTLYLQMNSLKPEDTAVYTCAASAIGSGALRRFEYDYSGQGTQVTVS

SEQ ID NO: 66 - protein, 123 aa, synthetic construct
EVQLVESGGGLVQAGDSLRLSCLASGRSFKDDAMGWFRQAPGKEREFVSGIDWRGNIVDAESVKGRFTISRENAKNTLYLQMNHLKPEDTAVYYCAASSVFSDLRYRKNPKYWGQGTQVTVSS

SEQ ID NO: 67 - protein, 126 aa, synthetic construct
EVQLVESGGGLVQAGGSLRRLSCAASGSIFRINAMGWYRQAPGKQRELVAAAISGGSTNYADFVKGRFTISRDNAKNTVYLQMNSLKPEDTAVYYCNALVVSHNYSDYVPFPDDYWGQGTQVTVSS

SEQ ID NO: 68 - protein, 128 aa, synthetic construct
EVQLVESGGGLVQPGGSLRLSCAASGFTLDYYAIGWFRQAPGKEREGVSCISSTDGSTYYADSVKGRFTISRDNAKNTVYLQMNSLNPEDTGVYTCAAVLTTAQAMGVPTRSYEYDYWGQGTQVTVSS

SEQ ID NO: 69 - protein, 126 aa, synthetic construct
EVQLVESGGGLVEAGGSLRLSCAAAGRTLSSYSMAWFRQAPGKEREFVAIIRGNPSRTYHSDSVKGRFTASRDNAKNTVYLQMNRLEPEDTAVYYCAADPPPFASDYSAPQSYDYWGQGTQVTVSS

SEQ ID NO: 70 - protein, 116 aa, synthetic construct
EVQLVESGGGLVQAGGSLNLSCNASGDIGSINAMGWHRQAPGQQREWVAVITDTDSTIYPDSVKGRFAISRDGAKNTVHLRMSSLKPEDTAVYYCNAYQAGWGDYWGQGTQVTVSS

SEQ ID NO: 71 - protein, 124 aa, synthetic construct
QVQLQESGGGVVQPGGSLTLSCTRTGFTASTNAYGWYRQGPGKKCEWVSYMTIPSGRTTYADAVKGRFAMSRDKAKSTVLLQMNSLKPEDTAVYYCGDVPFSTLPAMCTNDGPWGQGTQVTVSS

SEQ ID NO: 72 - protein, 124 aa, synthetic construct
QVQLQESGGGVVQPGGSLTLSCTRTGFTASTNAYGWYRQGPGKKCEWVSYMTIPSGRTTYADAVKGRFAMSRDKAKSTVFLQMNSLKPEDTAVYYCGDVPFSTLPAMCTNDGPWGQGTQVTVSS

SEQ ID NO: 73 - protein, 119 aa, synthetic construct
QVQLQESGGGLVQAGGPLRLSCAASWRTFSSYAMGWFRQAPGKEREFVAAISWSGGSTYYADSVKGRFTISRDNAKNTVYLQMNSLKPEDTAVYYCAVLHEDLYEYDYWGQGTQVTVSS

SEQ ID NO: 74 - protein, 124 aa, synthetic construct
QVQLQESGGGVVQPGGSLTLSCTRTGLTPSTGAYGWYRQAPGKKCELVSYITIPSGRTTYTDSVKGRFAISRDKAKNTVFLQMNSLKPEDTALYYCGDVPYSTIQAMCTDDGPWGQGTQVTVSS

SEQ ID NO: 75 - protein, 124 aa, synthetic construct
QVQLQESGGGVVQPGGSLTLSCTRTGLTASTNAYGWYRQAPGKKCELVSYITIPSGRTTYADSVKGRFAISRDKAKNTVFLQMNSLKPEDTALYYCGDVPYSTIQAMCTDDGPWGQGTQVTVSS

SEQ ID NO: 76 - protein, 114 aa, synthetic construct
QVQLQESGGGLVQSGGSLRLSCRASGFTFSHYPMSWYRQAPGKKRELVAGIYTDGSTNYADSVKGRFTISRDNAKNTVYLQMSSLKPEDTAVYYCRRSMVSVYWGQGTQVTVSS

SEQ ID NO: 77 - protein, 120 aa, synthetic construct
QVQLQESGGGLVQPGGSLRLSCAASGRTFSYYTMAWFRQAPGKEREFVASISWSGGITYYADSVKGRFTISRDNAKNTVYLQMNSLKPEDTAVYYCAARKEPGSAYFGSWGQGTQVTVSS

SEQ ID NO: 78 - protein, 124 aa, synthetic construct
QVQLQESGGGVVQPGGSLTLSCTRTGFTASTNAYGWYRQAPGKKCELVSYITIPSGRTTYADAVKGRFAISRDKAKNTVFLQMNSLKPEDTAVYYCGDVPFSTLPAMCTNDGPWGQGTQVTVSS

SEQ ID NO: 79 - protein, 666 aa, synthetic construct
LYLTFYLEKVMKKMLLIAGATVISSMAHPTFAVEDELNIFDECRSPCSLTPELGKPIQSKLSIPSDVVLDEGVLYYSMTINDEQNDIKDEDKGESIITIGEFATVRATRHYVNQDAPFGVINLDITTENGTKTYSYNRKEGEFAINWLVPIGEDSPASIKISVDELDQQRNIIEVPKLYSIDLDNQTLEQWKTQGNVSFSVTRPEHNIAISWPSVSYKAAQKEGSRHKRWAHWHTGLALCWLVPIDAIYNYITQQNCTLGDNWFGGSYETVAGTPKAITVKQGIEQKPVEQRIHFSKKNAMEALAAHRVCGVPLETLARSRKPRDLPDDLSCAYQAQNIVSLFVATRILFSHLDSVFTLNLDEQEPEVAERLSALRQINENNPGMVTQVLTVARQIYNDYVTHHPGLTPEQTSAGAQAADILSLFCPDADKPCVASNNDQANINIESRSGRSYLPENRAVITPQGVTNWTYQELEATHQALTREGYVFVGYHGTNHVAAQTIVNRIAPVPRGNNTENEEKWGGLYVATHAEVAHGYARIKEGTGEYGLPTRAERDARGVMLRVYIPRASLERFYRTNTPLENAEEHITQVIGHSLPLRNEAFTGPESAGGEDETVIGWDMAIHAVAIPSTIPGNAYEELAIDEEAVAKEQSISTKPPYKERKDELK

SEQ ID NO: 80 - protein, 365 aa, synthetic construct
EALAAHRVCGVPLETLARSRKPRDLPDDLSCAYQAQNIVSLFVATRILFSHLDSVFTLNLDEQEPEVAERLSALRQINENNPGMVTQVLTVARQIYNDYVTHHPGLTPEQTSAGAQAADILSLFCPDADKPCVASNNDQANINIESRSGRSYLPENRAVITPQGVTNWTYQELEATHQALTREGYVFVGYHGTNHVAAQTIVNRIAPVPRGNNTENEEKWGGLYVATHAEVAHGYARIKEGTGEYGLPTRAERDARGVMLRVYIPRASLERFYRTNTPLENAEEHITQVIGHSLPLRNEAFTGPESAGGEDETVIGWDMAIHAVAIPSTIPGNAYEELAIDEEAVAKEQSISTKPPYKERKDELK

SEQ ID NO: 81 - protein, 382 aa, synthetic construct
MVKIIFVFFIFLSSFSYANDDKLYRADSRPPDEIKQSGGLMPRGQSEYFDRGTQMNINLYDHARGTQTGFVRHDDGYVSTSISLRSAHLVGQTILSGHSTYYIYVIATAPNMFNVNDVLGAYSPHPDEQEVSALGGIPYSQIYGWYRVHFGVLDEQLHRNRGYRDRYYSNLDIAPAADGYGLAGFPPEHRAWREEPWIHHAPPGCGNAPRSSMSNTCDEKTQSLGVKFLDEYQSKVKRQIFSGYQSDIDTHNRIKDELMIKLKFGVFFTVLLSSAYAHGTPQNITDLCAESHNTQIYTLNDKIFSYTESLAGKREMAIITFKNGAIFQVEVPSSQHIDSQKKAIERMKDTLRIAYLTEAKVEKLCVWNNKTPHAIAAISMAN

SEQ ID NO: 82 - protein, 258 aa, synthetic construct
MKNITFIFFILLASPLYANGDRLYRADSRPPDEIKRSGGLMPRGHNEYFDRGTQMNINLYDHARGTQTGFVRYDDGYVSTSLSLRSAHLAGQSILSGYSTYYIYVIATAPNMFNVNDVLGVYSPHPYEQEVSALGGIPYSQIYGWYRVNFGVIDERLHRNREYRDRYYRNLNIAPAEDGYRLAGFPPDHQAWREEPWIHHAPQGCGNSSRTITGDTCNEETQNLSTIYLREYQSKVKRQIFSDYQSEVDIYNRIRDEL

SEQ ID NO: 83 - protein, 103 aa, synthetic construct
APQTITELCSEYRNTQIYTINDKILSYTESMAGKREMVIITFKSGETFQVEVPGSQHIDSQKKAIERMKDTLRITYLTETKIDKLCVWNNKTPNSIAAISMKN

SEQ ID NO: 84 - protein, 535 aa, synthetic construct
GADDVVDSSKSFVMENFSSYHGTKPGYVDSIQKGIQKPKSGTQGNYDDDWKGFYSTDNKYDAAGYSVDNENPLSGKAGGVVKVTYPGLTKVLALKVDNAETIKKELGLSLTEPLMEQVGTEEFIKRFGDGASRVVLSLPFAEGSSSVEYINNWEQAKALSVELEINFETRGKRGQDAMYEYMAQACAGNRVRRSVGSSLSCINLDWDVIRDKTKTKIESLKEHGPIKNKMSESPNKTVSEEKAKQYLEEFHQTALEHPELSELKTVTGTNPVFAGANYAAWAVNVAQVIDSETADNLEKTTAALSILPGIGSVMGIADGAVHHNTEEIVAQSIALSSLMVAQAIPLVGELVDIGFAAYNFVESIINLFQVVHNSYNRPAYSPGHKTQPFLHDGYAVSWNTVEDSIIRTGFQGESGHDIKITAENTPLPIAGVLLPTIPGKLDVNKSKTHISVNGRKIRMRCRAIDGDVTFCRPKSPVYVGNGVHANLHVAFHRSSSEKIHSNEISSDSIGVLGYQKTVDHTKVNSKLSLFFEIKS

SEQ ID NO: 85 - protein, 390 aa, synthetic construct
GADDVVDSSKSFVMENFSSYHGTKPGYVDSIQKGIQKPKSGTQGNYDDDWKGFYSTDNKYDAAGYSVDNENPLSGKAGGVVKVTYPGLTKVLALKVDNAETIKKELGLSLTEPLMEQVGTEEFIKRFGDGASRVVLSLPFAEGSSSVEYINNWEQAKALSVELEINFETRGKRGQDAMYEYMAQACAGNRVRRSVGSSLSCINLDWDVIRDKTKTKIESLKEHGPIKNKMSESPNKTVSEEKAKQYLEEFHQTALEHPELSELKTVTGTNPVFAGANYAAWAVNVAQVIDSETADNLEKTTAALSILPGIGSVMGIADGAVHHNTEEIVAQSIALSSLMVAQAIPLVGELVDIGFAAYNFVESIINLFQVVHNSYNRPAYSPGHKTQPFL

SEQ ID NO: 86 - protein, 287 aa, synthetic construct
KEFTLDFSTAKTYVDSLNVIRSAIGTPLQTISSGGTSLLMIDSGTGDNLFAVDVRGIDPEEGRFNNLRLIVERNNLYVTGFVNRTNNVFYRFADFSHVTFPGTTAVTLSGDSSYTTLQRVAGISRTGMQINRHSLTTSYLDLMSHSGTSLTQSVARAMLRFVTVTAEALRFRQIQRGFRTTLDDLSGRSYVMTAEDVDLTLNWGRLSSVLPDYHGQDSVRVGRISFGSINAILGSVALILNCHHHASRVARMASDEFPSMCPADGRVRGITHNKILWDSSTLGAILM

SEQ ID NO: 87 - protein, 69 aa, synthetic construct
TPDCVTGKVEYTKYNDDDTFTVKVGDKELFTNRWNLQSLLLSAQITGMTVTIKTNACHNGGGFSEVIFR

SEQ ID NO: 88 - protein, 800 aa, synthetic construct
MTRNKFIPNKFSIISFSVLLFAISSSQAIEVNAMNEHYTESDIKRNHKTEKNKTEKEKFKDSINNLVKTEFTNETLDKIQQTQDLLKKIPKDVLEIYSELGGEIYFTDIDLVEHKELQDLSEEEKNSMNSRGEKVPFASRFVFEKKRETPKLIINIKDYAINSEQSKEVYYEIGKGISLDIISKDKSLDPEFLNLIKSLSDDSDSSDLLFSQKFKEKLELNNKSIDINFIKENLTEFQHAFSLAFSYYFAPDHRTVLELYAPDMFEYMNKLEKGGFEKISESLKKEGVEKDRIDVLKGEKALKASGLVPEHADAFKKIARELNTYILFRPVNKLATNLIKSGVATKGLNVHGKSSDWGPVAGYIPFDQDLSKKHGQQLAVEKGNLENKKSITEHEGEIGKIPLKLDHLRIEELKENGIILKGKKEIDNGKKYYLLESNNQVYEFRISDENNEVQYKTKEGKITVLGEKFNWRNIEVMAKNVEGVLKPLTADYDLFALAPSLTEIKKQIPQKEWDKVVNTPNSLEKQKGVTNLLIKYGIERKPDSTKGTLSNWQKQMLDRLNEAVKYTGYTGGDVVNHGTEQDNEEFPEKDNEIFIINPEGEFILTKNWEMTGRFIEKNITGKDYLYYFNRSYNKIAPGNKAYIEWTDPITKAKINTIPTSAEFIKNLSSIRRSSNVGVYKDSGDKDEFAKKESVKKIAGYLSDYYNSANHIFSQEKKRKISIFRGIQAYNEIENVLKSKQIAPEYKNYFQYLKERITNQVQLLLTHQKSNIEFKLLYKQLNFTENETDNFEVFQKIIDEK

SEQ ID NO: 89 - protein, 809 aa, synthetic construct
MNIKKEFIKVISMSCLVTAITLSGPVFIPLVQGAGGHGDVGMHVKEKEKNKDENKRKDEERNKTQEEHLKEIMKHIVKIEVKGEEAVKKEAAEKLLEKVPSDVLEMYKAIGGKIYIVDGDITKHISLEALSEDKKKIKDIYGKDALLHEHYVYAKEGYEPVLVIQSSEDYVENTEKALNVYYEIGKILSRDILSKINQPYQKFLDVLNTIKNASDSDGQDLLFTNQLKEHPTDFSVEFLEQNSNEVQEVFAKAFAYYIEPQHRDVLQLYAPEAFNYMDKFNEQEINLSLEELKDQRMLARYEKWEKIKQHYQHWSDSLSEEGRGLLKKLQIPIEPKKDDIIHSLSQEEKELLKRIQIDSSDFLSTEEKEFLKKLQIDIRDSLSEEEKELLNRIQVDSSNPLSEKEKEFLKKLKLDIQPYDINQRLQDTGGLIDSPSINLDVRKQYKRDIQNIDALLHQSIGSTLYNKIYLYENMNINNLTATLGADLVDSTDNTKINRGIFNEFKKNFKYSISSNYMIVDINERPALDNERLKWRIQLSPDTRAGYLENGKLILQRNIGLEIKDVQIIKQSEKEYIRIDAKVVPKSKIDTKIQEAQLNINQEWNKALGLPKYTKLITFNVHNRYASNIVESAYLILNEWKNNIQSDLIKKVTNYLVDGNGRFVFTDITLPNIAEQYTHQDEIYEQVHSKGLYVPESRSILLHGPSKGVELRNDSEGFIHEFGHAVDDYAGYLLDKNQSDLVTNSKKFIDIFKEEGSNLTSYGRTNEAEFFAEAFRLMHSTDHAERLKVQKNAPKTFQFINDQIKFIINS

SEQ ID NO: 90 - protein, 764 aa, synthetic construct
MKKRKVLIPLMALSTILVSSTGNLEVIQAEVKQENRLLNESESSSQGLLGYYFSDLNFQAPMVVTSSTTGDLSIPSSELENIPSENQYFQSAIWSGFIKVKKSDEYTFATSADNHVTMWVDDQEVINKASNSNKIRLEKGRLYQIKIQYQRENPTEKGLDFKLYWTDSQNKKEVISSDNLQLPELKQKSSNSRKKRSTSAGPTVPDRDNDGIPDSLEVEGYTVDVKNKRTFLSPWISNIHEKKGLTKYKSSPEKWSTASDPYSDFEKVTGRIDKNVSPEARHPLVAAYPIVHVDMENIILSKNEDQSTQNTDSQTRTISKNTSTSRTHTSEVHGNAEVHASFFDIGGSVSAGFSNSNSSTVAIDHSLSLAGERTWAETMGLNTADTARLNANIRYVNTGTAPIYNVLPTTSLVLGKNQTLATIKAKENQLSQILAPNNYYPSKNLAPIALNAQDDFSSTPITMNYNQFLELEKTKQLRLDTDQVYGNIATYNFENGRVRVDTGSNWSEVLPQIQETTARIIFNGKDLNLVERRIAAVNPSDPLETTKPDMTLKEALKIAFGFNEPNGNLQYQGKDITEFDFNFDQQTSQNIKNQLAELNATNIYTVLDKIKLNAKMNILIRDKRFHYDRNNIAVGADESVVKEAHREVINSSTEGLLLNIDKDIRKILSGYIVEIEDTEGLKEVINDRYDMLNISSLRQDGKTFIDFKKYNDKLPLYISNPNYKVNVYAVTKENTIINPSENGDTSTNGIKKILIFSKKGYEIG

SEQ ID NO: 91 - protein, 271 aa, synthetic construct
SNAMIFPKQYPIINFTTAGATVQSYTNFIRAVRGRLTTGADVRHEIPVLPNRVGLPINQRFILVELSNHAELSVTLALDVTNAYVVGYRAGNSAYFFHPDNQEDAEAITHLFTDVQNRYTFAFGGNYDRLEQLAGNLRENIELGNGPLEEAISALYYYSTGGTQLPTLARSFIICIQMISEAARFQYIEGEMRTRIRYNRRSAPDPSVITLENSWGRLSTAIQESNQGAFASPIQLQRRNGSKFSVYDVSILIPIIALMVYRCAPPPSSQF

SEQ ID NO: 92 - DNA, 5464 bp, synthetic construct
  source 1..5464: mol_type = other DNA
tggcgaatgggacgcgccctgtagcggcgcattaagcgcggcgggtgtggtggttacgcgcagcgtgaccgctacacttgccagcgccctagcgcccgctcctttcgctttcttcccttcctttctcgccacgttcgccggctttccccgtcaagctctaaatcgggggctccctttagggttccgatttagtgctttacggcacctcgaccccaaaaaacttgattagggtgatggttcacgtagtgggccatcgccctgatagacggtttttcgccctttgacgttggagtccacgttctttaatagtggactcttgttccaaactggaacaacactcaaccctatctcggtctattcttttgatttataagggattttgccgatttcggcctattggttaaaaaatgagctgatttaacaaaaatttaacgcgaattttaacaaaatattaacgcttacaatttaggtggcacttttcggggaaatgtgcgcggaacccctatttgtttatttttctaaatacattcaaatatgtatccgctcatgaattaattcttagaaaaactcatcgagcatcaaatgaaactgcaatttattcatatcaggattatcaataccatatttttgaaaaagccgtttctgtaatgaaggagaaaactcaccgaggcagttccataggatggcaagatcctggtatcggtctgcgattccgactcgtccaacatcaatacaacctattaatttcccctcgtcaaaaataaggttatcaagtgagaaatcaccatgagtgacgactgaatccggtgagaatggcaaaagtttatgcatttctttccagacttgttcaacaggccagccattacgctcgtcatcaaaatcactcgcatcaaccaaaccgttattcattcgtgattgcgcctgagcgagacgaaatacgcgatcgctgttaaaaggacaattacaaacaggaatcgaatgcaaccggcgcaggaacactgccagcgcatcaacaatattttcacctgaatcaggatattcttctaatacctggaatgctgttttcccggggatcgcagtggtgagtaaccatgcatcatcaggagtacggataaaatgcttgatggtcggaagaggcataaattccgtcagccagtttagtctgaccatctcatctgtaacatcattggcaacgctacctttgccatgtttcagaaacaactctggcgcatcgggcttcccatacaatcgatagattgtcgcacctgattgcccgacattatcgcgagcccatttatacccatataaatcagcatccatgttggaatttaatcgcggcctagagcaagacgtttcccgttgaatatggctcataacaccccttgtattactgtttatgtaagcagacagttttattgttcatgaccaaaatcccttaacgtgagttttcgttccactgagcgtcagaccccgtagaaaagatcaaaggatcttcttgagatcctttttttctgcgcgtaatctgctgcttgcaaacaaaaaaaccaccgctaccagcggtggtttgtttgccggatcaagagctaccaactctttttccgaaggtaactggcttcagcagagcgcagataccaaatactgtccttctagtgtagccgtagttaggccaccacttcaagaactctgtagcaccgcctacatacctcgctctgctaatcctgttaccagtggctgctgccagtggcgataagtcgtgtcttaccgggttggactcaagacgatagttaccggataaggcgcagcggtcgggctgaacggggggttcgtgcacacagcccagcttggagcgaacgacctacaccgaactgagatacctacagcgtgagctatgagaaagcgccacgcttcccgaagggagaaaggcggacaggtatccggtaagcggcagggtcggaacaggagagcgcacgagggagcttccagggggaaacgcctggtatctttatagtcctgtcgggtttcgccacctctgacttgagcgtcgatttttgtgatgctcgtcaggggggcggagcctatggaaaaacgccagcaacgcggcctttttacggttcctggccttttgctggccttttgctcacatgttctttcctgcgttatcccctgattctgtggataaccgtattaccgcctttgagtgagctgataccgctcgccgcagccgaacgaccgagcgcagcgagtcagtgagcgaggaagcggaagagcgcctgatgcggtattttctccttacgcatctgtgcggtatttcacaccgcaatggtgcactctcagtacaatctgctctgatgccgcatagttaagccagtatacactccgctatcgctacgtgactgggtcatggctgcgccccgacacccgccaacacccgctgacgcgccctgacgggcttgtctgctcccggcatccgcttacagacaagctgtgaccgtctccgggagctgcatgtgtgatgcctccgtgtaagggggatttctgttcatgggggtaatgataccgatgaaacgagagaggatgctcacgatacgggttactgatgatgaacatgcccggttactggaacgttgtgagggtaaacaactggcggtatggatgcggcgggaccagagaaaaatcactcagggtcaatgccagcgcttcgttaatacagatgtaggtgttccacagggtagccagcagcatcctgcgatgcagatccggaacataatggtgcagggcgctgacttccgcgtttccagactttacgaaacacggaaaccgaagaccattcatgttgttgctcaggtcgcagacgttttgcagcagcagtcgcttcacgttcgctcgcgtatcggtgattcattctgctaaccagtaaggcaaccccgccagcctagccgggtcctcaacgacaggagcacgatcatgcgcacccgtggggccgccatgccggcgataatggcctgcttctcgccgaaacgtttggtggcgggaccagtgacgaaggcttgagcgagggcgtgcaagattccgaataccgcaagcgacaggccgatcatcgtcgcgctccagcgaaagcggtcctcgccgaaaatgacccagagcgctgccggcacctgtcctacgagttgcatgataaagaagacagtcataagtgcggcgacgatagtcatgccccgcgcccaccggaaggagctgactgggttgaaggctctcaagggcatcggtcgagatcccggtgcctaatgagtgagctaacttacattaattgcgttgcgctcactgcccgctttccagtcgggaaacctgtcgtgccagctgcattaatgaatcggccaacgcgcggggagaggcggtttgcgtattgggcgccagggtggtttttcttttcaccagtgagacgggcaacagctgattgcccttcaccgcctggccctgagagagttgcagcaagcggtccacgctggtttgccccagcaggcgaaaatcctgtttgatggtggttaacggcgggatataacatgagctgtcttcggtatcgtcgtatcccactaccgagatatccgcaccaacgcgcagcccggactcggtaatggcgcgcattgcgcccagcgccatctgatcgttggcaaccagcatcgcagtgggaacgatgccctcattcagcatttgcatggtttgttgaaaaccggacatggcactccagtcgccttcccgttccgctatcggctgaatttgattgcgagtgagatatttatgccagccagccagacgcagacgcgccgagacagaacttaatgggcccgctaacagcgcgatttgctggtgacccaatgcgaccagatgctccacgcccagtcgcgtaccgtcttcatgggagaaaataatactgttgatgggtgtctggtcagagacatcaagaaataacgccggaacattagtgcaggcagcttccacagcaatggcatcctggtcatccagcggatagttaatgatcagcccactgacgcgttgcgcgagaagattgtgcaccgccgctttacaggcttcgacgccgcttcgttctaccatcgacaccaccacgctggcacccagttgatcggcgcgagatttaatcgccgcgacaatttgcgacggcgcgtgcagggccagactggaggtggcaacgccaatcagcaacgactgtttgcccgccagttgttgtgccacgcggttgggaatgtaattcagctccgccatcgccgcttccactttttcccgcgttttcgcagaaacgtggctggcctggttcaccacgcgggaaacggtctgataagagacaccggcatactctgcgacatcgtataacgttactggtttcacattcaccaccctgaattgactctcttccgggcgctatcatgccataccgcgaaaggttttgcgccattcgatggtgtccgggatctcgacgctctcccttatgcgactcctgcattaggaagcagcccagtagtaggttgaggccgttgagcaccgccgccgcaaggaatggtgcatgcaaggagatggcgcccaacagtcccccggccacggggcctgccaccatacccacgccgaaacaagcgctcatgagcccgaagtggcgagcccgatcttccccatcggtgatgtcggcgatataggcgccagcaaccgcacctgtggcgccggtgatgccggccacgatgcgtccggcgtagaggatcgagatctcgatcccgcgaaattaatacgactcactataggggaattgtgagcggataacaattcccctctagaaataattttgtttaactttaagaaggagatatacatatgaaatacctgctgccgaccgctgctgctggtctgctgctcctcgctgcccagccggcgatggccgaagtgcaactggtggaaagcggtggaggccttgttcagaccggcggcagcctgcgtctgtcatgcgctgcaagcggctttacgttcagcagctacgcgatgagctgggtgcgccaggcaccgggcaaaggcttggaatgggttagcggcatcaagtcaagcggcgatagcaccagatatgccggaagcgttaaaggccgctttaccatttcacgcgataacgccaagaacatgctgtatctgcaaatgtatagcctgaaaccggaagataccgcagtgtattactgcgccaagagccgcgtgagtcgcacgggtctgtatacctatgacaaccgtggtcagggcacgcaggtgactgtgtcaagccatcatcaccatcatcattaagatccggctgctaacaaagcccgaaaggaagctgagttggctgctgccaccgctgagcaataactagcataaccccttggggcctctaaacgggtcttgaggggttttttgctgaaaggaggaactatatccggat

SEQ ID NO: 93 - DNA, 5482 bp, synthetic construct
  source 1..5482: mol_type = other DNA
tggcgaatgggacgcgccctgtagcggcgcattaagcgcggcgggtgtggtggttacgcgcagcgtgaccgctacacttgccagcgccctagcgcccgctcctttcgctttcttcccttcctttctcgccacgttcgccggctttccccgtcaagctctaaatcgggggctccctttagggttccgatttagtgctttacggcacctcgaccccaaaaaacttgattagggtgatggttcacgtagtgggccatcgccctgatagacggtttttcgccctttgacgttggagtccacgttctttaatagtggactcttgttccaaactggaacaacactcaaccctatctcggtctattcttttgatttataagggattttgccgatttcggcctattggttaaaaaatgagctgatttaacaaaaatttaacgcgaattttaacaaaatattaacgcttacaatttaggtggcacttttcggggaaatgtgcgcggaacccctatttgtttatttttctaaatacattcaaatatgtatccgctcatgaattaattcttagaaaaactcatcgagcatcaaatgaaactgcaatttattcatatcaggattatcaataccatatttttgaaaaagccgtttctgtaatgaaggagaaaactcaccgaggcagttccataggatggcaagatcctggtatcggtctgcgattccgactcgtccaacatcaatacaacctattaatttcccctcgtcaaaaataaggttatcaagtgagaaatcaccatgagtgacgactgaatccggtgagaatggcaaaagtttatgcatttctttccagacttgttcaacaggccagccattacgctcgtcatcaaaatcactcgcatcaaccaaaccgttattcattcgtgattgcgcctgagcgagacgaaatacgcgatcgctgttaaaaggacaattacaaacaggaatcgaatgcaaccggcgcaggaacactgccagcgcatcaacaatattttcacctgaatcaggatattcttctaatacctggaatgctgttttcccggggatcgcagtggtgagtaaccatgcatcatcaggagtacggataaaatgcttgatggtcggaagaggcataaattccgtcagccagtttagtctgaccatctcatctgtaacatcattggcaacgctacctttgccatgtttcagaaacaactctggcgcatcgggcttcccatacaatcgatagattgtcgcacctgattgcccgacattatcgcgagcccatttatacccatataaatcagcatccatgttggaatttaatcgcggcctagagcaagacgtttcccgttgaatatggctcataacaccccttgtattactgtttatgtaagcagacagttttattgttcatgaccaaaatcccttaacgtgagttttcgttccactgagcgtcagaccccgtagaaaagatcaaaggatcttcttgagatcctttttttctgcgcgtaatctgctgcttgcaaacaaaaaaaccaccgctaccagcggtggtttgtttgccggatcaagagctaccaactctttttccgaaggtaactggcttcagcagagcgcagataccaaatactgtccttctagtgtagccgtagttaggccaccacttcaagaactctgtagcaccgcctacatacctcgctctgctaatcctgttaccagtggctgctgccagtggcgataagtcgtgtcttaccgggttggactcaagacgatagttaccggataaggcgcagcggtcgggctgaacggggggttcgtgcacacagcccagcttggagcgaacgacctacaccgaactgagatacctacagcgtgagctatgagaaagcgccacgcttcccgaagggagaaaggcggacaggtatccggtaagcggcagggtcggaacaggagagcgcacgagggagcttccagggggaaacgcctggtatctttatagtcctgtcgggtttcgccacctctgacttgagcgtcgatttttgtgatgctcgtcaggggggcggagcctatggaaaaacgccagcaacgcggcctttttacggttcctggccttttgctggccttttgctcacatgttctttcctgcgttatcccctgattctgtggataaccgtattaccgcctttgagtgagctgataccgctcgccgcagccgaacgaccgagcgcagcgagtcagtgagcgaggaagcggaagagcgcctgatgcggtattttctccttacgcatctgtgcggtatttcacaccgcaatggtgcactctcagtacaatctgctctgatgccgcatagttaagccagtatacactccgctatcgctacgtgactgggtcatggctgcgccccgacacccgccaacacccgctgacgcgccctgacgggcttgtctgctcccggcatccgcttacagacaagctgtgaccgtctccgggagctgcatgtgtgatgcctccgtgtaagggggatttctgttcatgggggtaatgataccgatgaaacgagagaggatgctcacgatacgggttactgatgatgaacatgcccggttactggaacgttgtgagggtaaacaactggcggtatggatgcggcgggaccagagaaaaatcactcagggtcaatgccagcgcttcgttaatacagatgtaggtgttccacagggtagccagcagcatcctgcgatgcagatccggaacataatggtgcagggcgctgacttccgcgtttccagactttacgaaacacggaaaccgaagaccattcatgttgttgctcaggtcgcagacgttttgcagcagcagtcgcttcacgttcgctcgcgtatcggtgattcattctgctaaccagtaaggcaaccccgccagcctagccgggtcctcaacgacaggagcacgatcatgcgcacccgtggggccgccatgccggcgataatggcctgcttctcgccgaaacgtttggtggcgggaccagtgacgaaggcttgagcgagggcgtgcaagattccgaataccgcaagcgacaggccgatcatcgtcgcgctccagcgaaagcggtcctcgccgaaaatgacccagagcgctgccggcacctgtcctacgagttgcatgataaagaagacagtcataagtgcggcgacgatagtcatgccccgcgcccaccggaaggagctgactgggttgaaggctctcaagggcatcggtcgagatcccggtgcctaatgagtgagctaacttacattaattgcgttgcgctcactgcccgctttccagtcgggaaacctgtcgtgccagctgcattaatgaatcggccaacgcgcggggagaggcggtttgcgtattgggcgccagggtggtttttcttttcaccagtgagacgggcaacagctgattgcccttcaccgcctggccctgagagagttgcagcaagcggtccacgctggtttgccccagcaggcgaaaatcctgtttgatggtggttaacggcgggatataacatgagctgtcttcggtatcgtcgtatcccactaccgagatatccgcaccaacgcgcagcccggactcggtaatggcgcgcattgcgcccagcgccatctgatcgttggcaaccagcatcgcagtgggaacgatgccctcattcagcatttgcatggtttgttgaaaaccggacatggcactccagtcgccttcccgttccgctatcggctgaatttgattgcgagtgagatatttatgccagccagccagacgcagacgcgccgagacagaacttaatgggcccgctaacagcgcgatttgctggtgacccaatgcgaccagatgctccacgcccagtcgcgtaccgtcttcatgggagaaaataatactgttgatgggtgtctggtcagagacatcaagaaataacgccggaacattagtgcaggcagcttccacagcaatggcatcctggtcatccagcggatagttaatgatcagcccactgacgcgttgcgcgagaagattgtgcaccgccgctttacaggcttcgacgccgcttcgttctaccatcgacaccaccacgctggcacccagttgatcggcgcgagatttaatcgccgcgacaatttgcgacggcgcgtgcagggccagactggaggtggcaacgccaatcagcaacgactgtttgcccgccagttgttgtgccacgcggttgggaatgtaattcagctccgccatcgccgcttccactttttcccgcgttttcgcagaaacgtggctggcctggttcaccacgcgggaaacggtctgataagagacaccggcatactctgcgacatcgtataacgttactggtttcacattcaccaccctgaattgactctcttccgggcgctatcatgccataccgcgaaaggttttgcgccattcgatggtgtccgggatctcgacgctctcccttatgcgactcctgcattaggaagcagcccagtagtaggttgaggccgttgagcaccgccgccgcaaggaatggtgcatgcaaggagatggcgcccaacagtcccccggccacggggcctgccaccatacccacgccgaaacaagcgctcatgagcccgaagtggcgagcccgatcttccccatcggtgatgtcggcgatataggcgccagcaaccgcacctgtggcgccggtgatgccggccacgatgcgtccggcgtagaggatcgagatctcgatcccgcgaaattaatacgactcactataggggaattgtgagcggataacaattcccctctagaaataattttgtttaactttaagaaggagatatacatatgaaatacctgctgccgaccgctgctgctggtctgctgctcctcgctgcccagccggcgatggccgaagtccagctggttgaaagcggtggaggcctggttcagaccggcggaagcctgcgtctgagctgtgcagcctctggccgcacgtttaacaactacgcgatgggctggtttcgccgtgcaccgggcaaagaacgcgaatttgtggcggcaatcactcgtagcggtgtgagaagcggagtgtcagcgatctatggcgatagcgtgaaagatcgcttcaccatcagccgcgataacgccaagaacaccttgtacttgcagatgaacagcctgaaaccggaagatactgcggtgtatacctgcgccgcaagtgcgatcggcagcggtgcactgcgtcgtttcgaatacgactatagcggtcagggcacacaggtgaccgtgagcagccatcatcaccatcatcattaagatccggctgctaacaaagcccgaaaggaagctgagttggctgctgccaccgctgagcaataactagcataaccccttggggcctctaaacgggtcttgaggggttttttgctgaaaggaggaactatatccggat

SEQ ID NO: 94 - DNA, 5497 bp, synthetic construct
  source 1..5497: mol_type = other DNA
tggcgaatgggacgcgccctgtagcggcgcattaagcgcggcgggtgtggtggttacgcgcagcgtgaccgctacacttgccagcgccctagcgcccgctcctttcgctttcttcccttcctttctcgccacgttcgccggctttccccgtcaagctctaaatcgggggctccctttagggttccgatttagtgctttacggcacctcgaccccaaaaaacttgattagggtgatggttcacgtagtgggccatcgccctgatagacggtttttcgccctttgacgttggagtccacgttctttaatagtggactcttgttccaaactggaacaacactcaaccctatctcggtctattcttttgatttataagggattttgccgatttcggcctattggttaaaaaatgagctgatttaacaaaaatttaacgcgaattttaacaaaatattaacgcttacaatttaggtggcacttttcggggaaatgtgcgcggaacccctatttgtttatttttctaaatacattcaaatatgtatccgctcatgaattaattcttagaaaaactcatcgagcatcaaatgaaactgcaatttattcatatcaggattatcaataccatatttttgaaaaagccgtttctgtaatgaaggagaaaactcaccgaggcagttccataggatggcaagatcctggtatcggtctgcgattccgactcgtccaacatcaatacaacctattaatttcccctcgtcaaaaataaggttatcaagtgagaaatcaccatgagtgacgactgaatccggtgagaatggcaaaagtttatgcatttctttccagacttgttcaacaggccagccattacgctcgtcatcaaaatcactcgcatcaaccaaaccgttattcattcgtgattgcgcctgagcgagacgaaatacgcgatcgctgttaaaaggacaattacaaacaggaatcgaatgcaaccggcgcaggaacactgccagcgcatcaacaatattttcacctgaatcaggatattcttctaatacctggaatgctgttttcccggggatcgcagtggtgagtaaccatgcatcatcaggagtacggataaaatgcttgatggtcggaagaggcataaattccgtcagccagtttagtctgaccatctcatctgtaacatcattggcaacgctacctttgccatgtttcagaaacaactctggcgcatcgggcttcccatacaatcgatagattgtcgcacctgattgcccgacattatcgcgagcccatttatacccatataaatcagcatccatgttggaatttaatcgcggcctagagcaagacgtttcccgttgaatatggctcataacaccccttgtattactgtttatgtaagcagacagttttattgttcatgaccaaaatcccttaacgtgagttttcgttccactgagcgtcagaccccgtagaaaagatcaaaggatcttcttgagatcctttttttctgcgcgtaatctgctgcttgcaaacaaaaaaaccaccgctaccagcggtggtttgtttgccggatcaagagctaccaactctttttccgaaggtaactggcttcagcagagcgcagataccaaatactgtccttctagtgtagccgtagttaggccaccacttcaagaactctgtagcaccgcctacatacctcgctctgctaatcctgttaccagtggctgctgccagtggcgataagtcgtgtcttaccgggttggactcaagacgatagttaccggataaggcgcagcggtcgggctgaacggggggttcgtgcacacagcccagcttggagcgaacgacctacaccgaactgagatacctacagcgtgagctatgagaaagcgccacgcttcccgaagggagaaaggcggacaggtatccggtaagcggcagggtcggaacaggagagcgcacgagggagcttccagggggaaacgcctggtatctttatagtcctgtcgggtttcgccacctctgacttgagcgtcgatttttgtgatgctcgtcaggggggcggagcctatggaaaaacgccagcaacgcggcctttttacggttcctggccttttgctggccttttgctcacatgttctttcctgcgttatcccctgattctgtggataaccgtattaccgcctttgagtgagctgataccgctcgccgcagccgaacgaccgagcgcagcgagtcagtgagcgaggaagcggaagagcgcctgatgcggtattttctccttacgcatctgtgcggtatttcacaccgcaatggtgcactctcagtacaatctgctctgatgccgcatagttaagccagtatacactccgctatcgctacgtgactgggtcatggctgcgccccgacacccgccaacacccgctgacgcgccctgacgggcttgtctgctcccggcatccgcttacagacaagctgtgaccgtctccgggagctgcatgtgtgatgcctccgtgtaagggggatttctgttcatgggggtaatgataccgatgaaacgagagaggatgctcacgatacgggttactgatgatgaacatgcccggttactggaacgttgtgagggtaaacaactggcggtatggatgcggcgggaccagagaaaaatcactcagggtcaatgccagcgcttcgttaatacagatgtaggtgttccacagggtagccagcagcatcctgcgatgcagatccggaacataatggtgcagggcgctgacttccgcgtttccagactttacgaaacacggaaaccgaagaccattcatgttgttgctcaggtcgcagacgttttgcagcagcagtcgcttcacgttcgctcgcgtatcggtgattcattctgctaaccagtaaggcaaccccgccagcctagccgggtcctcaacgacaggagcacgatcatgcgcacccgtggggccgccatgccggcgataatggcctgcttctcgccgaaacgtttggtggcgggaccagtgacgaaggcttgagcgagggcgtgcaagattccgaataccgcaagcgacaggccgatcatcgtcgcgctccagcgaaagcggtcctcgccgaaaatgacccagagcgctgccggcacctgtcctacgagttgcatgataaagaagacagtcataagtgcggcgacgatagtcatgccccgcgcccaccggaaggagctgactgggttgaaggctctcaagggcatcggtcgagatcccggtgcctaatgagtgagctaacttacattaattgcgttgcgctcactgcccgctttccagtcgggaaacctgtcgtgccagctgcattaatgaatcggccaacgcgcggggagaggcggtttgcgtattgggcgccagggtggtttttcttttcaccagtgagacgggcaacagctgattgcccttcaccgcctggccctgagagagttgcagcaagcggtccacgctggtttgccccagcaggcgaaaatcctgtttgatggtggttaacggcgggatataacatgagctgtcttcggtatcgtcgtatcccactaccgagatatccgcaccaacgcgcagcccggactcggtaatggcgcgcattgcgcccagcgccatctgatcgttggcaaccagcatcgcagtgggaacgatgccctcattcagcatttgcatggtttgttgaaaaccggacatggcactccagtcgccttcccgttccgctatcggctgaatttgattgcgagtgagatatttatgccagccagccagacgcagacgcgccgagacagaacttaatgggcccgctaacagcgcgatttgctggtgacccaatgcgaccagatgctccacgcccagtcgcgtaccgtcttcatgggagaaaataatactgttgatgggtgtctggtcagagacatcaagaaataacgccggaacattagtgcaggcagcttccacagcaatggcatcctggtcatccagcggatagttaatgatcagcccactgacgcgttgcgcgagaagattgtgcaccgccgctttacaggcttcgacgccgcttcgttctaccatcgacaccaccacgctggcacccagttgatcggcgcgagatttaatcgccgcgacaatttgcgacggcgcgtgcagggccagactggaggtggcaacgccaatcagcaacgactgtttgcccgccagttgttgtgccacgcggttgggaatgtaattcagctccgccatcgccgcttccactttttcccgcgttttcgcagaaacgtggctggcctggttcaccacgcgggaaacggtctgataagagacaccggcatactctgcgacatcgtataacgttactggtttcacattcaccaccctgaattgactctcttccgggcgctatcatgccataccgcgaaaggttttgcgccattcgatggtgtccgggatctcgacgctctcccttatgcgactcctgcattaggaagcagcccagtagtaggttgaggccgttgagcaccgccgccgcaaggaatggtgcatgcaaggagatggcgcccaacagtcccccggccacggggcctgccaccatacccacgccgaaacaagcgctcatgagcccgaagtggcgagcccgatcttccccatcggtgatgtcggcgatataggcgccagcaaccgcacctgtggcgccggtgatgccggccacgatgcgtccggcgtagaggatcgagatctcgatcccgcgaaattaatacgactcactataggggaattgtgagcggataacaattcccctctagaaataattttgtttaactttaagaaggagatatacatatgaaatacctgctgccgaccgctgctgctggtctgctgctcctcgctgcccagccggcgatggcccaggttcagctgcaagaaagcggaggtggtctggttcagccgggaggtagcttacgcctgtcatgcgcagcaagcggtcgtacctttagcagctatgcgatgggctggtttcgtcaggcacctggcaaagaacgcgaatttgtggcggcaattcgctggtcaggcggctatacctactacaccgatagcgtgaaaggccgctttaccattagccgcgataacgccaagaccaccgtgtacctgcaaatgaacagcctgaaaccggaagataccgcagtgtactactgcgcagcgacctatctgagcagcgattatagccgctatgccttaccgcagcgtccgctggattacgactattggggccaaggtacgcaggttaccgttagcagcgcagcagcgcatcatcaccatcatcattaagatccggctgctaacaaagcccgaaaggaagctgagttggctgctgccaccgctgagcaataactagcataaccccttggggcctctaaacgggtcttgaggggttttttgctgaaaggaggaactatatccggat

SEQ ID NO: 95 - DNA, 5461 bp, synthetic construct
  source 1..5461: mol_type = other DNA
tggcgaatgggacgcgccctgtagcggcgcattaagcgcggcgggtgtggtggttacgcgcagcgtgaccgctacacttgccagcgccctagcgcccgctcctttcgctttcttcccttcctttctcgccacgttcgccggctttccccgtcaagctctaaatcgggggctccctttagggttccgatttagtgctttacggcacctcgaccccaaaaaacttgattagggtgatggttcacgtagtgggccatcgccctgatagacggtttttcgccctttgacgttggagtccacgttctttaatagtggactcttgttccaaactggaacaacactcaaccctatctcggtctattcttttgatttataagggattttgccgatttcggcctattggttaaaaaatgagctgatttaacaaaaatttaacgcgaattttaacaaaatattaacgcttacaatttaggtggcacttttcggggaaatgtgcgcggaacccctatttgtttatttttctaaatacattcaaatatgtatccgctcatgaattaattcttagaaaaactcatcgagcatcaaatgaaactgcaatttattcatatcaggattatcaataccatatttttgaaaaagccgtttctgtaatgaaggagaaaactcaccgaggcagttccataggatggcaagatcctggtatcggtctgcgattccgactcgtccaacatcaatacaacctattaatttcccctcgtcaaaaataaggttatcaagtgagaaatcaccatgagtgacgactgaatccggtgagaatggcaaaagtttatgcatttctttccagacttgttcaacaggccagccattacgctcgtcatcaaaatcactcgcatcaaccaaaccgttattcattcgtgattgcgcctgagcgagacgaaatacgcgatcgctgttaaaaggacaattacaaacaggaatcgaatgcaaccggcgcaggaacactgccagcgcatcaacaatattttcacctgaatcaggatattcttctaatacctggaatgctgttttcccggggatcgcagtggtgagtaaccatgcatcatcaggagtacggataaaatgcttgatggtcggaagaggcataaattccgtcagccagtttagtctgaccatctcatctgtaacatcattggcaacgctacctttgccatgtttcagaaacaactctggcgcatcgggcttcccatacaatcgatagattgtcgcacctgattgcccgacattatcgcgagcccatttatacccatataaatcagcatccatgttggaatttaatcgcggcctagagcaagacgtttcccgttgaatatggctcataacaccccttgtattactgtttatgtaagcagacagttttattgttcatgaccaaaatcccttaacgtgagttttcgttccactgagcgtcagaccccgtagaaaagatcaaaggatcttcttgagatcctttttttctgcgcgtaatctgctgcttgcaaacaaaaaaaccaccgctaccagcggtggtttgtttgccggatcaagagctaccaactctttttccgaaggtaactggcttcagcagagcgcagataccaaatactgtccttctagtgtagccgtagttaggccaccacttcaagaactctgtagcaccgcctacatacctcgctctgctaatcctgttaccagtggctgctgccagtggcgataagtcgtgtcttaccgggttggactcaagacgatagttaccggataaggcgcagcggtcgggctgaacggggggttcgtgcacacagcccagcttggagcgaacgacctacaccgaactgagatacctacagcgtgagctatgagaaagcgccacgcttcccgaagggagaaaggcggacaggtatccggtaagcggcagggtcggaacaggagagcgcacgagggagcttccagggggaaacgcctggtatctttatagtcctgtcgggtttcgccacctctgacttgagcgtcgatttttgtgatgctcgtcaggggggcggagcctatggaaaaacgccagcaacgcggcctttttacggttcctggccttttgctggccttttgctcacatgttctttcctgcgttatcccctgattctgtggataaccgtattaccgcctttgagtgagctgataccgctcgccgcagccgaacgaccgagcgcagcgagtcagtgagcgaggaagcggaagagcgcctgatgcggtattttctccttacgcatctgtgcggtatttcacaccgcaatggtgcactctcagtacaatctgctctgatgccgcatagttaagccagtatacactccgctatcgctacgtgactgggtcatggctgcgccccgacacccgccaacacccgctgacgcgccctgacgggcttgtctgctcccggcatccgcttacagacaagctgtgaccgtctccgggagctgcatgtgtgatgcctccgtgtaagggggatttctgttcatgggggtaatgataccgatgaaacgagagaggatgctcacgatacgggttactgatgatgaacatgcccggttactggaacgttgtgagggtaaacaactggcggtatggatgcggcgggaccagagaaaaatcactcagggtcaatgccagcgcttcgttaatacagatgtaggtgttccacagggtagccagcagcatcctgcgatgcagatccggaacataatggtgcagggcgctgacttccgcgtttccagactttacgaaacacggaaaccgaagaccattcatgttgttgctcaggtcgcagacgttttgcagcagcagtcgcttcacgttcgctcgcgtatcggtgattcattctgctaaccagtaaggcaaccccgccagcctagccgggtcctcaacgacaggagcacgatcatgcgcacccgtggggccgccatgccggcgataatggcctgcttctcgccgaaacgtttggtggcgggaccagtgacgaaggcttgagcgagggcgtgcaagattccgaataccgcaagcgacaggccgatcatcgtcgcgctccagcgaaagcggtcctcgccgaaaatgacccagagcgctgccggcacctgtcctacgagttgcatgataaagaagacagtcataagtgcggcgacgatagtcatgccccgcgcccaccggaaggagctgactgggttgaaggctctcaagggcatcggtcgagatcccggtgcctaatgagtgagctaacttacattaattgcgttgcgctcactgcccgctttccagtcgggaaacctgtcgtgccagctgcattaatgaatcggccaacgcgcggggagaggcggtttgcgtattgggcgccagggtggtttttcttttcaccagtgagacgggcaacagctgattgcccttcaccgcctggccctgagagagttgcagcaagcggtccacgctggtttgccccagcaggcgaaaatcctgtttgatggtggttaacggcgggatataacatgagctgtcttcggtatcgtcgtatcccactaccgagatatccgcaccaacgcgcagcccggactcggtaatggcgcgcattgcgcccagcgccatctgatcgttggcaaccagcatcgcagtgggaacgatgccctcattcagcatttgcatggtttgttgaaaaccggacatggcactccagtcgccttcccgttccgctatcggctgaatttgattgcgagtgagatatttatgccagccagccagacgcagacgcgccgagacagaacttaatgggcccgctaacagcgcgatttgctggtgacccaatgcgaccagatgctccacgcccagtcgcgtaccgtcttcatgggagaaaataatactgttgatgggtgtctggtcagagacatcaagaaataacgccggaacattagtgcaggcagcttccacagcaatggcatcctggtcatccagcggatagttaatgatcagcccactgacgcgttgcgcgagaagattgtgcaccgccgctttacaggcttcgacgccgcttcgttctaccatcgacaccaccacgctggcacccagttgatcggcgcgagatttaatcgccgcgacaatttgcgacggcgcgtgcagggccagactggaggtggcaacgccaatcagcaacgactgtttgcccgccagttgttgtgccacgcggttgggaatgtaattcagctccgccatcgccgcttccactttttcccgcgttttcgcagaaacgtggctggcctggttcaccacgcgggaaacggtctgataagagacaccggcatactctgcgacatcgtataacgttactggtttcacattcaccaccctgaattgactctcttccgggcgctatcatgccataccgcgaaaggttttgcgccattcgatggtgtccgggatctcgacgctctcccttatgcgactcctgcattaggaagcagcccagtagtaggttgaggccgttgagcaccgccgccgcaaggaatggtgcatgcaaggagatggcgcccaacagtcccccggccacggggcctgccaccatacccacgccgaaacaagcgctcatgagcccgaagtggcgagcccgatcttccccatcggtgatgtcggcgatataggcgccagcaaccgcacctgtggcgccggtgatgccggccacgatgcgtccggcgtagaggatcgagatctcgatcccgcgaaattaatacgactcactataggggaattgtgagcggataacaattcccctctagaaataattttgtttaactttaagaaggagatatacatatgaaatacctgctgccgaccgctgctgctggtctgctgctcctcgctgcccagccggcgatggccggcggtggcagcgttcaggcaggtggcagcctgaaactgagctgcgaagccagcctgcctagcacgaccacgccgtatagcatggcctggtttcgtcaggcgcctggacgtgaaagagaagcggtggccaccatcagcgcaagaggtggcactaaactgtacagcgattctgtgcgcgaacgcttcacgattagccgtgataaccgcaagaacacggtctacctgaagatggatcatctgaacaccgatgataccgccatctactattgcgccgcaacgggcagcattctgtttaatagccgtccattcgcggaaagcacgtatccgttctggggtcagggtactctggtcacggtgagcagccatcatcaccatcatcattaagatccggctgctaacaaagcccgaaaggaagctgagttggctgctgccaccgctgagcaataactagcataaccccttggggcctctaaacgggtcttgaggggttttttgctgaaaggaggaactatatccggat

SEQ ID NO: 96 - DNA, 5488 bp, synthetic construct
  source 1..5488: mol_type = other DNA
tggcgaatgggacgcgccctgtagcggcgcattaagcgcggcgggtgtggtggttacgcgcagcgtgaccgctacacttgccagcgccctagcgcccgctcctttcgctttcttcccttcctttctcgccacgttcgccggctttccccgtcaagctctaaatcgggggctccctttagggttccgatttagtgctttacggcacctcgaccccaaaaaacttgattagggtgatggttcacgtagtgggccatcgccctgatagacggtttttcgccctttgacgttggagtccacgttctttaatagtggactcttgttccaaactggaacaacactcaaccctatctcggtctattcttttgatttataagggattttgccgatttcggcctattggttaaaaaatgagctgatttaacaaaaatttaacgcgaattttaacaaaatattaacgcttacaatttaggtggcacttttcggggaaatgtgcgcggaacccctatttgtttatttttctaaatacattcaaatatgtatccgctcatgaattaattcttagaaaaactcatcgagcatcaaatgaaactgcaatttattcatatcaggattatcaataccatatttttgaaaaagccgtttctgtaatgaaggagaaaactcaccgaggcagttccataggatggcaagatcctggtatcggtctgcgattccgactcgtccaacatcaatacaacctattaatttcccctcgtcaaaaataaggttatcaagtgagaaatcaccatgagtgacgactgaatccggtgagaatggcaaaagtttatgcatttctttccagacttgttcaacaggccagccattacgctcgtcatcaaaatcactcgcatcaaccaaaccgttattcattcgtgattgcgcctgagcgagacgaaatacgcgatcgctgttaaaaggacaattacaaacaggaatcgaatgcaaccggcgcaggaacactgccagcgcatcaacaatattttcacctgaatcaggatattcttctaatacctggaatgctgttttcccggggatcgcagtggtgagtaaccatgcatcatcaggagtacggataaaatgcttgatggtcggaagaggcataaattccgtcagccagtttagtctgaccatctcatctgtaacatcattggcaacgctacctttgccatgtttcagaaacaactctggcgcatcgggcttcccatacaatcgatagattgtcgcacctgattgcccgacattatcgcgagcccatttatacccatataaatcagcatccatgttggaatttaatcgcggcctagagcaagacgtttcccgttgaatatggctcataacaccccttgtattactgtttatgtaagcagacagttttattgttcatgaccaaaatcccttaacgtgagttttcgttccactgagcgtcagaccccgtagaaaagatcaaaggatcttcttgagatcctttttttctgcgcgtaatctgctgcttgcaaacaaaaaaaccaccgctaccagcggtggtttgtttgccggatcaagagctaccaactctttttccgaaggtaactggcttcagcagagcgcagataccaaatactgtccttctagtgtagccgtagttaggccaccacttcaagaactctgtagcaccgcctacatacctcgctctgctaatcctgttaccagtggctgctgccagtggcgataagtcgtgtcttaccgggttggactcaagacgatagttaccggataaggcgcagcggtcgggctgaacggggggttcgtgcacacagcccagcttggagcgaacgacctacaccgaactgagatacctacagcgtgagctatgagaaagcgccacgcttcccgaagggagaaaggcggacaggtatccggtaagcggcagggtcggaacaggagagcgcacgagggagcttccagggggaaacgcctggtatctttatagtcctgtcgggtttcgccacctctgacttgagcgtcgatttttgtgatgctcgtcaggggggcggagcctatggaaaaacgccagcaacgcggcctttttacggttcctggccttttgctggccttttgctcacatgttctttcctgcgttatcccctgattctgtggataaccgtattaccgcctttgagtgagctgataccgctcgccgcagccgaacgaccgagcgcagcgagtcagtgagcgaggaagcggaagagcgcctgatgcggtattttctccttacgcatctgtgcggtatttcacaccgcaatggtgcactctcagtacaatctgctctgatgccgcatagttaagccagtatacactccgctatcgctacgtgactgggtcatggctgcgccccgacacccgccaacacccgctgacgcgccctgacgggcttgtctgctcccggcatccgcttacagacaagctgtgaccgtctccgggagctgcatgtgtgatgcctccgtgtaagggggatttctgttcatgggggtaatgataccgatgaaacgagagaggatgctcacgatacgggttactgatgatgaacatgcccggttactggaacgttgtgagggtaaacaactggcggtatggatgcggcgggaccagagaaaaatcactcagggtcaatgccagcgcttcgttaatacagatgtaggtgttccacagggtagccagcagcatcctgcgatgcagatccggaacataatggtgcagggcgctgacttccgcgtttccagactttacgaaacacggaaaccgaagaccattcatgttgttgctcaggtcgcagacgttttgcagcagcagtcgcttcacgttcgctcgcgtatcggtgattcattctgctaaccagtaaggcaaccccgccagcctagccgggtcctcaacgacaggagcacgatcatgcgcacccgtggggccgccatgccggcgataatggcctgcttctcgccgaaacgtttggtggcgggaccagtgacgaaggcttgagcgagggcgtgcaagattccgaataccgcaagcgacaggccgatcatcgtcgcgctccagcgaaagcggtcctcgccgaaaatgacccagagcgctgccggcacctgtcctacgagttgcatgataaagaagacagtcataagtgcggcgacgatagtcatgccccgcgcccaccggaaggagctgactgggttgaaggctctcaagggcatcggtcgagatcccggtgcctaatgagtgagctaacttacattaattgcgttgcgctcactgcccgctttccagtcgggaaacctgtcgtgccagctgcattaatgaatcggccaacgcgcggggagaggcggtttgcgtattgggcgccagggtggtttttcttttcaccagtgagacgggcaacagctgattgcccttcaccgcctggccctgagagagttgcagcaagcggtccacgctggtttgccccagcaggcgaaaatcctgtttgatggtggttaacggcgggatataacatgagctgtcttcggtatcgtcgtatcccactaccgagatatccgcaccaacgcgcagcccggactcggtaatggcgcgcattgcgcccagcgccatctgatcgttggcaaccagcatcgcagtgggaacgatgccctcattcagcatttgcatggtttgttgaaaaccggacatggcactccagtcgccttcccgttccgctatcggctgaatttgattgcgagtgagatatttatgccagccagccagacgcagacgcgccgagacagaacttaatgggcccgctaacagcgcgatttgctggtgacccaatgcgaccagatgctccacgcccagtcgcgtaccgtcttcatgggagaaaataatactgttgatgggtgtctggtcagagacatcaagaaataacgccggaacattagtgcaggcagcttccacagcaatggcatcctggtcatccagcggatagttaatgatcagcccactgacgcgttgcgcgagaagattgtgcaccgccgctttacaggcttcgacgccgcttcgttctaccatcgacaccaccacgctggcacccagttgatcggcgcgagatttaatcgccgcgacaatttgcgacggcgcgtgcagggccagactggaggtggcaacgccaatcagcaacgactgtttgcccgccagttgttgtgccacgcggttgggaatgtaattcagctccgccatcgccgcttccactttttcccgcgttttcgcagaaacgtggctggcctggttcaccacgcgggaaacggtctgataagagacaccggcatactctgcgacatcgtataacgttactggtttcacattcaccaccctgaattgactctcttccgggcgctatcatgccataccgcgaaaggttttgcgccattcgatggtgtccgggatctcgacgctctcccttatgcgactcctgcattaggaagcagcccagtagtaggttgaggccgttgagcaccgccgccgcaaggaatggtgcatgcaaggagatggcgcccaacagtcccccggccacggggcctgccaccatacccacgccgaaacaagcgctcatgagcccgaagtggcgagcccgatcttccccatcggtgatgtcggcgatataggcgccagcaaccgcacctgtggcgccggtgatgccggccacgatgcgtccggcgtagaggatcgagatctcgatcccgcgaaattaatacgactcactataggggaattgtgagcggataacaattcccctctagaaataattttgtttaactttaagaaggagatatacatatgaaatacctgctgccgaccgctgctgctggtctgctgctcctcgctgcccagccggcgatggccggcggtggcacggtacaggctggcggtagcctgaaactgagctgcgccgcgagaggttggcgctttagcggctattgcgtagcctggtttcgtcaagcaccgggcaaagaacgcgaagcggtagcgatcattccgggtgctggcgtgatgtataccgatgattctgtgaaaggccgtttcacctattcgcgcgataatgtgaagaacaccgttagtctgcaaatgaacagcctggaaccggaagataccgcaacgtactactgcgctgtggattgggcatacagccatagctgtccgaagaacacggaagattaccgttattggggccagggcacgcaggtgaccgtgtcatcatacccctatgacgtgcctgattacgccggctctggccaccaccaccaccaccactgagatccggctgctaacaaagcccgaaaggaagctgagttggctgctgccaccgctgagcaataactagcataaccccttggggcctctaaacgggtcttgaggggttttttgctgaaaggaggaactatatccggat

SEQ ID NO: 97 - DNA, 6229 bp, synthetic construct
  source 1..6229: mol_type = other DNA
tggcgaatgggacgcgccctgtagcggcgcattaagcgcggcgggtgtggtggttacgcgcagcgtgaccgctacacttgccagcgccctagcgcccgctcctttcgctttcttcccttcctttctcgccacgttcgccggctttccccgtcaagctctaaatcgggggctccctttagggttccgatttagtgctttacggcacctcgaccccaaaaaacttgattagggtgatggttcacgtagtgggccatcgccctgatagacggtttttcgccctttgacgttggagtccacgttctttaatagtggactcttgttccaaactggaacaacactcaaccctatctcggtctattcttttgatttataagggattttgccgatttcggcctattggttaaaaaatgagctgatttaacaaaaatttaacgcgaattttaacaaaatattaacgcttacaatttaggtggcacttttcggggaaatgtgcgcggaacccctatttgtttatttttctaaatacattcaaatatgtatccgctcatgaattaattcttagaaaaactcatcgagcatcaaatgaaactgcaatttattcatatcaggattatcaataccatatttttgaaaaagccgtttctgtaatgaaggagaaaactcaccgaggcagttccataggatggcaagatcctggtatcggtctgcgattccgactcgtccaacatcaatacaacctattaatttcccctcgtcaaaaataaggttatcaagtgagaaatcaccatgagtgacgactgaatccggtgagaatggcaaaagtttatgcatttctttccagacttgttcaacaggccagccattacgctcgtcatcaaaatcactcgcatcaaccaaaccgttattcattcgtgattgcgcctgagcgagacgaaatacgcgatcgctgttaaaaggacaattacaaacaggaatcgaatgcaaccggcgcaggaacactgccagcgcatcaacaatattttcacctgaatcaggatattcttctaatacctggaatgctgttttcccggggatcgcagtggtgagtaaccatgcatcatcaggagtacggataaaatgcttgatggtcggaagaggcataaattccgtcagccagtttagtctgaccatctcatctgtaacatcattggcaacgctacctttgccatgtttcagaaacaactctggcgcatcgggcttcccatacaatcgatagattgtcgcacctgattgcccgacattatcgcgagcccatttatacccatataaatcagcatccatgttggaatttaatcgcggcctagagcaagacgtttcccgttgaatatggctcataacaccccttgtattactgtttatgtaagcagacagttttattgttcatgaccaaaatcccttaacgtgagttttcgttccactgagcgtcagaccccgtagaaaagatcaaaggatcttcttgagatcctttttttctgcgcgtaatctgctgcttgcaaacaaaaaaaccaccgctaccagcggtggtttgtttgccggatcaagagctaccaactctttttccgaaggtaactggcttcagcagagcgcagataccaaatactgtccttctagtgtagccgtagttaggccaccacttcaagaactctgtagcaccgcctacatacctcgctctgctaatcctgttaccagtggctgctgccagtggcgataagtcgtgtcttaccgggttggactcaagacgatagttaccggataaggcgcagcggtcgggctgaacggggggttcgtgcacacagcccagcttggagcgaacgacctacaccgaactgagatacctacagcgtgagctatgagaaagcgccacgcttcccgaagggagaaaggcggacaggtatccggtaagcggcagggtcggaacaggagagcgcacgagggagcttccagggggaaacgcctggtatctttatagtcctgtcgggtttcgccacctctgacttgagcgtcgatttttgtgatgctcgtcaggggggcggagcctatggaaaaacgccagcaacgcggcctttttacggttcctggccttttgctggccttttgctcacatgttctttcctgcgttatcccctgattctgtggataaccgtattaccgcctttgagtgagctgataccgctcgccgcagccgaacgaccgagcgcagcgagtcagtgagcgaggaagcggaagagcgcctgatgcggtattttctccttacgcatctgtgcggtatttcacaccgcaatggtgcactctcagtacaatctgctctgatgccgcatagttaagccagtatacactccgctatcgctacgtgactgggtcatggctgcgccccgacacccgccaacacccgctgacgcgccctgacgggcttgtctgctcccggcatccgcttacagacaagctgtgaccgtctccgggagctgcatgtgtgatgcctccgtgtaagggggatttctgttcatgggggtaatgataccgatgaaacgagagaggatgctcacgatacgggttactgatgatgaacatgcccggttactggaacgttgtgagggtaaacaactggcggtatggatgcggcgggaccagagaaaaatcactcagggtcaatgccagcgcttcgttaatacagatgtaggtgttccacagggtagccagcagcatcctgcgatgcagatccggaacataatggtgcagggcgctgacttccgcgtttccagactttacgaaacacggaaaccgaagaccattcatgttgttgctcaggtcgcagacgttttgcagcagcagtcgcttcacgttcgctcgcgtatcggtgattcattctgctaaccagtaaggcaaccccgccagcctagccgggtcctcaacgacaggagcacgatcatgcgcacccgtggggccgccatgccggcgataatggcctgcttctcgccgaaacgtttggtggcgggaccagtgacgaaggcttgagcgagggcgtgcaagattccgaataccgcaagcgacaggccgatcatcgtcgcgctccagcgaaagcggtcctcgccgaaaatgacccagagcgctgccggcacctgtcctacgagttgcatgataaagaagacagtcataagtgcggcgacgatagtcatgccccgcgcccaccggaaggagctgactgggttgaaggctctcaagggcatcggtcgagatcccggtgcctaatgagtgagctaacttacattaattgcgttgcgctcactgcccgctttccagtcgggaaacctgtcgtgccagctgcattaatgaatcggccaacgcgcggggagaggcggtttgcgtattgggcgccagggtggtttttcttttcaccagtgagacgggcaacagctgattgcccttcaccgcctggccctgagagagttgcagcaagcggtccacgctggtttgccccagcaggcgaaaatcctgtttgatggtggttaacggcgggatataacatgagctgtcttcggtatcgtcgtatcccactaccgagatatccgcaccaacgcgcagcccggactcggtaatggcgcgcattgcgcccagcgccatctgatcgttggcaaccagcatcgcagtgggaacgatgccctcattcagcatttgcatggtttgttgaaaaccggacatggcactccagtcgccttcccgttccgctatcggctgaatttgattgcgagtgagatatttatgccagccagccagacgcagacgcgccgagacagaacttaatgggcccgctaacagcgcgatttgctggtgacccaatgcgaccagatgctccacgcccagtcgcgtaccgtcttcatgggagaaaataatactgttgatgggtgtctggtcagagacatcaagaaataacgccggaacattagtgcaggcagcttccacagcaatggcatcctggtcatccagcggatagttaatgatcagcccactgacgcgttgcgcgagaagattgtgcaccgccgctttacaggcttcgacgccgcttcgttctaccatcgacaccaccacgctggcacccagttgatcggcgcgagatttaatcgccgcgacaatttgcgacggcgcgtgcagggccagactggaggtggcaacgccaatcagcaacgactgtttgcccgccagttgttgtgccacgcggttgggaatgtaattcagctccgccatcgccgcttccactttttcccgcgttttcgcagaaacgtggctggcctggttcaccacgcgggaaacggtctgataagagacaccggcatactctgcgacatcgtataacgttactggtttcacattcaccaccctgaattgactctcttccgggcgctatcatgccataccgcgaaaggttttgcgccattcgatggtgtccgggatctcgacgctctcccttatgcgactcctgcattaggaagcagcccagtagtaggttgaggccgttgagcaccgccgccgcaaggaatggtgcatgcaaggagatggcgcccaacagtcccccggccacggggcctgccaccatacccacgccgaaacaagcgctcatgagcccgaagtggcgagcccgatcttccccatcggtgatgtcggcgatataggcgccagcaaccgcacctgtggcgccggtgatgccggccacgatgcgtccggcgtagaggatcgagatctcgatcccgcgaaattaatacgactcactataggggaattgtgagcggataacaattcccctctagaaataattttgtttaactttaagaaggagatatacatatgaaatacctgctgccgaccgctgctgctggtctgctgctcctcgctgcccagccggcgatggccgaagcactggcagcacatcgtgtttgcggagttccactggaaacgctggcacgtagccgtaaaccgcgtgatcttccggatgatctgtcatgcgcctatcaggcacagaacatcgttagcctgtttgtggcaacacgcatcttgttcagccatctggatagcgtgtttacgctgaacctggatgaacaagaaccggaagtggcagaacgccttagcgcactgagacagatcaacgagaacaatccgggcatggtgacacaggtgctgaccgttgcacgccagatttacaacgattacgtgacgcatcatccgggcttaactccggaacagactagcgcgggtgcacaagccgcagatatcttgagcctgttttgtccggatgcagataaaccgtgcgttgcgagcaacaacgatcaggcgaacatcaacatcgagtcacgtagcggacgcagctatctgccggagaatcgcgccgtgattacgcctcagggtgtgaccaactggacctatcaagaactggaagcaacgcatcaggcactgacacgcgaaggttatgtgtttgttggctatcatggcaccaaccatgttgcggcacagaccattgtgaaccgcattgcaccggttccacgtggtaacaacaccgaaaacgaagagaaatggggcggtctgtatgttgccacgcacgcagaagttgctcatggctatgcacgcatcaaagaaggtacgggcgaatatggcttaccgacgcgtgcagaacgtgatgccagaggcgttatgctgcgtgtgtacattccgagagcgagcttagaacgcttctatcgcaccaacacaccgctggaaaacgcggaagaacacattactcaggtgattggccatagcctgccgttacgcaacgaagcctttaccggtccggaaagcgcaggtggtgaagatgaaaccgtgattggctgggatatggcgattcatgccgttgccataccgagcaccataccgggcaatgcgtatgaagagctggcaattgacgaagaagcagttgccaaagaacagagcattagcaccaaaccgccgtataaagagcgcaaagacgaactgaagtacccctatgacgtgcctgattacgccggctctggccaccaccaccaccaccactgagatccggctgctaacaaagcccgaaaggaagctgagttggctgctgccaccgctgagcaataactagcataaccccttggggcctctaaacgggtcttgaggggttttttgctgaaaggaggaactatatccggat

SEQ ID NO: 98 - DNA, 6304 bp, synthetic construct
  source 1..6304: mol_type = other DNA
tggcgaatgggacgcgccctgtagcggcgcattaagcgcggcgggtgtggtggttacgcgcagcgtgaccgctacacttgccagcgccctagcgcccgctcctttcgctttcttcccttcctttctcgccacgttcgccggctttccccgtcaagctctaaatcgggggctccctttagggttccgatttagtgctttacggcacctcgaccccaaaaaacttgattagggtgatggttcacgtagtgggccatcgccctgatagacggtttttcgccctttgacgttggagtccacgttctttaatagtggactcttgttccaaactggaacaacactcaaccctatctcggtctattcttttgatttataagggattttgccgatttcggcctattggttaaaaaatgagctgatttaacaaaaatttaacgcgaattttaacaaaatattaacgcttacaatttaggtggcacttttcggggaaatgtgcgcggaacccctatttgtttatttttctaaatacattcaaatatgtatccgctcatgaattaattcttagaaaaactcatcgagcatcaaatgaaactgcaatttattcatatcaggattatcaataccatatttttgaaaaagccgtttctgtaatgaaggagaaaactcaccgaggcagttccataggatggcaagatcctggtatcggtctgcgattccgactcgtccaacatcaatacaacctattaatttcccctcgtcaaaaataaggttatcaagtgagaaatcaccatgagtgacgactgaatccggtgagaatggcaaaagtttatgcatttctttccagacttgttcaacaggccagccattacgctcgtcatcaaaatcactcgcatcaaccaaaccgttattcattcgtgattgcgcctgagcgagacgaaatacgcgatcgctgttaaaaggacaattacaaacaggaatcgaatgcaaccggcgcaggaacactgccagcgcatcaacaatattttcacctgaatcaggatattcttctaatacctggaatgctgttttcccggggatcgcagtggtgagtaaccatgcatcatcaggagtacggataaaatgcttgatggtcggaagaggcataaattccgtcagccagtttagtctgaccatctcatctgtaacatcattggcaacgctacctttgccatgtttcagaaacaactctggcgcatcgggcttcccatacaatcgatagattgtcgcacctgattgcccgacattatcgcgagcccatttatacccatataaatcagcatccatgttggaatttaatcgcggcctagagcaagacgtttcccgttgaatatggctcataacaccccttgtattactgtttatgtaagcagacagttttattgttcatgaccaaaatcccttaacgtgagttttcgttccactgagcgtcagaccccgtagaaaagatcaaaggatcttcttgagatcctttttttctgcgcgtaatctgctgcttgcaaacaaaaaaaccaccgctaccagcggtggtttgtttgccggatcaagagctaccaactctttttccgaaggtaactggcttcagcagagcgcagataccaaatactgtccttctagtgtagccgtagttaggccaccacttcaagaactctgtagcaccgcctacatacctcgctctgctaatcctgttaccagtggctgctgccagtggcgataagtcgtgtcttaccgggttggactcaagacgatagttaccggataaggcgcagcggtcgggctgaacggggggttcgtgcacacagcccagcttggagcgaacgacctacaccgaactgagatacctacagcgtgagctatgagaaagcgccacgcttcccgaagggagaaaggcggacaggtatccggtaagcggcagggtcggaacaggagagcgcacgagggagcttccagggggaaacgcctggtatctttatagtcctgtcgggtttcgccacctctgacttgagcgtcgatttttgtgatgctcgtcaggggggcggagcctatggaaaaacgccagcaacgcggcctttttacggttcctggccttttgctggccttttgctcacatgttctttcctgcgttatcccctgattctgtggataaccgtattaccgcctttgagtgagctgataccgctcgccgcagccgaacgaccgagcgcagcgagtcagtgagcgaggaagcggaagagcgcctgatgcggtattttctccttacgcatctgtgcggtatttcacaccgcaatggtgcactctcagtacaatctgctctgatgccgcatagttaagccagtatacactccgctatcgctacgtgactgggtcatggctgcgccccgacacccgccaacacccgctgacgcgccctgacgggcttgtctgctcccggcatccgcttacagacaagctgtgaccgtctccgggagctgcatgtgtgatgcctccgtgtaagggggatttctgttcatgggggtaatgataccgatgaaacgagagaggatgctcacgatacgggttactgatgatgaacatgcccggttactggaacgttgtgagggtaaacaactggcggtatggatgcggcgggaccagagaaaaatcactcagggtcaatgccagcgcttcgttaatacagatgtaggtgttccacagggtagccagcagcatcctgcgatgcagatccggaacataatggtgcagggcgctgacttccgcgtttccagactttacgaaacacggaaaccgaagaccattcatgttgttgctcaggtcgcagacgttttgcagcagcagtcgcttcacgttcgctcgcgtatcggtgattcattctgctaaccagtaaggcaaccccgccagcctagccgggtcctcaacgacaggagcacgatcatgcgcacccgtggggccgccatgccggcgataatggcctgcttctcgccgaaacgtttggtggcgggaccagtgacgaaggcttgagcgagggcgtgcaagattccgaataccgcaagcgacaggccgatcatcgtcgcgctccagcgaaagcggtcctcgccgaaaatgacccagagcgctgccggcacctgtcctacgagttgcatgataaagaagacagtcataagtgcggcgacgatagtcatgccccgcgcccaccggaaggagctgactgggttgaaggctctcaagggcatcggtcgagatcccggtgcctaatgagtgagctaacttacattaattgcgttgcgctcactgcccgctttccagtcgggaaacctgtcgtgccagctgcattaatgaatcggccaacgcgcggggagaggcggtttgcgtattgggcgccagggtggtttttcttttcaccagtgagacgggcaacagctgattgcccttcaccgcctggccctgagagagttgcagcaagcggtccacgctggtttgccccagcaggcgaaaatcctgtttgatggtggttaacggcgggatataacatgagctgtcttcggtatcgtcgtatcccactaccgagatatccgcaccaacgcgcagcccggactcggtaatggcgcgcattgcgcccagcgccatctgatcgttggcaaccagcatcgcagtgggaacgatgccctcattcagcatttgcatggtttgttgaaaaccggacatggcactccagtcgccttcccgttccgctatcggctgaatttgattgcgagtgagatatttatgccagccagccagacgcagacgcgccgagacagaacttaatgggcccgctaacagcgcgatttgctggtgacccaatgcgaccagatgctccacgcccagtcgcgtaccgtcttcatgggagaaaataatactgttgatgggtgtctggtcagagacatcaagaaataacgccggaacattagtgcaggcagcttccacagcaatggcatcctggtcatccagcggatagttaatgatcagcccactgacgcgttgcgcgagaagattgtgcaccgccgctttacaggcttcgacgccgcttcgttctaccatcgacaccaccacgctggcacccagttgatcggcgcgagatttaatcgccgcgacaatttgcgacggcgcgtgcagggccagactggaggtggcaacgccaatcagcaacgactgtttgcccgccagttgttgtgccacgcggttgggaatgtaattcagctccgccatcgccgcttccactttttcccgcgttttcgcagaaacgtggctggcctggttcaccacgcgggaaacggtctgataagagacaccggcatactctgcgacatcgtataacgttactggtttcacattcaccaccctgaattgactctcttccgggcgctatcatgccataccgcgaaaggttttgcgccattcgatggtgtccgggatctcgacgctctcccttatgcgactcctgcattaggaagcagcccagtagtaggttgaggccgttgagcaccgccgccgcaaggaatggtgcatgcaaggagatggcgcccaacagtcccccggccacggggcctgccaccatacccacgccgaaacaagcgctcatgagcccgaagtggcgagcccgatcttccccatcggtgatgtcggcgatataggcgccagcaaccgcacctgtggcgccggtgatgccggccacgatgcgtccggcgtagaggatcgagatctcgatcccgcgaaattaatacgactcactataggggaattgtgagcggataacaattcccctctagaaataattttgtttaactttaagaaggagatatacatatgaaatacctgctgccgaccgctgctgctggtctgctgctcctcgctgcccagccggcgatggccggcgcggatgatgtcgtggattcaagcaaatcatttgtcatggagaacttcagcagctatcacggcaccaaacctggctatgtggattcgattcagaaaggcattcagaaaccgaaatccggtacgcagggcaactatgacgatgattggaaaggcttctacagcaccgataacaagtacgatgcggcgggttactccgtggataatgagaatccactgagcggtaaagctggcggtgtggtgaaagtcacctatccgggcctgacgaaagtgctggcactgaaggtggataatgccgaaaccattaagaaagaactgggcctgagcctgaccgaacctctgatggaacaggttggcacagaagagtttatcaaacgctttggcgatggtgcgtcaagagttgtgctgagccttccgtttgccgaaggtagcagcagcgttgagtacatcaacaattgggaacaggccaaagcactgtcagtggaactggaaatcaactttgagacacgtggtaagagaggccaagatgccatgtacgagtacatggcgcaagcgtgcgcaggcaaccgcgttcgtagaagcgttggcagcagcctgagctgcatcaacctggactgggatgtgattcgcgataagaccaagacgaagatcgaaagcctgaaagaacacggaccaatcaagaacaagatgagcgaaagtccgaacaagacggtgagcgaagagaaagcgaaacagtatctggaagagtttcaccagaccgcactggaacatccggaactgagcgagcttaagaccgtgacgggcacaaatccggtgtttgcaggcgcaaactatgcggcatgggcggtgaacgtggcacaggtcattgacagcgaaactgcggataatctggagaaaacgaccgctgcactgagcatactgccgggaattggcagcgtaatgggcatcgcggatggtgctgttcaccacaacaccgaagagattgttgcgcagagcatcgcactgagcagcctgatggtggcacaagcgattccgctggtgggcgaattggtcgatatcggctttgcggcctataacttcgtcgaaagcattatcaacctgtttcaggtggttcacaacagctacaatcgtccggcctatagtccgggacacaagacgcagccgtttctgtacccctatgacgtgcctgattacgccggctctggccaccaccaccaccaccactgagatccggctgctaacaaagcccgaaaggaagctgagttggctgctgccaccgctgagcaataactagcataaccccttggggcctctaaacgggtcttgaggggttttttgctgaaaggaggaactatatccggat

SEQ ID NO: 99 - DNA, 6505 bp, synthetic construct
  source 1..6505: mol_type = other DNA
tggcgaatgggacgcgccctgtagcggcgcattaagcgcggcgggtgtggtggttacgcgcagcgtgaccgctacacttgccagcgccctagcgcccgctcctttcgctttcttcccttcctttctcgccacgttcgccggctttccccgtcaagctctaaatcgggggctccctttagggttccgatttagtgctttacggcacctcgaccccaaaaaacttgattagggtgatggttcacgtagtgggccatcgccctgatagacggtttttcgccctttgacgttggagtccacgttctttaatagtggactcttgttccaaactggaacaacactcaaccctatctcggtctattcttttgatttataagggattttgccgatttcggcctattggttaaaaaatgagctgatttaacaaaaatttaacgcgaattttaacaaaatattaacgcttacaatttaggtggcacttttcggggaaatgtgcgcggaacccctatttgtttatttttctaaatacattcaaatatgtatccgctcatgaattaattcttagaaaaactcatcgagcatcaaatgaaactgcaatttattcatatcaggattatcaataccatatttttgaaaaagccgtttctgtaatgaaggagaaaactcaccgaggcagttccataggatggcaagatcctggtatcggtctgcgattccgactcgtccaacatcaatacaacctattaatttcccctcgtcaaaaataaggttatcaagtgagaaatcaccatgagtgacgactgaatccggtgagaatggcaaaagtttatgcatttctttccagacttgttcaacaggccagccattacgctcgtcatcaaaatcactcgcatcaaccaaaccgttattcattcgtgattgcgcctgagcgagacgaaatacgcgatcgctgttaaaaggacaattacaaacaggaatcgaatgcaaccggcgcaggaacactgccagcgcatcaacaatattttcacctgaatcaggatattcttctaatacctggaatgctgttttcccggggatcgcagtggtgagtaaccatgcatcatcaggagtacggataaaatgcttgatggtcggaagaggcataaattccgtcagccagtttagtctgaccatctcatctgtaacatcattggcaacgctacctttgccatgtttcagaaacaactctggcgcatcgggcttcccatacaatcgatagattgtcgcacctgattgcccgacattatcgcgagcccatttatacccatataaatcagcatccatgttggaatttaatcgcggcctagagcaagacgtttcccgttgaatatggctcataacaccccttgtattactgtttatgtaagcagacagttttattgttcatgaccaaaatcccttaacgtgagttttcgttccactgagcgtcagaccccgtagaaaagatcaaaggatcttcttgagatcctttttttctgcgcgtaatctgctgcttgcaaacaaaaaaaccaccgctaccagcggtggtttgtttgccggatcaagagctaccaactctttttccgaaggtaactggcttcagcagagcgcagataccaaatactgtccttctagtgtagccgtagttaggccaccacttcaagaactctgtagcaccgcctacatacctcgctctgctaatcctgttaccagtggctgctgccagtggcgataagtcgtgtcttaccgggttggactcaagacgatagttaccggataaggcgcagcggtcgggctgaacggggggttcgtgcacacagcccagcttggagcgaacgacctacaccgaactgagatacctacagcgtgagctatgagaaagcgccacgcttcccgaagggagaaaggcggacaggtatccggtaagcggcagggtcggaacaggagagcgcacgagggagcttccagggggaaacgcctggtatctttatagtcctgtcgggtttcgccacctctgacttgagcgtcgatttttgtgatgctcgtcaggggggcggagcctatggaaaaacgccagcaacgcggcctttttacggttcctggccttttgctggccttttgctcacatgttctttcctgcgttatcccctgattctgtggataaccgtattaccgcctttgagtgagctgataccgctcgccgcagccgaacgaccgagcgcagcgagtcagtgagcgaggaagcggaagagcgcctgatgcggtattttctccttacgcatctgtgcggtatttcacaccgcaatggtgcactctcagtacaatctgctctgatgccgcatagttaagccagtatacactccgctatcgctacgtgactgggtcatggctgcgccccgacacccgccaacacccgctgacgcgccctgacgggcttgtctgctcccggcatccgcttacagacaagctgtgaccgtctccgggagctgcatgtgtgatgcctccgtgtaagggggatttctgttcatgggggtaatgataccgatgaaacgagagaggatgctcacgatacgggttactgatgatgaacatgcccggttactggaacgttgtgagggtaaacaactggcggtatggatgcggcgggaccagagaaaaatcactcagggtcaatgccagcgcttcgttaatacagatgtaggtgttccacagggtagccagcagcatcctgcgatgcagatccggaacataatggtgcagggcgctgacttccgcgtttccagactttacgaaacacggaaaccgaagaccattcatgttgttgctcaggtcgcagacgttttgcagcagcagtcgcttcacgttcgctcgcgtatcggtgattcattctgctaaccagtaaggcaaccccgccagcctagccgggtcctcaacgacaggagcacgatcatgcgcacccgtggggccgccatgccggcgataatggcctgcttctcgccgaaacgtttggtggcgggaccagtgacgaaggcttgagcgagggcgtgcaagattccgaataccgcaagcgacaggccgatcatcgtcgcgctccagcgaaagcggtcctcgccgaaaatgacccagagcgctgccggcacctgtcctacgagttgcatgataaagaagacagtcataagtgcggcgacgatagtcatgccccgcgcccaccggaaggagctgactgggttgaaggctctcaagggcatcggtcgagatcccggtgcctaatgagtgagctaacttacattaattgcgttgcgctcactgcccgctttccagtcgggaaacctgtcgtgccagctgcattaatgaatcggccaacgcgcggggagaggcggtttgcgtattgggcgccagggtggtttttcttttcaccagtgagacgggcaacagctgattgcccttcaccgcctggccctgagagagttgcagcaagcggtccacgctggtttgccccagcaggcgaaaatcctgtttgatggtggttaacggcgggatataacatgagctgtcttcggtatcgtcgtatcccactaccgagatatccgcaccaacgcgcagcccggactcggtaatggcgcgcattgcgcccagcgccatctgatcgttggcaaccagcatcgcagtgggaacgatgccctcattcagcatttgcatggtttgttgaaaaccggacatggcactccagtcgccttcccgttccgctatcggctgaatttgattgcgagtgagatatttatgccagccagccagacgcagacgcgccgagacagaacttaatgggcccgctaacagcgcgatttgctggtgacccaatgcgaccagatgctccacgcccagtcgcgtaccgtcttcatgggagaaaataatactgttgatgggtgtctggtcagagacatcaagaaataacgccggaacattagtgcaggcagcttccacagcaatggcatcctggtcatccagcggatagttaatgatcagcccactgacgcgttgcgcgagaagattgtgcaccgccgctttacaggcttcgacgccgcttcgttctaccatcgacaccaccacgctggcacccagttgatcggcgcgagatttaatcgccgcgacaatttgcgacggcgcgtgcagggccagactggaggtggcaacgccaatcagcaacgactgtttgcccgccagttgttgtgccacgcggttgggaatgtaattcagctccgccatcgccgcttccactttttcccgcgttttcgcagaaacgtggctggcctggttcaccacgcgggaaacggtctgataagagacaccggcatactctgcgacatcgtataacgttactggtttcacattcaccaccctgaattgactctcttccgggcgctatcatgccataccgcgaaaggttttgcgccattcgatggtgtccgggatctcgacgctctcccttatgcgactcctgcattaggaagcagcccagtagtaggttgaggccgttgagcaccgccgccgcaaggaatggtgcatgcaaggagatggcgcccaacagtcccccggccacggggcctgccaccatacccacgccgaaacaagcgctcatgagcccgaagtggcgagcccgatcttccccatcggtgatgtcggcgatataggcgccagcaaccgcacctgtggcgccggtgatgccggccacgatgcgtccggcgtagaggatcgagatctcgatcccgcgaaattaatacgactcactataggggaattgtgagcggataacaattcccctctagaaataattttgtttaactttaagaaggagatatacatatgaaatacctgctgccgaccgctgctgctggtctgctgctcctcgctgcccagccggcgatggccgaagtgcaactggtggaaagcggtggaggccttgttcagaccggcggcagcctgcgtctgtcatgcgctgcaagcggctttacgttcagcagctacgcgatgagctgggtgcgccaggcaccgggcaaaggcttggaatgggttagcggcatcaagtcaagcggcgatagcaccagatatgccggaagcgttaaaggccgctttaccatttcacgcgataacgccaagaacatgctgtatctgcaaatgtatagcctgaaaccggaagataccgcagtgtattactgcgccaagagccgcgtgagtcgcacgggtctgtatacctatgacaaccgtggtcagggcacgcaggtgactgtgtcaagccctgaaggtggtagcctggcggcactgaccgcacaccaagcatgtcatctgccactggaaacctttacccgtcatcgtcagccgcgtggctgggaacaactggaacaatgtggatatccggtgcagagactggtcgcattatatctggcagcacgtctgagttggaatcaggttgatcaagttattcgtaacgcacttgcctcaccgggtagcggtggtgatttaggtgaggcaattcgtgaacaacctgaacaggcacgcttagcattaacccttgcagccgcagaaagtgaaagatttgtgcgtcagggtactggtaatgatgaggccggtgcagcaaatgggccggcagacagcggagatgcattattagagagaaattatcctaccggcgcagaatttctgggtgatgggggtgatgttagtttttcaacacgcgggacacagaattggaccgtggaacgtttactgcaggcacatcgtcagctggaagaacgcggttatgtttttgttggttatcatgggacgtttctggaggcagcacagagcattgtctttggcggtgtgcgggcgcgtagccaggatcttgatgcaatttggcgtggtttttatattgcgggtgatcctgcgctggcgtatggatatgcgcaggatcaggagccggatgcgcgtggtcgtattcgtaatggtgccctgctgcgggtttatgttccgcgtagctcactgccggggttttatagaacaagcttaacactggctgcgccggaagcagcaggtgaagttgaacgtctgattggccatccgctgccgttacgtttagatgcaattactggtccggaagaagaaggtggtcgcctggaaaccattctgggttggccgctggcagaaagaaccgtggttataccttccgcaataccgaccgatcctcggaatgtggggggtgatttagatcctagcagcattcctgataaagaacaggcaatttctgctctgcctgattatgcatcacagccgggtaaaccgccgcgtgaagatttaaagcatcatcaccatcatcattaagatccggctgctaacaaagcccgaaaggaagctgagttggctgctgccaccgctgagcaataactagcataaccccttggggcctctaaacgggtcttgaggggttttttgctgaaaggaggaactatatccggat

SEQ ID NO: 100 - DNA, 6523 bp, synthetic construct
  source 1..6523: mol_type = other DNA
tggcgaatgggacgcgccctgtagcggcgcattaagcgcggcgggtgtggtggttacgcgcagcgtgaccgctacacttgccagcgccctagcgcccgctcctttcgctttcttcccttcctttctcgccacgttcgccggctttccccgtcaagctctaaatcgggggctccctttagggttccgatttagtgctttacggcacctcgaccccaaaaaacttgattagggtgatggttcacgtagtgggccatcgccctgatagacggtttttcgccctttgacgttggagtccacgttctttaatagtggactcttgttccaaactggaacaacactcaaccctatctcggtctattcttttgatttataagggattttgccgatttcggcctattggttaaaaaatgagctgatttaacaaaaatttaacgcgaattttaacaaaatattaacgcttacaatttaggtggcacttttcggggaaatgtgcgcggaacccctatttgtttatttttctaaatacattcaaatatgtatccgctcatgaattaattcttagaaaaactcatcgagcatcaaatgaaactgcaatttattcatatcaggattatcaataccatatttttgaaaaagccgtttctgtaatgaaggagaaaactcaccgaggcagttccataggatggcaagatcctggtatcggtctgcgattccgactcgtccaacatcaatacaacctattaatttcccctcgtcaaaaataaggttatcaagtgagaaatcaccatgagtgacgactgaatccggtgagaatggcaaaagtttatgcatttctttccagacttgttcaacaggccagccattacgctcgtcatcaaaatcactcgcatcaaccaaaccgttattcattcgtgattgcgcctgagcgagacgaaatacgcgatcgctgttaaaaggacaattacaaacaggaatcgaatgcaaccggcgcaggaacactgccagcgcatcaacaatattttcacctgaatcaggatattcttctaatacctggaatgctgttttcccggggatcgcagtggtgagtaaccatgcatcatcaggagtacggataaaatgcttgatggtcggaagaggcataaattccgtcagccagtttagtctgaccatctcatctgtaacatcattggcaacgctacctttgccatgtttcagaaacaactctggcgcatcgggcttcccatacaatcgatagattgtcgcacctgattgcccgacattatcgcgagcccatttatacccatataaatcagcatccatgttggaatttaatcgcggcctagagcaagacgtttcccgttgaatatggctcataacaccccttgtattactgtttatgtaagcagacagttttattgttcatgaccaaaatcccttaacgtgagttttcgttccactgagcgtcagaccccgtagaaaagatcaaaggatcttcttgagatcctttttttctgcgcgtaatctgctgcttgcaaacaaaaaaaccaccgctaccagcggtggtttgtttgccggatcaagagctaccaactctttttccgaaggtaactggcttcagcagagcgcagataccaaatactgtccttctagtgtagccgtagttaggccaccacttcaagaactctgtagcaccgcctacatacctcgctctgctaatcctgttaccagtggctgctgccagtggcgataagtcgtgtcttaccgggttggactcaagacgatagttaccggataaggcgcagcggtcgggctgaacggggggttcgtgcacacagcccagcttggagcgaacgacctacaccgaactgagatacctacagcgtgagctatgagaaagcgccacgcttcccgaagggagaaaggcggacaggtatccggtaagcggcagggtcggaacaggagagcgcacgagggagcttccagggggaaacgcctggtatctttatagtcctgtcgggtttcgccacctctgacttgagcgtcgatttttgtgatgctcgtcaggggggcggagcctatggaaaaacgccagcaacgcggcctttttacggttcctggccttttgctggccttttgctcacatgttctttcctgcgttatcccctgattctgtggataaccgtattaccgcctttgagtgagctgataccgctcgccgcagccgaacgaccgagcgcagcgagtcagtgagcgaggaagcggaagagcgcctgatgcggtattttctccttacgcatctgtgcggtatttcacaccgcaatggtgcactctcagtacaatctgctctgatgccgcatagttaagccagtatacactccgctatcgctacgtgactgggtcatggctgcgccccgacacccgccaacacccgctgacgcgccctgacgggcttgtctgctcccggcatccgcttacagacaagctgtgaccgtctccgggagctgcatgtgtgatgcctccgtgtaagggggatttctgttcatgggggtaatgataccgatgaaacgagagaggatgctcacgatacgggttactgatgatgaacatgcccggttactggaacgttgtgagggtaaacaactggcggtatggatgcggcgggaccagagaaaaatcactcagggtcaatgccagcgcttcgttaatacagatgtaggtgttccacagggtagccagcagcatcctgcgatgcagatccggaacataatggtgcagggcgctgacttccgcgtttccagactttacgaaacacggaaaccgaagaccattcatgttgttgctcaggtcgcagacgttttgcagcagcagtcgcttcacgttcgctcgcgtatcggtgattcattctgctaaccagtaaggcaaccccgccagcctagccgggtcctcaacgacaggagcacgatcatgcgcacccgtggggccgccatgccggcgataatggcctgcttctcgccgaaacgtttggtggcgggaccagtgacgaaggcttgagcgagggcgtgcaagattccgaataccgcaagcgacaggccgatcatcgtcgcgctccagcgaaagcggtcctcgccgaaaatgacccagagcgctgccggcacctgtcctacgagttgcatgataaagaagacagtcataagtgcggcgacgatagtcatgccccgcgcccaccggaaggagctgactgggttgaaggctctcaagggcatcggtcgagatcccggtgcctaatgagtgagctaacttacattaattgcgttgcgctcactgcccgctttccagtcgggaaacctgtcgtgccagctgcattaatgaatcggccaacgcgcggggagaggcggtttgcgtattgggcgccagggtggtttttcttttcaccagtgagacgggcaacagctgattgcccttcaccgcctggccctgagagagttgcagcaagcggtccacgctggtttgccccagcaggcgaaaatcctgtttgatggtggttaacggcgggatataacatgagctgtcttcggtatcgtcgtatcccactaccgagatatccgcaccaacgcgcagcccggactcggtaatggcgcgcattgcgcccagcgccatctgatcgttggcaaccagcatcgcagtgggaacgatgccctcattcagcatttgcatggtttgttgaaaaccggacatggcactccagtcgccttcccgttccgctatcggctgaatttgattgcgagtgagatatttatgccagccagccagacgcagacgcgccgagacagaacttaatgggcccgctaacagcgcgatttgctggtgacccaatgcgaccagatgctccacgcccagtcgcgtaccgtcttcatgggagaaaataatactgttgatgggtgtctggtcagagacatcaagaaataacgccggaacattagtgcaggcagcttccacagcaatggcatcctggtcatccagcggatagttaatgatcagcccactgacgcgttgcgcgagaagattgtgcaccgccgctttacaggcttcgacgccgcttcgttctaccatcgacaccaccacgctggcacccagttgatcggcgcgagatttaatcgccgcgacaatttgcgacggcgcgtgcagggccagactggaggtggcaacgccaatcagcaacgactgtttgcccgccagttgttgtgccacgcggttgggaatgtaattcagctccgccatcgccgcttccactttttcccgcgttttcgcagaaacgtggctggcctggttcaccacgcgggaaacggtctgataagagacaccggcatactctgcgacatcgtataacgttactggtttcacattcaccaccctgaattgactctcttccgggcgctatcatgccataccgcgaaaggttttgcgccattcgatggtgtccgggatctcgacgctctcccttatgcgactcctgcattaggaagcagcccagtagtaggttgaggccgttgagcaccgccgccgcaaggaatggtgcatgcaaggagatggcgcccaacagtcccccggccacggggcctgccaccatacccacgccgaaacaagcgctcatgagcccgaagtggcgagcccgatcttccccatcggtgatgtcggcgatataggcgccagcaaccgcacctgtggcgccggtgatgccggccacgatgcgtccggcgtagaggatcgagatctcgatcccgcgaaattaatacgactcactataggggaattgtgagcggataacaattcccctctagaaataattttgtttaactttaagaaggagatatacatatgaaatacctgctgccgaccgctgctgctggtctgctgctcctcgctgcccagccggcgatggccgaagtccagctggttgaaagcggtggaggcctggttcagaccggcggaagcctgcgtctgagctgtgcagcctctggccgcacgtttaacaactacgcgatgggctggtttcgccgtgcaccgggcaaagaacgcgaatttgtggcggcaatcactcgtagcggtgtgagaagcggagtgtcagcgatctatggcgatagcgtgaaagatcgcttcaccatcagccgcgataacgccaagaacaccttgtacttgcagatgaacagcctgaaaccggaagatactgcggtgtatacctgcgccgcaagtgcgatcggcagcggtgcactgcgtcgtttcgaatacgactatagcggtcagggcacacaggtgaccgtgagcagccctgaaggtggtagcctggcggcactgaccgcacaccaagcatgtcatctgccactggaaacctttacccgtcatcgtcagccgcgtggctgggaacaactggaacaatgtggatatccggtgcagagactggtcgcattatatctggcagcacgtctgagttggaatcaggttgatcaagttattcgtaacgcacttgcctcaccgggtagcggtggtgatttaggtgaggcaattcgtgaacaacctgaacaggcacgcttagcattaacccttgcagccgcagaaagtgaaagatttgtgcgtcagggtactggtaatgatgaggccggtgcagcaaatgggccggcagacagcggagatgcattattagagagaaattatcctaccggcgcagaatttctgggtgatgggggtgatgttagtttttcaacacgcgggacacagaattggaccgtggaacgtttactgcaggcacatcgtcagctggaagaacgcggttatgtttttgttggttatcatgggacgtttctggaggcagcacagagcattgtctttggcggtgtgcgggcgcgtagccaggatcttgatgcaatttggcgtggtttttatattgcgggtgatcctgcgctggcgtatggatatgcgcaggatcaggagccggatgcgcgtggtcgtattcgtaatggtgccctgctgcgggtttatgttccgcgtagctcactgccggggttttatagaacaagcttaacactggctgcgccggaagcagcaggtgaagttgaacgtctgattggccatccgctgccgttacgtttagatgcaattactggtccggaagaagaaggtggtcgcctggaaaccattctgggttggccgctggcagaaagaaccgtggttataccttccgcaataccgaccgatcctcggaatgtggggggtgatttagatcctagcagcattcctgataaagaacaggcaatttctgctctgcctgattatgcatcacagccgggtaaaccgccgcgtgaagatttaaagcatcatcaccatcatcattaagatccggctgctaacaaagcccgaaaggaagctgagttggctgctgccaccgctgagcaataactagcataaccccttggggcctctaaacgggtcttgaggggttttttgctgaaaggaggaactatatccggat

SEQ ID NO: 101 - DNA, 6538 bp, synthetic construct
  source 1..6538: mol_type = other DNA
tggcgaatgggacgcgccctgtagcggcgcattaagcgcggcgggtgtggtggttacgcgcagcgtgaccgctacacttgccagcgccctagcgcccgctcctttcgctttcttcccttcctttctcgccacgttcgccggctttccccgtcaagctctaaatcgggggctccctttagggttccgatttagtgctttacggcacctcgaccccaaaaaacttgattagggtgatggttcacgtagtgggccatcgccctgatagacggtttttcgccctttgacgttggagtccacgttctttaatagtggactcttgttccaaactggaacaacactcaaccctatctcggtctattcttttgatttataagggattttgccgatttcggcctattggttaaaaaatgagctgatttaacaaaaatttaacgcgaattttaacaaaatattaacgcttacaatttaggtggcacttttcggggaaatgtgcgcggaacccctatttgtttatttttctaaatacattcaaatatgtatccgctcatgaattaattcttagaaaaactcatcgagcatcaaatgaaactgcaatttattcatatcaggattatcaataccatatttttgaaaaagccgtttctgtaatgaaggagaaaactcaccgaggcagttccataggatggcaagatcctggtatcggtctgcgattccgactcgtccaacatcaatacaacctattaatttcccctcgtcaaaaataaggttatcaagtgagaaatcaccatgagtgacgactgaatccggtgagaatggcaaaagtttatgcatttctttccagacttgttcaacaggccagccattacgctcgtcatcaaaatcactcgcatcaaccaaaccgttattcattcgtgattgcgcctgagcgagacgaaatacgcgatcgctgttaaaaggacaattacaaacaggaatcgaatgcaaccggcgcaggaacactgccagcgcatcaacaatattttcacctgaatcaggatattcttctaatacctggaatgctgttttcccggggatcgcagtggtgagtaaccatgcatcatcaggagtacggataaaatgcttgatggtcggaagaggcataaattccgtcagccagtttagtctgaccatctcatctgtaacatcattggcaacgctacctttgccatgtttcagaaacaactctggcgcatcgggcttcccatacaatcgatagattgtcgcacctgattgcccgacattatcgcgagcccatttatacccatataaatcagcatccatgttggaatttaatcgcggcctagagcaagacgtttcccgttgaatatggctcataacaccccttgtattactgtttatgtaagcagacagttttattgttcatgaccaaaatcccttaacgtgagttttcgttccactgagcgtcagaccccgtagaaaagatcaaaggatcttcttgagatcctttttttctgcgcgtaatctgctgcttgcaaacaaaaaaaccaccgctaccagcggtggtttgtttgccggatcaagagctaccaactctttttccgaaggtaactggcttcagcagagcgcagataccaaatactgtccttctagtgtagccgtagttaggccaccacttcaagaactctgtagcaccgcctacatacctcgctctgctaatcctgttaccagtggctgctgccagtggcgataagtcgtgtcttaccgggttggactcaagacgatagttaccggataaggcgcagcggtcgggctgaacggggggttcgtgcacacagcccagcttggagcgaacgacctacaccgaactgagatacctacagcgtgagctatgagaaagcgccacgcttcccgaagggagaaaggcggacaggtatccggtaagcggcagggtcggaacaggagagcgcacgagggagcttccagggggaaacgcctggtatctttatagtcctgtcgggtttcgccacctctgacttgagcgtcgatttttgtgatgctcgtcaggggggcggagcctatggaaaaacgccagcaacgcggcctttttacggttcctggccttttgctggccttttgctcacatgttctttcctgcgttatcccctgattctgtggataaccgtattaccgcctttgagtgagctgataccgctcgccgcagccgaacgaccgagcgcagcgagtcagtgagcgaggaagcggaagagcgcctgatgcggtattttctccttacgcatctgtgcggtatttcacaccgcaatggtgcactctcagtacaatctgctctgatgccgcatagttaagccagtatacactccgctatcgctacgtgactgggtcatggctgcgccccgacacccgccaacacccgctgacgcgccctgacgggcttgtctgctcccggcatccgcttacagacaagctgtgaccgtctccgggagctgcatgtgtgatgcctccgtgtaagggggatttctgttcatgggggtaatgataccgatgaaacgagagaggatgctcacgatacgggttactgatgatgaacatgcccggttactggaacgttgtgagggtaaacaactggcggtatggatgcggcgggaccagagaaaaatcactcagggtcaatgccagcgcttcgttaatacagatgtaggtgttccacagggtagccagcagcatcctgcgatgcagatccggaacataatggtgcagggcgctgacttccgcgtttccagactttacgaaacacggaaaccgaagaccattcatgttgttgctcaggtcgcagacgttttgcagcagcagtcgcttcacgttcgctcgcgtatcggtgattcattctgctaaccagtaaggcaaccccgccagcctagccgggtcctcaacgacaggagcacgatcatgcgcacccgtggggccgccatgccggcgataatggcctgcttctcgccgaaacgtttggtggcgggaccagtgacgaaggcttgagcgagggcgtgcaagattccgaataccgcaagcgacaggccgatcatcgtcgcgctccagcgaaagcggtcctcgccgaaaatgacccagagcgctgccggcacctgtcctacgagttgcatgataaagaagacagtcataagtgcggcgacgatagtcatgccccgcgcccaccggaaggagctgactgggttgaaggctctcaagggcatcggtcgagatcccggtgcctaatgagtgagctaacttacattaattgcgttgcgctcactgcccgctttccagtcgggaaacctgtcgtgccagctgcattaatgaatcggccaacgcgcggggagaggcggtttgcgtattgggcgccagggtggtttttcttttcaccagtgagacgggcaacagctgattgcccttcaccgcctggccctgagagagttgcagcaagcggtccacgctggtttgccccagcaggcgaaaatcctgtttgatggtggttaacggcgggatataacatgagctgtcttcggtatcgtcgtatcccactaccgagatatccgcaccaacgcgcagcccggactcggtaatggcgcgcattgcgcccagcgccatctgatcgttggcaaccagcatcgcagtgggaacgatgccctcattcagcatttgcatggtttgttgaaaaccggacatggcactccagtcgccttcccgttccgctatcggctgaatttgattgcgagtgagatatttatgccagccagccagacgcagacgcgccgagacagaacttaatgggcccgctaacagcgcgatttgctggtgacccaatgcgaccagatgctccacgcccagtcgcgtaccgtcttcatgggagaaaataatactgttgatgggtgtctggtcagagacatcaagaaataacgccggaacattagtgcaggcagcttccacagcaatggcatcctggtcatccagcggatagttaatgatcagcccactgacgcgttgcgcgagaagattgtgcaccgccgctttacaggcttcgacgccgcttcgttctaccatcgacaccaccacgctggcacccagttgatcggcgcgagatttaatcgccgcgacaatttgcgacggcgcgtgcagggccagactggaggtggcaacgccaatcagcaacgactgtttgcccgccagttgttgtgccacgcggttgggaatgtaattcagctccgccatcgccgcttccactttttcccgcgttttcgcagaaacgtggctggcctggttcaccacgcgggaaacggtctgataagagacaccggcatactctgcgacatcgtataacgttactggtttcacattcaccaccctgaattgactctcttccgggcgctatcatgccataccgcgaaaggttttgcgccattcgatggtgtccgggatctcgacgctctcccttatgcgactcctgcattaggaagcagcccagtagtaggttgaggccgttgagcaccgccgccgcaaggaatggtgcatgcaaggagatggcgcccaacagtcccccggccacggggcctgccaccatacccacgccgaaacaagcgctcatgagcccgaagtggcgagcccgatcttccccatcggtgatgtcggcgatataggcgccagcaaccgcacctgtggcgccggtgatgccggccacgatgcgtccggcgtagaggatcgagatctcgatcccgcgaaattaatacgactcactataggggaattgtgagcggataacaattcccctctagaaataattttgtttaactttaagaaggagatatacatatgaaatacctgctgccgaccgctgctgctggtctgctgctcctcgctgcccagccggcgatggcccaggttcagctgcaagaaagcggaggtggtctggttcagccgggaggtagcttacgcctgtcatgcgcagcaagcggtcgtacctttagcagctatgcgatgggctggtttcgtcaggcacctggcaaagaacgcgaatttgtggcggcaattcgctggtcaggcggctatacctactacaccgatagcgtgaaaggccgctttaccattagccgcgataacgccaagaccaccgtgtacctgcaaatgaacagcctgaaaccggaagataccgcagtgtactactgcgcagcgacctatctgagcagcgattatagccgctatgccttaccgcagcgtccgctggattacgactattggggccaaggtacgcaggttaccgttagcagcgcagcagcgcctgaaggtggtagcctggcggcactgaccgcacaccaagcatgtcatctgccactggaaacctttacccgtcatcgtcagccgcgtggctgggaacaactggaacaatgtggatatccggtgcagagactggtcgcattatatctggcagcacgtctgagttggaatcaggttgatcaagttattcgtaacgcacttgcctcaccgggtagcggtggtgatttaggtgaggcaattcgtgaacaacctgaacaggcacgcttagcattaacccttgcagccgcagaaagtgaaagatttgtgcgtcagggtactggtaatgatgaggccggtgcagcaaatgggccggcagacagcggagatgcattattagagagaaattatcctaccggcgcagaatttctgggtgatgggggtgatgttagtttttcaacacgcgggacacagaattggaccgtggaacgtttactgcaggcacatcgtcagctggaagaacgcggttatgtttttgttggttatcatgggacgtttctggaggcagcacagagcattgtctttggcggtgtgcgggcgcgtagccaggatcttgatgcaatttggcgtggtttttatattgcgggtgatcctgcgctggcgtatggatatgcgcaggatcaggagccggatgcgcgtggtcgtattcgtaatggtgccctgctgcgggtttatgttccgcgtagctcactgccggggttttatagaacaagcttaacactggctgcgccggaagcagcaggtgaagttgaacgtctgattggccatccgctgccgttacgtttagatgcaattactggtccggaagaagaaggtggtcgcctggaaaccattctgggttggccgctggcagaaagaaccgtggttataccttccgcaataccgaccgatcctcggaatgtggggggtgatttagatcctagcagcattcctgataaagaacaggcaatttctgctctgcctgattatgcatcacagccgggtaaaccgccgcgtgaagatttaaagcatcatcaccatcatcattaagatccggctgctaacaaagcccgaaaggaagctgagttggctgctgccaccgctgagcaataactagcataaccccttggggcctctaaacgggtcttgaggggttttttgctgaaaggaggaactatatccggat

SEQ ID NO: 102 - DNA, 6502 bp, synthetic construct
  source 1..6502: mol_type = other DNA
tggcgaatgggacgcgccctgtagcggcgcattaagcgcggcgggtgtggtggttacgcgcagcgtgaccgctacacttgccagcgccctagcgcccgctcctttcgctttcttcccttcctttctcgccacgttcgccggctttccccgtcaagctctaaatcgggggctccctttagggttccgatttagtgctttacggcacctcgaccccaaaaaacttgattagggtgatggttcacgtagtgggccatcgccctgatagacggtttttcgccctttgacgttggagtccacgttctttaatagtggactcttgttccaaactggaacaacactcaaccctatctcggtctattcttttgatttataagggattttgccgatttcggcctattggttaaaaaatgagctgatttaacaaaaatttaacgcgaattttaacaaaatattaacgcttacaatttaggtggcacttttcggggaaatgtgcgcggaacccctatttgtttatttttctaaatacattcaaatatgtatccgctcatgaattaattcttagaaaaactcatcgagcatcaaatgaaactgcaatttattcatatcaggattatcaataccatatttttgaaaaagccgtttctgtaatgaaggagaaaactcaccgaggcagttccataggatggcaagatcctggtatcggtctgcgattccgactcgtccaacatcaatacaacctattaatttcccctcgtcaaaaataaggttatcaagtgagaaatcaccatgagtgacgactgaatccggtgagaatggcaaaagtttatgcatttctttccagacttgttcaacaggccagccattacgctcgtcatcaaaatcactcgcatcaaccaaaccgttattcattcgtgattgcgcctgagcgagacgaaatacgcgatcgctgttaaaaggacaattacaaacaggaatcgaatgcaaccggcgcaggaacactgccagcgcatcaacaatattttcacctgaatcaggatattcttctaatacctggaatgctgttttcccggggatcgcagtggtgagtaaccatgcatcatcaggagtacggataaaatgcttgatggtcggaagaggcataaattccgtcagccagtttagtctgaccatctcatctgtaacatcattggcaacgctacctttgccatgtttcagaaacaactctggcgcatcgggcttcccatacaatcgatagattgtcgcacctgattgcccgacattatcgcgagcccatttatacccatataaatcagcatccatgttggaatttaatcgcggcctagagcaagacgtttcccgttgaatatggctcataacaccccttgtattactgtttatgtaagcagacagttttattgttcatgaccaaaatcccttaacgtgagttttcgttccactgagcgtcagaccccgtagaaaagatcaaaggatcttcttgagatcctttttttctgcgcgtaatctgctgcttgcaaacaaaaaaaccaccgctaccagcggtggtttgtttgccggatcaagagctaccaactctttttccgaaggtaactggcttcagcagagcgcagataccaaatactgtccttctagtgtagccgtagttaggccaccacttcaagaactctgtagcaccgcctacatacctcgctctgctaatcctgttaccagtggctgctgccagtggcgataagtcgtgtcttaccgggttggactcaagacgatagttaccggataaggcgcagcggtcgggctgaacggggggttcgtgcacacagcccagcttggagcgaacgacctacaccgaactgagatacctacagcgtgagctatgagaaagcgccacgcttcccgaagggagaaaggcggacaggtatccggtaagcggcagggtcggaacaggagagcgcacgagggagcttccagggggaaacgcctggtatctttatagtcctgtcgggtttcgccacctctgacttgagcgtcgatttttgtgatgctcgtcaggggggcggagcctatggaaaaacgccagcaacgcggcctttttacggttcctggccttttgctggccttttgctcacatgttctttcctgcgttatcccctgattctgtggataaccgtattaccgcctttgagtgagctgataccgctcgccgcagccgaacgaccgagcgcagcgagtcagtgagcgaggaagcggaagagcgcctgatgcggtattttctccttacgcatctgtgcggtatttcacaccgcaatggtgcactctcagtacaatctgctctgatgccgcatagttaagccagtatacactccgctatcgctacgtgactgggtcatggctgcgccccgacacccgccaacacccgctgacgcgccctgacgggcttgtctgctcccggcatccgcttacagacaagctgtgaccgtctccgggagctgcatgtgtgatgcctccgtgtaagggggatttctgttcatgggggtaatgataccgatgaaacgagagaggatgctcacgatacgggttactgatgatgaacatgcccggttactggaacgttgtgagggtaaacaactggcggtatggatgcggcgggaccagagaaaaatcactcagggtcaatgccagcgcttcgttaatacagatgtaggtgttccacagggtagccagcagcatcctgcgatgcagatccggaacataatggtgcagggcgctgacttccgcgtttccagactttacgaaacacggaaaccgaagaccattcatgttgttgctcaggtcgcagacgttttgcagcagcagtcgcttcacgttcgctcgcgtatcggtgattcattctgctaaccagtaaggcaaccccgccagcctagccgggtcctcaacgacaggagcacgatcatgcgcacccgtggggccgccatgccggcgataatggcctgcttctcgccgaaacgtttggtggcgggaccagtgacgaaggcttgagcgagggcgtgcaagattccgaataccgcaagcgacaggccgatcatcgtcgcgctccagcgaaagcggtcctcgccgaaaatgacccagagcgctgccggcacctgtcctacgagttgcatgataaagaagacagtcataagtgcggcgacgatagtcatgccccgcgcccaccggaaggagctgactgggttgaaggctctcaagggcatcggtcgagatcccggtgcctaatgagtgagctaacttacattaattgcgttgcgctcactgcccgctttccagtcgggaaacctgtcgtgccagctgcattaatgaatcggccaacgcgcggggagaggcggtttgcgtattgggcgccagggtggtttttcttttcaccagtgagacgggcaacagctgattgcccttcaccgcctggccctgagagagttgcagcaagcggtccacgctggtttgccccagcaggcgaaaatcctgtttgatggtggttaacggcgggatataacatgagctgtcttcggtatcgtcgtatcccactaccgagatatccgcaccaacgcgcagcccggactcggtaatggcgcgcattgcgcccagcgccatctgatcgttggcaaccagcatcgcagtgggaacgatgccctcattcagcatttgcatggtttgttgaaaaccggacatggcactccagtcgccttcccgttccgctatcggctgaatttgattgcgagtgagatatttatgccagccagccagacgcagacgcgccgagacagaacttaatgggcccgctaacagcgcgatttgctggtgacccaatgcgaccagatgctccacgcccagtcgcgtaccgtcttcatgggagaaaataatactgttgatgggtgtctggtcagagacatcaagaaataacgccggaacattagtgcaggcagcttccacagcaatggcatcctggtcatccagcggatagttaatgatcagcccactgacgcgttgcgcgagaagattgtgcaccgccgctttacaggcttcgacgccgcttcgttctaccatcgacaccaccacgctggcacccagttgatcggcgcgagatttaatcgccgcgacaatttgcgacggcgcgtgcagggccagactggaggtggcaacgccaatcagcaacgactgtttgcccgccagttgttgtgccacgcggttgggaatgtaattcagctccgccatcgccgcttccactttttcccgcgttttcgcagaaacgtggctggcctggttcaccacgcgggaaacggtctgataagagacaccggcatactctgcgacatcgtataacgttactggtttcacattcaccaccctgaattgactctcttccgggcgctatcatgccataccgcgaaaggttttgcgccattcgatggtgtccgggatctcgacgctctcccttatgcgactcctgcattaggaagcagcccagtagtaggttgaggccgttgagcaccgccgccgcaaggaatggtgcatgcaaggagatggcgcccaacagtcccccggccacggggcctgccaccatacccacgccgaaacaagcgctcatgagcccgaagtggcgagcccgatcttccccatcggtgatgtcggcgatataggcgccagcaaccgcacctgtggcgccggtgatgccggccacgatgcgtccggcgtagaggatcgagatctcgatcccgcgaaattaatacgactcactataggggaattgtgagcggataacaattcccctctagaaataattttgtttaactttaagaaggagatatacatatgaaatacctgctgccgaccgctgctgctggtctgctgctcctcgctgcccagccggcgatggccggcggtggcagcgttcaggcaggtggcagcctgaaactgagctgcgaagccagcctgcctagcacgaccacgccgtatagcatggcctggtttcgtcaggcgcctggacgtgaaagagaagcggtggccaccatcagcgcaagaggtggcactaaactgtacagcgattctgtgcgcgaacgcttcacgattagccgtgataaccgcaagaacacggtctacctgaagatggatcatctgaacaccgatgataccgccatctactattgcgccgcaacgggcagcattctgtttaatagccgtccattcgcggaaagcacgtatccgttctggggtcagggtactctggtcacggtgagcagccctgaaggtggtagcctggcggcactgaccgcacaccaagcatgtcatctgccactggaaacctttacccgtcatcgtcagccgcgtggctgggaacaactggaacaatgtggatatccggtgcagagactggtcgcattatatctggcagcacgtctgagttggaatcaggttgatcaagttattcgtaacgcacttgcctcaccgggtagcggtggtgatttaggtgaggcaattcgtgaacaacctgaacaggcacgcttagcattaacccttgcagccgcagaaagtgaaagatttgtgcgtcagggtactggtaatgatgaggccggtgcagcaaatgggccggcagacagcggagatgcattattagagagaaattatcctaccggcgcagaatttctgggtgatgggggtgatgttagtttttcaacacgcgggacacagaattggaccgtggaacgtttactgcaggcacatcgtcagctggaagaacgcggttatgtttttgttggttatcatgggacgtttctggaggcagcacagagcattgtctttggcggtgtgcgggcgcgtagccaggatcttgatgcaatttggcgtggtttttatattgcgggtgatcctgcgctggcgtatggatatgcgcaggatcaggagccggatgcgcgtggtcgtattcgtaatggtgccctgctgcgggtttatgttccgcgtagctcactgccggggttttatagaacaagcttaacactggctgcgccggaagcagcaggtgaagttgaacgtctgattggccatccgctgccgttacgtttagatgcaattactggtccggaagaagaaggtggtcgcctggaaaccattctgggttggccgctggcagaaagaaccgtggttataccttccgcaataccgaccgatcctcggaatgtggggggtgatttagatcctagcagcattcctgataaagaacaggcaatttctgctctgcctgattatgcatcacagccgggtaaaccgccgcgtgaagatttaaagcatcatcaccatcatcattaagatccggctgctaacaaagcccgaaaggaagctgagttggctgctgccaccgctgagcaataactagcataaccccttggggcctctaaacgggtcttgaggggttttttgctgaaaggaggaactatatccggat

SEQ ID NO: 103 - DNA, 6493 bp, synthetic construct
  source 1..6493: mol_type = other DNA
tggcgaatgggacgcgccctgtagcggcgcattaagcgcggcgggtgtggtggttacgcgcagcgtgaccgctacacttgccagcgccctagcgcccgctcctttcgctttcttcccttcctttctcgccacgttcgccggctttccccgtcaagctctaaatcgggggctccctttagggttccgatttagtgctttacggcacctcgaccccaaaaaacttgattagggtgatggttcacgtagtgggccatcgccctgatagacggtttttcgccctttgacgttggagtccacgttctttaatagtggactcttgttccaaactggaacaacactcaaccctatctcggtctattcttttgatttataagggattttgccgatttcggcctattggttaaaaaatgagctgatttaacaaaaatttaacgcgaattttaacaaaatattaacgcttacaatttaggtggcacttttcggggaaatgtgcgcggaacccctatttgtttatttttctaaatacattcaaatatgtatccgctcatgaattaattcttagaaaaactcatcgagcatcaaatgaaactgcaatttattcatatcaggattatcaataccatatttttgaaaaagccgtttctgtaatgaaggagaaaactcaccgaggcagttccataggatggcaagatcctggtatcggtctgcgattccgactcgtccaacatcaatacaacctattaatttcccctcgtcaaaaataaggttatcaagtgagaaatcaccatgagtgacgactgaatccggtgagaatggcaaaagtttatgcatttctttccagacttgttcaacaggccagccattacgctcgtcatcaaaatcactcgcatcaaccaaaccgttattcattcgtgattgcgcctgagcgagacgaaatacgcgatcgctgttaaaaggacaattacaaacaggaatcgaatgcaaccggcgcaggaacactgccagcgcatcaacaatattttcacctgaatcaggatattcttctaatacctggaatgctgttttcccggggatcgcagtggtgagtaaccatgcatcatcaggagtacggataaaatgcttgatggtcggaagaggcataaattccgtcagccagtttagtctgaccatctcatctgtaacatcattggcaacgctacctttgccatgtttcagaaacaactctggcgcatcgggcttcccatacaatcgatagattgtcgcacctgattgcccgacattatcgcgagcccatttatacccatataaatcagcatccatgttggaatttaatcgcggcctagagcaagacgtttcccgttgaatatggctcataacaccccttgtattactgtttatgtaagcagacagttttattgttcatgaccaaaatcccttaacgtgagttttcgttccactgagcgtcagaccccgtagaaaagatcaaaggatcttcttgagatcctttttttctgcgcgtaatctgctgcttgcaaacaaaaaaaccaccgctaccagcggtggtttgtttgccggatcaagagctaccaactctttttccgaaggtaactggcttcagcagagcgcagataccaaatactgtccttctagtgtagccgtagttaggccaccacttcaagaactctgtagcaccgcctacatacctcgctctgctaatcctgttaccagtggctgctgccagtggcgataagtcgtgtcttaccgggttggactcaagacgatagttaccggataaggcgcagcggtcgggctgaacggggggttcgtgcacacagcccagcttggagcgaacgacctacaccgaactgagatacctacagcgtgagctatgagaaagcgccacgcttcccgaagggagaaaggcggacaggtatccggtaagcggcagggtcggaacaggagagcgcacgagggagcttccagggggaaacgcctggtatctttatagtcctgtcgggtttcgccacctctgacttgagcgtcgatttttgtgatgctcgtcaggggggcggagcctatggaaaaacgccagcaacgcggcctttttacggttcctggccttttgctggccttttgctcacatgttctttcctgcgttatcccctgattctgtggataaccgtattaccgcctttgagtgagctgataccgctcgccgcagccgaacgaccgagcgcagcgagtcagtgagcgaggaagcggaagagcgcctgatgcggtattttctccttacgcatctgtgcggtatttcacaccgcaatggtgcactctcagtacaatctgctctgatgccgcatagttaagccagtatacactccgctatcgctacgtgactgggtcatggctgcgccccgacacccgccaacacccgctgacgcgccctgacgggcttgtctgctcccggcatccgcttacagacaagctgtgaccgtctccgggagctgcatgtgtgatgcctccgtgtaagggggatttctgttcatgggggtaatgataccgatgaaacgagagaggatgctcacgatacgggttactgatgatgaacatgcccggttactggaacgttgtgagggtaaacaactggcggtatggatgcggcgggaccagagaaaaatcactcagggtcaatgccagcgcttcgttaatacagatgtaggtgttccacagggtagccagcagcatcctgcgatgcagatccggaacataatggtgcagggcgctgacttccgcgtttccagactttacgaaacacggaaaccgaagaccattcatgttgttgctcaggtcgcagacgttttgcagcagcagtcgcttcacgttcgctcgcgtatcggtgattcattctgctaaccagtaaggcaaccccgccagcctagccgggtcctcaacgacaggagcacgatcatgcgcacccgtggggccgccatgccggcgataatggcctgcttctcgccgaaacgtttggtggcgggaccagtgacgaaggcttgagcgagggcgtgcaagattccgaataccgcaagcgacaggccgatcatcgtcgcgctccagcgaaagcggtcctcgccgaaaatgacccagagcgctgccggcacctgtcctacgagttgcatgataaagaagacagtcataagtgcggcgacgatagtcatgccccgcgcccaccggaaggagctgactgggttgaaggctctcaagggcatcggtcgagatcccggtgcctaatgagtgagctaacttacattaattgcgttgcgctcactgcccgctttccagtcgggaaacctgtcgtgccagctgcattaatgaatcggccaacgcgcggggagaggcggtttgcgtattgggcgccagggtggtttttcttttcaccagtgagacgggcaacagctgattgcccttcaccgcctggccctgagagagttgcagcaagcggtccacgctggtttgccccagcaggcgaaaatcctgtttgatggtggttaacggcgggatataacatgagctgtcttcggtatcgtcgtatcccactaccgagatatccgcaccaacgcgcagcccggactcggtaatggcgcgcattgcgcccagcgccatctgatcgttggcaaccagcatcgcagtgggaacgatgccctcattcagcatttgcatggtttgttgaaaaccggacatggcactccagtcgccttcccgttccgctatcggctgaatttgattgcgagtgagatatttatgccagccagccagacgcagacgcgccgagacagaacttaatgggcccgctaacagcgcgatttgctggtgacccaatgcgaccagatgctccacgcccagtcgcgtaccgtcttcatgggagaaaataatactgttgatgggtgtctggtcagagacatcaagaaataacgccggaacattagtgcaggcagcttccacagcaatggcatcctggtcatccagcggatagttaatgatcagcccactgacgcgttgcgcgagaagattgtgcaccgccgctttacaggcttcgacgccgcttcgttctaccatcgacaccaccacgctggcacccagttgatcggcgcgagatttaatcgccgcgacaatttgcgacggcgcgtgcagggccagactggaggtggcaacgccaatcagcaacgactgtttgcccgccagttgttgtgccacgcggttgggaatgtaattcagctccgccatcgccgcttccactttttcccgcgttttcgcagaaacgtggctggcctggttcaccacgcgggaaacggtctgataagagacaccggcatactctgcgacatcgtataacgttactggtttcacattcaccaccctgaattgactctcttccgggcgctatcatgccataccgcgaaaggttttgcgccattcgatggtgtccgggatctcgacgctctcccttatgcgactcctgcattaggaagcagcccagtagtaggttgaggccgttgagcaccgccgccgcaaggaatggtgcatgcaaggagatggcgcccaacagtcccccggccacggggcctgccaccatacccacgccgaaacaagcgctcatgagcccgaagtggcgagcccgatcttccccatcggtgatgtcggcgatataggcgccagcaaccgcacctgtggcgccggtgatgccggccacgatgcgtccggcgtagaggatcgagatctcgatcccgcgaaattaatacgactcactataggggaattgtgagcggataacaattcccctctagaaataattttgtttaactttaagaaggagatatacatatgaaatacctgctgccgaccgctgctgctggtctgctgctcctcgctgcccagccggcgatggccggcggtggcacggtacaggctggcggtagcctgaaactgagctgcgccgcgagaggttggcgctttagcggctattgcgtagcctggtttcgtcaagcaccgggcaaagaacgcgaagcggtagcgatcattccgggtgctggcgtgatgtataccgatgattctgtgaaaggccgtttcacctattcgcgcgataatgtgaagaacaccgttagtctgcaaatgaacagcctggaaccggaagataccgcaacgtactactgcgctgtggattgggcatacagccatagctgtccgaagaacacggaagattaccgttattggggccagggcacgcaggtgaccgtgtcatcacctgaaggtggtagcctggcggcactgaccgcacaccaagcatgtcatctgccactggaaacctttacccgtcatcgtcagccgcgtggctgggaacaactggaacaatgtggatatccggtgcagagactggtcgcattatatctggcagcacgtctgagttggaatcaggttgatcaagttattcgtaacgcacttgcctcaccgggtagcggtggtgatttaggtgaggcaattcgtgaacaacctgaacaggcacgcttagcattaacccttgcagccgcagaaagtgaaagatttgtgcgtcagggtactggtaatgatgaggccggtgcagcaaatgggccggcagacagcggagatgcattattagagagaaattatcctaccggcgcagaatttctgggtgatgggggtgatgttagtttttcaacacgcgggacacagaattggaccgtggaacgtttactgcaggcacatcgtcagctggaagaacgcggttatgtttttgttggttatcatgggacgtttctggaggcagcacagagcattgtctttggcggtgtgcgggcgcgtagccaggatcttgatgcaatttggcgtggtttttatattgcgggtgatcctgcgctggcgtatggatatgcgcaggatcaggagccggatgcgcgtggtcgtattcgtaatggtgccctgctgcgggtttatgttccgcgtagctcactgccggggttttatagaacaagcttaacactggctgcgccggaagcagcaggtgaagttgaacgtctgattggccatccgctgccgttacgtttagatgcaattactggtccggaagaagaaggtggtcgcctggaaaccattctgggttggccgctggcagaaagaaccgtggttataccttccgcaataccgaccgatcctcggaatgtggggggtgatttagatcctagcagcattcctgataaagaacaggcaatttctgctctgcctgattatgcatcacagccgggtaaaccgccgcgtgaagatttaaagcatcatcaccatcatcattaagatccggctgctaacaaagcccgaaaggaagctgagttggctgctgccaccgctgagcaataactagcataaccccttggggcctctaaacgggtcttgaggggttttttgctgaaaggaggaactatatccggat

SEQ ID NO: 104 - DNA, 6583 bp, synthetic construct
  source 1..6583: mol_type = other DNA
tggcgaatgggacgcgccctgtagcggcgcattaagcgcggcgggtgtggtggttacgcgcagcgtgaccgctacacttgccagcgccctagcgcccgctcctttcgctttcttcccttcctttctcgccacgttcgccggctttccccgtcaagctctaaatcgggggctccctttagggttccgatttagtgctttacggcacctcgaccccaaaaaacttgattagggtgatggttcacgtagtgggccatcgccctgatagacggtttttcgccctttgacgttggagtccacgttctttaatagtggactcttgttccaaactggaacaacactcaaccctatctcggtctattcttttgatttataagggattttgccgatttcggcctattggttaaaaaatgagctgatttaacaaaaatttaacgcgaattttaacaaaatattaacgcttacaatttaggtggcacttttcggggaaatgtgcgcggaacccctatttgtttatttttctaaatacattcaaatatgtatccgctcatgaattaattcttagaaaaactcatcgagcatcaaatgaaactgcaatttattcatatcaggattatcaataccatatttttgaaaaagccgtttctgtaatgaaggagaaaactcaccgaggcagttccataggatggcaagatcctggtatcggtctgcgattccgactcgtccaacatcaatacaacctattaatttcccctcgtcaaaaataaggttatcaagtgagaaatcaccatgagtgacgactgaatccggtgagaatggcaaaagtttatgcatttctttccagacttgttcaacaggccagccattacgctcgtcatcaaaatcactcgcatcaaccaaaccgttattcattcgtgattgcgcctgagcgagacgaaatacgcgatcgctgttaaaaggacaattacaaacaggaatcgaatgcaaccggcgcaggaacactgccagcgcatcaacaatattttcacctgaatcaggatattcttctaatacctggaatgctgttttcccggggatcgcagtggtgagtaaccatgcatcatcaggagtacggataaaatgcttgatggtcggaagaggcataaattccgtcagccagtttagtctgaccatctcatctgtaacatcattggcaacgctacctttgccatgtttcagaaacaactctggcgcatcgggcttcccatacaatcgatagattgtcgcacctgattgcccgacattatcgcgagcccatttatacccatataaatcagcatccatgttggaatttaatcgcggcctagagcaagacgtttcccgttgaatatggctcataacaccccttgtattactgtttatgtaagcagacagttttattgttcatgaccaaaatcccttaacgtgagttttcgttccactgagcgtcagaccccgtagaaaagatcaaaggatcttcttgagatcctttttttctgcgcgtaatctgctgcttgcaaacaaaaaaaccaccgctaccagcggtggtttgtttgccggatcaagagctaccaactctttttccgaaggtaactggcttcagcagagcgcagataccaaatactgtccttctagtgtagccgtagttaggccaccacttcaagaactctgtagcaccgcctacatacctcgctctgctaatcctgttaccagtggctgctgccagtggcgataagtcgtgtcttaccgggttggactcaagacgatagttaccggataaggcgcagcggtcgggctgaacggggggttcgtgcacacagcccagcttggagcgaacgacctacaccgaactgagatacctacagcgtgagctatgagaaagcgccacgcttcccgaagggagaaaggcggacaggtatccggtaagcggcagggtcggaacaggagagcgcacgagggagcttccagggggaaacgcctggtatctttatagtcctgtcgggtttcgccacctctgacttgagcgtcgatttttgtgatgctcgtcaggggggcggagcctatggaaaaacgccagcaacgcggcctttttacggttcctggccttttgctggccttttgctcacatgttctttcctgcgttatcccctgattctgtggataaccgtattaccgcctttgagtgagctgataccgctcgccgcagccgaacgaccgagcgcagcgagtcagtgagcgaggaagcggaagagcgcctgatgcggtattttctccttacgcatctgtgcggtatttcacaccgcaatggtgcactctcagtacaatctgctctgatgccgcatagttaagccagtatacactccgctatcgctacgtgactgggtcatggctgcgccccgacacccgccaacacccgctgacgcgccctgacgggcttgtctgctcccggcatccgcttacagacaagctgtgaccgtctccgggagctgcatgtgtgatgcctccgtgtaagggggatttctgttcatgggggtaatgataccgatgaaacgagagaggatgctcacgatacgggttactgatgatgaacatgcccggttactggaacgttgtgagggtaaacaactggcggtatggatgcggcgggaccagagaaaaatcactcagggtcaatgccagcgcttcgttaatacagatgtaggtgttccacagggtagccagcagcatcctgcgatgcagatccggaacataatggtgcagggcgctgacttccgcgtttccagactttacgaaacacggaaaccgaagaccattcatgttgttgctcaggtcgcagacgttttgcagcagcagtcgcttcacgttcgctcgcgtatcggtgattcattctgctaaccagtaaggcaaccccgccagcctagccgggtcctcaacgacaggagcacgatcatgcgcacccgtggggccgccatgccggcgataatggcctgcttctcgccgaaacgtttggtggcgggaccagtgacgaaggcttgagcgagggcgtgcaagattccgaataccgcaagcgacaggccgatcatcgtcgcgctccagcgaaagcggtcctcgccgaaaatgacccagagcgctgccggcacctgtcctacgagttgcatgataaagaagacagtcataagtgcggcgacgatagtcatgccccgcgcccaccggaaggagctgactgggttgaaggctctcaagggcatcggtcgagatcccggtgcctaatgagtgagctaacttacattaattgcgttgcgctcactgcccgctttccagtcgggaaacctgtcgtgccagctgcattaatgaatcggccaacgcgcggggagaggcggtttgcgtattgggcgccagggtggtttttcttttcaccagtgagacgggcaacagctgattgcccttcaccgcctggccctgagagagttgcagcaagcggtccacgctggtttgccccagcaggcgaaaatcctgtttgatggtggttaacggcgggatataacatgagctgtcttcggtatcgtcgtatcccactaccgagatatccgcaccaacgcgcagcccggactcggtaatggcgcgcattgcgcccagcgccatctgatcgttggcaaccagcatcgcagtgggaacgatgccctcattcagcatttgcatggtttgttgaaaaccggacatggcactccagtcgccttcccgttccgctatcggctgaatttgattgcgagtgagatatttatgccagccagccagacgcagacgcgccgagacagaacttaatgggcccgctaacagcgcgatttgctggtgacccaatgcgaccagatgctccacgcccagtcgcgtaccgtcttcatgggagaaaataatactgttgatgggtgtctggtcagagacatcaagaaataacgccggaacattagtgcaggcagcttccacagcaatggcatcctggtcatccagcggatagttaatgatcagcccactgacgcgttgcgcgagaagattgtgcaccgccgctttacaggcttcgacgccgcttcgttctaccatcgacaccaccacgctggcacccagttgatcggcgcgagatttaatcgccgcgacaatttgcgacggcgcgtgcagggccagactggaggtggcaacgccaatcagcaacgactgtttgcccgccagttgttgtgccacgcggttgggaatgtaattcagctccgccatcgccgcttccactttttcccgcgttttcgcagaaacgtggctggcctggttcaccacgcgggaaacggtctgataagagacaccggcatactctgcgacatcgtataacgttactggtttcacattcaccaccctgaattgactctcttccgggcgctatcatgccataccgcgaaaggttttgcgccattcgatggtgtccgggatctcgacgctctcccttatgcgactcctgcattaggaagcagcccagtagtaggttgaggccgttgagcaccgccgccgcaaggaatggtgcatgcaaggagatggcgcccaacagtcccccggccacggggcctgccaccatacccacgccgaaacaagcgctcatgagcccgaagtggcgagcccgatcttccccatcggtgatgtcggcgatataggcgccagcaaccgcacctgtggcgccggtgatgccggccacgatgcgtccggcgtagaggatcgagatctcgatcccgcgaaattaatacgactcactataggggaattgtgagcggataacaattcccctctagaaataattttgtttaactttaagaaggagatatacatatgaaatacctgctgccgaccgctgctgctggtctgctgctcctcgctgcccagccggcgatggccgaggttcaattagtggaatctggcgggggattggttcaagccggtgagtccttgcgtttgagctgcgccgcatctgggagcacatttgatttcaaagtgatgggctggtatcgtcagccgcccggaaaacagcgcgagggtgtagcagccatccgcttgagcggaaatatgcactacgccgagtctgtaaaagggcgctttgctatttccaaagcgaacgctaagaacacagtgtatcttcagatgaactccttgcgtcccgaagacactgccgtttattattgcaaagtaaacatccgtgggcaagactactggggtcaaggaacgcaggtcacagtctcttctggctctggcgaagcactggcagcacatcgtgtttgcggagttccactggaaacgctggcacgtagccgtaaaccgcgtgatcttccggatgatctgtcatgcgcctatcaggcacagaacatcgttagcctgtttgtggcaacacgcatcttgttcagccatctggatagcgtgtttacgctgaacctggatgaacaagaaccggaagtggcagaacgccttagcgcactgagacagatcaacgagaacaatccgggcatggtgacacaggtgctgaccgttgcacgccagatttacaacgattacgtgacgcatcatccgggcttaactccggaacagactagcgcgggtgcacaagccgcagatatcttgagcctgttttgtccggatgcagataaaccgtgcgttgcgagcaacaacgatcaggcgaacatcaacatcgagtcacgtagcggacgcagctatctgccggagaatcgcgccgtgattacgcctcagggtgtgaccaactggacctatcaagaactggaagcaacgcatcaggcactgacacgcgaaggttatgtgtttgttggctatcatggcaccaaccatgttgcggcacagaccattgtgaaccgcattgcaccggttccacgtggtaacaacaccgaaaacgaagagaaatggggcggtctgtatgttgccacgcacgcagaagttgctcatggctatgcacgcatcaaagaaggtacgggcgaatatggcttaccgacgcgtgcagaacgtgatgccagaggcgttatgctgcgtgtgtacattccgagagcgagcttagaacgcttctatcgcaccaacacaccgctggaaaacgcggaagaacacattactcaggtgattggccatagcctgccgttacgcaacgaagcctttaccggtccggaaagcgcaggtggtgaagatgaaaccgtgattggctgggatatggcgattcatgccgttgccataccgagcaccataccgggcaatgcgtatgaagagctggcaattgacgaagaagcagttgccaaagaacagagcattagcaccaaaccgccgtataaagagcgcaaagacgaactgaagtacccctatgacgtgcctgattacgccggctctggccaccaccaccaccaccactgagatccggctgctaacaaagcccgaaaggaagctgagttggctgctgccaccgctgagcaataactagcataaccccttggggcctctaaacgggtcttgaggggttttttgctgaaaggaggaactatatccggat

SEQ ID NO: 105 - DNA, 6658 bp, synthetic construct
  source 1..6658: mol_type = other DNA
tggcgaatgggacgcgccctgtagcggcgcattaagcgcggcgggtgtggtggttacgcgcagcgtgaccgctacacttgccagcgccctagcgcccgctcctttcgctttcttcccttcctttctcgccacgttcgccggctttccccgtcaagctctaaatcgggggctccctttagggttccgatttagtgctttacggcacctcgaccccaaaaaacttgattagggtgatggttcacgtagtgggccatcgccctgatagacggtttttcgccctttgacgttggagtccacgttctttaatagtggactcttgttccaaactggaacaacactcaaccctatctcggtctattcttttgatttataagggattttgccgatttcggcctattggttaaaaaatgagctgatttaacaaaaatttaacgcgaattttaacaaaatattaacgcttacaatttaggtggcacttttcggggaaatgtgcgcggaacccctatttgtttatttttctaaatacattcaaatatgtatccgctcatgaattaattcttagaaaaactcatcgagcatcaaatgaaactgcaatttattcatatcaggattatcaataccatatttttgaaaaagccgtttctgtaatgaaggagaaaactcaccgaggcagttccataggatggcaagatcctggtatcggtctgcgattccgactcgtccaacatcaatacaacctattaatttcccctcgtcaaaaataaggttatcaagtgagaaatcaccatgagtgacgactgaatccggtgagaatggcaaaagtttatgcatttctttccagacttgttcaacaggccagccattacgctcgtcatcaaaatcactcgcatcaaccaaaccgttattcattcgtgattgcgcctgagcgagacgaaatacgcgatcgctgttaaaaggacaattacaaacaggaatcgaatgcaaccggcgcaggaacactgccagcgcatcaacaatattttcacctgaatcaggatattcttctaatacctggaatgctgttttcccggggatcgcagtggtgagtaaccatgcatcatcaggagtacggataaaatgcttgatggtcggaagaggcataaattccgtcagccagtttagtctgaccatctcatctgtaacatcattggcaacgctacctttgccatgtttcagaaacaactctggcgcatcgggcttcccatacaatcgatagattgtcgcacctgattgcccgacattatcgcgagcccatttatacccatataaatcagcatccatgttggaatttaatcgcggcctagagcaagacgtttcccgttgaatatggctcataacaccccttgtattactgtttatgtaagcagacagttttattgttcatgaccaaaatcccttaacgtgagttttcgttccactgagcgtcagaccccgtagaaaagatcaaaggatcttcttgagatcctttttttctgcgcgtaatctgctgcttgcaaacaaaaaaaccaccgctaccagcggtggtttgtttgccggatcaagagctaccaactctttttccgaaggtaactggcttcagcagagcgcagataccaaatactgtccttctagtgtagccgtagttaggccaccacttcaagaactctgtagcaccgcctacatacctcgctctgctaatcctgttaccagtggctgctgccagtggcgataagtcgtgtcttaccgggttggactcaagacgatagttaccggataaggcgcagcggtcgggctgaacggggggttcgtgcacacagcccagcttggagcgaacgacctacaccgaactgagatacctacagcgtgagctatgagaaagcgccacgcttcccgaagggagaaaggcggacaggtatccggtaagcggcagggtcggaacaggagagcgcacgagggagcttccagggggaaacgcctggtatctttatagtcctgtcgggtttcgccacctctgacttgagcgtcgatttttgtgatgctcgtcaggggggcggagcctatggaaaaacgccagcaacgcggcctttttacggttcctggccttttgctggccttttgctcacatgttctttcctgcgttatcccctgattctgtggataaccgtattaccgcctttgagtgagctgataccgctcgccgcagccgaacgaccgagcgcagcgagtcagtgagcgaggaagcggaagagcgcctgatgcggtattttctccttacgcatctgtgcggtatttcacaccgcaatggtgcactctcagtacaatctgctctgatgccgcatagttaagccagtatacactccgctatcgctacgtgactgggtcatggctgcgccccgacacccgccaacacccgctgacgcgccctgacgggcttgtctgctcccggcatccgcttacagacaagctgtgaccgtctccgggagctgcatgtgtgatgcctccgtgtaagggggatttctgttcatgggggtaatgataccgatgaaacgagagaggatgctcacgatacgggttactgatgatgaacatgcccggttactggaacgttgtgagggtaaacaactggcggtatggatgcggcgggaccagagaaaaatcactcagggtcaatgccagcgcttcgttaatacagatgtaggtgttccacagggtagccagcagcatcctgcgatgcagatccggaacataatggtgcagggcgctgacttccgcgtttccagactttacgaaacacggaaaccgaagaccattcatgttgttgctcaggtcgcagacgttttgcagcagcagtcgcttcacgttcgctcgcgtatcggtgattcattctgctaaccagtaaggcaaccccgccagcctagccgggtcctcaacgacaggagcacgatcatgcgcacccgtggggccgccatgccggcgataatggcctgcttctcgccgaaacgtttggtggcgggaccagtgacgaaggcttgagcgagggcgtgcaagattccgaataccgcaagcgacaggccgatcatcgtcgcgctccagcgaaagcggtcctcgccgaaaatgacccagagcgctgccggcacctgtcctacgagttgcatgataaagaagacagtcataagtgcggcgacgatagtcatgccccgcgcccaccggaaggagctgactgggttgaaggctctcaagggcatcggtcgagatcccggtgcctaatgagtgagctaacttacattaattgcgttgcgctcactgcccgctttccagtcgggaaacctgtcgtgccagctgcattaatgaatcggccaacgcgcggggagaggcggtttgcgtattgggcgccagggtggtttttcttttcaccagtgagacgggcaacagctgattgcccttcaccgcctggccctgagagagttgcagcaagcggtccacgctggtttgccccagcaggcgaaaatcctgtttgatggtggttaacggcgggatataacatgagctgtcttcggtatcgtcgtatcccactaccgagatatccgcaccaacgcgcagcccggactcggtaatggcgcgcattgcgcccagcgccatctgatcgttggcaaccagcatcgcagtgggaacgatgccctcattcagcatttgcatggtttgttgaaaaccggacatggcactccagtcgccttcccgttccgctatcggctgaatttgattgcgagtgagatatttatgccagccagccagacgcagacgcgccgagacagaacttaatgggcccgctaacagcgcgatttgctggtgacccaatgcgaccagatgctccacgcccagtcgcgtaccgtcttcatgggagaaaataatactgttgatgggtgtctggtcagagacatcaagaaataacgccggaacattagtgcaggcagcttccacagcaatggcatcctggtcatccagcggatagttaatgatcagcccactgacgcgttgcgcgagaagattgtgcaccgccgctttacaggcttcgacgccgcttcgttctaccatcgacaccaccacgctggcacccagttgatcggcgcgagatttaatcgccgcgacaatttgcgacggcgcgtgcagggccagactggaggtggcaacgccaatcagcaacgactgtttgcccgccagttgttgtgccacgcggttgggaatgtaattcagctccgccatcgccgcttccactttttcccgcgttttcgcagaaacgtggctggcctggttcaccacgcgggaaacggtctgataagagacaccggcatactctgcgacatcgtataacgttactggtttcacattcaccaccctgaattgactctcttccgggcgctatcatgccataccgcgaaaggttttgcgccattcgatggtgtccgggatctcgacgctctcccttatgcgactcctgcattaggaagcagcccagtagtaggttgaggccgttgagcaccgccgccgcaaggaatggtgcatgcaaggagatggcgcccaacagtcccccggccacggggcctgccaccatacccacgccgaaacaagcgctcatgagcccgaagtggcgagcccgatcttccccatcggtgatgtcggcgatataggcgccagcaaccgcacctgtggcgccggtgatgccggccacgatgcgtccggcgtagaggatcgagatctcgatcccgcgaaattaatacgactcactataggggaattgtgagcggataacaattcccctctagaaataattttgtttaactttaagaaggagatatacatatgaaatacctgctgccgaccgctgctgctggtctgctgctcctcgctgcccagccggcgatggccgaggttcaattagtggaatctggcgggggattggttcaagccggtgagtccttgcgtttgagctgcgccgcatctgggagcacatttgatttcaaagtgatgggctggtatcgtcagccgcccggaaaacagcgcgagggtgtagcagccatccgcttgagcggaaatatgcactacgccgagtctgtaaaagggcgctttgctatttccaaagcgaacgctaagaacacagtgtatcttcagatgaactccttgcgtcccgaagacactgccgtttattattgcaaagtaaacatccgtgggcaagactactggggtcaaggaacgcaggtcacagtctcttctggctctggcggcgcggatgatgtcgtggattcaagcaaatcatttgtcatggagaacttcagcagctatcacggcaccaaacctggctatgtggattcgattcagaaaggcattcagaaaccgaaatccggtacgcagggcaactatgacgatgattggaaaggcttctacagcaccgataacaagtacgatgcggcgggttactccgtggataatgagaatccactgagcggtaaagctggcggtgtggtgaaagtcacctatccgggcctgacgaaagtgctggcactgaaggtggataatgccgaaaccattaagaaagaactgggcctgagcctgaccgaacctctgatggaacaggttggcacagaagagtttatcaaacgctttggcgatggtgcgtcaagagttgtgctgagccttccgtttgccgaaggtagcagcagcgttgagtacatcaacaattgggaacaggccaaagcactgtcagtggaactggaaatcaactttgagacacgtggtaagagaggccaagatgccatgtacgagtacatggcgcaagcgtgcgcaggcaaccgcgttcgtagaagcgttggcagcagcctgagctgcatcaacctggactgggatgtgattcgcgataagaccaagacgaagatcgaaagcctgaaagaacacggaccaatcaagaacaagatgagcgaaagtccgaacaagacggtgagcgaagagaaagcgaaacagtatctggaagagtttcaccagaccgcactggaacatccggaactgagcgagcttaagaccgtgacgggcacaaatccggtgtttgcaggcgcaaactatgcggcatgggcggtgaacgtggcacaggtcattgacagcgaaactgcggataatctggagaaaacgaccgctgcactgagcatactgccgggaattggcagcgtaatgggcatcgcggatggtgctgttcaccacaacaccgaagagattgttgcgcagagcatcgcactgagcagcctgatggtggcacaagcgattccgctggtgggcgaattggtcgatatcggctttgcggcctataacttcgtcgaaagcattatcaacctgtttcaggtggttcacaacagctacaatcgtccggcctatagtccgggacacaagacgcagccgtttctgtacccctatgacgtgcctgattacgccggctctggccaccaccaccaccaccactgagatccggctgctaacaaagcccgaaaggaagctgagttggctgctgccaccgctgagcaataactagcataaccccttggggcctctaaacgggtcttgaggggttttttgctgaaaggaggaactatatccggat

SEQ ID NO: 106 - DNA, 4801 bp, synthetic construct
  source 1..4801: mol_type = other DNA
catggtcatagctgtttcctttaatgcccatggcgtttaccaatgcttaatcagtgaggcacctatctcagcgatctgtctatttcgttcatccatagttgcctgactccccgtcgtgtagataactacgatacgggagggcttaccatctggccccagtgctgcaatgataccgcgacttccacgctcaccggctccagatttatcagcaataaaccagccagccggaagggccgagcgcagaagtggtcctgcaactttatccgcctccatccagtctattaattgttgccgggaagctagagtaagtagttcgccagttaatagtttgcgcaacgttgttgccattgctacaggcatcgtggtgtcacgctcgtcgtttggtatggcttcattcagctccggttcccaacgatcaaggcgagttacatgatcccccatgttgtgcaaaaaagcggttagctccttcggtcctccgatcgttgtcagaagtaagttggccgcagtgttatcactcatggttatggcagcactgcataattctcttactgtcatgccatccgtaagatgcttttctgtgactggtgagtactcaaccaagtcattctgagaatagtgtatgcggcgaccgagttgctcttgcccggcgtcaatacgggataataccgcgccacatagcagaactttaaaagtgctcatcattggaaaacgttcttcggggcgaaaactctcaaggatcttaccgctgttgagatccagttcgatgtaacccactcgtgcacccaactgatcttcagcatcttttactttcaccagcgtttctgggtgagcaaaaacaggaaggcaaaatgccgcaaaaaagggaataagggcgacacggaaatgttgaatactcatactcttcctttttcaatattattgaagcatttatcagggttattgtctcatgagcggatacatatttgaatgtatttagaaaaataaacaaataggggttccgcgcacatttccccgaaaagtgccacctgacgtctaagaaaccattattatcatgacattaacctataaaaataggcgtatcacgaggcccttaggccaaataggccgttcagatccttccgtatttagccagtatgttctctagtgtggttcgttgtttttgcgtgagccatgagaacgaaccattgagatcatgcttactttgcatgtcactcaaaaattttgcctcaaaactggtgagctgaatttttgcagttaaagcatcgtgtagtgtttttcttagtccgttacgtaggtaggaatctgatgtaatggttgttggtattttgtcaccattcatttttatctggttgttctcaagttcggttacgagatccatttgtctatctagttcaacttggaaaatcaacgtatcagtcgggcggcctcgcttatcaaccaccaatttcatattgctgtaagtgtttaaatctttacttattggtttcaaaacccattggttaagccttttaaactcatggtagttattttcaagcattaacatgaacttaaattcatcaaggctaatctctatatttgccttgtgagttttcttttgtgttagttcttttaataaccactcataaatcctcatagagtatttgttttcaaaagacttaacatgttccagattatattttatgaatttttttaactggaaaagataaggcaatatctcttcactaaaaactaattctaatttttcgcttgagaacttggcatagtttgtccactggaaaatctcaaagcctttaaccaaaggattcctgatttccacagttctcgtcatcagctctctggttgctttagctaatacaccataagcattttccctactgatgttcatcatctgagcgtattggttataagtgaacgataccgtccgttctttccttgtagggttttcaatcgtggggttgagtagtgccacacagcataaaattagcttggtttcatgctccgttaagtcatagcgactaatcgctagttcatttgctttgaaaacaactaattcagacatacatctcaattggtctaggtgattttaatcactataccaattgagatgggctagtcaatgataattactagtccttttcctttgagttgtgggtatctgtaaattctgctagacctttgctggaaaacttgtaaattctgctagaccctctgtaaattccgctagacctttgtgtgttttttttgtttatattcaagtggttataatttatagaataaagaaagaataaaaaaagataaaaagaatagatcccagccctgtgtataactcactactttagtcagttccgcagtattacaaaaggatgtcgcaaacgctgtttgctcctctacaaaacagaccttaaaaccctaaaggcttaagtagcaccctcgcaagctcgggcaaatcgctgaatattccttttgtctccgaccatcaggcacctgagtcgctgtctttttcgtgacattcagttcgctgcgctcacggctctggcagtgaatgggggtaaatggcactacaggcgccttttatggattcatgcaaggaaactacccataatacaagaaaagcccgtcacgggcttctcagggcgttttatggcgggtctgctatgtggtgctatctgactttttgctgttcagcagttcctgccctctgattttccagtctgaccacttcggattatcccgtgacaggtcattcagactggctaatgcacccagtaaggcagcggtatcatcaacaggcttacccgtcttactgtcaagaggacatccggtcagataaccgtcatcttcggctactgtctagggcggcggatttgtcctactcaggagagcgttcaccgacaaacaacagataaaacgaaaggcccagtctttcgactgagcctttcgttttatttgatgcactagtgccgatcatattcaataacccttaatataacttcgtataatgtatgctatacgaagttattaggtctgaagaggagtttacgtcccatatgggcgagctcgatatcaaattacgccccgccctgccactcatcgcagtactgttgtaattcattaagcattctgccgacatggaagccatcacagacggcatgatgaacctgaatcgccagcggcatcagcaccttgtcgccttgcgtataatatttgcccatggtgaaaacgggggcgaagaagttgtccatattggccacgtttaaatcaaaactggtgaaactcacccagggattggctgagacgaaaaacatattctcaataaaccctttagggaaataggccaggttttcaccgtaacacgccacatcttgcgaatatatgtgtagaaactgccggaaatcgtcgtggtattcactccagagcgatgaaaacgtttcagtttgctcatggaaaacggtgtaacaagggtgaacactatcccatatcaccagctcaccgtctttcattgccatacgaaattccggatgagcattcatcaggcgggcaagaatgtgaataaaggccggataaaacttgtgcttatttttctttacggtctttaaaaaggccgtaatatccagctgaacggtctggttataggtacattgagcaactgactgaaatgcctcaaaatgttctttacgatgccattgggatatatcaacggtggtatatccagtgatttttttctccattttagcttccttagctcctgaaaatctcgataactcaaaaaatacgcccggtagtgatcttatttcattatggtgaaagttggaacctcttacgtgccgatcaacgtctcattttcgccagatatcgccaagcttaggatccggaacccttaatataacttcgtataatgtatgctatacgaagttattaggtccctcgaagaggttcactagctatctagagcttggactcctgttgatagatccagtaatgacctcagaactccatctggatttgttcagaacgctcggttgccgccgggcgttttttattggtgagaatccaagcccgggaaacgggatcctgatcttgatccgccgcaaagtttgagcgaagtcaataaactctctacccattcagggcaatatctctcttgcaggtgaatgcaacgtcaagcgatggcctacttgcggcctcacacaggaaagtactagatgaaatacctgctgccgaccgctgctgctggtctgctgctcctcgctgcccagccggcgatggccgaagtgcaactggtggaaagcggtggaggccttgttcagaccggcggcagcctgcgtctgtcatgcgctgcaagcggctttacgttcagcagctacgcgatgagctgggtgcgccaggcaccgggcaaaggcttggaatgggttagcggcatcaagtcaagcggcgatagcaccagatatgccggaagcgttaaaggccgctttaccatttcacgcgataacgccaagaacatgctgtatctgcaaatgtatagcctgaaaccggaagataccgcagtgtattactgcgccaagagccgcgtgagtcgcacgggtctgtatacctatgacaaccgtggtcagggcacgcaggtgactgtgtcaagccatcatcaccatcatcattaagatccggggctctggaagatccgcgcgtaccgagttctaattcactggccgtcgttttacaacatacgatgaaggcgataagtcgcgtaagttgctagcccacgcggctcaccttcacgggtgggcctttcttcgcgatccacatg

SEQ ID NO: 107 - DNA, 4819 bp, synthetic construct
  source 1..4819: mol_type = other DNA
catggtcatagctgtttcctttaatgcccatggcgtttaccaatgcttaatcagtgaggcacctatctcagcgatctgtctatttcgttcatccatagttgcctgactccccgtcgtgtagataactacgatacgggagggcttaccatctggccccagtgctgcaatgataccgcgacttccacgctcaccggctccagatttatcagcaataaaccagccagccggaagggccgagcgcagaagtggtcctgcaactttatccgcctccatccagtctattaattgttgccgggaagctagagtaagtagttcgccagttaatagtttgcgcaacgttgttgccattgctacaggcatcgtggtgtcacgctcgtcgtttggtatggcttcattcagctccggttcccaacgatcaaggcgagttacatgatcccccatgttgtgcaaaaaagcggttagctccttcggtcctccgatcgttgtcagaagtaagttggccgcagtgttatcactcatggttatggcagcactgcataattctcttactgtcatgccatccgtaagatgcttttctgtgactggtgagtactcaaccaagtcattctgagaatagtgtatgcggcgaccgagttgctcttgcccggcgtcaatacgggataataccgcgccacatagcagaactttaaaagtgctcatcattggaaaacgttcttcggggcgaaaactctcaaggatcttaccgctgttgagatccagttcgatgtaacccactcgtgcacccaactgatcttcagcatcttttactttcaccagcgtttctgggtgagcaaaaacaggaaggcaaaatgccgcaaaaaagggaataagggcgacacggaaatgttgaatactcatactcttcctttttcaatattattgaagcatttatcagggttattgtctcatgagcggatacatatttgaatgtatttagaaaaataaacaaataggggttccgcgcacatttccccgaaaagtgccacctgacgtctaagaaaccattattatcatgacattaacctataaaaataggcgtatcacgaggcccttaggccaaataggccgttcagatccttccgtatttagccagtatgttctctagtgtggttcgttgtttttgcgtgagccatgagaacgaaccattgagatcatgcttactttgcatgtcactcaaaaattttgcctcaaaactggtgagctgaatttttgcagttaaagcatcgtgtagtgtttttcttagtccgttacgtaggtaggaatctgatgtaatggttgttggtattttgtcaccattcatttttatctggttgttctcaagttcggttacgagatccatttgtctatctagttcaacttggaaaatcaacgtatcagtcgggcggcctcgcttatcaaccaccaatttcatattgctgtaagtgtttaaatctttacttattggtttcaaaacccattggttaagccttttaaactcatggtagttattttcaagcattaacatgaacttaaattcatcaaggctaatctctatatttgccttgtgagttttcttttgtgttagttcttttaataaccactcataaatcctcatagagtatttgttttcaaaagacttaacatgttccagattatattttatgaatttttttaactggaaaagataaggcaatatctcttcactaaaaactaattctaatttttcgcttgagaacttggcatagtttgtccactggaaaatctcaaagcctttaaccaaaggattcctgatttccacagttctcgtcatcagctctctggttgctttagctaatacaccataagcattttccctactgatgttcatcatctgagcgtattggttataagtgaacgataccgtccgttctttccttgtagggttttcaatcgtggggttgagtagtgccacacagcataaaattagcttggtttcatgctccgttaagtcatagcgactaatcgctagttcatttgctttgaaaacaactaattcagacatacatctcaattggtctaggtgattttaatcactataccaattgagatgggctagtcaatgataattactagtccttttcctttgagttgtgggtatctgtaaattctgctagacctttgctggaaaacttgtaaattctgctagaccctctgtaaattccgctagacctttgtgtgttttttttgtttatattcaagtggttataatttatagaataaagaaagaataaaaaaagataaaaagaatagatcccagccctgtgtataactcactactttagtcagttccgcagtattacaaaaggatgtcgcaaacgctgtttgctcctctacaaaacagaccttaaaaccctaaaggcttaagtagcaccctcgcaagctcgggcaaatcgctgaatattccttttgtctccgaccatcaggcacctgagtcgctgtctttttcgtgacattcagttcgctgcgctcacggctctggcagtgaatgggggtaaatggcactacaggcgccttttatggattcatgcaaggaaactacccataatacaagaaaagcccgtcacgggcttctcagggcgttttatggcgggtctgctatgtggtgctatctgactttttgctgttcagcagttcctgccctctgattttccagtctgaccacttcggattatcccgtgacaggtcattcagactggctaatgcacccagtaaggcagcggtatcatcaacaggcttacccgtcttactgtcaagaggacatccggtcagataaccgtcatcttcggctactgtctagggcggcggatttgtcctactcaggagagcgttcaccgacaaacaacagataaaacgaaaggcccagtctttcgactgagcctttcgttttatttgatgcactagtgccgatcatattcaataacccttaatataacttcgtataatgtatgctatacgaagttattaggtctgaagaggagtttacgtcccatatgggcgagctcgatatcaaattacgccccgccctgccactcatcgcagtactgttgtaattcattaagcattctgccgacatggaagccatcacagacggcatgatgaacctgaatcgccagcggcatcagcaccttgtcgccttgcgtataatatttgcccatggtgaaaacgggggcgaagaagttgtccatattggccacgtttaaatcaaaactggtgaaactcacccagggattggctgagacgaaaaacatattctcaataaaccctttagggaaataggccaggttttcaccgtaacacgccacatcttgcgaatatatgtgtagaaactgccggaaatcgtcgtggtattcactccagagcgatgaaaacgtttcagtttgctcatggaaaacggtgtaacaagggtgaacactatcccatatcaccagctcaccgtctttcattgccatacgaaattccggatgagcattcatcaggcgggcaagaatgtgaataaaggccggataaaacttgtgcttatttttctttacggtctttaaaaaggccgtaatatccagctgaacggtctggttataggtacattgagcaactgactgaaatgcctcaaaatgttctttacgatgccattgggatatatcaacggtggtatatccagtgatttttttctccattttagcttccttagctcctgaaaatctcgataactcaaaaaatacgcccggtagtgatcttatttcattatggtgaaagttggaacctcttacgtgccgatcaacgtctcattttcgccagatatcgccaagcttaggatccggaacccttaatataacttcgtataatgtatgctatacgaagttattaggtccctcgaagaggttcactagctatctagagcttggactcctgttgatagatccagtaatgacctcagaactccatctggatttgttcagaacgctcggttgccgccgggcgttttttattggtgagaatccaagcccgggaaacgggatcctgatcttgatccgccgcaaagtttgagcgaagtcaataaactctctacccattcagggcaatatctctcttgcaggtgaatgcaacgtcaagcgatggcctacttgcggcctcacacaggaaagtactagatgaaatacctgctgccgaccgctgctgctggtctgctgctcctcgctgcccagccggcgatggccgaagtccagctggttgaaagcggtggaggcctggttcagaccggcggaagcctgcgtctgagctgtgcagcctctggccgcacgtttaacaactacgcgatgggctggtttcgccgtgcaccgggcaaagaacgcgaatttgtggcggcaatcactcgtagcggtgtgagaagcggagtgtcagcgatctatggcgatagcgtgaaagatcgcttcaccatcagccgcgataacgccaagaacaccttgtacttgcagatgaacagcctgaaaccggaagatactgcggtgtatacctgcgccgcaagtgcgatcggcagcggtgcactgcgtcgtttcgaatacgactatagcggtcagggcacacaggtgaccgtgagcagccatcatcaccatcatcattaagatccggggctctggaagatccgcgcgtaccgagttctaattcactggccgtcgttttacaacatacgatgaaggcgataagtcgcgtaagttgctagcccacgcggctcaccttcacgggtgggcctttcttcgcgatccacatg

SEQ ID NO: 108 - DNA, 4834 bp, synthetic construct
  source 1..4834: mol_type = other DNA
catggtcatagctgtttcctttaatgcccatggcgtttaccaatgcttaatcagtgaggcacctatctcagcgatctgtctatttcgttcatccatagttgcctgactccccgtcgtgtagataactacgatacgggagggcttaccatctggccccagtgctgcaatgataccgcgacttccacgctcaccggctccagatttatcagcaataaaccagccagccggaagggccgagcgcagaagtggtcctgcaactttatccgcctccatccagtctattaattgttgccgggaagctagagtaagtagttcgccagttaatagtttgcgcaacgttgttgccattgctacaggcatcgtggtgtcacgctcgtcgtttggtatggcttcattcagctccggttcccaacgatcaaggcgagttacatgatcccccatgttgtgcaaaaaagcggttagctccttcggtcctccgatcgttgtcagaagtaagttggccgcagtgttatcactcatggttatggcagcactgcataattctcttactgtcatgccatccgtaagatgcttttctgtgactggtgagtactcaaccaagtcattctgagaatagtgtatgcggcgaccgagttgctcttgcccggcgtcaatacgggataataccgcgccacatagcagaactttaaaagtgctcatcattggaaaacgttcttcggggcgaaaactctcaaggatcttaccgctgttgagatccagttcgatgtaacccactcgtgcacccaactgatcttcagcatcttttactttcaccagcgtttctgggtgagcaaaaacaggaaggcaaaatgccgcaaaaaagggaataagggcgacacggaaatgttgaatactcatactcttcctttttcaatattattgaagcatttatcagggttattgtctcatgagcggatacatatttgaatgtatttagaaaaataaacaaataggggttccgcgcacatttccccgaaaagtgccacctgacgtctaagaaaccattattatcatgacattaacctataaaaataggcgtatcacgaggcccttaggccaaataggccgttcagatccttccgtatttagccagtatgttctctagtgtggttcgttgtttttgcgtgagccatgagaacgaaccattgagatcatgcttactttgcatgtcactcaaaaattttgcctcaaaactggtgagctgaatttttgcagttaaagcatcgtgtagtgtttttcttagtccgttacgtaggtaggaatctgatgtaatggttgttggtattttgtcaccattcatttttatctggttgttctcaagttcggttacgagatccatttgtctatctagttcaacttggaaaatcaacgtatcagtcgggcggcctcgcttatcaaccaccaatttcatattgctgtaagtgtttaaatctttacttattggtttcaaaacccattggttaagccttttaaactcatggtagttattttcaagcattaacatgaacttaaattcatcaaggctaatctctatatttgccttgtgagttttcttttgtgttagttcttttaataaccactcataaatcctcatagagtatttgttttcaaaagacttaacatgttccagattatattttatgaatttttttaactggaaaagataaggcaatatctcttcactaaaaactaattctaatttttcgcttgagaacttggcatagtttgtccactggaaaatctcaaagcctttaaccaaaggattcctgatttccacagttctcgtcatcagctctctggttgctttagctaatacaccataagcattttccctactgatgttcatcatctgagcgtattggttataagtgaacgataccgtccgttctttccttgtagggttttcaatcgtggggttgagtagtgccacacagcataaaattagcttggtttcatgctccgttaagtcatagcgactaatcgctagttcatttgctttgaaaacaactaattcagacatacatctcaattggtctaggtgattttaatcactataccaattgagatgggctagtcaatgataattactagtccttttcctttgagttgtgggtatctgtaaattctgctagacctttgctggaaaacttgtaaattctgctagaccctctgtaaattccgctagacctttgtgtgttttttttgtttatattcaagtggttataatttatagaataaagaaagaataaaaaaagataaaaagaatagatcccagccctgtgtataactcactactttagtcagttccgcagtattacaaaaggatgtcgcaaacgctgtttgctcctctacaaaacagaccttaaaaccctaaaggcttaagtagcaccctcgcaagctcgggcaaatcgctgaatattccttttgtctccgaccatcaggcacctgagtcgctgtctttttcgtgacattcagttcgctgcgctcacggctctggcagtgaatgggggtaaatggcactacaggcgccttttatggattcatgcaaggaaactacccataatacaagaaaagcccgtcacgggcttctcagggcgttttatggcgggtctgctatgtggtgctatctgactttttgctgttcagcagttcctgccctctgattttccagtctgaccacttcggattatcccgtgacaggtcattcagactggctaatgcacccagtaaggcagcggtatcatcaacaggcttacccgtcttactgtcaagaggacatccggtcagataaccgtcatcttcggctactgtctagggcggcggatttgtcctactcaggagagcgttcaccgacaaacaacagataaaacgaaaggcccagtctttcgactgagcctttcgttttatttgatgcactagtgccgatcatattcaataacccttaatataacttcgtataatgtatgctatacgaagttattaggtctgaagaggagtttacgtcccatatgggcgagctcgatatcaaattacgccccgccctgccactcatcgcagtactgttgtaattcattaagcattctgccgacatggaagccatcacagacggcatgatgaacctgaatcgccagcggcatcagcaccttgtcgccttgcgtataatatttgcccatggtgaaaacgggggcgaagaagttgtccatattggccacgtttaaatcaaaactggtgaaactcacccagggattggctgagacgaaaaacatattctcaataaaccctttagggaaataggccaggttttcaccgtaacacgccacatcttgcgaatatatgtgtagaaactgccggaaatcgtcgtggtattcactccagagcgatgaaaacgtttcagtttgctcatggaaaacggtgtaacaagggtgaacactatcccatatcaccagctcaccgtctttcattgccatacgaaattccggatgagcattcatcaggcgggcaagaatgtgaataaaggccggataaaacttgtgcttatttttctttacggtctttaaaaaggccgtaatatccagctgaacggtctggttataggtacattgagcaactgactgaaatgcctcaaaatgttctttacgatgccattgggatatatcaacggtggtatatccagtgatttttttctccattttagcttccttagctcctgaaaatctcgataactcaaaaaatacgcccggtagtgatcttatttcattatggtgaaagttggaacctcttacgtgccgatcaacgtctcattttcgccagatatcgccaagcttaggatccggaacccttaatataacttcgtataatgtatgctatacgaagttattaggtccctcgaagaggttcactagctatctagagcttggactcctgttgatagatccagtaatgacctcagaactccatctggatttgttcagaacgctcggttgccgccgggcgttttttattggtgagaatccaagcccgggaaacgggatcctgatcttgatccgccgcaaagtttgagcgaagtcaataaactctctacccattcagggcaatatctctcttgcaggtgaatgcaacgtcaagcgatggcctacttgcggcctcacacaggaaagtactagatgaaatacctgctgccgaccgctgctgctggtctgctgctcctcgctgcccagccggcgatggcccaggttcagctgcaagaaagcggaggtggtctggttcagccgggaggtagcttacgcctgtcatgcgcagcaagcggtcgtacctttagcagctatgcgatgggctggtttcgtcaggcacctggcaaagaacgcgaatttgtggcggcaattcgctggtcaggcggctatacctactacaccgatagcgtgaaaggccgctttaccattagccgcgataacgccaagaccaccgtgtacctgcaaatgaacagcctgaaaccggaagataccgcagtgtactactgcgcagcgacctatctgagcagcgattatagccgctatgccttaccgcagcgtccgctggattacgactattggggccaaggtacgcaggttaccgttagcagcgcagcagcgcatcatcaccatcatcattaagatccggggctctggaagatccgcgcgtaccgagttctaattcactggccgtcgttttacaacatacgatgaaggcgataagtcgcgtaagttgctagcccacgcggctcaccttcacgggtgggcctttcttcgcgatccacatg

SEQ ID NO: 109 - DNA, 4798 bp, synthetic construct
  source 1..4798: mol_type = other DNA
catggtcatagctgtttcctttaatgcccatggcgtttaccaatgcttaatcagtgaggcacctatctcagcgatctgtctatttcgttcatccatagttgcctgactccccgtcgtgtagataactacgatacgggagggcttaccatctggccccagtgctgcaatgataccgcgacttccacgctcaccggctccagatttatcagcaataaaccagccagccggaagggccgagcgcagaagtggtcctgcaactttatccgcctccatccagtctattaattgttgccgggaagctagagtaagtagttcgccagttaatagtttgcgcaacgttgttgccattgctacaggcatcgtggtgtcacgctcgtcgtttggtatggcttcattcagctccggttcccaacgatcaaggcgagttacatgatcccccatgttgtgcaaaaaagcggttagctccttcggtcctccgatcgttgtcagaagtaagttggccgcagtgttatcactcatggttatggcagcactgcataattctcttactgtcatgccatccgtaagatgcttttctgtgactggtgagtactcaaccaagtcattctgagaatagtgtatgcggcgaccgagttgctcttgcccggcgtcaatacgggataataccgcgccacatagcagaactttaaaagtgctcatcattggaaaacgttcttcggggcgaaaactctcaaggatcttaccgctgttgagatccagttcgatgtaacccactcgtgcacccaactgatcttcagcatcttttactttcaccagcgtttctgggtgagcaaaaacaggaaggcaaaatgccgcaaaaaagggaataagggcgacacggaaatgttgaatactcatactcttcctttttcaatattattgaagcatttatcagggttattgtctcatgagcggatacatatttgaatgtatttagaaaaataaacaaataggggttccgcgcacatttccccgaaaagtgccacctgacgtctaagaaaccattattatcatgacattaacctataaaaataggcgtatcacgaggcccttaggccaaataggccgttcagatccttccgtatttagccagtatgttctctagtgtggttcgttgtttttgcgtgagccatgagaacgaaccattgagatcatgcttactttgcatgtcactcaaaaattttgcctcaaaactggtgagctgaatttttgcagttaaagcatcgtgtagtgtttttcttagtccgttacgtaggtaggaatctgatgtaatggttgttggtattttgtcaccattcatttttatctggttgttctcaagttcggttacgagatccatttgtctatctagttcaacttggaaaatcaacgtatcagtcgggcggcctcgcttatcaaccaccaatttcatattgctgtaagtgtttaaatctttacttattggtttcaaaacccattggttaagccttttaaactcatggtagttattttcaagcattaacatgaacttaaattcatcaaggctaatctctatatttgccttgtgagttttcttttgtgttagttcttttaataaccactcataaatcctcatagagtatttgttttcaaaagacttaacatgttccagattatattttatgaatttttttaactggaaaagataaggcaatatctcttcactaaaaactaattctaatttttcgcttgagaacttggcatagtttgtccactggaaaatctcaaagcctttaaccaaaggattcctgatttccacagttctcgtcatcagctctctggttgctttagctaatacaccataagcattttccctactgatgttcatcatctgagcgtattggttataagtgaacgataccgtccgttctttccttgtagggttttcaatcgtggggttgagtagtgccacacagcataaaattagcttggtttcatgctccgttaagtcatagcgactaatcgctagttcatttgctttgaaaacaactaattcagacatacatctcaattggtctaggtgattttaatcactataccaattgagatgggctagtcaatgataattactagtccttttcctttgagttgtgggtatctgtaaattctgctagacctttgctggaaaacttgtaaattctgctagaccctctgtaaattccgctagacctttgtgtgttttttttgtttatattcaagtggttataatttatagaataaagaaagaataaaaaaagataaaaagaatagatcccagccctgtgtataactcactactttagtcagttccgcagtattacaaaaggatgtcgcaaacgctgtttgctcctctacaaaacagaccttaaaaccctaaaggcttaagtagcaccctcgcaagctcgggcaaatcgctgaatattccttttgtctccgaccatcaggcacctgagtcgctgtctttttcgtgacattcagttcgctgcgctcacggctctggcagtgaatgggggtaaatggcactacaggcgccttttatggattcatgcaaggaaactacccataatacaagaaaagcccgtcacgggcttctcagggcgttttatggcgggtctgctatgtggtgctatctgactttttgctgttcagcagttcctgccctctgattttccagtctgaccacttcggattatcccgtgacaggtcattcagactggctaatgcacccagtaaggcagcggtatcatcaacaggcttacccgtcttactgtcaagaggacatccggtcagataaccgtcatcttcggctactgtctagggcggcggatttgtcctactcaggagagcgttcaccgacaaacaacagataaaacgaaaggcccagtctttcgactgagcctttcgttttatttgatgcactagtgccgatcatattcaataacccttaatataacttcgtataatgtatgctatacgaagttattaggtctgaagaggagtttacgtcccatatgggcgagctcgatatcaaattacgccccgccctgccactcatcgcagtactgttgtaattcattaagcattctgccgacatggaagccatcacagacggcatgatgaacctgaatcgccagcggcatcagcaccttgtcgccttgcgtataatatttgcccatggtgaaaacgggggcgaagaagttgtccatattggccacgtttaaatcaaaactggtgaaactcacccagggattggctgagacgaaaaacatattctcaataaaccctttagggaaataggccaggttttcaccgtaacacgccacatcttgcgaatatatgtgtagaaactgccggaaatcgtcgtggtattcactccagagcgatgaaaacgtttcagtttgctcatggaaaacggtgtaacaagggtgaacactatcccatatcaccagctcaccgtctttcattgccatacgaaattccggatgagcattcatcaggcgggcaagaatgtgaataaaggccggataaaacttgtgcttatttttctttacggtctttaaaaaggccgtaatatccagctgaacggtctggttataggtacattgagcaactgactgaaatgcctcaaaatgttctttacgatgccattgggatatatcaacggtggtatatccagtgatttttttctccattttagcttccttagctcctgaaaatctcgataactcaaaaaatacgcccggtagtgatcttatttcattatggtgaaagttggaacctcttacgtgccgatcaacgtctcattttcgccagatatcgccaagcttaggatccggaacccttaatataacttcgtataatgtatgctatacgaagttattaggtccctcgaagaggttcactagctatctagagcttggactcctgttgatagatccagtaatgacctcagaactccatctggatttgttcagaacgctcggttgccgccgggcgttttttattggtgagaatccaagcccgggaaacgggatcctgatcttgatccgccgcaaagtttgagcgaagtcaataaactctctacccattcagggcaatatctctcttgcaggtgaatgcaacgtcaagcgatggcctacttgcggcctcacacaggaaagtactagatgaaatacctgctgccgaccgctgctgctggtctgctgctcctcgctgcccagccggcgatggccggcggtggcagcgttcaggcaggtggcagcctgaaactgagctgcgaagccagcctgcctagcacgaccacgccgtatagcatggcctggtttcgtcaggcgcctggacgtgaaagagaagcggtggccaccatcagcgcaagaggtggcactaaactgtacagcgattctgtgcgcgaacgcttcacgattagccgtgataaccgcaagaacacggtctacctgaagatggatcatctgaacaccgatgataccgccatctactattgcgccgcaacgggcagcattctgtttaatagccgtccattcgcggaaagcacgtatccgttctggggtcagggtactctggtcacggtgagcagccatcatcaccatcatcattaagatccggggctctggaagatccgcgcgtaccgagttctaattcactggccgtcgttttacaacatacgatgaaggcgataagtcgcgtaagttgctagcccacgcggctcaccttcacgggtgggcctttcttcgcgatccacatg

SEQ ID NO: 110 - DNA, 4787 bp, synthetic construct
  source 1..4787: mol_type = other DNA
catggtcatagctgtttcctttaatgcccatggcgtttaccaatgcttaatcagtgaggcacctatctcagcgatctgtctatttcgttcatccatagttgcctgactccccgtcgtgtagataactacgatacgggagggcttaccatctggccccagtgctgcaatgataccgcgacttccacgctcaccggctccagatttatcagcaataaaccagccagccggaagggccgagcgcagaagtggtcctgcaactttatccgcctccatccagtctattaattgttgccgggaagctagagtaagtagttcgccagttaatagtttgcgcaacgttgttgccattgctacaggcatcgtggtgtcacgctcgtcgtttggtatggcttcattcagctccggttcccaacgatcaaggcgagttacatgatcccccatgttgtgcaaaaaagcggttagctccttcggtcctccgatcgttgtcagaagtaagttggccgcagtgttatcactcatggttatggcagcactgcataattctcttactgtcatgccatccgtaagatgcttttctgtgactggtgagtactcaaccaagtcattctgagaatagtgtatgcggcgaccgagttgctcttgcccggcgtcaatacgggataataccgcgccacatagcagaactttaaaagtgctcatcattggaaaacgttcttcggggcgaaaactctcaaggatcttaccgctgttgagatccagttcgatgtaacccactcgtgcacccaactgatcttcagcatcttttactttcaccagcgtttctgggtgagcaaaaacaggaaggcaaaatgccgcaaaaaagggaataagggcgacacggaaatgttgaatactcatactcttcctttttcaatattattgaagcatttatcagggttattgtctcatgagcggatacatatttgaatgtatttagaaaaataaacaaataggggttccgcgcacatttccccgaaaagtgccacctgacgtctaagaaaccattattatcatgacattaacctataaaaataggcgtatcacgaggcccttaggccaaataggccgttcagatccttccgtatttagccagtatgttctctagtgtggttcgttgtttttgcgtgagccatgagaacgaaccattgagatcatgcttactttgcatgtcactcaaaaattttgcctcaaaactggtgagctgaatttttgcagttaaagcatcgtgtagtgtttttcttagtccgttacgtaggtaggaatctgatgtaatggttgttggtattttgtcaccattcatttttatctggttgttctcaagttcggttacgagatccatttgtctatctagttcaacttggaaaatcaacgtatcagtcgggcggcctcgcttatcaaccaccaatttcatattgctgtaagtgtttaaatctttacttattggtttcaaaacccattggttaagccttttaaactcatggtagttattttcaagcattaacatgaacttaaattcatcaaggctaatctctatatttgccttgtgagttttcttttgtgttagttcttttaataaccactcataaatcctcatagagtatttgttttcaaaagacttaacatgttccagattatattttatgaatttttttaactggaaaagataaggcaatatctcttcactaaaaactaattctaatttttcgcttgagaacttggcatagtttgtccactggaaaatctcaaagcctttaaccaaaggattcctgatttccacagttctcgtcatcagctctctggttgctttagctaatacaccataagcattttccctactgatgttcatcatctgagcgtattggttataagtgaacgataccgtccgttctttccttgtagggttttcaatcgtggggttgagtagtgccacacagcataaaattagcttggtttcatgctccgttaagtcatagcgactaatcgctagttcatttgctttgaaaacaactaattcagacatacatctcaattggtctaggtgattttaatcactataccaattgagatgggctagtcaatgataattactagtccttttcctttgagttgtgggtatctgtaaattctgctagacctttgctggaaaacttgtaaattctgctagaccctctgtaaattccgctagacctttgtgtgttttttttgtttatattcaagtggttataatttatagaataaagaaagaataaaaaaagataaaaagaatagatcccagccctgtgtataactcactactttagtcagttccgcagtattacaaaaggatgtcgcaaacgctgtttgctcctctacaaaacagaccttaaaaccctaaaggcttaagtagcaccctcgcaagctcgggcaaatcgctgaatattccttttgtctccgaccatcaggcacctgagtcgctgtctttttcgtgacattcagttcgctgcgctcacggctctggcagtgaatgggggtaaatggcactacaggcgccttttatggattcatgcaaggaaactacccataatacaagaaaagcccgtcacgggcttctcagggcgttttatggcgggtctgctatgtggtgctatctgactttttgctgttcagcagttcctgccctctgattttccagtctgaccacttcggattatcccgtgacaggtcattcagactggctaatgcacccagtaaggcagcggtatcatcaacaggcttacccgtcttactgtcaagaggacatccggtcagataaccgtcatcttcggctactgtctagggcggcggatttgtcctactcaggagagcgttcaccgacaaacaacagataaaacgaaaggcccagtctttcgactgagcctttcgttttatttgatgcactagtgccgatcatattcaataacccttaatataacttcgtataatgtatgctatacgaagttattaggtctgaagaggagtttacgtcccatatgggcgagctcgatatcaaattacgccccgccctgccactcatcgcagtactgttgtaattcattaagcattctgccgacatggaagccatcacagacggcatgatgaacctgaatcgccagcggcatcagcaccttgtcgccttgcgtataatatttgcccatggtgaaaacgggggcgaagaagttgtccatattggccacgtttaaatcaaaactggtgaaactcacccagggattggctgagacgaaaaacatattctcaataaaccctttagggaaataggccaggttttcaccgtaacacgccacatcttgcgaatatatgtgtagaaactgccggaaatcgtcgtggtattcactccagagcgatgaaaacgtttcagtttgctcatggaaaacggtgtaacaagggtgaacactatcccatatcaccagctcaccgtctttcattgccatacgaaattccggatgagcattcatcaggcgggcaagaatgtgaataaaggccggataaaacttgtgcttatttttctttacggtctttaaaaaggccgtaatatccagctgaacggtctggttataggtacattgagcaactgactgaaatgcctcaaaatgttctttacgatgccattgggatatatcaacggtggtatatccagtgatttttttctccattttagcttccttagctcctgaaaatctcgataactcaaaaaatacgcccggtagtgatcttatttcattatggtgaaagttggaacctcttacgtgccgatcaacgtctcattttcgccagatatcgccaagcttaggatccggaacccttaatataacttcgtataatgtatgctatacgaagttattaggtccctcgaagaggttcactagctatctagagcttggactcctgttgatagatccagtaatgacctcagaactccatctggatttgttcagaacgctcggttgccgccgggcgttttttattggtgagaatccaagcccgggaaacgggatcctgatcttgatccgccgcaaagtttgagcgaagtcaataaactctctacccattcagggcaatatctctcttgcaggtgaatgcaacgtcaagcgatggcctacttgcggcctcacacaggaaagtactagatgaaatacctgctgccgaccgctgctgctggtctgctgctcctcgctgcccagccggcgatggccggcggtggcacggtacaggctggcggtagcctgaaactgagctgcgccgcgagaggttggcgctttagcggctattgcgtagcctggtttcgtcaagcaccgggcaaagaacgcgaagcggtagcgatcattccgggtgctggcgtgatgtataccgatgattctgtgaaaggccgtttcacctattcgcgcgataatgtgaagaacaccgttagtctgcaaatgaacagcctggaaccggaagataccgcaacgtactactgcgctgtggattgggcatacagccatagctgtccgaagaacacggaagattaccgttattggggccagggcacgcaggtgaccgtgtcatcacatcatcaccatcatcattaagatccggctctggaagatccgcgcgtaccgagttctaattcactggccgtcgttttacaacatacgatgaaggcgataagtcgcgtaagttgctagcccacgcggctcaccttcacgggtgggcctttcttcgcgatccacatg

SEQ ID NO: 111 - DNA, 5842 bp, synthetic construct
  source 1..5842: mol_type = other DNA
catggtcatagctgtttcctttaatgcccatggcgtttaccaatgcttaatcagtgaggcacctatctcagcgatctgtctatttcgttcatccatagttgcctgactccccgtcgtgtagataactacgatacgggagggcttaccatctggccccagtgctgcaatgataccgcgacttccacgctcaccggctccagatttatcagcaataaaccagccagccggaagggccgagcgcagaagtggtcctgcaactttatccgcctccatccagtctattaattgttgccgggaagctagagtaagtagttcgccagttaatagtttgcgcaacgttgttgccattgctacaggcatcgtggtgtcacgctcgtcgtttggtatggcttcattcagctccggttcccaacgatcaaggcgagttacatgatcccccatgttgtgcaaaaaagcggttagctccttcggtcctccgatcgttgtcagaagtaagttggccgcagtgttatcactcatggttatggcagcactgcataattctcttactgtcatgccatccgtaagatgcttttctgtgactggtgagtactcaaccaagtcattctgagaatagtgtatgcggcgaccgagttgctcttgcccggcgtcaatacgggataataccgcgccacatagcagaactttaaaagtgctcatcattggaaaacgttcttcggggcgaaaactctcaaggatcttaccgctgttgagatccagttcgatgtaacccactcgtgcacccaactgatcttcagcatcttttactttcaccagcgtttctgggtgagcaaaaacaggaaggcaaaatgccgcaaaaaagggaataagggcgacacggaaatgttgaatactcatactcttcctttttcaatattattgaagcatttatcagggttattgtctcatgagcggatacatatttgaatgtatttagaaaaataaacaaataggggttccgcgcacatttccccgaaaagtgccacctgacgtctaagaaaccattattatcatgacattaacctataaaaataggcgtatcacgaggcccttaggccaaataggccgttcagatccttccgtatttagccagtatgttctctagtgtggttcgttgtttttgcgtgagccatgagaacgaaccattgagatcatgcttactttgcatgtcactcaaaaattttgcctcaaaactggtgagctgaatttttgcagttaaagcatcgtgtagtgtttttcttagtccgttacgtaggtaggaatctgatgtaatggttgttggtattttgtcaccattcatttttatctggttgttctcaagttcggttacgagatccatttgtctatctagttcaacttggaaaatcaacgtatcagtcgggcggcctcgcttatcaaccaccaatttcatattgctgtaagtgtttaaatctttacttattggtttcaaaacccattggttaagccttttaaactcatggtagttattttcaagcattaacatgaacttaaattcatcaaggctaatctctatatttgccttgtgagttttcttttgtgttagttcttttaataaccactcataaatcctcatagagtatttgttttcaaaagacttaacatgttccagattatattttatgaatttttttaactggaaaagataaggcaatatctcttcactaaaaactaattctaatttttcgcttgagaacttggcatagtttgtccactggaaaatctcaaagcctttaaccaaaggattcctgatttccacagttctcgtcatcagctctctggttgctttagctaatacaccataagcattttccctactgatgttcatcatctgagcgtattggttataagtgaacgataccgtccgttctttccttgtagggttttcaatcgtggggttgagtagtgccacacagcataaaattagcttggtttcatgctccgttaagtcatagcgactaatcgctagttcatttgctttgaaaacaactaattcagacatacatctcaattggtctaggtgattttaatcactataccaattgagatgggctagtcaatgataattactagtccttttcctttgagttgtgggtatctgtaaattctgctagacctttgctggaaaacttgtaaattctgctagaccctctgtaaattccgctagacctttgtgtgttttttttgtttatattcaagtggttataatttatagaataaagaaagaataaaaaaagataaaaagaatagatcccagccctgtgtataactcactactttagtcagttccgcagtattacaaaaggatgtcgcaaacgctgtttgctcctctacaaaacagaccttaaaaccctaaaggcttaagtagcaccctcgcaagctcgggcaaatcgctgaatattccttttgtctccgaccatcaggcacctgagtcgctgtctttttcgtgacattcagttcgctgcgctcacggctctggcagtgaatgggggtaaatggcactacaggcgccttttatggattcatgcaaggaaactacccataatacaagaaaagcccgtcacgggcttctcagggcgttttatggcgggtctgctatgtggtgctatctgactttttgctgttcagcagttcctgccctctgattttccagtctgaccacttcggattatcccgtgacaggtcattcagactggctaatgcacccagtaaggcagcggtatcatcaacaggcttacccgtcttactgtcaagaggacatccggtcagataaccgtcatcttcggctactgtctagggcggcggatttgtcctactcaggagagcgttcaccgacaaacaacagataaaacgaaaggcccagtctttcgactgagcctttcgttttatttgatgcactagtgccgatcatattcaataacccttaatataacttcgtataatgtatgctatacgaagttattaggtctgaagaggagtttacgtcccatatgggcgagctcgatatcaaattacgccccgccctgccactcatcgcagtactgttgtaattcattaagcattctgccgacatggaagccatcacagacggcatgatgaacctgaatcgccagcggcatcagcaccttgtcgccttgcgtataatatttgcccatggtgaaaacgggggcgaagaagttgtccatattggccacgtttaaatcaaaactggtgaaactcacccagggattggctgagacgaaaaacatattctcaataaaccctttagggaaataggccaggttttcaccgtaacacgccacatcttgcgaatatatgtgtagaaactgccggaaatcgtcgtggtattcactccagagcgatgaaaacgtttcagtttgctcatggaaaacggtgtaacaagggtgaacactatcccatatcaccagctcaccgtctttcattgccatacgaaattccggatgagcattcatcaggcgggcaagaatgtgaataaaggccggataaaacttgtgcttatttttctttacggtctttaaaaaggccgtaatatccagctgaacggtctggttataggtacattgagcaactgactgaaatgcctcaaaatgttctttacgatgccattgggatatatcaacggtggtatatccagtgatttttttctccattttagcttccttagctcctgaaaatctcgataactcaaaaaatacgcccggtagtgatcttatttcattatggtgaaagttggaacctcttacgtgccgatcaacgtctcattttcgccagatatcgccaagcttaggatccggaacccttaatataacttcgtataatgtatgctatacgaagttattaggtccctcgaagaggttcactagctatctagagcttggactcctgttgatagatccagtaatgacctcagaactccatctggatttgttcagaacgctcggttgccgccgggcgttttttattggtgagaatccaagcccgggaaacgggatcctgatcttgatccgccgcaaagtttgagcgaagtcaataaactctctacccattcagggcaatatctctcttgcaggtgaatgcaacgtcaagcgatggcctacttgcggcctcacacaggaaagtactagatgaaatacctgctgccgaccgctgctgctggtctgctgctcctcgctgcccagccggcgatggccgaagtgcaactggtggaaagcggtggaggccttgttcagaccggcggcagcctgcgtctgtcatgcgctgcaagcggctttacgttcagcagctacgcgatgagctgggtgcgccaggcaccgggcaaaggcttggaatgggttagcggcatcaagtcaagcggcgatagcaccagatatgccggaagcgttaaaggccgctttaccatttcacgcgataacgccaagaacatgctgtatctgcaaatgtatagcctgaaaccggaagataccgcagtgtattactgcgccaagagccgcgtgagtcgcacgggtctgtatacctatgacaaccgtggtcagggcacgcaggtgactgtgtcaagccctgaaggtggtagcctggcggcactgaccgcacaccaagcatgtcatctgccactggaaacctttacccgtcatcgtcagccgcgtggctgggaacaactggaacaatgtggatatccggtgcagagactggtcgcattatatctggcagcacgtctgagttggaatcaggttgatcaagttattcgtaacgcacttgcctcaccgggtagcggtggtgatttaggtgaggcaattcgtgaacaacctgaacaggcacgcttagcattaacccttgcagccgcagaaagtgaaagatttgtgcgtcagggtactggtaatgatgaggccggtgcagcaaatgggccggcagacagcggagatgcattattagagagaaattatcctaccggcgcagaatttctgggtgatgggggtgatgttagtttttcaacacgcgggacacagaattggaccgtggaacgtttactgcaggcacatcgtcagctggaagaacgcggttatgtttttgttggttatcatgggacgtttctggaggcagcacagagcattgtctttggcggtgtgcgggcgcgtagccaggatcttgatgcaatttggcgtggtttttatattgcgggtgatcctgcgctggcgtatggatatgcgcaggatcaggagccggatgcgcgtggtcgtattcgtaatggtgccctgctgcgggtttatgttccgcgtagctcactgccggggttttatagaacaagcttaacactggctgcgccggaagcagcaggtgaagttgaacgtctgattggccatccgctgccgttacgtttagatgcaattactggtccggaagaagaaggtggtcgcctggaaaccattctgggttggccgctggcagaaagaaccgtggttataccttccgcaataccgaccgatcctcggaatgtggggggtgatttagatcctagcagcattcctgataaagaacaggcaatttctgctctgcctgattatgcatcacagccgggtaaaccgccgcgtgaagatttaaagcatcatcaccatcatcattaagatccggggctctggaagatccgcgcgtaccgagttctaattcactggccgtcgttttacaacatacgatgaaggcgataagtcgcgtaagttgctagcccacgcggctcaccttcacgggtgggcctttcttcgcgatccacatg

SEQ ID NO: 112 - DNA, 5860 bp, synthetic construct
  source 1..5860: mol_type = other DNA
catggtcatagctgtttcctttaatgcccatggcgtttaccaatgcttaatcagtgaggcacctatctcagcgatctgtctatttcgttcatccatagttgcctgactccccgtcgtgtagataactacgatacgggagggcttaccatctggccccagtgctgcaatgataccgcgacttccacgctcaccggctccagatttatcagcaataaaccagccagccggaagggccgagcgcagaagtggtcctgcaactttatccgcctccatccagtctattaattgttgccgggaagctagagtaagtagttcgccagttaatagtttgcgcaacgttgttgccattgctacaggcatcgtggtgtcacgctcgtcgtttggtatggcttcattcagctccggttcccaacgatcaaggcgagttacatgatcccccatgttgtgcaaaaaagcggttagctccttcggtcctccgatcgttgtcagaagtaagttggccgcagtgttatcactcatggttatggcagcactgcataattctcttactgtcatgccatccgtaagatgcttttctgtgactggtgagtactcaaccaagtcattctgagaatagtgtatgcggcgaccgagttgctcttgcccggcgtcaatacgggataataccgcgccacatagcagaactttaaaagtgctcatcattggaaaacgttcttcggggcgaaaactctcaaggatcttaccgctgttgagatccagttcgatgtaacccactcgtgcacccaactgatcttcagcatcttttactttcaccagcgtttctgggtgagcaaaaacaggaaggcaaaatgccgcaaaaaagggaataagggcgacacggaaatgttgaatactcatactcttcctttttcaatattattgaagcatttatcagggttattgtctcatgagcggatacatatttgaatgtatttagaaaaataaacaaataggggttccgcgcacatttccccgaaaagtgccacctgacgtctaagaaaccattattatcatgacattaacctataaaaataggcgtatcacgaggcccttaggccaaataggccgttcagatccttccgtatttagccagtatgttctctagtgtggttcgttgtttttgcgtgagccatgagaacgaaccattgagatcatgcttactttgcatgtcactcaaaaattttgcctcaaaactggtgagctgaatttttgcagttaaagcatcgtgtagtgtttttcttagtccgttacgtaggtaggaatctgatgtaatggttgttggtattttgtcaccattcatttttatctggttgttctcaagttcggttacgagatccatttgtctatctagttcaacttggaaaatcaacgtatcagtcgggcggcctcgcttatcaaccaccaatttcatattgctgtaagtgtttaaatctttacttattggtttcaaaacccattggttaagccttttaaactcatggtagttattttcaagcattaacatgaacttaaattcatcaaggctaatctctatatttgccttgtgagttttcttttgtgttagttcttttaataaccactcataaatcctcatagagtatttgttttcaaaagacttaacatgttccagattatattttatgaatttttttaactggaaaagataaggcaatatctcttcactaaaaactaattctaatttttcgcttgagaacttggcatagtttgtccactggaaaatctcaaagcctttaaccaaaggattcctgatttccacagttctcgtcatcagctctctggttgctttagctaatacaccataagcattttccctactgatgttcatcatctgagcgtattggttataagtgaacgataccgtccgttctttccttgtagggttttcaatcgtggggttgagtagtgccacacagcataaaattagcttggtttcatgctccgttaagtcatagcgactaatcgctagttcatttgctttgaaaacaactaattcagacatacatctcaattggtctaggtgattttaatcactataccaattgagatgggctagtcaatgataattactagtccttttcctttgagttgtgggtatctgtaaattctgctagacctttgctggaaaacttgtaaattctgctagaccctctgtaaattccgctagacctttgtgtgttttttttgtttatattcaagtggttataatttatagaataaagaaagaataaaaaaagataaaaagaatagatcccagccctgtgtataactcactactttagtcagttccgcagtattacaaaaggatgtcgcaaacgctgtttgctcctctacaaaacagaccttaaaaccctaaaggcttaagtagcaccctcgcaagctcgggcaaatcgctgaatattccttttgtctccgaccatcaggcacctgagtcgctgtctttttcgtgacattcagttcgctgcgctcacggctctggcagtgaatgggggtaaatggcactacaggcgccttttatggattcatgcaaggaaactacccataatacaagaaaagcccgtcacgggcttctcagggcgttttatggcgggtctgctatgtggtgctatctgactttttgctgttcagcagttcctgccctctgattttccagtctgaccacttcggattatcccgtgacaggtcattcagactggctaatgcacccagtaaggcagcggtatcatcaacaggcttacccgtcttactgtcaagaggacatccggtcagataaccgtcatcttcggctactgtctagggcggcggatttgtcctactcaggagagcgttcaccgacaaacaacagataaaacgaaaggcccagtctttcgactgagcctttcgttttatttgatgcactagtgccgatcatattcaataacccttaatataacttcgtataatgtatgctatacgaagttattaggtctgaagaggagtttacgtcccatatgggcgagctcgatatcaaattacgccccgccctgccactcatcgcagtactgttgtaattcattaagcattctgccgacatggaagccatcacagacggcatgatgaacctgaatcgccagcggcatcagcaccttgtcgccttgcgtataatatttgcccatggtgaaaacgggggcgaagaagttgtccatattggccacgtttaaatcaaaactggtgaaactcacccagggattggctgagacgaaaaacatattctcaataaaccctttagggaaataggccaggttttcaccgtaacacgccacatcttgcgaatatatgtgtagaaactgccggaaatcgtcgtggtattcactccagagcgatgaaaacgtttcagtttgctcatggaaaacggtgtaacaagggtgaacactatcccatatcaccagctcaccgtctttcattgccatacgaaattccggatgagcattcatcaggcgggcaagaatgtgaataaaggccggataaaacttgtgcttatttttctttacggtctttaaaaaggccgtaatatccagctgaacggtctggttataggtacattgagcaactgactgaaatgcctcaaaatgttctttacgatgccattgggatatatcaacggtggtatatccagtgatttttttctccattttagcttccttagctcctgaaaatctcgataactcaaaaaatacgcccggtagtgatcttatttcattatggtgaaagttggaacctcttacgtgccgatcaacgtctcattttcgccagatatcgccaagcttaggatccggaacccttaatataacttcgtataatgtatgctatacgaagttattaggtccctcgaagaggttcactagctatctagagcttggactcctgttgatagatccagtaatgacctcagaactccatctggatttgttcagaacgctcggttgccgccgggcgttttttattggtgagaatccaagcccgggaaacgggatcctgatcttgatccgccgcaaagtttgagcgaagtcaataaactctctacccattcagggcaatatctctcttgcaggtgaatgcaacgtcaagcgatggcctacttgcggcctcacacaggaaagtactagatgaaatacctgctgccgaccgctgctgctggtctgctgctcctcgctgcccagccggcgatggccgaagtccagctggttgaaagcggtggaggcctggttcagaccggcggaagcctgcgtctgagctgtgcagcctctggccgcacgtttaacaactacgcgatgggctggtttcgccgtgcaccgggcaaagaacgcgaatttgtggcggcaatcactcgtagcggtgtgagaagcggagtgtcagcgatctatggcgatagcgtgaaagatcgcttcaccatcagccgcgataacgccaagaacaccttgtacttgcagatgaacagcctgaaaccggaagatactgcggtgtatacctgcgccgcaagtgcgatcggcagcggtgcactgcgtcgtttcgaatacgactatagcggtcagggcacacaggtgaccgtgagcagccctgaaggtggtagcctggcggcactgaccgcacaccaagcatgtcatctgccactggaaacctttacccgtcatcgtcagccgcgtggctgggaacaactggaacaatgtggatatccggtgcagagactggtcgcattatatctggcagcacgtctgagttggaatcaggttgatcaagttattcgtaacgcacttgcctcaccgggtagcggtggtgatttaggtgaggcaattcgtgaacaacctgaacaggcacgcttagcattaacccttgcagccgcagaaagtgaaagatttgtgcgtcagggtactggtaatgatgaggccggtgcagcaaatgggccggcagacagcggagatgcattattagagagaaattatcctaccggcgcagaatttctgggtgatgggggtgatgttagtttttcaacacgcgggacacagaattggaccgtggaacgtttactgcaggcacatcgtcagctggaagaacgcggttatgtttttgttggttatcatgggacgtttctggaggcagcacagagcattgtctttggcggtgtgcgggcgcgtagccaggatcttgatgcaatttggcgtggtttttatattgcgggtgatcctgcgctggcgtatggatatgcgcaggatcaggagccggatgcgcgtggtcgtattcgtaatggtgccctgctgcgggtttatgttccgcgtagctcactgccggggttttatagaacaagcttaacactggctgcgccggaagcagcaggtgaagttgaacgtctgattggccatccgctgccgttacgtttagatgcaattactggtccggaagaagaaggtggtcgcctggaaaccattctgggttggccgctggcagaaagaaccgtggttataccttccgcaataccgaccgatcctcggaatgtggggggtgatttagatcctagcagcattcctgataaagaacaggcaatttctgctctgcctgattatgcatcacagccgggtaaaccgccgcgtgaagatttaaagcatcatcaccatcatcattaagatccggggctctggaagatccgcgcgtaccgagttctaattcactggccgtcgttttacaacatacgatgaaggcgataagtcgcgtaagttgctagcccacgcggctcaccttcacgggtgggcctttcttcgcgatccacatg

SEQ ID NO: 113 - DNA, 5875 bp, synthetic construct
  source 1..5875: mol_type = other DNA
catggtcatagctgtttcctttaatgcccatggcgtttaccaatgcttaatcagtgaggcacctatctcagcgatctgtctatttcgttcatccatagttgcctgactccccgtcgtgtagataactacgatacgggagggcttaccatctggccccagtgctgcaatgataccgcgacttccacgctcaccggctccagatttatcagcaataaaccagccagccggaagggccgagcgcagaagtggtcctgcaactttatccgcctccatccagtctattaattgttgccgggaagctagagtaagtagttcgccagttaatagtttgcgcaacgttgttgccattgctacaggcatcgtggtgtcacgctcgtcgtttggtatggcttcattcagctccggttcccaacgatcaaggcgagttacatgatcccccatgttgtgcaaaaaagcggttagctccttcggtcctccgatcgttgtcagaagtaagttggccgcagtgttatcactcatggttatggcagcactgcataattctcttactgtcatgccatccgtaagatgcttttctgtgactggtgagtactcaaccaagtcattctgagaatagtgtatgcggcgaccgagttgctcttgcccggcgtcaatacgggataataccgcgccacatagcagaactttaaaagtgctcatcattggaaaacgttcttcggggcgaaaactctcaaggatcttaccgctgttgagatccagttcgatgtaacccactcgtgcacccaactgatcttcagcatcttttactttcaccagcgtttctgggtgagcaaaaacaggaaggcaaaatgccgcaaaaaagggaataagggcgacacggaaatgttgaatactcatactcttcctttttcaatattattgaagcatttatcagggttattgtctcatgagcggatacatatttgaatgtatttagaaaaataaacaaataggggttccgcgcacatttccccgaaaagtgccacctgacgtctaagaaaccattattatcatgacattaacctataaaaataggcgtatcacgaggcccttaggccaaataggccgttcagatccttccgtatttagccagtatgttctctagtgtggttcgttgtttttgcgtgagccatgagaacgaaccattgagatcatgcttactttgcatgtcactcaaaaattttgcctcaaaactggtgagctgaatttttgcagttaaagcatcgtgtagtgtttttcttagtccgttacgtaggtaggaatctgatgtaatggttgttggtattttgtcaccattcatttttatctggttgttctcaagttcggttacgagatccatttgtctatctagttcaacttggaaaatcaacgtatcagtcgggcggcctcgcttatcaaccaccaatttcatattgctgtaagtgtttaaatctttacttattggtttcaaaacccattggttaagccttttaaactcatggtagttattttcaagcattaacatgaacttaaattcatcaaggctaatctctatatttgccttgtgagttttcttttgtgttagttcttttaataaccactcataaatcctcatagagtatttgttttcaaaagacttaacatgttccagattatattttatgaatttttttaactggaaaagataaggcaatatctcttcactaaaaactaattctaatttttcgcttgagaacttggcatagtttgtccactggaaaatctcaaagcctttaaccaaaggattcctgatttccacagttctcgtcatcagctctctggttgctttagctaatacaccataagcattttccctactgatgttcatcatctgagcgtattggttataagtgaacgataccgtccgttctttccttgtagggttttcaatcgtggggttgagtagtgccacacagcataaaattagcttggtttcatgctccgttaagtcatagcgactaatcgctagttcatttgctttgaaaacaactaattcagacatacatctcaattggtctaggtgattttaatcactataccaattgagatgggctagtcaatgataattactagtccttttcctttgagttgtgggtatctgtaaattctgctagacctttgctggaaaacttgtaaattctgctagaccctctgtaaattccgctagacctttgtgtgttttttttgtttatattcaagtggttataatttatagaataaagaaagaataaaaaaagataaaaagaatagatcccagccctgtgtataactcactactttagtcagttccgcagtattacaaaaggatgtcgcaaacgctgtttgctcctctacaaaacagaccttaaaaccctaaaggcttaagtagcaccctcgcaagctcgggcaaatcgctgaatattccttttgtctccgaccatcaggcacctgagtcgctgtctttttcgtgacattcagttcgctgcgctcacggctctggcagtgaatgggggtaaatggcactacaggcgccttttatggattcatgcaaggaaactacccataatacaagaaaagcccgtcacgggcttctcagggcgttttatggcgggtctgctatgtggtgctatctgactttttgctgttcagcagttcctgccctctgattttccagtctgaccacttcggattatcccgtgacaggtcattcagactggctaatgcacccagtaaggcagcggtatcatcaacaggcttacccgtcttactgtcaagaggacatccggtcagataaccgtcatcttcggctactgtctagggcggcggatttgtcctactcaggagagcgttcaccgacaaacaacagataaaacgaaaggcccagtctttcgactgagcctttcgttttatttgatgcactagtgccgatcatattcaataacccttaatataacttcgtataatgtatgctatacgaagttattaggtctgaagaggagtttacgtcccatatgggcgagctcgatatcaaattacgccccgccctgccactcatcgcagtactgttgtaattcattaagcattctgccgacatggaagccatcacagacggcatgatgaacctgaatcgccagcggcatcagcaccttgtcgccttgcgtataatatttgcccatggtgaaaacgggggcgaagaagttgtccatattggccacgtttaaatcaaaactggtgaaactcacccagggattggctgagacgaaaaacatattctcaataaaccctttagggaaataggccaggttttcaccgtaacacgccacatcttgcgaatatatgtgtagaaactgccggaaatcgtcgtggtattcactccagagcgatgaaaacgtttcagtttgctcatggaaaacggtgtaacaagggtgaacactatcccatatcaccagctcaccgtctttcattgccatacgaaattccggatgagcattcatcaggcgggcaagaatgtgaataaaggccggataaaacttgtgcttatttttctttacggtctttaaaaaggccgtaatatccagctgaacggtctggttataggtacattgagcaactgactgaaatgcctcaaaatgttctttacgatgccattgggatatatcaacggtggtatatccagtgatttttttctccattttagcttccttagctcctgaaaatctcgataactcaaaaaatacgcccggtagtgatcttatttcattatggtgaaagttggaacctcttacgtgccgatcaacgtctcattttcgccagatatcgccaagcttaggatccggaacccttaatataacttcgtataatgtatgctatacgaagttattaggtccctcgaagaggttcactagctatctagagcttggactcctgttgatagatccagtaatgacctcagaactccatctggatttgttcagaacgctcggttgccgccgggcgttttttattggtgagaatccaagcccgggaaacgggatcctgatcttgatccgccgcaaagtttgagcgaagtcaataaactctctacccattcagggcaatatctctcttgcaggtgaatgcaacgtcaagcgatggcctacttgcggcctcacacaggaaagtactagatgaaatacctgctgccgaccgctgctgctggtctgctgctcctcgctgcccagccggcgatggcccaggttcagctgcaagaaagcggaggtggtctggttcagccgggaggtagcttacgcctgtcatgcgcagcaagcggtcgtacctttagcagctatgcgatgggctggtttcgtcaggcacctggcaaagaacgcgaatttgtggcggcaattcgctggtcaggcggctatacctactacaccgatagcgtgaaaggccgctttaccattagccgcgataacgccaagaccaccgtgtacctgcaaatgaacagcctgaaaccggaagataccgcagtgtactactgcgcagcgacctatctgagcagcgattatagccgctatgccttaccgcagcgtccgctggattacgactattggggccaaggtacgcaggttaccgttagcagcgcagcagcgcctgaaggtggtagcctggcggcactgaccgcacaccaagcatgtcatctgccactggaaacctttacccgtcatcgtcagccgcgtggctgggaacaactggaacaatgtggatatccggtgcagagactggtcgcattatatctggcagcacgtctgagttggaatcaggttgatcaagttattcgtaacgcacttgcctcaccgggtagcggtggtgatttaggtgaggcaattcgtgaacaacctgaacaggcacgcttagcattaacccttgcagccgcagaaagtgaaagatttgtgcgtcagggtactggtaatgatgaggccggtgcagcaaatgggccggcagacagcggagatgcattattagagagaaattatcctaccggcgcagaatttctgggtgatgggggtgatgttagtttttcaacacgcgggacacagaattggaccgtggaacgtttactgcaggcacatcgtcagctggaagaacgcggttatgtttttgttggttatcatgggacgtttctggaggcagcacagagcattgtctttggcggtgtgcgggcgcgtagccaggatcttgatgcaatttggcgtggtttttatattgcgggtgatcctgcgctggcgtatggatatgcgcaggatcaggagccggatgcgcgtggtcgtattcgtaatggtgccctgctgcgggtttatgttccgcgtagctcactgccggggttttatagaacaagcttaacactggctgcgccggaagcagcaggtgaagttgaacgtctgattggccatccgctgccgttacgtttagatgcaattactggtccggaagaagaaggtggtcgcctggaaaccattctgggttggccgctggcagaaagaaccgtggttataccttccgcaataccgaccgatcctcggaatgtggggggtgatttagatcctagcagcattcctgataaagaacaggcaatttctgctctgcctgattatgcatcacagccgggtaaaccgccgcgtgaagatttaaagcatcatcaccatcatcattaagatccggggctctggaagatccgcgcgtaccgagttctaattcactggccgtcgttttacaacatacgatgaaggcgataagtcgcgtaagttgctagcccacgcggctcaccttcacgggtgggcctttcttcgcgatccacatg

SEQ ID NO: 114 - DNA, 5839 bp, synthetic construct
  source 1..5839: mol_type = other DNA
catggtcatagctgtttcctttaatgcccatggcgtttaccaatgcttaatcagtgaggcacctatctcagcgatctgtctatttcgttcatccatagttgcctgactccccgtcgtgtagataactacgatacgggagggcttaccatctggccccagtgctgcaatgataccgcgacttccacgctcaccggctccagatttatcagcaataaaccagccagccggaagggccgagcgcagaagtggtcctgcaactttatccgcctccatccagtctattaattgttgccgggaagctagagtaagtagttcgccagttaatagtttgcgcaacgttgttgccattgctacaggcatcgtggtgtcacgctcgtcgtttggtatggcttcattcagctccggttcccaacgatcaaggcgagttacatgatcccccatgttgtgcaaaaaagcggttagctccttcggtcctccgatcgttgtcagaagtaagttggccgcagtgttatcactcatggttatggcagcactgcataattctcttactgtcatgccatccgtaagatgcttttctgtgactggtgagtactcaaccaagtcattctgagaatagtgtatgcggcgaccgagttgctcttgcccggcgtcaatacgggataataccgcgccacatagcagaactttaaaagtgctcatcattggaaaacgttcttcggggcgaaaactctcaaggatcttaccgctgttgagatccagttcgatgtaacccactcgtgcacccaactgatcttcagcatcttttactttcaccagcgtttctgggtgagcaaaaacaggaaggcaaaatgccgcaaaaaagggaataagggcgacacggaaatgttgaatactcatactcttcctttttcaatattattgaagcatttatcagggttattgtctcatgagcggatacatatttgaatgtatttagaaaaataaacaaataggggttccgcgcacatttccccgaaaagtgccacctgacgtctaagaaaccattattatcatgacattaacctataaaaataggcgtatcacgaggcccttaggccaaataggccgttcagatccttccgtatttagccagtatgttctctagtgtggttcgttgtttttgcgtgagccatgagaacgaaccattgagatcatgcttactttgcatgtcactcaaaaattttgcctcaaaactggtgagctgaatttttgcagttaaagcatcgtgtagtgtttttcttagtccgttacgtaggtaggaatctgatgtaatggttgttggtattttgtcaccattcatttttatctggttgttctcaagttcggttacgagatccatttgtctatctagttcaacttggaaaatcaacgtatcagtcgggcggcctcgcttatcaaccaccaatttcatattgctgtaagtgtttaaatctttacttattggtttcaaaacccattggttaagccttttaaactcatggtagttattttcaagcattaacatgaacttaaattcatcaaggctaatctctatatttgccttgtgagttttcttttgtgttagttcttttaataaccactcataaatcctcatagagtatttgttttcaaaagacttaacatgttccagattatattttatgaatttttttaactggaaaagataaggcaatatctcttcactaaaaactaattctaatttttcgcttgagaacttggcatagtttgtccactggaaaatctcaaagcctttaaccaaaggattcctgatttccacagttctcgtcatcagctctctggttgctttagctaatacaccataagcattttccctactgatgttcatcatctgagcgtattggttataagtgaacgataccgtccgttctttccttgtagggttttcaatcgtggggttgagtagtgccacacagcataaaattagcttggtttcatgctccgttaagtcatagcgactaatcgctagttcatttgctttgaaaacaactaattcagacatacatctcaattggtctaggtgattttaatcactataccaattgagatgggctagtcaatgataattactagtccttttcctttgagttgtgggtatctgtaaattctgctagacctttgctggaaaacttgtaaattctgctagaccctctgtaaattccgctagacctttgtgtgttttttttgtttatattcaagtggttataatttatagaataaagaaagaataaaaaaagataaaaagaatagatcccagccctgtgtataactcactactttagtcagttccgcagtattacaaaaggatgtcgcaaacgctgtttgctcctctacaaaacagaccttaaaaccctaaaggcttaagtagcaccctcgcaagctcgggcaaatcgctgaatattccttttgtctccgaccatcaggcacctgagtcgctgtctttttcgtgacattcagttcgctgcgctcacggctctggcagtgaatgggggtaaatggcactacaggcgccttttatggattcatgcaaggaaactacccataatacaagaaaagcccgtcacgggcttctcagggcgttttatggcgggtctgctatgtggtgctatctgactttttgctgttcagcagttcctgccctctgattttccagtctgaccacttcggattatcccgtgacaggtcattcagactggctaatgcacccagtaaggcagcggtatcatcaacaggcttacccgtcttactgtcaagaggacatccggtcagataaccgtcatcttcggctactgtctagggcggcggatttgtcctactcaggagagcgttcaccgacaaacaacagataaaacgaaaggcccagtctttcgactgagcctttcgttttatttgatgcactagtgccgatcatattcaataacccttaatataacttcgtataatgtatgctatacgaagttattaggtctgaagaggagtttacgtcccatatgggcgagctcgatatcaaattacgccccgccctgccactcatcgcagtactgttgtaattcattaagcattctgccgacatggaagccatcacagacggcatgatgaacctgaatcgccagcggcatcagcaccttgtcgccttgcgtataatatttgcccatggtgaaaacgggggcgaagaagttgtccatattggccacgtttaaatcaaaactggtgaaactcacccagggattggctgagacgaaaaacatattctcaataaaccctttagggaaataggccaggttttcaccgtaacacgccacatcttgcgaatatatgtgtagaaactgccggaaatcgtcgtggtattcactccagagcgatgaaaacgtttcagtttgctcatggaaaacggtgtaacaagggtgaacactatcccatatcaccagctcaccgtctttcattgccatacgaaattccggatgagcattcatcaggcgggcaagaatgtgaataaaggccggataaaacttgtgcttatttttctttacggtctttaaaaaggccgtaatatccagctgaacggtctggttataggtacattgagcaactgactgaaatgcctcaaaatgttctttacgatgccattgggatatatcaacggtggtatatccagtgatttttttctccattttagcttccttagctcctgaaaatctcgataactcaaaaaatacgcccggtagtgatcttatttcattatggtgaaagttggaacctcttacgtgccgatcaacgtctcattttcgccagatatcgccaagcttaggatccggaacccttaatataacttcgtataatgtatgctatacgaagttattaggtccctcgaagaggttcactagctatctagagcttggactcctgttgatagatccagtaatgacctcagaactccatctggatttgttcagaacgctcggttgccgccgggcgttttttattggtgagaatccaagcccgggaaacgggatcctgatcttgatccgccgcaaagtttgagcgaagtcaataaactctctacccattcagggcaatatctctcttgcaggtgaatgcaacgtcaagcgatggcctacttgcggcctcacacaggaaagtactagatgaaatacctgctgccgaccgctgctgctggtctgctgctcctcgctgcccagccggcgatggccggcggtggcagcgttcaggcaggtggcagcctgaaactgagctgcgaagccagcctgcctagcacgaccacgccgtatagcatggcctggtttcgtcaggcgcctggacgtgaaagagaagcggtggccaccatcagcgcaagaggtggcactaaactgtacagcgattctgtgcgcgaacgcttcacgattagccgtgataaccgcaagaacacggtctacctgaagatggatcatctgaacaccgatgataccgccatctactattgcgccgcaacgggcagcattctgtttaatagccgtccattcgcggaaagcacgtatccgttctggggtcagggtactctggtcacggtgagcagccctgaaggtggtagcctggcggcactgaccgcacaccaagcatgtcatctgccactggaaacctttacccgtcatcgtcagccgcgtggctgggaacaactggaacaatgtggatatccggtgcagagactggtcgcattatatctggcagcacgtctgagttggaatcaggttgatcaagttattcgtaacgcacttgcctcaccgggtagcggtggtgatttaggtgaggcaattcgtgaacaacctgaacaggcacgcttagcattaacccttgcagccgcagaaagtgaaagatttgtgcgtcagggtactggtaatgatgaggccggtgcagcaaatgggccggcagacagcggagatgcattattagagagaaattatcctaccggcgcagaatttctgggtgatgggggtgatgttagtttttcaacacgcgggacacagaattggaccgtggaacgtttactgcaggcacatcgtcagctggaagaacgcggttatgtttttgttggttatcatgggacgtttctggaggcagcacagagcattgtctttggcggtgtgcgggcgcgtagccaggatcttgatgcaatttggcgtggtttttatattgcgggtgatcctgcgctggcgtatggatatgcgcaggatcaggagccggatgcgcgtggtcgtattcgtaatggtgccctgctgcgggtttatgttccgcgtagctcactgccggggttttatagaacaagcttaacactggctgcgccggaagcagcaggtgaagttgaacgtctgattggccatccgctgccgttacgtttagatgcaattactggtccggaagaagaaggtggtcgcctggaaaccattctgggttggccgctggcagaaagaaccgtggttataccttccgcaataccgaccgatcctcggaatgtggggggtgatttagatcctagcagcattcctgataaagaacaggcaatttctgctctgcctgattatgcatcacagccgggtaaaccgccgcgtgaagatttaaagcatcatcaccatcatcattaagatccggggctctggaagatccgcgcgtaccgagttctaattcactggccgtcgttttacaacatacgatgaaggcgataagtcgcgtaagttgctagcccacgcggctcaccttcacgggtgggcctttcttcgcgatccacatg

SEQ ID NO: 115 - DNA, 5830 bp, synthetic construct
  source 1..5830: mol_type = other DNA
catggtcatagctgtttcctttaatgcccatggcgtttaccaatgcttaatcagtgaggcacctatctcagcgatctgtctatttcgttcatccatagttgcctgactccccgtcgtgtagataactacgatacgggagggcttaccatctggccccagtgctgcaatgataccgcgacttccacgctcaccggctccagatttatcagcaataaaccagccagccggaagggccgagcgcagaagtggtcctgcaactttatccgcctccatccagtctattaattgttgccgggaagctagagtaagtagttcgccagttaatagtttgcgcaacgttgttgccattgctacaggcatcgtggtgtcacgctcgtcgtttggtatggcttcattcagctccggttcccaacgatcaaggcgagttacatgatcccccatgttgtgcaaaaaagcggttagctccttcggtcctccgatcgttgtcagaagtaagttggccgcagtgttatcactcatggttatggcagcactgcataattctcttactgtcatgccatccgtaagatgcttttctgtgactggtgagtactcaaccaagtcattctgagaatagtgtatgcggcgaccgagttgctcttgcccggcgtcaatacgggataataccgcgccacatagcagaactttaaaagtgctcatcattggaaaacgttcttcggggcgaaaactctcaaggatcttaccgctgttgagatccagttcgatgtaacccactcgtgcacccaactgatcttcagcatcttttactttcaccagcgtttctgggtgagcaaaaacaggaaggcaaaatgccgcaaaaaagggaataagggcgacacggaaatgttgaatactcatactcttcctttttcaatattattgaagcatttatcagggttattgtctcatgagcggatacatatttgaatgtatttagaaaaataaacaaataggggttccgcgcacatttccccgaaaagtgccacctgacgtctaagaaaccattattatcatgacattaacctataaaaataggcgtatcacgaggcccttaggccaaataggccgttcagatccttccgtatttagccagtatgttctctagtgtggttcgttgtttttgcgtgagccatgagaacgaaccattgagatcatgcttactttgcatgtcactcaaaaattttgcctcaaaactggtgagctgaatttttgcagttaaagcatcgtgtagtgtttttcttagtccgttacgtaggtaggaatctgatgtaatggttgttggtattttgtcaccattcatttttatctggttgttctcaagttcggttacgagatccatttgtctatctagttcaacttggaaaatcaacgtatcagtcgggcggcctcgcttatcaaccaccaatttcatattgctgtaagtgtttaaatctttacttattggtttcaaaacccattggttaagccttttaaactcatggtagttattttcaagcattaacatgaacttaaattcatcaaggctaatctctatatttgccttgtgagttttcttttgtgttagttcttttaataaccactcataaatcctcatagagtatttgttttcaaaagacttaacatgttccagattatattttatgaatttttttaactggaaaagataaggcaatatctcttcactaaaaactaattctaatttttcgcttgagaacttggcatagtttgtccactggaaaatctcaaagcctttaaccaaaggattcctgatttccacagttctcgtcatcagctctctggttgctttagctaatacaccataagcattttccctactgatgttcatcatctgagcgtattggttataagtgaacgataccgtccgttctttccttgtagggttttcaatcgtggggttgagtagtgccacacagcataaaattagcttggtttcatgctccgttaagtcatagcgactaatcgctagttcatttgctttgaaaacaactaattcagacatacatctcaattggtctaggtgattttaatcactataccaattgagatgggctagtcaatgataattactagtccttttcctttgagttgtgggtatctgtaaattctgctagacctttgctggaaaacttgtaaattctgctagaccctctgtaaattccgctagacctttgtgtgttttttttgtttatattcaagtggttataatttatagaataaagaaagaataaaaaaagataaaaagaatagatcccagccctgtgtataactcactactttagtcagttccgcagtattacaaaaggatgtcgcaaacgctgtttgctcctctacaaaacagaccttaaaaccctaaaggcttaagtagcaccctcgcaagctcgggcaaatcgctgaatattccttttgtctccgaccatcaggcacctgagtcgctgtctttttcgtgacattcagttcgctgcgctcacggctctggcagtgaatgggggtaaatggcactacaggcgccttttatggattcatgcaaggaaactacccataatacaagaaaagcccgtcacgggcttctcagggcgttttatggcgggtctgctatgtggtgctatctgactttttgctgttcagcagttcctgccctctgattttccagtctgaccacttcggattatcccgtgacaggtcattcagactggctaatgcacccagtaaggcagcggtatcatcaacaggcttacccgtcttactgtcaagaggacatccggtcagataaccgtcatcttcggctactgtctagggcggcggatttgtcctactcaggagagcgttcaccgacaaacaacagataaaacgaaaggcccagtctttcgactgagcctttcgttttatttgatgcactagtgccgatcatattcaataacccttaatataacttcgtataatgtatgctatacgaagttattaggtctgaagaggagtttacgtcccatatgggcgagctcgatatcaaattacgccccgccctgccactcatcgcagtactgttgtaattcattaagcattctgccgacatggaagccatcacagacggcatgatgaacctgaatcgccagcggcatcagcaccttgtcgccttgcgtataatatttgcccatggtgaaaacgggggcgaagaagttgtccatattggccacgtttaaatcaaaactggtgaaactcacccagggattggctgagacgaaaaacatattctcaataaaccctttagggaaataggccaggttttcaccgtaacacgccacatcttgcgaatatatgtgtagaaactgccggaaatcgtcgtggtattcactccagagcgatgaaaacgtttcagtttgctcatggaaaacggtgtaacaagggtgaacactatcccatatcaccagctcaccgtctttcattgccatacgaaattccggatgagcattcatcaggcgggcaagaatgtgaataaaggccggataaaacttgtgcttatttttctttacggtctttaaaaaggccgtaatatccagctgaacggtctggttataggtacattgagcaactgactgaaatgcctcaaaatgttctttacgatgccattgggatatatcaacggtggtatatccagtgatttttttctccattttagcttccttagctcctgaaaatctcgataactcaaaaaatacgcccggtagtgatcttatttcattatggtgaaagttggaacctcttacgtgccgatcaacgtctcattttcgccagatatcgccaagcttaggatccggaacccttaatataacttcgtataatgtatgctatacgaagttattaggtccctcgaagaggttcactagctatctagagcttggactcctgttgatagatccagtaatgacctcagaactccatctggatttgttcagaacgctcggttgccgccgggcgttttttattggtgagaatccaagcccgggaaacgggatcctgatcttgatccgccgcaaagtttgagcgaagtcaataaactctctacccattcagggcaatatctctcttgcaggtgaatgcaacgtcaagcgatggcctacttgcggcctcacacaggaaagtactagatgaaatacctgctgccgaccgctgctgctggtctgctgctcctcgctgcccagccggcgatggccggcggtggcacggtacaggctggcggtagcctgaaactgagctgcgccgcgagaggttggcgctttagcggctattgcgtagcctggtttcgtcaagcaccgggcaaagaacgcgaagcggtagcgatcattccgggtgctggcgtgatgtataccgatgattctgtgaaaggccgtttcacctattcgcgcgataatgtgaagaacaccgttagtctgcaaatgaacagcctggaaccggaagataccgcaacgtactactgcgctgtggattgggcatacagccatagctgtccgaagaacacggaagattaccgttattggggccagggcacgcaggtgaccgtgtcatcacctgaaggtggtagcctggcggcactgaccgcacaccaagcatgtcatctgccactggaaacctttacccgtcatcgtcagccgcgtggctgggaacaactggaacaatgtggatatccggtgcagagactggtcgcattatatctggcagcacgtctgagttggaatcaggttgatcaagttattcgtaacgcacttgcctcaccgggtagcggtggtgatttaggtgaggcaattcgtgaacaacctgaacaggcacgcttagcattaacccttgcagccgcagaaagtgaaagatttgtgcgtcagggtactggtaatgatgaggccggtgcagcaaatgggccggcagacagcggagatgcattattagagagaaattatcctaccggcgcagaatttctgggtgatgggggtgatgttagtttttcaacacgcgggacacagaattggaccgtggaacgtttactgcaggcacatcgtcagctggaagaacgcggttatgtttttgttggttatcatgggacgtttctggaggcagcacagagcattgtctttggcggtgtgcgggcgcgtagccaggatcttgatgcaatttggcgtggtttttatattgcgggtgatcctgcgctggcgtatggatatgcgcaggatcaggagccggatgcgcgtggtcgtattcgtaatggtgccctgctgcgggtttatgttccgcgtagctcactgccggggttttatagaacaagcttaacactggctgcgccggaagcagcaggtgaagttgaacgtctgattggccatccgctgccgttacgtttagatgcaattactggtccggaagaagaaggtggtcgcctggaaaccattctgggttggccgctggcagaaagaaccgtggttataccttccgcaataccgaccgatcctcggaatgtggggggtgatttagatcctagcagcattcctgataaagaacaggcaatttctgctctgcctgattatgcatcacagccgggtaaaccgccgcgtgaagatttaaagcatcatcaccatcatcattaagatccggggctctggaagatccgcgcgtaccgagttctaattcactggccgtcgttttacaacatacgatgaaggcgataagtcgcgtaagttgctagcccacgcggctcaccttcacgggtgggcctttcttcgcgatccacatg

SEQ ID NO: 116 - DNA, 5528 bp, synthetic construct
  source 1..5528: mol_type = other DNA
catggtcatagctgtttcctttaatgcccatggcgtttaccaatgcttaatcagtgaggcacctatctcagcgatctgtctatttcgttcatccatagttgcctgactccccgtcgtgtagataactacgatacgggagggcttaccatctggccccagtgctgcaatgataccgcgacttccacgctcaccggctccagatttatcagcaataaaccagccagccggaagggccgagcgcagaagtggtcctgcaactttatccgcctccatccagtctattaattgttgccgggaagctagagtaagtagttcgccagttaatagtttgcgcaacgttgttgccattgctacaggcatcgtggtgtcacgctcgtcgtttggtatggcttcattcagctccggttcccaacgatcaaggcgagttacatgatcccccatgttgtgcaaaaaagcggttagctccttcggtcctccgatcgttgtcagaagtaagttggccgcagtgttatcactcatggttatggcagcactgcataattctcttactgtcatgccatccgtaagatgcttttctgtgactggtgagtactcaaccaagtcattctgagaatagtgtatgcggcgaccgagttgctcttgcccggcgtcaatacgggataataccgcgccacatagcagaactttaaaagtgctcatcattggaaaacgttcttcggggcgaaaactctcaaggatcttaccgctgttgagatccagttcgatgtaacccactcgtgcacccaactgatcttcagcatcttttactttcaccagcgtttctgggtgagcaaaaacaggaaggcaaaatgccgcaaaaaagggaataagggcgacacggaaatgttgaatactcatactcttcctttttcaatattattgaagcatttatcagggttattgtctcatgagcggatacatatttgaatgtatttagaaaaataaacaaataggggttccgcgcacatttccccgaaaagtgccacctgacgtctaagaaaccattattatcatgacattaacctataaaaataggcgtatcacgaggcccttaggccaaataggccgttcagatccttccgtatttagccagtatgttctctagtgtggttcgttgtttttgcgtgagccatgagaacgaaccattgagatcatgcttactttgcatgtcactcaaaaattttgcctcaaaactggtgagctgaatttttgcagttaaagcatcgtgtagtgtttttcttagtccgttacgtaggtaggaatctgatgtaatggttgttggtattttgtcaccattcatttttatctggttgttctcaagttcggttacgagatccatttgtctatctagttcaacttggaaaatcaacgtatcagtcgggcggcctcgcttatcaaccaccaatttcatattgctgtaagtgtttaaatctttacttattggtttcaaaacccattggttaagccttttaaactcatggtagttattttcaagcattaacatgaacttaaattcatcaaggctaatctctatatttgccttgtgagttttcttttgtgttagttcttttaataaccactcataaatcctcatagagtatttgttttcaaaagacttaacatgttccagattatattttatgaatttttttaactggaaaagataaggcaatatctcttcactaaaaactaattctaatttttcgcttgagaacttggcatagtttgtccactggaaaatctcaaagcctttaaccaaaggattcctgatttccacagttctcgtcatcagctctctggttgctttagctaatacaccataagcattttccctactgatgttcatcatctgagcgtattggttataagtgaacgataccgtccgttctttccttgtagggttttcaatcgtggggttgagtagtgccacacagcataaaattagcttggtttcatgctccgttaagtcatagcgactaatcgctagttcatttgctttgaaaacaactaattcagacatacatctcaattggtctaggtgattttaatcactataccaattgagatgggctagtcaatgataattactagtccttttcctttgagttgtgggtatctgtaaattctgctagacctttgctggaaaacttgtaaattctgctagaccctctgtaaattccgctagacctttgtgtgttttttttgtttatattcaagtggttataatttatagaataaagaaagaataaaaaaagataaaaagaatagatcccagccctgtgtataactcactactttagtcagttccgcagtattacaaaaggatgtcgcaaacgctgtttgctcctctacaaaacagaccttaaaaccctaaaggcttaagtagcaccctcgcaagctcgggcaaatcgctgaatattccttttgtctccgaccatcaggcacctgagtcgctgtctttttcgtgacattcagttcgctgcgctcacggctctggcagtgaatgggggtaaatggcactacaggcgccttttatggattcatgcaaggaaactacccataatacaagaaaagcccgtcacgggcttctcagggcgttttatggcgggtctgctatgtggtgctatctgactttttgctgttcagcagttcctgccctctgattttccagtctgaccacttcggattatcccgtgacaggtcattcagactggctaatgcacccagtaaggcagcggtatcatcaacaggcttacccgtcttactgtcaagaggacatccggtcagataaccgtcatcttcggctactgtctagggcggcggatttgtcctactcaggagagcgttcaccgacaaacaacagataaaacgaaaggcccagtctttcgactgagcctttcgttttatttgatgcactagtgccgatcatattcaataacccttaatataacttcgtataatgtatgctatacgaagttattaggtctgaagaggagtttacgtcccatatgggcgagctcgatatcaaattacgccccgccctgccactcatcgcagtactgttgtaattcattaagcattctgccgacatggaagccatcacagacggcatgatgaacctgaatcgccagcggcatcagcaccttgtcgccttgcgtataatatttgcccatggtgaaaacgggggcgaagaagttgtccatattggccacgtttaaatcaaaactggtgaaactcacccagggattggctgagacgaaaaacatattctcaataaaccctttagggaaataggccaggttttcaccgtaacacgccacatcttgcgaatatatgtgtagaaactgccggaaatcgtcgtggtattcactccagagcgatgaaaacgtttcagtttgctcatggaaaacggtgtaacaagggtgaacactatcccatatcaccagctcaccgtctttcattgccatacgaaattccggatgagcattcatcaggcgggcaagaatgtgaataaaggccggataaaacttgtgcttatttttctttacggtctttaaaaaggccgtaatatccagctgaacggtctggttataggtacattgagcaactgactgaaatgcctcaaaatgttctttacgatgccattgggatatatcaacggtggtatatccagtgatttttttctccattttagcttccttagctcctgaaaatctcgataactcaaaaaatacgcccggtagtgatcttatttcattatggtgaaagttggaacctcttacgtgccgatcaacgtctcattttcgccagatatcgccaagcttaggatccggaacccttaatataacttcgtataatgtatgctatacgaagttattaggtccctcgaagaggttcactagctatctagagcttggactcctgttgatagatccagtaatgacctcagaactccatctggatttgttcagaacgctcggttgccgccgggcgttttttattggtgagaatccaagcccgggaaacgggatcctgatcttgatccgccgcaaagtttgagcgaagtcaataaactctctacccattcagggcaatatctctcttgcaggtgaatgcaacgtcaagcgatggcctacttgcggcctcacacaggaaagtactagatgaaatacctgctgccgaccgctgctgctggtctgctgctcctcgctgcccagccggcgatggccgaagcactggcagcacatcgtgtttgcggagttccactggaaacgctggcacgtagccgtaaaccgcgtgatcttccggatgatctgtcatgcgcctatcaggcacagaacatcgttagcctgtttgtggcaacacgcatcttgttcagccatctggatagcgtgtttacgctgaacctggatgaacaagaaccggaagtggcagaacgccttagcgcactgagacagatcaacgagaacaatccgggcatggtgacacaggtgctgaccgttgcacgccagatttacaacgattacgtgacgcatcatccgggcttaactccggaacagactagcgcgggtgcacaagccgcagatatcttgagcctgttttgtccggatgcagataaaccgtgcgttgcgagcaacaacgatcaggcgaacatcaacatcgagtcacgtagcggacgcagctatctgccggagaatcgcgccgtgattacgcctcagggtgtgaccaactggacctatcaagaactggaagcaacgcatcaggcactgacacgcgaaggttatgtgtttgttggctatcatggcaccaaccatgttgcggcacagaccattgtgaaccgcattgcaccggttccacgtggtaacaacaccgaaaacgaagagaaatggggcggtctgtatgttgccacgcacgcagaagttgctcatggctatgcacgcatcaaagaaggtacgggcgaatatggcttaccgacgcgtgcagaacgtgatgccagaggcgttatgctgcgtgtgtacattccgagagcgagcttagaacgcttctatcgcaccaacacaccgctggaaaacgcggaagaacacattactcaggtgattggccatagcctgccgttacgcaacgaagcctttaccggtccggaaagcgcaggtggtgaagatgaaaccgtgattggctgggatatggcgattcatgccgttgccataccgagcaccataccgggcaatgcgtatgaagagctggcaattgacgaagaagcagttgccaaagaacagagcattagcaccaaaccgccgtataaagagcgcaaagacgaactgaagcatcatcaccatcatcattaagatccggctctggaagatccgcgcgtaccgagttctaattcactggccgtcgttttacaacatacgatgaaggcgataagtcgcgtaagttgctagcccacgcggctcaccttcacgggtgggcctttcttcgcgatccacatg

SEQ ID NO: 117 - DNA, 5603 bp, synthetic construct
  source 1..5603: mol_type = other DNA
catggtcatagctgtttcctttaatgcccatggcgtttaccaatgcttaatcagtgaggcacctatctcagcgatctgtctatttcgttcatccatagttgcctgactccccgtcgtgtagataactacgatacgggagggcttaccatctggccccagtgctgcaatgataccgcgacttccacgctcaccggctccagatttatcagcaataaaccagccagccggaagggccgagcgcagaagtggtcctgcaactttatccgcctccatccagtctattaattgttgccgggaagctagagtaagtagttcgccagttaatagtttgcgcaacgttgttgccattgctacaggcatcgtggtgtcacgctcgtcgtttggtatggcttcattcagctccggttcccaacgatcaaggcgagttacatgatcccccatgttgtgcaaaaaagcggttagctccttcggtcctccgatcgttgtcagaagtaagttggccgcagtgttatcactcatggttatggcagcactgcataattctcttactgtcatgccatccgtaagatgcttttctgtgactggtgagtactcaaccaagtcattctgagaatagtgtatgcggcgaccgagttgctcttgcccggcgtcaatacgggataataccgcgccacatagcagaactttaaaagtgctcatcattggaaaacgttcttcggggcgaaaactctcaaggatcttaccgctgttgagatccagttcgatgtaacccactcgtgcacccaactgatcttcagcatcttttactttcaccagcgtttctgggtgagcaaaaacaggaaggcaaaatgccgcaaaaaagggaataagggcgacacggaaatgttgaatactcatactcttcctttttcaatattattgaagcatttatcagggttattgtctcatgagcggatacatatttgaatgtatttagaaaaataaacaaataggggttccgcgcacatttccccgaaaagtgccacctgacgtctaagaaaccattattatcatgacattaacctataaaaataggcgtatcacgaggcccttaggccaaataggccgttcagatccttccgtatttagccagtatgttctctagtgtggttcgttgtttttgcgtgagccatgagaacgaaccattgagatcatgcttactttgcatgtcactcaaaaattttgcctcaaaactggtgagctgaatttttgcagttaaagcatcgtgtagtgtttttcttagtccgttacgtaggtaggaatctgatgtaatggttgttggtattttgtcaccattcatttttatctggttgttctcaagttcggttacgagatccatttgtctatctagttcaacttggaaaatcaacgtatcagtcgggcggcctcgcttatcaaccaccaatttcatattgctgtaagtgtttaaatctttacttattggtttcaaaacccattggttaagccttttaaactcatggtagttattttcaagcattaacatgaacttaaattcatcaaggctaatctctatatttgccttgtgagttttcttttgtgttagttcttttaataaccactcataaatcctcatagagtatttgttttcaaaagacttaacatgttccagattatattttatgaatttttttaactggaaaagataaggcaatatctcttcactaaaaactaattctaatttttcgcttgagaacttggcatagtttgtccactggaaaatctcaaagcctttaaccaaaggattcctgatttccacagttctcgtcatcagctctctggttgctttagctaatacaccataagcattttccctactgatgttcatcatctgagcgtattggttataagtgaacgataccgtccgttctttccttgtagggttttcaatcgtggggttgagtagtgccacacagcataaaattagcttggtttcatgctccgttaagtcatagcgactaatcgctagttcatttgctttgaaaacaactaattcagacatacatctcaattggtctaggtgattttaatcactataccaattgagatgggctagtcaatgataattactagtccttttcctttgagttgtgggtatctgtaaattctgctagacctttgctggaaaacttgtaaattctgctagaccctctgtaaattccgctagacctttgtgtgttttttttgtttatattcaagtggttataatttatagaataaagaaagaataaaaaaagataaaaagaatagatcccagccctgtgtataactcactactttagtcagttccgcagtattacaaaaggatgtcgcaaacgctgtttgctcctctacaaaacagaccttaaaaccctaaaggcttaagtagcaccctcgcaagctcgggcaaatcgctgaatattccttttgtctccgaccatcaggcacctgagtcgctgtctttttcgtgacattcagttcgctgcgctcacggctctggcagtgaatgggggtaaatggcactacaggcgccttttatggattcatgcaaggaaactacccataatacaagaaaagcccgtcacgggcttctcagggcgttttatggcgggtctgctatgtggtgctatctgactttttgctgttcagcagttcctgccctctgattttccagtctgaccacttcggattatcccgtgacaggtcattcagactggctaatgcacccagtaaggcagcggtatcatcaacaggcttacccgtcttactgtcaagaggacatccggtcagataaccgtcatcttcggctactgtctagggcggcggatttgtcctactcaggagagcgttcaccgacaaacaacagataaaacgaaaggcccagtctttcgactgagcctttcgttttatttgatgcactagtgccgatcatattcaataacccttaatataacttcgtataatgtatgctatacgaagttattaggtctgaagaggagtttacgtcccatatgggcgagctcgatatcaaattacgccccgccctgccactcatcgcagtactgttgtaattcattaagcattctgccgacatggaagccatcacagacggcatgatgaacctgaatcgccagcggcatcagcaccttgtcgccttgcgtataatatttgcccatggtgaaaacgggggcgaagaagttgtccatattggccacgtttaaatcaaaactggtgaaactcacccagggattggctgagacgaaaaacatattctcaataaaccctttagggaaataggccaggttttcaccgtaacacgccacatcttgcgaatatatgtgtagaaactgccggaaatcgtcgtggtattcactccagagcgatgaaaacgtttcagtttgctcatggaaaacggtgtaacaagggtgaacactatcccatatcaccagctcaccgtctttcattgccatacgaaattccggatgagcattcatcaggcgggcaagaatgtgaataaaggccggataaaacttgtgcttatttttctttacggtctttaaaaaggccgtaatatccagctgaacggtctggttataggtacattgagcaactgactgaaatgcctcaaaatgttctttacgatgccattgggatatatcaacggtggtatatccagtgatttttttctccattttagcttccttagctcctgaaaatctcgataactcaaaaaatacgcccggtagtgatcttatttcattatggtgaaagttggaacctcttacgtgccgatcaacgtctcattttcgccagatatcgccaagcttaggatccggaacccttaatataacttcgtataatgtatgctatacgaagttattaggtccctcgaagaggttcactagctatctagagcttggactcctgttgatagatccagtaatgacctcagaactccatctggatttgttcagaacgctcggttgccgccgggcgttttttattggtgagaatccaagcccgggaaacgggatcctgatcttgatccgccgcaaagtttgagcgaagtcaataaactctctacccattcagggcaatatctctcttgcaggtgaatgcaacgtcaagcgatggcctacttgcggcctcacacaggaaagtactagatgaaatacctgctgccgaccgctgctgctggtctgctgctcctcgctgcccagccggcgatggccggcgcggatgatgtcgtggattcaagcaaatcatttgtcatggagaacttcagcagctatcacggcaccaaacctggctatgtggattcgattcagaaaggcattcagaaaccgaaatccggtacgcagggcaactatgacgatgattggaaaggcttctacagcaccgataacaagtacgatgcggcgggttactccgtggataatgagaatccactgagcggtaaagctggcggtgtggtgaaagtcacctatccgggcctgacgaaagtgctggcactgaaggtggataatgccgaaaccattaagaaagaactgggcctgagcctgaccgaacctctgatggaacaggttggcacagaagagtttatcaaacgctttggcgatggtgcgtcaagagttgtgctgagccttccgtttgccgaaggtagcagcagcgttgagtacatcaacaattgggaacaggccaaagcactgtcagtggaactggaaatcaactttgagacacgtggtaagagaggccaagatgccatgtacgagtacatggcgcaagcgtgcgcaggcaaccgcgttcgtagaagcgttggcagcagcctgagctgcatcaacctggactgggatgtgattcgcgataagaccaagacgaagatcgaaagcctgaaagaacacggaccaatcaagaacaagatgagcgaaagtccgaacaagacggtgagcgaagagaaagcgaaacagtatctggaagagtttcaccagaccgcactggaacatccggaactgagcgagcttaagaccgtgacgggcacaaatccggtgtttgcaggcgcaaactatgcggcatgggcggtgaacgtggcacaggtcattgacagcgaaactgcggataatctggagaaaacgaccgctgcactgagcatactgccgggaattggcagcgtaatgggcatcgcggatggtgctgttcaccacaacaccgaagagattgttgcgcagagcatcgcactgagcagcctgatggtggcacaagcgattccgctggtgggcgaattggtcgatatcggctttgcggcctataacttcgtcgaaagcattatcaacctgtttcaggtggttcacaacagctacaatcgtccggcctatagtccgggacacaagacgcagccgtttctgcatcatcaccatcatcattaagatccggctctggaagatccgcgcgtaccgagttctaattcactggccgtcgttttacaacatacgatgaaggcgataagtcgcgtaagttgctagcccacgcggctcaccttcacgggtgggcctttcttcgcgatccacatg

SEQ ID NO: 118 - DNA, 5957 bp, synthetic construct
  source 1..5957: mol_type = other DNA
catggtcatagctgtttcctttaatgcccatggcgtttaccaatgcttaatcagtgaggcacctatctcagcgatctgtctatttcgttcatccatagttgcctgactccccgtcgtgtagataactacgatacgggagggcttaccatctggccccagtgctgcaatgataccgcgacttccacgctcaccggctccagatttatcagcaataaaccagccagccggaagggccgagcgcagaagtggtcctgcaactttatccgcctccatccagtctattaattgttgccgggaagctagagtaagtagttcgccagttaatagtttgcgcaacgttgttgccattgctacaggcatcgtggtgtcacgctcgtcgtttggtatggcttcattcagctccggttcccaacgatcaaggcgagttacatgatcccccatgttgtgcaaaaaagcggttagctccttcggtcctccgatcgttgtcagaagtaagttggccgcagtgttatcactcatggttatggcagcactgcataattctcttactgtcatgccatccgtaagatgcttttctgtgactggtgagtactcaaccaagtcattctgagaatagtgtatgcggcgaccgagttgctcttgcccggcgtcaatacgggataataccgcgccacatagcagaactttaaaagtgctcatcattggaaaacgttcttcggggcgaaaactctcaaggatcttaccgctgttgagatccagttcgatgtaacccactcgtgcacccaactgatcttcagcatcttttactttcaccagcgtttctgggtgagcaaaaacaggaaggcaaaatgccgcaaaaaagggaataagggcgacacggaaatgttgaatactcatactcttcctttttcaatattattgaagcatttatcagggttattgtctcatgagcggatacatatttgaatgtatttagaaaaataaacaaataggggttccgcgcacatttccccgaaaagtgccacctgacgtctaagaaaccattattatcatgacattaacctataaaaataggcgtatcacgaggcccttaggccaaataggccgttcagatccttccgtatttagccagtatgttctctagtgtggttcgttgtttttgcgtgagccatgagaacgaaccattgagatcatgcttactttgcatgtcactcaaaaattttgcctcaaaactggtgagctgaatttttgcagttaaagcatcgtgtagtgtttttcttagtccgttacgtaggtaggaatctgatgtaatggttgttggtattttgtcaccattcatttttatctggttgttctcaagttcggttacgagatccatttgtctatctagttcaacttggaaaatcaacgtatcagtcgggcggcctcgcttatcaaccaccaatttcatattgctgtaagtgtttaaatctttacttattggtttcaaaacccattggttaagccttttaaactcatggtagttattttcaagcattaacatgaacttaaattcatcaaggctaatctctatatttgccttgtgagttttcttttgtgttagttcttttaataaccactcataaatcctcatagagtatttgttttcaaaagacttaacatgttccagattatattttatgaatttttttaactggaaaagataaggcaatatctcttcactaaaaactaattctaatttttcgcttgagaacttggcatagtttgtccactggaaaatctcaaagcctttaaccaaaggattcctgatttccacagttctcgtcatcagctctctggttgctttagctaatacaccataagcattttccctactgatgttcatcatctgagcgtattggttataagtgaacgataccgtccgttctttccttgtagggttttcaatcgtggggttgagtagtgccacacagcataaaattagcttggtttcatgctccgttaagtcatagcgactaatcgctagttcatttgctttgaaaacaactaattcagacatacatctcaattggtctaggtgattttaatcactataccaattgagatgggctagtcaatgataattactagtccttttcctttgagttgtgggtatctgtaaattctgctagacctttgctggaaaacttgtaaattctgctagaccctctgtaaattccgctagacctttgtgtgttttttttgtttatattcaagtggttataatttatagaataaagaaagaataaaaaaagataaaaagaatagatcccagccctgtgtataactcactactttagtcagttccgcagtattacaaaaggatgtcgcaaacgctgtttgctcctctacaaaacagaccttaaaaccctaaaggcttaagtagcaccctcgcaagctcgggcaaatcgctgaatattccttttgtctccgaccatcaggcacctgagtcgctgtctttttcgtgacattcagttcgctgcgctcacggctctggcagtgaatgggggtaaatggcactacaggcgccttttatggattcatgcaaggaaactacccataatacaagaaaagcccgtcacgggcttctcagggcgttttatggcgggtctgctatgtggtgctatctgactttttgctgttcagcagttcctgccctctgattttccagtctgaccacttcggattatcccgtgacaggtcattcagactggctaatgcacccagtaaggcagcggtatcatcaacaggcttacccgtcttactgtcaagaggacatccggtcagataaccgtcatcttcggctactgtctagggcggcggatttgtcctactcaggagagcgttcaccgacaaacaacagataaaacgaaaggcccagtctttcgactgagcctttcgttttatttgatgcactagtgccgatcatattcaataacccttaatataacttcgtataatgtatgctatacgaagttattaggtctgaagaggagtttacgtcccatatgggcgagctcgatatcaaattacgccccgccctgccactcatcgcagtactgttgtaattcattaagcattctgccgacatggaagccatcacagacggcatgatgaacctgaatcgccagcggcatcagcaccttgtcgccttgcgtataatatttgcccatggtgaaaacgggggcgaagaagttgtccatattggccacgtttaaatcaaaactggtgaaactcacccagggattggctgagacgaaaaacatattctcaataaaccctttagggaaataggccaggttttcaccgtaacacgccacatcttgcgaatatatgtgtagaaactgccggaaatcgtcgtggtattcactccagagcgatgaaaacgtttcagtttgctcatggaaaacggtgtaacaagggtgaacactatcccatatcaccagctcaccgtctttcattgccatacgaaattccggatgagcattcatcaggcgggcaagaatgtgaataaaggccggataaaacttgtgcttatttttctttacggtctttaaaaaggccgtaatatccagctgaacggtctggttataggtacattgagcaactgactgaaatgcctcaaaatgttctttacgatgccattgggatatatcaacggtggtatatccagtgatttttttctccattttagcttccttagctcctgaaaatctcgataactcaaaaaatacgcccggtagtgatcttatttcattatggtgaaagttggaacctcttacgtgccgatcaacgtctcattttcgccagatatcgccaagcttaggatccggaacccttaatataacttcgtataatgtatgctatacgaagttattaggtccctcgaagaggttcactagctatctagagcttggactcctgttgatagatccagtaatgacctcagaactccatctggatttgttcagaacgctcggttgccgccgggcgttttttattggtgagaatccaagcccgggaaacgggatcctgatcttgatccgccgcaaagtttgagcgaagtcaataaactctctacccattcagggcaatatctctcttgcaggtgaatgcaacgtcaagcgatggcctacttgcggcctcacacaggaaagtactagatgaaatacctgctgccgaccgctgctgctggtctgctgctcctcgctgcccagccggcgatggccgaggttcaattagtggaatctggcgggggattggttcaagccggtgagtccttgcgtttgagctgcgccgcatctgggagcacatttgatttcaaagtgatgggctggtatcgtcagccgcccggaaaacagcgcgagggtgtagcagccatccgcttgagcggaaatatgcactacgccgagtctgtaaaagggcgctttgctatttccaaagcgaacgctaagaacacagtgtatcttcagatgaactccttgcgtcccgaagacactgccgtttattattgcaaagtaaacatccgtgggcaagactactggggtcaaggaacgcaggtcacagtctcttctggctctggcggcgcggatgatgtcgtggattcaagcaaatcatttgtcatggagaacttcagcagctatcacggcaccaaacctggctatgtggattcgattcagaaaggcattcagaaaccgaaatccggtacgcagggcaactatgacgatgattggaaaggcttctacagcaccgataacaagtacgatgcggcgggttactccgtggataatgagaatccactgagcggtaaagctggcggtgtggtgaaagtcacctatccgggcctgacgaaagtgctggcactgaaggtggataatgccgaaaccattaagaaagaactgggcctgagcctgaccgaacctctgatggaacaggttggcacagaagagtttatcaaacgctttggcgatggtgcgtcaagagttgtgctgagccttccgtttgccgaaggtagcagcagcgttgagtacatcaacaattgggaacaggccaaagcactgtcagtggaactggaaatcaactttgagacacgtggtaagagaggccaagatgccatgtacgagtacatggcgcaagcgtgcgcaggcaaccgcgttcgtagaagcgttggcagcagcctgagctgcatcaacctggactgggatgtgattcgcgataagaccaagacgaagatcgaaagcctgaaagaacacggaccaatcaagaacaagatgagcgaaagtccgaacaagacggtgagcgaagagaaagcgaaacagtatctggaagagtttcaccagaccgcactggaacatccggaactgagcgagcttaagaccgtgacgggcacaaatccggtgtttgcaggcgcaaactatgcggcatgggcggtgaacgtggcacaggtcattgacagcgaaactgcggataatctggagaaaacgaccgctgcactgagcatactgccgggaattggcagcgtaatgggcatcgcggatggtgctgttcaccacaacaccgaagagattgttgcgcagagcatcgcactgagcagcctgatggtggcacaagcgattccgctggtgggcgaattggtcgatatcggctttgcggcctataacttcgtcgaaagcattatcaacctgtttcaggtggttcacaacagctacaatcgtccggcctatagtccgggacacaagacgcagccgtttctgcatcatcaccatcatcattaagatccggctctggaagatccgcgcgtaccgagttctaattcactggccgtcgttttacaacatacgatgaaggcgataagtcgcgtaagttgctagcccacgcggctcaccttcacgggtgggcctttcttcgcgatccacatg

SEQ ID NO: 119 - DNA, 5882 bp, synthetic construct
  source 1..5882: mol_type = other DNA
catggtcatagctgtttcctttaatgcccatggcgtttaccaatgcttaatcagtgaggcacctatctcagcgatctgtctatttcgttcatccatagttgcctgactccccgtcgtgtagataactacgatacgggagggcttaccatctggccccagtgctgcaatgataccgcgacttccacgctcaccggctccagatttatcagcaataaaccagccagccggaagggccgagcgcagaagtggtcctgcaactttatccgcctccatccagtctattaattgttgccgggaagctagagtaagtagttcgccagttaatagtttgcgcaacgttgttgccattgctacaggcatcgtggtgtcacgctcgtcgtttggtatggcttcattcagctccggttcccaacgatcaaggcgagttacatgatcccccatgttgtgcaaaaaagcggttagctccttcggtcctccgatcgttgtcagaagtaagttggccgcagtgttatcactcatggttatggcagcactgcataattctcttactgtcatgccatccgtaagatgcttttctgtgactggtgagtactcaaccaagtcattctgagaatagtgtatgcggcgaccgagttgctcttgcccggcgtcaatacgggataataccgcgccacatagcagaactttaaaagtgctcatcattggaaaacgttcttcggggcgaaaactctcaaggatcttaccgctgttgagatccagttcgatgtaacccactcgtgcacccaactgatcttcagcatcttttactttcaccagcgtttctgggtgagcaaaaacaggaaggcaaaatgccgcaaaaaagggaataagggcgacacggaaatgttgaatactcatactcttcctttttcaatattattgaagcatttatcagggttattgtctcatgagcggatacatatttgaatgtatttagaaaaataaacaaataggggttccgcgcacatttccccgaaaagtgccacctgacgtctaagaaaccattattatcatgacattaacctataaaaataggcgtatcacgaggcccttaggccaaataggccgttcagatccttccgtatttagccagtatgttctctagtgtggttcgttgtttttgcgtgagccatgagaacgaaccattgagatcatgcttactttgcatgtcactcaaaaattttgcctcaaaactggtgagctgaatttttgcagttaaagcatcgtgtagtgtttttcttagtccgttacgtaggtaggaatctgatgtaatggttgttggtattttgtcaccattcatttttatctggttgttctcaagttcggttacgagatccatttgtctatctagttcaacttggaaaatcaacgtatcagtcgggcggcctcgcttatcaaccaccaatttcatattgctgtaagtgtttaaatctttacttattggtttcaaaacccattggttaagccttttaaactcatggtagttattttcaagcattaacatgaacttaaattcatcaaggctaatctctatatttgccttgtgagttttcttttgtgttagttcttttaataaccactcataaatcctcatagagtatttgttttcaaaagacttaacatgttccagattatattttatgaatttttttaactggaaaagataaggcaatatctcttcactaaaaactaattctaatttttcgcttgagaacttggcatagtttgtccactggaaaatctcaaagcctttaaccaaaggattcctgatttccacagttctcgtcatcagctctctggttgctttagctaatacaccataagcattttccctactgatgttcatcatctgagcgtattggttataagtgaacgataccgtccgttctttccttgtagggttttcaatcgtggggttgagtagtgccacacagcataaaattagcttggtttcatgctccgttaagtcatagcgactaatcgctagttcatttgctttgaaaacaactaattcagacatacatctcaattggtctaggtgattttaatcactataccaattgagatgggctagtcaatgataattactagtccttttcctttgagttgtgggtatctgtaaattctgctagacctttgctggaaaacttgtaaattctgctagaccctctgtaaattccgctagacctttgtgtgttttttttgtttatattcaagtggttataatttatagaataaagaaagaataaaaaaagataaaaagaatagatcccagccctgtgtataactcactactttagtcagttccgcagtattacaaaaggatgtcgcaaacgctgtttgctcctctacaaaacagaccttaaaaccctaaaggcttaagtagcaccctcgcaagctcgggcaaatcgctgaatattccttttgtctccgaccatcaggcacctgagtcgctgtctttttcgtgacattcagttcgctgcgctcacggctctggcagtgaatgggggtaaatggcactacaggcgccttttatggattcatgcaaggaaactacccataatacaagaaaagcccgtcacgggcttctcagggcgttttatggcgggtctgctatgtggtgctatctgactttttgctgttcagcagttcctgccctctgattttccagtctgaccacttcggattatcccgtgacaggtcattcagactggctaatgcacccagtaaggcagcggtatcatcaacaggcttacccgtcttactgtcaagaggacatccggtcagataaccgtcatcttcggctactgtctagggcggcggatttgtcctactcaggagagcgttcaccgacaaacaacagataaaacgaaaggcccagtctttcgactgagcctttcgttttatttgatgcactagtgccgatcatattcaataacccttaatataacttcgtataatgtatgctatacgaagttattaggtctgaagaggagtttacgtcccatatgggcgagctcgatatcaaattacgccccgccctgccactcatcgcagtactgttgtaattcattaagcattctgccgacatggaagccatcacagacggcatgatgaacctgaatcgccagcggcatcagcaccttgtcgccttgcgtataatatttgcccatggtgaaaacgggggcgaagaagttgtccatattggccacgtttaaatcaaaactggtgaaactcacccagggattggctgagacgaaaaacatattctcaataaaccctttagggaaataggccaggttttcaccgtaacacgccacatcttgcgaatatatgtgtagaaactgccggaaatcgtcgtggtattcactccagagcgatgaaaacgtttcagtttgctcatggaaaacggtgtaacaagggtgaacactatcccatatcaccagctcaccgtctttcattgccatacgaaattccggatgagcattcatcaggcgggcaagaatgtgaataaaggccggataaaacttgtgcttatttttctttacggtctttaaaaaggccgtaatatccagctgaacggtctggttataggtacattgagcaactgactgaaatgcctcaaaatgttctttacgatgccattgggatatatcaacggtggtatatccagtgatttttttctccattttagcttccttagctcctgaaaatctcgataactcaaaaaatacgcccggtagtgatcttatttcattatggtgaaagttggaacctcttacgtgccgatcaacgtctcattttcgccagatatcgccaagcttaggatccggaacccttaatataacttcgtataatgtatgctatacgaagttattaggtccctcgaagaggttcactagctatctagagcttggactcctgttgatagatccagtaatgacctcagaactccatctggatttgttcagaacgctcggttgccgccgggcgttttttattggtgagaatccaagcccgggaaacgggatcctgatcttgatccgccgcaaagtttgagcgaagtcaataaactctctacccattcagggcaatatctctcttgcaggtgaatgcaacgtcaagcgatggcctacttgcggcctcacacaggaaagtactagatgaaatacctgctgccgaccgctgctgctggtctgctgctcctcgctgcccagccggcgatggccgaggttcaattagtggaatctggcgggggattggttcaagccggtgagtccttgcgtttgagctgcgccgcatctgggagcacatttgatttcaaagtgatgggctggtatcgtcagccgcccggaaaacagcgcgagggtgtagcagccatccgcttgagcggaaatatgcactacgccgagtctgtaaaagggcgctttgctatttccaaagcgaacgctaagaacacagtgtatcttcagatgaactccttgcgtcccgaagacactgccgtttattattgcaaagtaaacatccgtgggcaagactactggggtcaaggaacgcaggtcacagtctcttctggctctggcgaagcactggcagcacatcgtgtttgcggagttccactggaaacgctggcacgtagccgtaaaccgcgtgatcttccggatgatctgtcatgcgcctatcaggcacagaacatcgttagcctgtttgtggcaacacgcatcttgttcagccatctggatagcgtgtttacgctgaacctggatgaacaagaaccggaagtggcagaacgccttagcgcactgagacagatcaacgagaacaatccgggcatggtgacacaggtgctgaccgttgcacgccagatttacaacgattacgtgacgcatcatccgggcttaactccggaacagactagcgcgggtgcacaagccgcagatatcttgagcctgttttgtccggatgcagataaaccgtgcgttgcgagcaacaacgatcaggcgaacatcaacatcgagtcacgtagcggacgcagctatctgccggagaatcgcgccgtgattacgcctcagggtgtgaccaactggacctatcaagaactggaagcaacgcatcaggcactgacacgcgaaggttatgtgtttgttggctatcatggcaccaaccatgttgcggcacagaccattgtgaaccgcattgcaccggttccacgtggtaacaacaccgaaaacgaagagaaatggggcggtctgtatgttgccacgcacgcagaagttgctcatggctatgcacgcatcaaagaaggtacgggcgaatatggcttaccgacgcgtgcagaacgtgatgccagaggcgttatgctgcgtgtgtacattccgagagcgagcttagaacgcttctatcgcaccaacacaccgctggaaaacgcggaagaacacattactcaggtgattggccatagcctgccgttacgcaacgaagcctttaccggtccggaaagcgcaggtggtgaagatgaaaccgtgattggctgggatatggcgattcatgccgttgccataccgagcaccataccgggcaatgcgtatgaagagctggcaattgacgaagaagcagttgccaaagaacagagcattagcaccaaaccgccgtataaagagcgcaaagacgaactgaagcatcatcaccatcatcattaagatccggctctggaagatccgcgcgtaccgagttctaattcactggccgtcgttttacaacatacgatgaaggcgataagtcgcgtaagttgctagcccacgcggctcaccttcacgggtgggcctttcttcgcgatccacatg

SEQ ID NO: 120 - DNA, 18 bp, synthetic construct
  source 1..18: mol_type = other DNA
ggctctggaagatccgcg

SEQ ID NO: 121 - DNA, 18 bp, synthetic construct
  source 1..18: mol_type = other DNA
ggccgcaagtaggccatc

SEQ ID NO: 122 - DNA, 57 bp, synthetic construct
  source 1..57: mol_type = other DNA
gatggcctacttgcggcctcacacaggaaagtactagatgaaatacctgctgccgac

SEQ ID NO: 123 - DNA, 43 bp, synthetic construct
  source 1..43: mol_type = other DNA
cgcggatcttccagagccccggatcttaatgatgatggtgatg